European Patent Application EP 4 410 969 A1, published August 7, 2024. Title: 재조합된 약독화 RSV 생백신 및 이를 제조하는 방법. Applicant: 에스케이바이오사이언스(주). Application KR. The sequence listing filed with the application follows.

SEQUENCE LISTING (58 sequences)

SEQ ID NO: 1 - DNA, 15311 bp, respiratory syncytial virus
  source 1..15311: mol_type = genomic DNA
acgcgaaaaaatgcgtacaacaaacttgcgtaaaccaaaaaaatggggcaaataagaatttgataagtaccacttaaatttaactcctttggttagaggcgcgccatgggcagcaactcattgagtatgataaaagttagattgcaaaatctgtttgacaatgatgaagtagcattgttaaaaataacatgctatactgacaaattaatacagttaactaatgctttggctaaggcagttatacatacaatcaaattgaatggcattgtatttgtgcatgttattacaagtagtgatatttgccctaataataatattgtagtgaaatccaatttcacaacaatgccagtattacaaaatggaggttatatatgggaaatgatggaattaacacactgctctcaacctaatggcctaatagatgacaattgtgaaattaaattctccaaaaaactaagtgattcaacaatgaccaattatatgaatcaattatctgaattacttggatttgacctcaatccataaatcataataaatatcaactagcaaatcaatgtcactaacaccattagttaatataaaacttgacagaagataaaaatggggcaaataaatcaattcagccgacccaaccatggacacaacacacaatgataccacaccacaaagactgatgatcacagacatgaggccattatcgcttgagactataataacatctctaaccagagatatcataacacataaatttatatacttgataaatcatgaatgcatagtaagaaaacttgatgaaagacaggccacatttacatttctggtcaactatgaaatgaaactattgcacaaagtgggaagcactaaatataaaaaatatactgaatacaacacaaaatatggcactttccctatgccaatatttatcaatcatgatgggttcttagaatgcattggcattaagcctaccaagcacacacccataatatacaagtatgatctcaatccatgaatatcaaaccaagattcaaacaatccgaaataacaactttatgcataatcacactccatagtccaaatggagcctgaaaattatagttatttaaaattcctgcaggaaggagagacataagatgaaagatggggcaaatacaaaaatggctcttagcaaagtcaagttgaatgatacactcaacaaagatcaacttctatcatccagcaaatataccatccaacggagcacaggagacagcattgacactcctaattatgatgtgcagaaacacattaataagttatgtggcatgttattaatcacagaagatgctaatcataaattcactgggttaataggtatgttatatgctatgtctagattaggaagagaagacaccataaaaatactcaaagatgcgggatatcatgttaaggcaaatggagtggatgtaacaacacatcgtcaagacattaatgggaaagaaatgaaatttgaagtgttaacattagcaagcttaacaactgaaattcaaatcaacattgagatagaatctagaaaatcctacaaaaaaatgctaaaagaaatgggagaggtggctccagaatacaggcatgactctcctgattgtgggatgataatattatgtatagcggcattagtaataaccaaattagcagcaggagatagatcaggtcttacagctgtgattaggagagctaataatgtcctaaaaaatgaaatgaaacgttataaaggtttattacccaaggatatagccaacagcttctatgaagtgtttgaaaaatatcctcactttatagatgtttttgttcattttggtatagcacaatcttctaccagaggtggcagtagagttgaagggatttttgcaggattgtttatgaatgcctatggtgcagggcaagtgatgttacggtggggggtcttagcaaaatcagttaaaaacattatgttaggacacgctagtgtacaagcagaaatggaacaagttgtggaggtgtatgagtatgctcagaaattgggtggagaagcaggattctaccatatattgaacaacccaaaagcatcactattatctttgactcaatttcctcacttctctagtgtagtattgggcaatgctgctggcctaggcataatgggagaatacagaggtacaccaaggaatcaagatttatatgatgctgcaaaagcatatgctgaacaactcaaagaaaatggtgtgattaactacagtgtattagatttgacagcagaagaactagaggctatcaaacatcagcttaatccaaaagataatgatgtagagctttgagttaataaaaaagtggggcaaataaatcatcatggaaaagtttgctcctgaattccatggagaagatgcaaacaacagagccaccaaattcctagaatcaataaagggcaaattcacatcacccaaagatcccaagaaaaaagatagtatcatatctgtcaactcaatagatatagaagtaaccaaagaaagccctataacatcaaattcaaccattataaacccaataaatgagacagatgatactgtagggaacaagcccaattatcaaagaaagcctctagtaagtttcaaagaagaccctacgccaagtgataatcctttttcaaaactatacaaagaaaccatagaaacatttgataacaatgaagaagaatctagctattcatatgaagaaataaatgatcagacaaacgataatataacagcaagattagataggattgatgagaaattaagtgaaatactaggaatgcttcacacattagtagtagcgagtgcaggacccacatctgctcgggatggtataagagatgccatggttggtttaagagaagaaatgatagaaaaaatcagaactgaagcattaatgaccaatgacagactagaagctatggcaagactcaggaatgaagaaagtgaaaagatggcaaaagacacatcagatgaagtgtctctcaatccaacatcagagaaactgaacaacctgttggaagggaatgatagtgacaatgatctatcacttgaagatttctgattagctaccaaactgtacatcaaaacacaacaccaatagaaaaccaacaaacaaaccaactcacccatccaaccaaacatctatctgctgattagccaaccagccaaaaaacaaccagccaatctaaaactagccacccggaaaaaatcgatactatagttacaaaaaaagatggggcaaatatggaaacatacgtgaataaacttcacgagggctccacatacacagctgctgttcaatacaatgtcctagaaaaagacgatgatcctgcatcacttacaatatgggtgcccatgttccaatcatccatgccagcagatctactcataaaagaactagccaatgtcaatatactagtgaaacaaatatccacacccaagggaccctcattaagagtcatgataaactcaagaagtgcagtgctagcacaaatgcccagcaaatttaccatatgtgccaatgtgtccttggatgaaagaagcaagctggcatatgatgtaaccacaccctgtgaaattaaggcatgcagtctaacatgcctaaaatcaaaaaatatgttaactacagttaaagatctcactatgaaaacactcaacccaacacatgacatcattgctttatgtgaatttgaaaatatagtaacatcaaaaaaagtcataataccaacatacctaagatctatcagcgtcagaaataaagatctgaacacacttgaaaatataacaaccactgaattcaaaaatgccattacaaatgcaaaaatcatcccttactcaggattattgttagtcatcacagtgactgacaacaaaggagcattcaaatacataaagccacaaagtcaattcatagtagatcttggagcttacctagaaaaagaaagtatatattatgttacaacaaattggaagcacacagctacacgatttgcaatcaaacccatggaagattaacctttttcctctacatcaatgagtagattcatacaaactttctaactacattcttcacttcacaatcataatcaccaaccctctgtggttcaatcaatcaaacaaaactcatcaagagttccagatcatcccaagtcattgttcatcagatccagtactcaaataagttaataaaaaatccacatggggcaaataatcattgagggaaatccaactaatcacaacatctgtcaacatagacaagtcaacacgctagataaaatcaaccaatggaaaatacatccataactatagaattctcaagcaaattctggccttactttacactaatacacatgataacaacaataatctctttgataatcataatctccatcatgattgcaatactaaacaaactctgcgaatataatgtattccataacaaaacctttgagctaccaagagctcgagtcaatacatagcattcaccaatctgatagctcaaaacagtaaccttgcatttgtaaatgaactaccctcacttcttcacaaaaccacatcaacatctcaccatgcaagccatcatctataccataaagtagttaattaaaaatggccggccagtcataacaatgaactaggatattaagaccaaaaacaacgctggggcaaatgcaaacatgtccaaaaccgaggaccaacgcaccgccaagacactagaaaggacctgggacacttttaatcatctattattcatatcatcgtgcttatacaagttaaatcttaaatctatagcacaaatcacattatctattttggcaattataatctcaacctcacttataattgcagccatcatattcatagcctcggcaaaccacaaagtcacactaacaactgcaatcatacaagatgcaacgaaccagatcaagaacacaaccccaacatacctcacccagaatccccagcatggaatcagcttctccaatctgtccggaactacatcacaatccaccaccatactagcttcaacaacaccaagtgctgattcaaccccacaatccacaacagtcaagatcaaaaacacaacaacaacccaaatattacctagcaaacccaccacaaaacaacgccaaaataaaccacaaaacaaacccaacaatgattttcactttgaagtgttcaattttgtaccctgcagcatatgcagcaacaatccaacctgctgggccatctgcaagagaataccaaacaaaaaacctggaaagaaaaccaccaccaagcccacaaaaaaaccaaccctcaagacaaccaaaaaagatcccaaatcccaaaccacaaaaccaaaggaagtactcactaccaagcctacaggaaagccaaccatcaacaccactaaaacaaacatcagaactacactgctcacctccaacaccaaaggaaatccagaacacacaagtcaagaggaaaccctccactcaaccacctccgaaggctatccaagcccatcacaagtccacacaacatccggtcaagaggaaaccctccactcaaccacctccgaaggctatccaagcccatcacaagtctacacaacatccgagtacctatcacaatctctatcttcatccaacacaacaaaatgatagtcattaaaaagcacgcgtgtattgttgcaaaaagccatgaccaaatcaaacagaatcaaaatcaactctggggcaaataacaatggagttgccaatcctcaaaacaaatgctattaccacaatccttgctgcagtcacactctgtttcgcttccagtcaaaacatcactgaagaattttatcaatcaacatgcagtgcagtcagcaaaggctatcttagtgctctaagaactggttggtatactagtgttataactatagaattaagtaatatcaaggaaaataagtgtaatggtacagacgctaaggtaaaattaataaaacaagaattagataaatataaaaatgctgtaacagaattgcagttgctcatgcaaagcacaccagcagccaacaatcgagccagaagagaactaccaagatttatgaattatacactcaacaataccaaaaacaccaatgtaacattaagtaagaaaaggaaaagaagatttcttggatttttgttaggtgttggatctgcaatcgccagtggcattgccgtatccaaggtcctgcacctagaaggggaagtgaacaaaatcaaaagtgctctactatccacaaacaaggctgtagtcagcttatctaatggagtcagtgtcttaaccagcaaggtgttagacctcaaaaactatatagataaacagttgttacctattgttaacaagcaaagctgcagcatatcaaacattgaaactgtgatagagttccaacaaaagaacaacagactactagagattaccagagaatttagtgttaatgcaggtgtaactactcctgtaagcacttatatgttaactaatagtgagttattatcattaatcaatgatatgcctataacaaatgatcagaaaaagttaatgtccagcaatgttcaaatagttagacagcaaagttactctatcatgtcaataataaaagaggaagtcttggcatatgtagtacaattaccactatatggtgtaatagatactccttgttggaaactacacacatcccctttatgtacaaccaacacaaaggaaggatccaacatctgcttaacaagaaccgacagaggatggtactgtgacaatgcaggatcagtatcctttttcccacaagctgaaacatgtaaagttcaatcgaatcgggtgttttgtgacacaatgaacagtttaacattaccaagtgaggtaaatctctgcaacattgacatattcaaccccaaatatgattgcaaaattatgacttcaaaaacagatgtaagcagctccgttatcacatctctaggagccattgtgtcatgctatggcaaaaccaaatgtacagcatccaataaaaatcgtgggatcataaagacattctctaacgggtgtgattatgtatcaaataagggggtggatactgtgtctgtaggtaatacattatattatgtaaataagcaagaaggcaaaagtctctatgtaaaaggtgaaccaataataaatttctatgatccattagtgttcccctctgatgaatttgatgcatcaatatctcaagtcaatgagaaaattaatcagagtctagcatttatccgtaaatcagatgaattattacataatgtaaatgctggtaaatccaccacaaatatcatgataactaccataattatagtaattatagtaatattgttagcattaattgcagttggactgcttctatactgcaaggccagaagcacaccagtcacattaagtaaggatcaactgagtggtataaataatattgcatttagtaactgaataaaaatagcacctaatcatattcttacaatggttcgctatttgaccatagataacccatctatcattagattatcctaaaatttgaacttcatcacaactttcatctataaaccatctcacttacactttttaagtagatttctattttatagttatataaaacagggcccattgaataccaaattaacttactatttgtaaaaatgagaattggggcaaatatgtcacgaaggaatccttgcaaattcgaaattcgaggtcattgcttgaatggtaaaaggtgtcattttagtcataattattttgaatggccaccccatgcactgcttgtaagacaaaactttatgttaaacagaatacttaagtctatggataaaagcatagatactttgtcagaaataagtggagctgcagagttggacagaacagaagagtatgccctcggtgtagttggagtgctagagagttatataggatcaataaataatataactaaacaatcagcatgtgttgccatgagcaaactccttactgaactcaacagcgatgacatcaaaaaactaagggacaatgaagagccaaactcacccaaagtaagagtgtacaatactgtcatatcatatattgaaagcaacaggaagaacaataaacaaactatccatctgttaaaaagattgccagcagacgtattgaagaaaaccatcaaaaacacattggatatccacaagagcataaccatcaataacccaaaagaatcaactgttagtgatacgaacgaccatgccaaaaataatgatactacctgacaaatatccttgtagtataaattccatactaataacaagtaattgtagagtcactatgtataatcaaaaaaacacactatatatcaatcaaaacaaccaaaatagccatatatacccaccggatcaaccattcaatgaaatccattggacctctcaagacttgattgatgcaactcaaaattttctacaacatctaggtattactgatgatatatacacaatatatatattagtgtcataatactcaatcctaatacttaccacatcatcaaattattaactcaaacaattcaagctatgggacaaaatggatcccattattagtggaaattctgctaatgtttatctaactgatagttatttaaaaggtgttatttctttctcagaatgtaacgctttaggaagttacatattcaatggtccttatctcaaaaatgattataccaacttaattagtagacaaaatccattaatagaacacataaatctaaagaaactaaatataacacagtccttaatatctaagtatcataaaggtgaaataaaaatagaagaacctacttactttcagtcattacttatgacatacaagagtatgacctcttcagaacagactactactactaatttacttaaaaagataataagaagagctatagaaatcagtgatgtcaaagtctatgctatattgaataaactggggctcaaagaaaaagacaagattaaatccaataatggacaagatgaagacaactcagtcattactaccataatcaaagatgatatacttttagctgtcaaggataatcaatctcatcttaaagcagacaaaaatcaatccacaaaacaaaaagatacaatcaaaacaacacttttgaagaaattaatgtgttcgatgcaacatcctccatcatggttaatacattggtttaatttatacacaaaattaaacagcatattaacacaatatcgatctagtgaggtaaaaaaccatggttttatattgatagataatcatactcttagtggattccaatttattttgaatcaatatggttgtatagtttatcataaggaactcaaaagaattactgtgacaacttataatcaattcttgacatggaaagatattagccttagtagattaaatgtttgtttgattacatggattagtaactgtttgaacacattaaacaaaagcttaggcttaagatgtggattcaataatgttatcttgacacaattattcctttatggagattgtatactaaaactattccacaatgaggggttctacataataaaagaggtagagggatttattatgtctctaattttaaatataacagaagaagatcaattcagaaaacggttttataatagtatgctcaacaacatcacagatgccgccaacaaagctcaaaaaaatctgctatcaagagtatgtcatacattattagataagacaatatcagataatataataaatggcagatggataattctattgagtaagttcctaaaattaattaagcttgcaggtgacaataacctcaacaatctgagtgaattatattttttgttcagaatatttggacacccaatggtagatgaaagacaagccatggatgctgttaaagttaattgcaacgagaccaaattttatttgttaagtagtttgagtatgttaagaggagcttttatatatagaattataaaagggtttgtaaataattacaacagatggcctactttaagaaatgccattgtcttacccttaagatggttaacttactataaactaaacacttatccttccttgttggaacttacagaaagagatttgattgttctatcaggactacgtttctatcgagagtttcggttgcctaaaaaagtggatcttgaaatgatcataaatgataaggctatatcacctcctaaaaatttaatatggactagtttccctagaaattatatgccgtcacacatacaaaattatatagaacatgaaaaattaaaattctctgatagtgataaatcaagaagagtattagagtattatttaagagataacaaattcaatgaatgtgatttacacaactgtgtagttaatcaaagttatcttaacaacccgaatcatgtggtatcattgacaggcaaagaaagagaactcagtgtaggtagaatgtttgcaatgcaaccaggaatgttcagacaagttcaaatattagcagagaaaatgatagcagaaaacatattacaatttttccctgaaagtcttacaagatatggtgatctagaactacagaaaatattagaattgaaagcaggaataagtaacaaatcaaatcgttacaatgataattacaacaattacattagtaagtgctctatcatcacagatctcagcaaattcaatcaagcatttcgatatgaaacatcatgtatttgtagtgatgtactggatgaactgcatggtgtacaatctctattttcctggttacatttaactattcctcatgtcacaataatatgcacatataggcatgcacccccctatataaaggatcatattgtagatcttaacaatgtagatgagcaaagtggactatatagatatcatatgggtggtatcgaagggtggtgtcaaaaactatggaccatagaagctatatcactattagatctaatatctctcaaagggaaattctcaattactgctttaattaatggtgacaatcaatcaatagatataagtaaaccagtcagactcatggaaggtcaaactcatgctcaagcagattatttgctagcattaaatagtctcaaattactgtataaagagtatgcaggaataggccacaaattaaaaggaactgagacttatatatcgagagatatgcaatttatgagtaaaacgatccaacataacggtgtatattacccagctagtataaagaaagtcctaagagtgggaccgtggataaacactatacttgatgacttcaaagtgagtctagaatctataggtagtttgacacaagaattagaatatagaggtgaaagtctattatgcagtttaatatttagaaatgtatggttatataatcaaattgcattacaacttaaaaatcatgcattatgtaacaacaaattatatttggatatattaaaagttctaaaacacttaaaaaccttttttaatcttgataacattgatacagcattaacattgtatatgaatttgcccatgttatttggtggtggtgatcccaacttgttatatcgaagtttctatagaagaactcctgatttcctcacagaggctatagttcactctgtgttcatacttagttattatacaaaccatgatttaaaagataaacttcaagatctgtcagatgatagattgaataagttcttaacatgcataatcacgtttgataaaaaccccaatgctgaattcgttacattgatgagagatcctcaagctttaggatctgagaggcaagctaaaattactagcgaaatcaatagactggcagttaccgaggttttgagcacagctccaaacaaaatattttccaaaagtgcacaacactataccactacagagatagatcttaatgatattatgcaaaatatagaacctacatatcctcacgggctaagagttgtttatgagagtttacccttttataaagcagagaaaatagtaaatcttatatccggtacaaaatctataactaacatactggaaaagacttctgccatagacttaacagatattgatagagccactgagatgatgaggaaaaacataactttgcttataaggatattaccattagattgtaacagagataaaagagaaatattgagtatggaaaacctaagtattactgaattaagcaaatacgttagagaaagatcttggtctttatccaatatagttggtgttacatcacccagtatcatgtatacaatggacataaaatatacaacaagcactatagctagtggcataatcatagagaaatataatgtcaacagtttaacacgtggtgagagaggacccactaaaccatgggttggttcatctacacaagagaaaaagacaatgccagtttataatagacaagttttaaccaaaaaacagagagatcaaatagatctattagcaaaattggattgggtgtatgcatctatagataacaaggatgaatttatggaggaacttagcataggaactcttgggttaacatatgagaaggccaaaaaattattcccacaatatttgagtgttaactatttgcatcgtcttacagtcagtagtagaccatgtgaattccctgcatctataccagcttatagaactacaaattatcactttgatactagccctattaatcgcatattaacagaaaagtatggtgatgaagatattgatatagtattccaaaactgtataagctttggccttagcttaatgtctgtagtagaacaatttactaatgtatgtcctaacagaattattctcatacccaagcttaatgagatacatttgatgaaacctcccatattcacaggcgatgttgatattcacaagttaaaacaagtgatacaaaaacaacatatgtttttaccagacaaaataagtttgactcaatatgtggaattattcttaagtaataaaacactcaaatctggatctaatgttaattctaatttaatattggcgcataagatatctgactattttcataatacttacattttgagtactaatttagctggacattggattcttattatacaacttatgaaagattctaagggtatttttgaaaaagattggggagagggatatataactgatcatatgttcattaatttgaaagttttcttcaatgcttataagacatatctcttgtgttttcataaaggttacggcagagcaaagctggagtgtgatatgaatacttcagatctcctatgtgtattggaattaatagacagtagttattggaagtctatgtctaaggtgtttttagaacaaaaagttatcaaatacattcttagccaggatgcaagtttacatagagtaaaaggatgtcatagcttcaaactatggtttcttaaacgtcttaatgtagcagaattcacagtttgcccttgggttgttaacatagattatcatccaacacatatgaaagcaatattaacttatattgatcttgttagaatgggattgataaatatagatagaatatacattaaaaataaacacaagttcaatgatgagttttatacttctaatctgttttacattaattataacttctcagataatactcatctattaactaaacatataaggattgctaattccgaattagaaagtaattacaacaaattatatcatcctacaccagaaaccctagaaaatatactaaccaatccggttaaaagtaatgagaaaaagacactgagtgactattgtataggtaaaaatgttgactcaataatgttaccatcgttatctaataagaagcttattaaatcgtctacaatgattagaaccaattacagcagacaagatttgtataatttatttcctacggttgtgattgataaaattatagatcattcaggtaatacagccaaatctaaccaactttacactactacttctcatcaaatatccttagtgcacaatagcacatcactttattgcatgcttccttggcatcatattaatagattcaattttgtatttagttctacaggttgtaaaattagtatagagtatattttaaaagatcttaaaattaaggatcctaattgtatagcattcataggtgaaggagcagggaatttattattgcgtacagtagtggaacttcatcctgatataagatatatttacagaagtctgaaagattgcaatgatcatagtttaccaattgagtttttaaggctgtacaatggacatatcaacattgattatggtgaaaatttgaccattcctgctacagatgcaaccaacaacattcattggtcttatttacatataaagtttgctgaacctatcagtctttttgtctgtgatgctgaattgcctgtaacagtcaactggagtaagattataatagagtggagcaagcatgtaagaaaatgcaagtactgttcttcagttaataaatgtacattgatagtaaaatatcatgctcaagatgatatcgatttcaaattagacaacataactatattaaaaacttatgtatgcttaggtagtaagttaaagggatctgaagtttacttagtccttacaataggtcctgcaaatgtgttcccagtatttaatgtagtacaaaatgctaaattgatactatcaagaactaaaaatttcatcatgcctaaaaaagctgataaagagtctattgatgcaaatattaagagtttgataccctttctttgttaccctataacaaaaaaaggaattaatactgcattgtctaaattaaagagtgttgttagtggagatatactatcatattctatagctggacgtaatgaagttttcagcaataaacttataaatcataagcatatgaacatcttaaagtggttcaatcatgttttaaatttcagatcaacagaattaaactataatcatttatatatggtagaatctacttatcctcatctaagtgaattgttaaacagcttgacaaccaatgaacttaaaaaactgattaaaatcacaggtagtttgttatacaacttttataatgaataatgagcaaaaatcttataacaaaaatagctacacactaacattgtattcaattatagttattgaaaattaataattatataatttttaataacttctagtgaactaatcctaaaattatcattttgatctaggaagaataagtttaaatccaaatctaattggtttatatgtatattaactaaattacgagatattagtttttgacactttttttctcgt

SEQ ID NO: 2 - protein, 514 aa, synthetic construct
  REGION 1..514: note = Chimeric G protein of Vesicular stomatitis Indiana virus
MKCLLYLAFLFIGVNCKFTIVFPHNQKGNWKNVPSNYHYCPSSSDLNWHNDLIGTALQVKMPKSHKAIQADGWMCHASKWVTTCDFRWYGPKYITHSIRSFTPSVEQCKESIEQTKQGTWLNPGFPPQSCGYATVTDAEAVIVQVTPHHVLVDEYTGEWVDSQFINGKCSNYICPTVHNSTTWHSDYKVKGLCDSNLISMDITFFSEDGELSSLGKEGTGFRSNYFAYETGGKACKMQYCKHWGVRLPSGVWFEMADKDLFAAARFPECPEGSSISAPSQTSVDVSLIQDVERILDYSLCQETWSKIRAGLPISPVDLSYLAPKNPGTGPAFTIINGTLKYFETRYIRVDIAAPILSRMVGMISGTTTERELWDDWAPYEDVEIGPNGVLRTSSGYKFPLYMIGHGMLDSDLHLSSKAQVFEHPHIQDAASQLPDDESLFFGDTGLSKNPIELVEGWFSSWKSSIASFFFIIGLIIGLFLVLRVGIHLCIKARSTPVTLSKDQLSGINNIAFSN

SEQ ID NO: 3 - DNA, 1545 bp, synthetic construct
  misc_feature 1..1545: note = cDNA encoding a Chimeric G protein of Vesicular stomatitisIndiana virus
  source 1..1545: mol_type = other DNA
atgaagtgccttttgtacttagcctttttattcattggggtgaattgcaagttcaccatagtttttccacacaaccaaaaaggaaactggaaaaatgttccttctaattaccattattgcccgtcaagctcagatttaaattggcataatgacttaataggcacagccttacaagtcaaaatgcccaagagtcacaaggctattcaagcagacggttggatgtgtcatgcttccaaatgggtcactacttgtgatttccgctggtatggaccgaagtatataacacattccatccgatccttcactccatctgtagaacaatgcaaggaaagcattgaacaaacgaaacaaggaacttggctgaatccaggcttccctcctcaaagttgtggatatgcaactgtgacggatgccgaagcagtgattgtccaggtgactcctcaccatgtgctggttgatgaatacacaggagaatgggttgattcacagttcatcaacggaaaatgcagcaattacatatgccccactgtccataactctacaacctggcattctgactataaggtcaaagggctatgtgattctaacctcatttccatggacatcaccttcttctcagaggacggagagctatcatccctgggaaaggagggcacagggttcagaagtaactactttgcttatgaaactggaggcaaggcctgcaaaatgcaatactgcaagcattggggagtcagactcccatcaggtgtctggttcgagatggctgataaggatctctttgctgcagccagattccctgaatgcccagaagggtcaagtatctctgctccatctcagacctcagtggatgtaagtctaattcaggacgttgagaggatcttggattattccctctgccaagaaacctggagcaaaatcagagcgggtcttccaatctctccagtggatctcagctatcttgctcctaaaaacccaggaaccggtcctgctttcaccataatcaatggtaccctaaaatactttgagaccagatacatcagagtcgatattgctgctccaatcctctcaagaatggtcggaatgatcagtggaactaccacagaaagggaactgtgggatgactgggcaccatatgaagacgtggaaattggacccaatggagttctgaggaccagttcaggatataagtttcctttatacatgattggacatggtatgttggactccgatcttcatcttagctcaaaggctcaggtgttcgaacatcctcacattcaagacgctgcttcgcaacttcctgatgatgagagtttattttttggtgatactgggctatccaaaaatccaatcgagcttgtagaaggttggttcagtagttggaaaagctctattgcctcttttttctttatcatagggttaatcattggactattcttggttctccgagttggtatccatctttgcattaaagccagaagcacaccagtcacattaagtaaggatcaactgagtggtataaataatattgcatttagtaactaa

SEQ ID NO: 4 - DNA, 1869 bp, synthetic construct
  misc_feature 1..1869: note = G/F inter-gene - F 5UTR - preF ectodomain-foldon fusion gene - F3UTR
  source 1..1869: mol_type = other DNA
gtattgttgcaaaaagccatgaccaaatcaaacagaatcaaaatcaactctggggcaaataacaatggagttgccaatcctcaaaacaaatgctattaccacaatccttgctgcagtcacactctgtttcgcttccagtcaaaacatcactgaagaattttatcaatcaacatgcagtgcagtcagcaaaggctatcttagtgctctaagaactggttggtatactagtgttataactatagaattaagtaatatcaaggaaaataagtgtaatggtacagacgctaaggtaaaattaataaaacaagaattagataaatataaaaatgctgtaacagaattgcagttgctcatgcaaagcacaccagcagccaacaatcgagccagaagagaactaccaagatttatgaattatacactcaacaataccaaaaacaccaatgtaacattaagtaagaaaaggaaaagaagatttcttggatttttgttaggtgttggatctgcaatcgccagtggcattgccgtatccaaggtcctgcacctagaaggggaagtgaacaaaatcaaaagtgctctactatccacaaacaaggctgtagtcagcttatctaatggagtcagtgtcttaaccagcaaggtgttagacctcaaaaactatatagataaacagttgttacctattgttaacaagcaaagctgcagcatatcaaacattgaaactgtgatagagttccaacaaaagaacaacagactactagagattaccagagaatttagtgttaatgcaggtgtaactactcctgtaagcacttatatgttaactaatagtgagttattatcattaatcaatgatatgcctataacaaatgatcagaaaaagttaatgtccagcaatgttcaaatagttagacagcaaagttactctatcatgtcaataataaaagaggaagtcttggcatatgtagtacaattaccactatatggtgtaatagatactccttgttggaaactacacacatcccctttatgtacaaccaacacaaaggaaggatccaacatctgcttaacaagaaccgacagaggatggtactgtgacaatgcaggatcagtatcctttttcccacaagctgaaacatgtaaagttcaatcgaatcgggtgttttgtgacacaatgaacagtttaacattaccaagtgaggtaaatctctgcaacattgacatattcaaccccaaatatgattgcaaaattatgacttcaaaaacagatgtaagcagctccgttatcacatctctaggagccattgtgtcatgctatggcaaaaccaaatgtacagcatccaataaaaatcgtgggatcataaagacattctctaacgggtgtgattatgtatcaaataagggggtggatactgtgtctgtaggtaatacattatattatgtaaataagcaagaaggcaaaagtctctatgtaaaaggtgaaccaataataaatttctatgatccattagtgttcccctctctcctgtgggatgcatcaatatctcaagtcaatgagaaaattaatcagagtctagcatttatccgtaaatcagatgaattattaggctctggcggaagcggatacatccctgaggcaccaagggacggacaggcctacgtgcgcaaggatggcgagtgggtgctgctgtccacctttctgtgaataaaaatagcacctaatcatattcttacaatggttcgctatttgaccatagataacccatctatcattagattatcctaaaatttgaacttcatcacaactttcatctataaaccatctcacttacactttttaagtagatttctattttatagttatataaaaca

SEQ ID NO: 5 - DNA, 1887 bp, synthetic construct
  misc_feature 1..1887: note = Single chain PreF
  source 1..1887: mol_type = other DNA
gtattgttgcaaaaagccatgaccaaatcaaacagaatcaaaatcaactctggggcaaataacaatggagttgccaatcctcaaaacaaatgctattaccacaatccttgctgcagtcacactctgtttcgcttccagtcaaaacatcactgaagaattttatcaatcaacatgcagtgcagtcagcaaaggctatcttagtgctctaagaactggttggtatactagtgttataactatagaattaagtaatatcaaggaaaataagtgtaatggtacagacgctaaggtaaaattaataaaacaagaattagataaatataaaaatgctgtaacagaattgcagttgctcatgcaaagcacaccagcagccaacaatggagccagaggctctggcggaagcggacttggatttttgttaggtgttggatctgcaatcgccagtggcattgccgtatccaaggtcctgcacctagaaggggaagtgaacaaaatcaaaagtgctctactatccacaaacaaggctgtagtcagcttatctaatggagtcagtgtcttaaccagcaaggtgttagacctcaaaaactatatagataaacagttgttacctattgttaacaagcaaagctgcagcatatcaaacattgaaactgtgatagagttccaacaaaagaacaacagactactagagattaccagagaatttagtgttaatgcaggtgtaactactcctgtaagcacttatatgttaactaatagtgagttattatcattaatcaatgatatgcctataacaaatgatcagaaaaagttaatgtccagcaatgttcaaatagttagacagcaaagttactctatcatgtcaataataaaagaggaagtcttggcatatgtagtacaattaccactatatggtgtaatagatactccttgttggaaactacacacatcccctttatgtacaaccaacacaaaggaaggatccaacatctgcttaacaagaaccgacagaggatggtactgtgacaatgcaggatcagtatcctttttcccacaagctgaaacatgtaaagttcaatcgaatcgggtgttttgtgacacaatgaacagtttaacattaccaagtgaggtaaatctctgcaacattgacatattcaaccccaaatatgattgcaaaattatgacttcaaaaacagatgtaagcagctccgttatcacatctctaggagccattgtgtcatgctatggcaaaaccaaatgtacagcatccaataaaaatcgtgggatcataaagacattctctaacgggtgtgattatgtatcaaataagggggtggatactgtgtctgtaggtaatacattatattatgtaaataagcaagaaggcaaaagtctctatgtaaaaggtgaaccaataataaatttctatgatccattagtgttcccctctgatgaatttgatgcatcaatatctcaagtcaatgagaaaattaatcagagtctagcatttatccgtaaatcagatgaattattacataatgtaaatgctggtaaatccaccacaaatatcatgataactaccataattatagtaattatagtaatattgttagcattaattgcagttggactgcttctatactgcaaggccagaagcacaccagtcacattaagtaaggatcaactgagtggtataaataatattgcatttagtaactgaataaaaatagcacctaatcatattcttacaatggttcgctatttgaccatagataacccatctatcattagattatcctaaaatttgaacttcatcacaactttcatctataaaccatctcacttacactttttaagtagatttctattttatagttatataaaaca

SEQ ID NO: 6 - DNA, 16912 bp, synthetic construct
  misc_feature 1..16912: note = Modified RSV anti-genome with chimeric VSV G protein inserted
  source 1..16912: mol_type = other DNA
acgcgaaaaaatgcgtacaacaaacttgcgtaaaccaaaaaaatggggcaaataagaatttgataagtaccacttaaatttaactcctttggttagaggcgcgccatgggcagcaactcattgagtatgataaaagttagattgcaaaatctgtttgacaatgatgaagtagcattgttaaaaataacatgctatactgacaaattaatacagttaactaatgctttggctaaggcagttatacatacaatcaaattgaatggcattgtatttgtgcatgttattacaagtagtgatatttgccctaataataatattgtagtgaaatccaatttcacaacaatgccagtattacaaaatggaggttatatatgggaaatgatggaattaacacactgctctcaacctaatggcctaatagatgacaattgtgaaattaaattctccaaaaaactaagtgattcaacaatgaccaattatatgaatcaattatctgaattacttggatttgacctcaatccataaatcataataaatatcaactagcaaatcaatgtcactaacaccattagttaatataaaacttgacagaagataaaaatggggcaaataaatcaattcagccgacccaaccatggacacaacacacaatgataccacaccacaaagactgatgatcacagacatgaggccattatcgcttgagactataataacatctctaaccagagatatcataacacataaatttatatacttgataaatcatgaatgcatagtaagaaaacttgatgaaagacaggccacatttacatttctggtcaactatgaaatgaaactattgcacaaagtgggaagcactaaatataaaaaatatactgaatacaacacaaaatatggcactttccctatgccaatatttatcaatcatgatgggttcttagaatgcattggcattaagcctaccaagcacacacccataatatacaagtatgatctcaatccatgaatatcaaaccaagattcaaacaatccgaaataacaactttatgcataatcacactccatagtccaaatggagcctgaaaattatagttatttaaaattcctgcaggaaggagagacataagatgaaagatggggcaaatacaaaaatggctcttagcaaagtcaagttgaatgatacactcaacaaagatcaacttctatcatccagcaaatataccatccaacggagcacaggagacagcattgacactcctaattatgatgtgcagaaacacattaataagttatgtggcatgttattaatcacagaagatgctaatcataaattcactgggttaataggtatgttatatgctatgtctagattaggaagagaagacaccataaaaatactcaaagatgcgggatatcatgttaaggcaaatggagtggatgtaacaacacatcgtcaagacattaatgggaaagaaatgaaatttgaagtgttaacattagcaagcttaacaactgaaattcaaatcaacattgagatagaatctagaaaatcctacaaaaaaatgctaaaagaaatgggagaggtggctccagaatacaggcatgactctcctgattgtgggatgataatattatgtatagcggcattagtaataaccaaattagcagcaggagatagatcaggtcttacagctgtgattaggagagctaataatgtcctaaaaaatgaaatgaaacgttataaaggtttattacccaaggatatagccaacagcttctatgaagtgtttgaaaaatatcctcactttatagatgtttttgttcattttggtatagcacaatcttctaccagaggtggcagtagagttgaagggatttttgcaggattgtttatgaatgcctatggtgcagggcaagtgatgttacggtggggggtcttagcaaaatcagttaaaaacattatgttaggacacgctagtgtacaagcagaaatggaacaagttgtggaggtgtatgagtatgctcagaaattgggtggagaagcaggattctaccatatattgaacaacccaaaagcatcactattatctttgactcaatttcctcacttctctagtgtagtattgggcaatgctgctggcctaggcataatgggagaatacagaggtacaccaaggaatcaagatttatatgatgctgcaaaagcatatgctgaacaactcaaagaaaatggtgtgattaactacagtgtattagatttgacagcagaagaactagaggctatcaaacatcagcttaatccaaaagataatgatgtagagctttgagttaataaaaaagtggggcaaataaatcatcatggaaaagtttgctcctgaattccatggagaagatgcaaacaacagagccaccaaattcctagaatcaataaagggcaaattcacatcacccaaagatcccaagaaaaaagatagtatcatatctgtcaactcaatagatatagaagtaaccaaagaaagccctataacatcaaattcaaccattataaacccaataaatgagacagatgatactgtagggaacaagcccaattatcaaagaaagcctctagtaagtttcaaagaagaccctacgccaagtgataatcctttttcaaaactatacaaagaaaccatagaaacatttgataacaatgaagaagaatctagctattcatatgaagaaataaatgatcagacaaacgataatataacagcaagattagataggattgatgagaaattaagtgaaatactaggaatgcttcacacattagtagtagcgagtgcaggacccacatctgctcgggatggtataagagatgccatggttggtttaagagaagaaatgatagaaaaaatcagaactgaagcattaatgaccaatgacagactagaagctatggcaagactcaggaatgaagaaagtgaaaagatggcaaaagacacatcagatgaagtgtctctcaatccaacatcagagaaactgaacaacctgttggaagggaatgatagtgacaatgatctatcacttgaagatttctgattagctaccaaactgtacatcaaaacacaacaccaatagaaaaccaacaaacaaaccaactcacccatccaaccaaacatctatctgctgattagccaaccagccaaaaaacaaccagccaatctaaaactagccacccggaaaaaatcgatactatagttacaaaaaaagatggggcaaatatggaaacatacgtgaataaacttcacgagggctccacatacacagctgctgttcaatacaatgtcctagaaaaagacgatgatcctgcatcacttacaatatgggtgcccatgttccaatcatccatgccagcagatctactcataaaagaactagccaatgtcaatatactagtgaaacaaatatccacacccaagggaccctcattaagagtcatgataaactcaagaagtgcagtgctagcacaaatgcccagcaaatttaccatatgtgccaatgtgtccttggatgaaagaagcaagctggcatatgatgtaaccacaccctgtgaaattaaggcatgcagtctaacatgcctaaaatcaaaaaatatgttaactacagttaaagatctcactatgaaaacactcaacccaacacatgacatcattgctttatgtgaatttgaaaatatagtaacatcaaaaaaagtcataataccaacatacctaagatctatcagcgtcagaaataaagatctgaacacacttgaaaatataacaaccactgaattcaaaaatgccattacaaatgcaaaaatcatcccttactcaggattattgttagtcatcacagtgactgacaacaaaggagcattcaaatacataaagccacaaagtcaattcatagtagatcttggagcttacctagaaaaagaaagtatatattatgttacaacaaattggaagcacacagctacacgatttgcaatcaaacccatggaagattaacctttttcctctacatcaatgagtagattcatacaaactttctaactacattcttcacttcacaatcataatcaccaaccctctgtggttcaatcaatcaaacaaaactcatcaagagttccagatcatcccaagtcattgttcatcagatccagtactcaaataagttaataaaaaatccacatggggcaaataatcattgagggaaatccaactaatcacaacatctgtcaacatagacaagtcaacacgctagataaaatcaaccaatggaaaatacatccataactatagaattctcaagcaaattctggccttactttacactaatacacatgataacaacaataatctctttgataatcataatctccatcatgattgcaatactaaacaaactctgcgaatataatgtattccataacaaaacctttgagctaccaagagctcgagtcaatacatagcattcaccaatctgatagctcaaaacagtaaccttgcatttgtaaatgaactaccctcacttcttcacaaaaccacatcaacatctcaccatgcaagccatcatctataccataaagtagttaattaaaaatggccggccttgacagaagataaaaatggggcaaatgcaaacatgaagtgccttttgtacttagcctttttattcattggggtgaattgcaagttcaccatagtttttccacacaaccaaaaaggaaactggaaaaatgttccttctaattaccattattgcccgtcaagctcagatttaaattggcataatgacttaataggcacagccttacaagtcaaaatgcccaagagtcacaaggctattcaagcagacggttggatgtgtcatgcttccaaatgggtcactacttgtgatttccgctggtatggaccgaagtatataacacattccatccgatccttcactccatctgtagaacaatgcaaggaaagcattgaacaaacgaaacaaggaacttggctgaatccaggcttccctcctcaaagttgtggatatgcaactgtgacggatgccgaagcagtgattgtccaggtgactcctcaccatgtgctggttgatgaatacacaggagaatgggttgattcacagttcatcaacggaaaatgcagcaattacatatgccccactgtccataactctacaacctggcattctgactataaggtcaaagggctatgtgattctaacctcatttccatggacatcaccttcttctcagaggacggagagctatcatccctgggaaaggagggcacagggttcagaagtaactactttgcttatgaaactggaggcaaggcctgcaaaatgcaatactgcaagcattggggagtcagactcccatcaggtgtctggttcgagatggctgataaggatctctttgctgcagccagattccctgaatgcccagaagggtcaagtatctctgctccatctcagacctcagtggatgtaagtctaattcaggacgttgagaggatcttggattattccctctgccaagaaacctggagcaaaatcagagcgggtcttccaatctctccagtggatctcagctatcttgctcctaaaaacccaggaaccggtcctgctttcaccataatcaatggtaccctaaaatactttgagaccagatacatcagagtcgatattgctgctccaatcctctcaagaatggtcggaatgatcagtggaactaccacagaaagggaactgtgggatgactgggcaccatatgaagacgtggaaattggacccaatggagttctgaggaccagttcaggatataagtttcctttatacatgattggacatggtatgttggactccgatcttcatcttagctcaaaggctcaggtgttcgaacatcctcacattcaagacgctgcttcgcaacttcctgatgatgagagtttattttttggtgatactgggctatccaaaaatccaatcgagcttgtagaaggttggttcagtagttggaaaagctctattgcctcttttttctttatcatagggttaatcattggactattcttggttctccgagttggtatccatctttgcattaaagccagaagcacaccagtcacattaagtaaggatcaactgagtggtataaataatattgcatttagtaactaatagtcattaaaaagcggccggccagtcataacaatgaactaggatattaagaccaaaaacaacgctggggcaaatgcaaacatgtccaaaaccgaggaccaacgcaccgccaagacactagaaaggacctgggacacttttaatcatctattattcatatcatcgtgcttatacaagttaaatcttaaatctatagcacaaatcacattatctattttggcaattataatctcaacctcacttataattgcagccatcatattcatagcctcggcaaaccacaaagtcacactaacaactgcaatcatacaagatgcaacgaaccagatcaagaacacaaccccaacatacctcacccagaatccccagcatggaatcagcttctccaatctgtccggaactacatcacaatccaccaccatactagcttcaacaacaccaagtgctgattcaaccccacaatccacaacagtcaagatcaaaaacacaacaacaacccaaatattacctagcaaacccaccacaaaacaacgccaaaataaaccacaaaacaaacccaacaatgattttcactttgaagtgttcaattttgtaccctgcagcatatgcagcaacaatccaacctgctgggccatctgcaagagaataccaaacaaaaaacctggaaagaaaaccaccaccaagcccacaaaaaaaccaaccctcaagacaaccaaaaaagatcccaaatcccaaaccacaaaaccaaaggaagtactcactaccaagcctacaggaaagccaaccatcaacaccactaaaacaaacatcagaactacactgctcacctccaacaccaaaggaaatccagaacacacaagtcaagaggaaaccctccactcaaccacctccgaaggctatccaagcccatcacaagtccacacaacatccggtcaagaggaaaccctccactcaaccacctccgaaggctatccaagcccatcacaagtctacacaacatccgagtacctatcacaatctctatcttcatccaacacaacaaaatgatagtcattaaaaagcacgcgtgtattgttgcaaaaagccatgaccaaatcaaacagaatcaaaatcaactctggggcaaataacaatggagttgccaatcctcaaaacaaatgctattaccacaatccttgctgcagtcacactctgtttcgcttccagtcaaaacatcactgaagaattttatcaatcaacatgcagtgcagtcagcaaaggctatcttagtgctctaagaactggttggtatactagtgttataactatagaattaagtaatatcaaggaaaataagtgtaatggtacagacgctaaggtaaaattaataaaacaagaattagataaatataaaaatgctgtaacagaattgcagttgctcatgcaaagcacaccagcagccaacaatcgagccagaagagaactaccaagatttatgaattatacactcaacaataccaaaaacaccaatgtaacattaagtaagaaaaggaaaagaagatttcttggatttttgttaggtgttggatctgcaatcgccagtggcattgccgtatccaaggtcctgcacctagaaggggaagtgaacaaaatcaaaagtgctctactatccacaaacaaggctgtagtcagcttatctaatggagtcagtgtcttaaccagcaaggtgttagacctcaaaaactatatagataaacagttgttacctattgttaacaagcaaagctgcagcatatcaaacattgaaactgtgatagagttccaacaaaagaacaacagactactagagattaccagagaatttagtgttaatgcaggtgtaactactcctgtaagcacttatatgttaactaatagtgagttattatcattaatcaatgatatgcctataacaaatgatcagaaaaagttaatgtccagcaatgttcaaatagttagacagcaaagttactctatcatgtcaataataaaagaggaagtcttggcatatgtagtacaattaccactatatggtgtaatagatactccttgttggaaactacacacatcccctttatgtacaaccaacacaaaggaaggatccaacatctgcttaacaagaaccgacagaggatggtactgtgacaatgcaggatcagtatcctttttcccacaagctgaaacatgtaaagttcaatcgaatcgggtgttttgtgacacaatgaacagtttaacattaccaagtgaggtaaatctctgcaacattgacatattcaaccccaaatatgattgcaaaattatgacttcaaaaacagatgtaagcagctccgttatcacatctctaggagccattgtgtcatgctatggcaaaaccaaatgtacagcatccaataaaaatcgtgggatcataaagacattctctaacgggtgtgattatgtatcaaataagggggtggatactgtgtctgtaggtaatacattatattatgtaaataagcaagaaggcaaaagtctctatgtaaaaggtgaaccaataataaatttctatgatccattagtgttcccctctgatgaatttgatgcatcaatatctcaagtcaatgagaaaattaatcagagtctagcatttatccgtaaatcagatgaattattacataatgtaaatgctggtaaatccaccacaaatatcatgataactaccataattatagtaattatagtaatattgttagcattaattgcagttggactgcttctatactgcaaggccagaagcacaccagtcacattaagtaaggatcaactgagtggtataaataatattgcatttagtaactgaataaaaatagcacctaatcatattcttacaatggttcgctatttgaccatagataacccatctatcattagattatcctaaaatttgaacttcatcacaactttcatctataaaccatctcacttacactttttaagtagatttctattttatagttatataaaacagggcccattgaataccaaattaacttactatttgtaaaaatgagaattggggcaaatatgtcacgaaggaatccttgcaaattcgaaattcgaggtcattgcttgaatggtaaaaggtgtcattttagtcataattattttgaatggccaccccatgcactgcttgtaagacaaaactttatgttaaacagaatacttaagtctatggataaaagcatagatactttgtcagaaataagtggagctgcagagttggacagaacagaagagtatgccctcggtgtagttggagtgctagagagttatataggatcaataaataatataactaaacaatcagcatgtgttgccatgagcaaactccttactgaactcaacagcgatgacatcaaaaaactaagggacaatgaagagccaaactcacccaaagtaagagtgtacaatactgtcatatcatatattgaaagcaacaggaagaacaataaacaaactatccatctgttaaaaagattgccagcagacgtattgaagaaaaccatcaaaaacacattggatatccacaagagcataaccatcaataacccaaaagaatcaactgttagtgatacgaacgaccatgccaaaaataatgatactacctgacaaatatccttgtagtataaattccatactaataacaagtaattgtagagtcactatgtataatcaaaaaaacacactatatatcaatcaaaacaaccaaaatagccatatatacccaccggatcaaccattcaatgaaatccattggacctctcaagacttgattgatgcaactcaaaattttctacaacatctaggtattactgatgatatatacacaatatatatattagtgtcataatactcaatcctaatacttaccacatcatcaaattattaactcaaacaattcaagctatgggacaaaatggatcccattattagtggaaattctgctaatgtttatctaactgatagttatttaaaaggtgttatttctttctcagaatgtaacgctttaggaagttacatattcaatggtccttatctcaaaaatgattataccaacttaattagtagacaaaatccattaatagaacacataaatctaaagaaactaaatataacacagtccttaatatctaagtatcataaaggtgaaataaaaatagaagaacctacttactttcagtcattacttatgacatacaagagtatgacctcttcagaacagactactactactaatttacttaaaaagataataagaagagctatagaaatcagtgatgtcaaagtctatgctatattgaataaactggggctcaaagaaaaagacaagattaaatccaataatggacaagatgaagacaactcagtcattactaccataatcaaagatgatatacttttagctgtcaaggataatcaatctcatcttaaagcagacaaaaatcaatccacaaaacaaaaagatacaatcaaaacaacacttttgaagaaattaatgtgttcgatgcaacatcctccatcatggttaatacattggtttaatttatacacaaaattaaacagcatattaacacaatatcgatctagtgaggtaaaaaaccatggttttatattgatagataatcatactcttagtggattccaatttattttgaatcaatatggttgtatagtttatcataaggaactcaaaagaattactgtgacaacttataatcaattcttgacatggaaagatattagccttagtagattaaatgtttgtttgattacatggattagtaactgtttgaacacattaaacaaaagcttaggcttaagatgtggattcaataatgttatcttgacacaattattcctttatggagattgtatactaaaactattccacaatgaggggttctacataataaaagaggtagagggatttattatgtctctaattttaaatataacagaagaagatcaattcagaaaacggttttataatagtatgctcaacaacatcacagatgccgccaacaaagctcaaaaaaatctgctatcaagagtatgtcatacattattagataagacaatatcagataatataataaatggcagatggataattctattgagtaagttcctaaaattaattaagcttgcaggtgacaataacctcaacaatctgagtgaattatattttttgttcagaatatttggacacccaatggtagatgaaagacaagccatggatgctgttaaagttaattgcaacgagaccaaattttatttgttaagtagtttgagtatgttaagaggagcttttatatatagaattataaaagggtttgtaaataattacaacagatggcctactttaagaaatgccattgtcttacccttaagatggttaacttactataaactaaacacttatccttccttgttggaacttacagaaagagatttgattgttctatcaggactacgtttctatcgagagtttcggttgcctaaaaaagtggatcttgaaatgatcataaatgataaggctatatcacctcctaaaaatttaatatggactagtttccctagaaattatatgccgtcacacatacaaaattatatagaacatgaaaaattaaaattctctgatagtgataaatcaagaagagtattagagtattatttaagagataacaaattcaatgaatgtgatttacacaactgtgtagttaatcaaagttatcttaacaacccgaatcatgtggtatcattgacaggcaaagaaagagaactcagtgtaggtagaatgtttgcaatgcaaccaggaatgttcagacaagttcaaatattagcagagaaaatgatagcagaaaacatattacaatttttccctgaaagtcttacaagatatggtgatctagaactacagaaaatattagaattgaaagcaggaataagtaacaaatcaaatcgttacaatgataattacaacaattacattagtaagtgctctatcatcacagatctcagcaaattcaatcaagcatttcgatatgaaacatcatgtatttgtagtgatgtactggatgaactgcatggtgtacaatctctattttcctggttacatttaactattcctcatgtcacaataatatgcacatataggcatgcacccccctatataaaggatcatattgtagatcttaacaatgtagatgagcaaagtggactatatagatatcatatgggtggtatcgaagggtggtgtcaaaaactatggaccatagaagctatatcactattagatctaatatctctcaaagggaaattctcaattactgctttaattaatggtgacaatcaatcaatagatataagtaaaccagtcagactcatggaaggtcaaactcatgctcaagcagattatttgctagcattaaatagtctcaaattactgtataaagagtatgcaggaataggccacaaattaaaaggaactgagacttatatatcgagagatatgcaatttatgagtaaaacgatccaacataacggtgtatattacccagctagtataaagaaagtcctaagagtgggaccgtggataaacactatacttgatgacttcaaagtgagtctagaatctataggtagtttgacacaagaattagaatatagaggtgaaagtctattatgcagtttaatatttagaaatgtatggttatataatcaaattgcattacaacttaaaaatcatgcattatgtaacaacaaattatatttggatatattaaaagttctaaaacacttaaaaaccttttttaatcttgataacattgatacagcattaacattgtatatgaatttgcccatgttatttggtggtggtgatcccaacttgttatatcgaagtttctatagaagaactcctgatttcctcacagaggctatagttcactctgtgttcatacttagttattatacaaaccatgatttaaaagataaacttcaagatctgtcagatgatagattgaataagttcttaacatgcataatcacgtttgataaaaaccccaatgctgaattcgttacattgatgagagatcctcaagctttaggatctgagaggcaagctaaaattactagcgaaatcaatagactggcagttaccgaggttttgagcacagctccaaacaaaatattttccaaaagtgcacaacactataccactacagagatagatcttaatgatattatgcaaaatatagaacctacatatcctcacgggctaagagttgtttatgagagtttacccttttataaagcagagaaaatagtaaatcttatatccggtacaaaatctataactaacatactggaaaagacttctgccatagacttaacagatattgatagagccactgagatgatgaggaaaaacataactttgcttataaggatattaccattagattgtaacagagataaaagagaaatattgagtatggaaaacctaagtattactgaattaagcaaatacgttagagaaagatcttggtctttatccaatatagttggtgttacatcacccagtatcatgtatacaatggacataaaatatacaacaagcactatagctagtggcataatcatagagaaatataatgtcaacagtttaacacgtggtgagagaggacccactaaaccatgggttggttcatctacacaagagaaaaagacaatgccagtttataatagacaagttttaaccaaaaaacagagagatcaaatagatctattagcaaaattggattgggtgtatgcatctatagataacaaggatgaatttatggaggaacttagcataggaactcttgggttaacatatgagaaggccaaaaaattattcccacaatatttgagtgttaactatttgcatcgtcttacagtcagtagtagaccatgtgaattccctgcatctataccagcttatagaactacaaattatcactttgatactagccctattaatcgcatattaacagaaaagtatggtgatgaagatattgatatagtattccaaaactgtataagctttggccttagcttaatgtctgtagtagaacaatttactaatgtatgtcctaacagaattattctcatacccaagcttaatgagatacatttgatgaaacctcccatattcacaggcgatgttgatattcacaagttaaaacaagtgatacaaaaacaacatatgtttttaccagacaaaataagtttgactcaatatgtggaattattcttaagtaataaaacactcaaatctggatctaatgttaattctaatttaatattggcgcataagatatctgactattttcataatacttacattttgagtactaatttagctggacattggattcttattatacaacttatgaaagattctaagggtatttttgaaaaagattggggagagggatatataactgatcatatgttcattaatttgaaagttttcttcaatgcttataagacatatctcttgtgttttcataaaggttacggcagagcaaagctggagtgtgatatgaatacttcagatctcctatgtgtattggaattaatagacagtagttattggaagtctatgtctaaggtgtttttagaacaaaaagttatcaaatacattcttagccaggatgcaagtttacatagagtaaaaggatgtcatagcttcaaactatggtttcttaaacgtcttaatgtagcagaattcacagtttgcccttgggttgttaacatagattatcatccaacacatatgaaagcaatattaacttatattgatcttgttagaatgggattgataaatatagatagaatatacattaaaaataaacacaagttcaatgatgagttttatacttctaatctgttttacattaattataacttctcagataatactcatctattaactaaacatataaggattgctaattccgaattagaaagtaattacaacaaattatatcatcctacaccagaaaccctagaaaatatactaaccaatccggttaaaagtaatgagaaaaagacactgagtgactattgtataggtaaaaatgttgactcaataatgttaccatcgttatctaataagaagcttattaaatcgtctacaatgattagaaccaattacagcagacaagatttgtataatttatttcctacggttgtgattgataaaattatagatcattcaggtaatacagccaaatctaaccaactttacactactacttctcatcaaatatccttagtgcacaatagcacatcactttattgcatgcttccttggcatcatattaatagattcaattttgtatttagttctacaggttgtaaaattagtatagagtatattttaaaagatcttaaaattaaggatcctaattgtatagcattcataggtgaaggagcagggaatttattattgcgtacagtagtggaacttcatcctgatataagatatatttacagaagtctgaaagattgcaatgatcatagtttaccaattgagtttttaaggctgtacaatggacatatcaacattgattatggtgaaaatttgaccattcctgctacagatgcaaccaacaacattcattggtcttatttacatataaagtttgctgaacctatcagtctttttgtctgtgatgctgaattgcctgtaacagtcaactggagtaagattataatagagtggagcaagcatgtaagaaaatgcaagtactgttcttcagttaataaatgtacattgatagtaaaatatcatgctcaagatgatatcgatttcaaattagacaacataactatattaaaaacttatgtatgcttaggtagtaagttaaagggatctgaagtttacttagtccttacaataggtcctgcaaatgtgttcccagtatttaatgtagtacaaaatgctaaattgatactatcaagaactaaaaatttcatcatgcctaaaaaagctgataaagagtctattgatgcaaatattaagagtttgataccctttctttgttaccctataacaaaaaaaggaattaatactgcattgtctaaattaaagagtgttgttagtggagatatactatcatattctatagctggacgtaatgaagttttcagcaataaacttataaatcataagcatatgaacatcttaaagtggttcaatcatgttttaaatttcagatcaacagaattaaactataatcatttatatatggtagaatctacttatcctcatctaagtgaattgttaaacagcttgacaaccaatgaacttaaaaaactgattaaaatcacaggtagtttgttatacaacttttataatgaataatgagcaaaaatcttataacaaaaatagctacacactaacattgtattcaattatagttattgaaaattaataattatataatttttaataacttctagtgaactaatcctaaaattatcattttgatctaggaagaataagtttaaatccaaatctaattggtttatatgtatattaactaaattacgagatattagtttttgacactttttttctcgt

SEQ ID NO: 7 - DNA, 16494 bp, synthetic construct
  misc_feature 1..16494: note = Sequence in which the SH gene is deleted in SEQ ID NO: 6
  source 1..16494: mol_type = other DNA
acgcgaaaaaatgcgtacaacaaacttgcgtaaaccaaaaaaatggggcaaataagaatttgataagtaccacttaaatttaactcctttggttagaggcgcgccatgggcagcaactcattgagtatgataaaagttagattgcaaaatctgtttgacaatgatgaagtagcattgttaaaaataacatgctatactgacaaattaatacagttaactaatgctttggctaaggcagttatacatacaatcaaattgaatggcattgtatttgtgcatgttattacaagtagtgatatttgccctaataataatattgtagtgaaatccaatttcacaacaatgccagtattacaaaatggaggttatatatgggaaatgatggaattaacacactgctctcaacctaatggcctaatagatgacaattgtgaaattaaattctccaaaaaactaagtgattcaacaatgaccaattatatgaatcaattatctgaattacttggatttgacctcaatccataaatcataataaatatcaactagcaaatcaatgtcactaacaccattagttaatataaaacttgacagaagataaaaatggggcaaataaatcaattcagccgacccaaccatggacacaacacacaatgataccacaccacaaagactgatgatcacagacatgaggccattatcgcttgagactataataacatctctaaccagagatatcataacacataaatttatatacttgataaatcatgaatgcatagtaagaaaacttgatgaaagacaggccacatttacatttctggtcaactatgaaatgaaactattgcacaaagtgggaagcactaaatataaaaaatatactgaatacaacacaaaatatggcactttccctatgccaatatttatcaatcatgatgggttcttagaatgcattggcattaagcctaccaagcacacacccataatatacaagtatgatctcaatccatgaatatcaaaccaagattcaaacaatccgaaataacaactttatgcataatcacactccatagtccaaatggagcctgaaaattatagttatttaaaattcctgcaggaaggagagacataagatgaaagatggggcaaatacaaaaatggctcttagcaaagtcaagttgaatgatacactcaacaaagatcaacttctatcatccagcaaatataccatccaacggagcacaggagacagcattgacactcctaattatgatgtgcagaaacacattaataagttatgtggcatgttattaatcacagaagatgctaatcataaattcactgggttaataggtatgttatatgctatgtctagattaggaagagaagacaccataaaaatactcaaagatgcgggatatcatgttaaggcaaatggagtggatgtaacaacacatcgtcaagacattaatgggaaagaaatgaaatttgaagtgttaacattagcaagcttaacaactgaaattcaaatcaacattgagatagaatctagaaaatcctacaaaaaaatgctaaaagaaatgggagaggtggctccagaatacaggcatgactctcctgattgtgggatgataatattatgtatagcggcattagtaataaccaaattagcagcaggagatagatcaggtcttacagctgtgattaggagagctaataatgtcctaaaaaatgaaatgaaacgttataaaggtttattacccaaggatatagccaacagcttctatgaagtgtttgaaaaatatcctcactttatagatgtttttgttcattttggtatagcacaatcttctaccagaggtggcagtagagttgaagggatttttgcaggattgtttatgaatgcctatggtgcagggcaagtgatgttacggtggggggtcttagcaaaatcagttaaaaacattatgttaggacacgctagtgtacaagcagaaatggaacaagttgtggaggtgtatgagtatgctcagaaattgggtggagaagcaggattctaccatatattgaacaacccaaaagcatcactattatctttgactcaatttcctcacttctctagtgtagtattgggcaatgctgctggcctaggcataatgggagaatacagaggtacaccaaggaatcaagatttatatgatgctgcaaaagcatatgctgaacaactcaaagaaaatggtgtgattaactacagtgtattagatttgacagcagaagaactagaggctatcaaacatcagcttaatccaaaagataatgatgtagagctttgagttaataaaaaagtggggcaaataaatcatcatggaaaagtttgctcctgaattccatggagaagatgcaaacaacagagccaccaaattcctagaatcaataaagggcaaattcacatcacccaaagatcccaagaaaaaagatagtatcatatctgtcaactcaatagatatagaagtaaccaaagaaagccctataacatcaaattcaaccattataaacccaataaatgagacagatgatactgtagggaacaagcccaattatcaaagaaagcctctagtaagtttcaaagaagaccctacgccaagtgataatcctttttcaaaactatacaaagaaaccatagaaacatttgataacaatgaagaagaatctagctattcatatgaagaaataaatgatcagacaaacgataatataacagcaagattagataggattgatgagaaattaagtgaaatactaggaatgcttcacacattagtagtagcgagtgcaggacccacatctgctcgggatggtataagagatgccatggttggtttaagagaagaaatgatagaaaaaatcagaactgaagcattaatgaccaatgacagactagaagctatggcaagactcaggaatgaagaaagtgaaaagatggcaaaagacacatcagatgaagtgtctctcaatccaacatcagagaaactgaacaacctgttggaagggaatgatagtgacaatgatctatcacttgaagatttctgattagctaccaaactgtacatcaaaacacaacaccaatagaaaaccaacaaacaaaccaactcacccatccaaccaaacatctatctgctgattagccaaccagccaaaaaacaaccagccaatctaaaactagccacccggaaaaaatcgatactatagttacaaaaaaagatggggcaaatatggaaacatacgtgaataaacttcacgagggctccacatacacagctgctgttcaatacaatgtcctagaaaaagacgatgatcctgcatcacttacaatatgggtgcccatgttccaatcatccatgccagcagatctactcataaaagaactagccaatgtcaatatactagtgaaacaaatatccacacccaagggaccctcattaagagtcatgataaactcaagaagtgcagtgctagcacaaatgcccagcaaatttaccatatgtgccaatgtgtccttggatgaaagaagcaagctggcatatgatgtaaccacaccctgtgaaattaaggcatgcagtctaacatgcctaaaatcaaaaaatatgttaactacagttaaagatctcactatgaaaacactcaacccaacacatgacatcattgctttatgtgaatttgaaaatatagtaacatcaaaaaaagtcataataccaacatacctaagatctatcagcgtcagaaataaagatctgaacacacttgaaaatataacaaccactgaattcaaaaatgccattacaaatgcaaaaatcatcccttactcaggattattgttagtcatcacagtgactgacaacaaaggagcattcaaatacataaagccacaaagtcaattcatagtagatcttggagcttacctagaaaaagaaagtatatattatgttacaacaaattggaagcacacagctacacgatttgcaatcaaacccatggaagattaacctttttcctctacatcaatgagtagattcatacaaactttctaactacattcttcacttcacaatcataatcaccaaccctctgtggttcaatcaatcaaacaaaactcatcaagagttccagatcatcccaagtcattgttcatcagatccagtactcaaataagttaataaaaaatcggtccgttgacagaagataaaaatggggcaaatgcaaacatgaagtgccttttgtacttagcctttttattcattggggtgaattgcaagttcaccatagtttttccacacaaccaaaaaggaaactggaaaaatgttccttctaattaccattattgcccgtcaagctcagatttaaattggcataatgacttaataggcacagccttacaagtcaaaatgcccaagagtcacaaggctattcaagcagacggttggatgtgtcatgcttccaaatgggtcactacttgtgatttccgctggtatggaccgaagtatataacacattccatccgatccttcactccatctgtagaacaatgcaaggaaagcattgaacaaacgaaacaaggaacttggctgaatccaggcttccctcctcaaagttgtggatatgcaactgtgacggatgccgaagcagtgattgtccaggtgactcctcaccatgtgctggttgatgaatacacaggagaatgggttgattcacagttcatcaacggaaaatgcagcaattacatatgccccactgtccataactctacaacctggcattctgactataaggtcaaagggctatgtgattctaacctcatttccatggacatcaccttcttctcagaggacggagagctatcatccctgggaaaggagggcacagggttcagaagtaactactttgcttatgaaactggaggcaaggcctgcaaaatgcaatactgcaagcattggggagtcagactcccatcaggtgtctggttcgagatggctgataaggatctctttgctgcagccagattccctgaatgcccagaagggtcaagtatctctgctccatctcagacctcagtggatgtaagtctaattcaggacgttgagaggatcttggattattccctctgccaagaaacctggagcaaaatcagagcgggtcttccaatctctccagtggatctcagctatcttgctcctaaaaacccaggaaccggtcctgctttcaccataatcaatggtaccctaaaatactttgagaccagatacatcagagtcgatattgctgctccaatcctctcaagaatggtcggaatgatcagtggaactaccacagaaagggaactgtgggatgactgggcaccatatgaagacgtggaaattggacccaatggagttctgaggaccagttcaggatataagtttcctttatacatgattggacatggtatgttggactccgatcttcatcttagctcaaaggctcaggtgttcgaacatcctcacattcaagacgctgcttcgcaacttcctgatgatgagagtttattttttggtgatactgggctatccaaaaatccaatcgagcttgtagaaggttggttcagtagttggaaaagctctattgcctcttttttctttatcatagggttaatcattggactattcttggttctccgagttggtatccatctttgcattaaagccagaagcacaccagtcacattaagtaaggatcaactgagtggtataaataatattgcatttagtaactaatagtcattaaaaagcggccggccagtcataacaatgaactaggatattaagaccaaaaacaacgctggggcaaatgcaaacatgtccaaaaccgaggaccaacgcaccgccaagacactagaaaggacctgggacacttttaatcatctattattcatatcatcgtgcttatacaagttaaatcttaaatctatagcacaaatcacattatctattttggcaattataatctcaacctcacttataattgcagccatcatattcatagcctcggcaaaccacaaagtcacactaacaactgcaatcatacaagatgcaacgaaccagatcaagaacacaaccccaacatacctcacccagaatccccagcatggaatcagcttctccaatctgtccggaactacatcacaatccaccaccatactagcttcaacaacaccaagtgctgattcaaccccacaatccacaacagtcaagatcaaaaacacaacaacaacccaaatattacctagcaaacccaccacaaaacaacgccaaaataaaccacaaaacaaacccaacaatgattttcactttgaagtgttcaattttgtaccctgcagcatatgcagcaacaatccaacctgctgggccatctgcaagagaataccaaacaaaaaacctggaaagaaaaccaccaccaagcccacaaaaaaaccaaccctcaagacaaccaaaaaagatcccaaatcccaaaccacaaaaccaaaggaagtactcactaccaagcctacaggaaagccaaccatcaacaccactaaaacaaacatcagaactacactgctcacctccaacaccaaaggaaatccagaacacacaagtcaagaggaaaccctccactcaaccacctccgaaggctatccaagcccatcacaagtccacacaacatccggtcaagaggaaaccctccactcaaccacctccgaaggctatccaagcccatcacaagtctacacaacatccgagtacctatcacaatctctatcttcatccaacacaacaaaatgatagtcattaaaaagcacgcgtgtattgttgcaaaaagccatgaccaaatcaaacagaatcaaaatcaactctggggcaaataacaatggagttgccaatcctcaaaacaaatgctattaccacaatccttgctgcagtcacactctgtttcgcttccagtcaaaacatcactgaagaattttatcaatcaacatgcagtgcagtcagcaaaggctatcttagtgctctaagaactggttggtatactagtgttataactatagaattaagtaatatcaaggaaaataagtgtaatggtacagacgctaaggtaaaattaataaaacaagaattagataaatataaaaatgctgtaacagaattgcagttgctcatgcaaagcacaccagcagccaacaatcgagccagaagagaactaccaagatttatgaattatacactcaacaataccaaaaacaccaatgtaacattaagtaagaaaaggaaaagaagatttcttggatttttgttaggtgttggatctgcaatcgccagtggcattgccgtatccaaggtcctgcacctagaaggggaagtgaacaaaatcaaaagtgctctactatccacaaacaaggctgtagtcagcttatctaatggagtcagtgtcttaaccagcaaggtgttagacctcaaaaactatatagataaacagttgttacctattgttaacaagcaaagctgcagcatatcaaacattgaaactgtgatagagttccaacaaaagaacaacagactactagagattaccagagaatttagtgttaatgcaggtgtaactactcctgtaagcacttatatgttaactaatagtgagttattatcattaatcaatgatatgcctataacaaatgatcagaaaaagttaatgtccagcaatgttcaaatagttagacagcaaagttactctatcatgtcaataataaaagaggaagtcttggcatatgtagtacaattaccactatatggtgtaatagatactccttgttggaaactacacacatcccctttatgtacaaccaacacaaaggaaggatccaacatctgcttaacaagaaccgacagaggatggtactgtgacaatgcaggatcagtatcctttttcccacaagctgaaacatgtaaagttcaatcgaatcgggtgttttgtgacacaatgaacagtttaacattaccaagtgaggtaaatctctgcaacattgacatattcaaccccaaatatgattgcaaaattatgacttcaaaaacagatgtaagcagctccgttatcacatctctaggagccattgtgtcatgctatggcaaaaccaaatgtacagcatccaataaaaatcgtgggatcataaagacattctctaacgggtgtgattatgtatcaaataagggggtggatactgtgtctgtaggtaatacattatattatgtaaataagcaagaaggcaaaagtctctatgtaaaaggtgaaccaataataaatttctatgatccattagtgttcccctctgatgaatttgatgcatcaatatctcaagtcaatgagaaaattaatcagagtctagcatttatccgtaaatcagatgaattattacataatgtaaatgctggtaaatccaccacaaatatcatgataactaccataattatagtaattatagtaatattgttagcattaattgcagttggactgcttctatactgcaaggccagaagcacaccagtcacattaagtaaggatcaactgagtggtataaataatattgcatttagtaactgaataaaaatagcacctaatcatattcttacaatggttcgctatttgaccatagataacccatctatcattagattatcctaaaatttgaacttcatcacaactttcatctataaaccatctcacttacactttttaagtagatttctattttatagttatataaaacagggcccattgaataccaaattaacttactatttgtaaaaatgagaattggggcaaatatgtcacgaaggaatccttgcaaattcgaaattcgaggtcattgcttgaatggtaaaaggtgtcattttagtcataattattttgaatggccaccccatgcactgcttgtaagacaaaactttatgttaaacagaatacttaagtctatggataaaagcatagatactttgtcagaaataagtggagctgcagagttggacagaacagaagagtatgccctcggtgtagttggagtgctagagagttatataggatcaataaataatataactaaacaatcagcatgtgttgccatgagcaaactccttactgaactcaacagcgatgacatcaaaaaactaagggacaatgaagagccaaactcacccaaagtaagagtgtacaatactgtcatatcatatattgaaagcaacaggaagaacaataaacaaactatccatctgttaaaaagattgccagcagacgtattgaagaaaaccatcaaaaacacattggatatccacaagagcataaccatcaataacccaaaagaatcaactgttagtgatacgaacgaccatgccaaaaataatgatactacctgacaaatatccttgtagtataaattccatactaataacaagtaattgtagagtcactatgtataatcaaaaaaacacactatatatcaatcaaaacaaccaaaatagccatatatacccaccggatcaaccattcaatgaaatccattggacctctcaagacttgattgatgcaactcaaaattttctacaacatctaggtattactgatgatatatacacaatatatatattagtgtcataatactcaatcctaatacttaccacatcatcaaattattaactcaaacaattcaagctatgggacaaaatggatcccattattagtggaaattctgctaatgtttatctaactgatagttatttaaaaggtgttatttctttctcagaatgtaacgctttaggaagttacatattcaatggtccttatctcaaaaatgattataccaacttaattagtagacaaaatccattaatagaacacataaatctaaagaaactaaatataacacagtccttaatatctaagtatcataaaggtgaaataaaaatagaagaacctacttactttcagtcattacttatgacatacaagagtatgacctcttcagaacagactactactactaatttacttaaaaagataataagaagagctatagaaatcagtgatgtcaaagtctatgctatattgaataaactggggctcaaagaaaaagacaagattaaatccaataatggacaagatgaagacaactcagtcattactaccataatcaaagatgatatacttttagctgtcaaggataatcaatctcatcttaaagcagacaaaaatcaatccacaaaacaaaaagatacaatcaaaacaacacttttgaagaaattaatgtgttcgatgcaacatcctccatcatggttaatacattggtttaatttatacacaaaattaaacagcatattaacacaatatcgatctagtgaggtaaaaaaccatggttttatattgatagataatcatactcttagtggattccaatttattttgaatcaatatggttgtatagtttatcataaggaactcaaaagaattactgtgacaacttataatcaattcttgacatggaaagatattagccttagtagattaaatgtttgtttgattacatggattagtaactgtttgaacacattaaacaaaagcttaggcttaagatgtggattcaataatgttatcttgacacaattattcctttatggagattgtatactaaaactattccacaatgaggggttctacataataaaagaggtagagggatttattatgtctctaattttaaatataacagaagaagatcaattcagaaaacggttttataatagtatgctcaacaacatcacagatgccgccaacaaagctcaaaaaaatctgctatcaagagtatgtcatacattattagataagacaatatcagataatataataaatggcagatggataattctattgagtaagttcctaaaattaattaagcttgcaggtgacaataacctcaacaatctgagtgaattatattttttgttcagaatatttggacacccaatggtagatgaaagacaagccatggatgctgttaaagttaattgcaacgagaccaaattttatttgttaagtagtttgagtatgttaagaggagcttttatatatagaattataaaagggtttgtaaataattacaacagatggcctactttaagaaatgccattgtcttacccttaagatggttaacttactataaactaaacacttatccttccttgttggaacttacagaaagagatttgattgttctatcaggactacgtttctatcgagagtttcggttgcctaaaaaagtggatcttgaaatgatcataaatgataaggctatatcacctcctaaaaatttaatatggactagtttccctagaaattatatgccgtcacacatacaaaattatatagaacatgaaaaattaaaattctctgatagtgataaatcaagaagagtattagagtattatttaagagataacaaattcaatgaatgtgatttacacaactgtgtagttaatcaaagttatcttaacaacccgaatcatgtggtatcattgacaggcaaagaaagagaactcagtgtaggtagaatgtttgcaatgcaaccaggaatgttcagacaagttcaaatattagcagagaaaatgatagcagaaaacatattacaatttttccctgaaagtcttacaagatatggtgatctagaactacagaaaatattagaattgaaagcaggaataagtaacaaatcaaatcgttacaatgataattacaacaattacattagtaagtgctctatcatcacagatctcagcaaattcaatcaagcatttcgatatgaaacatcatgtatttgtagtgatgtactggatgaactgcatggtgtacaatctctattttcctggttacatttaactattcctcatgtcacaataatatgcacatataggcatgcacccccctatataaaggatcatattgtagatcttaacaatgtagatgagcaaagtggactatatagatatcatatgggtggtatcgaagggtggtgtcaaaaactatggaccatagaagctatatcactattagatctaatatctctcaaagggaaattctcaattactgctttaattaatggtgacaatcaatcaatagatataagtaaaccagtcagactcatggaaggtcaaactcatgctcaagcagattatttgctagcattaaatagtctcaaattactgtataaagagtatgcaggaataggccacaaattaaaaggaactgagacttatatatcgagagatatgcaatttatgagtaaaacgatccaacataacggtgtatattacccagctagtataaagaaagtcctaagagtgggaccgtggataaacactatacttgatgacttcaaagtgagtctagaatctataggtagtttgacacaagaattagaatatagaggtgaaagtctattatgcagtttaatatttagaaatgtatggttatataatcaaattgcattacaacttaaaaatcatgcattatgtaacaacaaattatatttggatatattaaaagttctaaaacacttaaaaaccttttttaatcttgataacattgatacagcattaacattgtatatgaatttgcccatgttatttggtggtggtgatcccaacttgttatatcgaagtttctatagaagaactcctgatttcctcacagaggctatagttcactctgtgttcatacttagttattatacaaaccatgatttaaaagataaacttcaagatctgtcagatgatagattgaataagttcttaacatgcataatcacgtttgataaaaaccccaatgctgaattcgttacattgatgagagatcctcaagctttaggatctgagaggcaagctaaaattactagcgaaatcaatagactggcagttaccgaggttttgagcacagctccaaacaaaatattttccaaaagtgcacaacactataccactacagagatagatcttaatgatattatgcaaaatatagaacctacatatcctcacgggctaagagttgtttatgagagtttacccttttataaagcagagaaaatagtaaatcttatatccggtacaaaatctataactaacatactggaaaagacttctgccatagacttaacagatattgatagagccactgagatgatgaggaaaaacataactttgcttataaggatattaccattagattgtaacagagataaaagagaaatattgagtatggaaaacctaagtattactgaattaagcaaatacgttagagaaagatcttggtctttatccaatatagttggtgttacatcacccagtatcatgtatacaatggacataaaatatacaacaagcactatagctagtggcataatcatagagaaatataatgtcaacagtttaacacgtggtgagagaggacccactaaaccatgggttggttcatctacacaagagaaaaagacaatgccagtttataatagacaagttttaaccaaaaaacagagagatcaaatagatctattagcaaaattggattgggtgtatgcatctatagataacaaggatgaatttatggaggaacttagcataggaactcttgggttaacatatgagaaggccaaaaaattattcccacaatatttgagtgttaactatttgcatcgtcttacagtcagtagtagaccatgtgaattccctgcatctataccagcttatagaactacaaattatcactttgatactagccctattaatcgcatattaacagaaaagtatggtgatgaagatattgatatagtattccaaaactgtataagctttggccttagcttaatgtctgtagtagaacaatttactaatgtatgtcctaacagaattattctcatacccaagcttaatgagatacatttgatgaaacctcccatattcacaggcgatgttgatattcacaagttaaaacaagtgatacaaaaacaacatatgtttttaccagacaaaataagtttgactcaatatgtggaattattcttaagtaataaaacactcaaatctggatctaatgttaattctaatttaatattggcgcataagatatctgactattttcataatacttacattttgagtactaatttagctggacattggattcttattatacaacttatgaaagattctaagggtatttttgaaaaagattggggagagggatatataactgatcatatgttcattaatttgaaagttttcttcaatgcttataagacatatctcttgtgttttcataaaggttacggcagagcaaagctggagtgtgatatgaatacttcagatctcctatgtgtattggaattaatagacagtagttattggaagtctatgtctaaggtgtttttagaacaaaaagttatcaaatacattcttagccaggatgcaagtttacatagagtaaaaggatgtcatagcttcaaactatggtttcttaaacgtcttaatgtagcagaattcacagtttgcccttgggttgttaacatagattatcatccaacacatatgaaagcaatattaacttatattgatcttgttagaatgggattgataaatatagatagaatatacattaaaaataaacacaagttcaatgatgagttttatacttctaatctgttttacattaattataacttctcagataatactcatctattaactaaacatataaggattgctaattccgaattagaaagtaattacaacaaattatatcatcctacaccagaaaccctagaaaatatactaaccaatccggttaaaagtaatgagaaaaagacactgagtgactattgtataggtaaaaatgttgactcaataatgttaccatcgttatctaataagaagcttattaaatcgtctacaatgattagaaccaattacagcagacaagatttgtataatttatttcctacggttgtgattgataaaattatagatcattcaggtaatacagccaaatctaaccaactttacactactacttctcatcaaatatccttagtgcacaatagcacatcactttattgcatgcttccttggcatcatattaatagattcaattttgtatttagttctacaggttgtaaaattagtatagagtatattttaaaagatcttaaaattaaggatcctaattgtatagcattcataggtgaaggagcagggaatttattattgcgtacagtagtggaacttcatcctgatataagatatatttacagaagtctgaaagattgcaatgatcatagtttaccaattgagtttttaaggctgtacaatggacatatcaacattgattatggtgaaaatttgaccattcctgctacagatgcaaccaacaacattcattggtcttatttacatataaagtttgctgaacctatcagtctttttgtctgtgatgctgaattgcctgtaacagtcaactggagtaagattataatagagtggagcaagcatgtaagaaaatgcaagtactgttcttcagttaataaatgtacattgatagtaaaatatcatgctcaagatgatatcgatttcaaattagacaacataactatattaaaaacttatgtatgcttaggtagtaagttaaagggatctgaagtttacttagtccttacaataggtcctgcaaatgtgttcccagtatttaatgtagtacaaaatgctaaattgatactatcaagaactaaaaatttcatcatgcctaaaaaagctgataaagagtctattgatgcaaatattaagagtttgataccctttctttgttaccctataacaaaaaaaggaattaatactgcattgtctaaattaaagagtgttgttagtggagatatactatcatattctatagctggacgtaatgaagttttcagcaataaacttataaatcataagcatatgaacatcttaaagtggttcaatcatgttttaaatttcagatcaacagaattaaactataatcatttatatatggtagaatctacttatcctcatctaagtgaattgttaaacagcttgacaaccaatgaacttaaaaaactgattaaaatcacaggtagtttgttatacaacttttataatgaataatgagcaaaaatcttataacaaaaatagctacacactaacattgtattcaattatagttattgaaaattaataattatataatttttaataacttctagtgaactaatcctaaaattatcattttgatctaggaagaataagtttaaatccaaatctaattggtttatatgtatattaactaaattacgagatattagtttttgacactttttttctcgt

SEQ ID NO: 8 - DNA, 15506 bp, synthetic construct
  misc_feature 1..15506: note = Sequence in which the G gene is deleted in SEQ ID NO: 7
  source 1..15506: mol_type = other DNA
acgcgaaaaaatgcgtacaacaaacttgcgtaaaccaaaaaaatggggcaaataagaatttgataagtaccacttaaatttaactcctttggttagaggcgcgccatgggcagcaactcattgagtatgataaaagttagattgcaaaatctgtttgacaatgatgaagtagcattgttaaaaataacatgctatactgacaaattaatacagttaactaatgctttggctaaggcagttatacatacaatcaaattgaatggcattgtatttgtgcatgttattacaagtagtgatatttgccctaataataatattgtagtgaaatccaatttcacaacaatgccagtattacaaaatggaggttatatatgggaaatgatggaattaacacactgctctcaacctaatggcctaatagatgacaattgtgaaattaaattctccaaaaaactaagtgattcaacaatgaccaattatatgaatcaattatctgaattacttggatttgacctcaatccataaatcataataaatatcaactagcaaatcaatgtcactaacaccattagttaatataaaacttgacagaagataaaaatggggcaaataaatcaattcagccgacccaaccatggacacaacacacaatgataccacaccacaaagactgatgatcacagacatgaggccattatcgcttgagactataataacatctctaaccagagatatcataacacataaatttatatacttgataaatcatgaatgcatagtaagaaaacttgatgaaagacaggccacatttacatttctggtcaactatgaaatgaaactattgcacaaagtgggaagcactaaatataaaaaatatactgaatacaacacaaaatatggcactttccctatgccaatatttatcaatcatgatgggttcttagaatgcattggcattaagcctaccaagcacacacccataatatacaagtatgatctcaatccatgaatatcaaaccaagattcaaacaatccgaaataacaactttatgcataatcacactccatagtccaaatggagcctgaaaattatagttatttaaaattcctgcaggaaggagagacataagatgaaagatggggcaaatacaaaaatggctcttagcaaagtcaagttgaatgatacactcaacaaagatcaacttctatcatccagcaaatataccatccaacggagcacaggagacagcattgacactcctaattatgatgtgcagaaacacattaataagttatgtggcatgttattaatcacagaagatgctaatcataaattcactgggttaataggtatgttatatgctatgtctagattaggaagagaagacaccataaaaatactcaaagatgcgggatatcatgttaaggcaaatggagtggatgtaacaacacatcgtcaagacattaatgggaaagaaatgaaatttgaagtgttaacattagcaagcttaacaactgaaattcaaatcaacattgagatagaatctagaaaatcctacaaaaaaatgctaaaagaaatgggagaggtggctccagaatacaggcatgactctcctgattgtgggatgataatattatgtatagcggcattagtaataaccaaattagcagcaggagatagatcaggtcttacagctgtgattaggagagctaataatgtcctaaaaaatgaaatgaaacgttataaaggtttattacccaaggatatagccaacagcttctatgaagtgtttgaaaaatatcctcactttatagatgtttttgttcattttggtatagcacaatcttctaccagaggtggcagtagagttgaagggatttttgcaggattgtttatgaatgcctatggtgcagggcaagtgatgttacggtggggggtcttagcaaaatcagttaaaaacattatgttaggacacgctagtgtacaagcagaaatggaacaagttgtggaggtgtatgagtatgctcagaaattgggtggagaagcaggattctaccatatattgaacaacccaaaagcatcactattatctttgactcaatttcctcacttctctagtgtagtattgggcaatgctgctggcctaggcataatgggagaatacagaggtacaccaaggaatcaagatttatatgatgctgcaaaagcatatgctgaacaactcaaagaaaatggtgtgattaactacagtgtattagatttgacagcagaagaactagaggctatcaaacatcagcttaatccaaaagataatgatgtagagctttgagttaataaaaaagtggggcaaataaatcatcatggaaaagtttgctcctgaattccatggagaagatgcaaacaacagagccaccaaattcctagaatcaataaagggcaaattcacatcacccaaagatcccaagaaaaaagatagtatcatatctgtcaactcaatagatatagaagtaaccaaagaaagccctataacatcaaattcaaccattataaacccaataaatgagacagatgatactgtagggaacaagcccaattatcaaagaaagcctctagtaagtttcaaagaagaccctacgccaagtgataatcctttttcaaaactatacaaagaaaccatagaaacatttgataacaatgaagaagaatctagctattcatatgaagaaataaatgatcagacaaacgataatataacagcaagattagataggattgatgagaaattaagtgaaatactaggaatgcttcacacattagtagtagcgagtgcaggacccacatctgctcgggatggtataagagatgccatggttggtttaagagaagaaatgatagaaaaaatcagaactgaagcattaatgaccaatgacagactagaagctatggcaagactcaggaatgaagaaagtgaaaagatggcaaaagacacatcagatgaagtgtctctcaatccaacatcagagaaactgaacaacctgttggaagggaatgatagtgacaatgatctatcacttgaagatttctgattagctaccaaactgtacatcaaaacacaacaccaatagaaaaccaacaaacaaaccaactcacccatccaaccaaacatctatctgctgattagccaaccagccaaaaaacaaccagccaatctaaaactagccacccggaaaaaatcgatactatagttacaaaaaaagatggggcaaatatggaaacatacgtgaataaacttcacgagggctccacatacacagctgctgttcaatacaatgtcctagaaaaagacgatgatcctgcatcacttacaatatgggtgcccatgttccaatcatccatgccagcagatctactcataaaagaactagccaatgtcaatatactagtgaaacaaatatccacacccaagggaccctcattaagagtcatgataaactcaagaagtgcagtgctagcacaaatgcccagcaaatttaccatatgtgccaatgtgtccttggatgaaagaagcaagctggcatatgatgtaaccacaccctgtgaaattaaggcatgcagtctaacatgcctaaaatcaaaaaatatgttaactacagttaaagatctcactatgaaaacactcaacccaacacatgacatcattgctttatgtgaatttgaaaatatagtaacatcaaaaaaagtcataataccaacatacctaagatctatcagcgtcagaaataaagatctgaacacacttgaaaatataacaaccactgaattcaaaaatgccattacaaatgcaaaaatcatcccttactcaggattattgttagtcatcacagtgactgacaacaaaggagcattcaaatacataaagccacaaagtcaattcatagtagatcttggagcttacctagaaaaagaaagtatatattatgttacaacaaattggaagcacacagctacacgatttgcaatcaaacccatggaagattaacctttttcctctacatcaatgagtagattcatacaaactttctaactacattcttcacttcacaatcataatcaccaaccctctgtggttcaatcaatcaaacaaaactcatcaagagttccagatcatcccaagtcattgttcatcagatccagtactcaaataagttaataaaaaatcggtccgttgacagaagataaaaatggggcaaatgcaaacatgaagtgccttttgtacttagcctttttattcattggggtgaattgcaagttcaccatagtttttccacacaaccaaaaaggaaactggaaaaatgttccttctaattaccattattgcccgtcaagctcagatttaaattggcataatgacttaataggcacagccttacaagtcaaaatgcccaagagtcacaaggctattcaagcagacggttggatgtgtcatgcttccaaatgggtcactacttgtgatttccgctggtatggaccgaagtatataacacattccatccgatccttcactccatctgtagaacaatgcaaggaaagcattgaacaaacgaaacaaggaacttggctgaatccaggcttccctcctcaaagttgtggatatgcaactgtgacggatgccgaagcagtgattgtccaggtgactcctcaccatgtgctggttgatgaatacacaggagaatgggttgattcacagttcatcaacggaaaatgcagcaattacatatgccccactgtccataactctacaacctggcattctgactataaggtcaaagggctatgtgattctaacctcatttccatggacatcaccttcttctcagaggacggagagctatcatccctgggaaaggagggcacagggttcagaagtaactactttgcttatgaaactggaggcaaggcctgcaaaatgcaatactgcaagcattggggagtcagactcccatcaggtgtctggttcgagatggctgataaggatctctttgctgcagccagattccctgaatgcccagaagggtcaagtatctctgctccatctcagacctcagtggatgtaagtctaattcaggacgttgagaggatcttggattattccctctgccaagaaacctggagcaaaatcagagcgggtcttccaatctctccagtggatctcagctatcttgctcctaaaaacccaggaaccggtcctgctttcaccataatcaatggtaccctaaaatactttgagaccagatacatcagagtcgatattgctgctccaatcctctcaagaatggtcggaatgatcagtggaactaccacagaaagggaactgtgggatgactgggcaccatatgaagacgtggaaattggacccaatggagttctgaggaccagttcaggatataagtttcctttatacatgattggacatggtatgttggactccgatcttcatcttagctcaaaggctcaggtgttcgaacatcctcacattcaagacgctgcttcgcaacttcctgatgatgagagtttattttttggtgatactgggctatccaaaaatccaatcgagcttgtagaaggttggttcagtagttggaaaagctctattgcctcttttttctttatcatagggttaatcattggactattcttggttctccgagttggtatccatctttgcattaaagccagaagcacaccagtcacattaagtaaggatcaactgagtggtataaataatattgcatttagtaactaatagtcattaaaaagcggccggccgtattgttgcaaaaagccatgaccaaatcaaacagaatcaaaatcaactctacgcgtgtattgttgcaaaaagccatgaccaaatcaaacagaatcaaaatcaactctggggcaaataacaatggagttgccaatcctcaaaacaaatgctattaccacaatccttgctgcagtcacactctgtttcgcttccagtcaaaacatcactgaagaattttatcaatcaacatgcagtgcagtcagcaaaggctatcttagtgctctaagaactggttggtatactagtgttataactatagaattaagtaatatcaaggaaaataagtgtaatggtacagacgctaaggtaaaattaataaaacaagaattagataaatataaaaatgctgtaacagaattgcagttgctcatgcaaagcacaccagcagccaacaatcgagccagaagagaactaccaagatttatgaattatacactcaacaataccaaaaacaccaatgtaacattaagtaagaaaaggaaaagaagatttcttggatttttgttaggtgttggatctgcaatcgccagtggcattgccgtatccaaggtcctgcacctagaaggggaagtgaacaaaatcaaaagtgctctactatccacaaacaaggctgtagtcagcttatctaatggagtcagtgtcttaaccagcaaggtgttagacctcaaaaactatatagataaacagttgttacctattgttaacaagcaaagctgcagcatatcaaacattgaaactgtgatagagttccaacaaaagaacaacagactactagagattaccagagaatttagtgttaatgcaggtgtaactactcctgtaagcacttatatgttaactaatagtgagttattatcattaatcaatgatatgcctataacaaatgatcagaaaaagttaatgtccagcaatgttcaaatagttagacagcaaagttactctatcatgtcaataataaaagaggaagtcttggcatatgtagtacaattaccactatatggtgtaatagatactccttgttggaaactacacacatcccctttatgtacaaccaacacaaaggaaggatccaacatctgcttaacaagaaccgacagaggatggtactgtgacaatgcaggatcagtatcctttttcccacaagctgaaacatgtaaagttcaatcgaatcgggtgttttgtgacacaatgaacagtttaacattaccaagtgaggtaaatctctgcaacattgacatattcaaccccaaatatgattgcaaaattatgacttcaaaaacagatgtaagcagctccgttatcacatctctaggagccattgtgtcatgctatggcaaaaccaaatgtacagcatccaataaaaatcgtgggatcataaagacattctctaacgggtgtgattatgtatcaaataagggggtggatactgtgtctgtaggtaatacattatattatgtaaataagcaagaaggcaaaagtctctatgtaaaaggtgaaccaataataaatttctatgatccattagtgttcccctctgatgaatttgatgcatcaatatctcaagtcaatgagaaaattaatcagagtctagcatttatccgtaaatcagatgaattattacataatgtaaatgctggtaaatccaccacaaatatcatgataactaccataattatagtaattatagtaatattgttagcattaattgcagttggactgcttctatactgcaaggccagaagcacaccagtcacattaagtaaggatcaactgagtggtataaataatattgcatttagtaactgaataaaaatagcacctaatcatattcttacaatggttcgctatttgaccatagataacccatctatcattagattatcctaaaatttgaacttcatcacaactttcatctataaaccatctcacttacactttttaagtagatttctattttatagttatataaaacagggcccattgaataccaaattaacttactatttgtaaaaatgagaattggggcaaatatgtcacgaaggaatccttgcaaattcgaaattcgaggtcattgcttgaatggtaaaaggtgtcattttagtcataattattttgaatggccaccccatgcactgcttgtaagacaaaactttatgttaaacagaatacttaagtctatggataaaagcatagatactttgtcagaaataagtggagctgcagagttggacagaacagaagagtatgccctcggtgtagttggagtgctagagagttatataggatcaataaataatataactaaacaatcagcatgtgttgccatgagcaaactccttactgaactcaacagcgatgacatcaaaaaactaagggacaatgaagagccaaactcacccaaagtaagagtgtacaatactgtcatatcatatattgaaagcaacaggaagaacaataaacaaactatccatctgttaaaaagattgccagcagacgtattgaagaaaaccatcaaaaacacattggatatccacaagagcataaccatcaataacccaaaagaatcaactgttagtgatacgaacgaccatgccaaaaataatgatactacctgacaaatatccttgtagtataaattccatactaataacaagtaattgtagagtcactatgtataatcaaaaaaacacactatatatcaatcaaaacaaccaaaatagccatatatacccaccggatcaaccattcaatgaaatccattggacctctcaagacttgattgatgcaactcaaaattttctacaacatctaggtattactgatgatatatacacaatatatatattagtgtcataatactcaatcctaatacttaccacatcatcaaattattaactcaaacaattcaagctatgggacaaaatggatcccattattagtggaaattctgctaatgtttatctaactgatagttatttaaaaggtgttatttctttctcagaatgtaacgctttaggaagttacatattcaatggtccttatctcaaaaatgattataccaacttaattagtagacaaaatccattaatagaacacataaatctaaagaaactaaatataacacagtccttaatatctaagtatcataaaggtgaaataaaaatagaagaacctacttactttcagtcattacttatgacatacaagagtatgacctcttcagaacagactactactactaatttacttaaaaagataataagaagagctatagaaatcagtgatgtcaaagtctatgctatattgaataaactggggctcaaagaaaaagacaagattaaatccaataatggacaagatgaagacaactcagtcattactaccataatcaaagatgatatacttttagctgtcaaggataatcaatctcatcttaaagcagacaaaaatcaatccacaaaacaaaaagatacaatcaaaacaacacttttgaagaaattaatgtgttcgatgcaacatcctccatcatggttaatacattggtttaatttatacacaaaattaaacagcatattaacacaatatcgatctagtgaggtaaaaaaccatggttttatattgatagataatcatactcttagtggattccaatttattttgaatcaatatggttgtatagtttatcataaggaactcaaaagaattactgtgacaacttataatcaattcttgacatggaaagatattagccttagtagattaaatgtttgtttgattacatggattagtaactgtttgaacacattaaacaaaagcttaggcttaagatgtggattcaataatgttatcttgacacaattattcctttatggagattgtatactaaaactattccacaatgaggggttctacataataaaagaggtagagggatttattatgtctctaattttaaatataacagaagaagatcaattcagaaaacggttttataatagtatgctcaacaacatcacagatgccgccaacaaagctcaaaaaaatctgctatcaagagtatgtcatacattattagataagacaatatcagataatataataaatggcagatggataattctattgagtaagttcctaaaattaattaagcttgcaggtgacaataacctcaacaatctgagtgaattatattttttgttcagaatatttggacacccaatggtagatgaaagacaagccatggatgctgttaaagttaattgcaacgagaccaaattttatttgttaagtagtttgagtatgttaagaggagcttttatatatagaattataaaagggtttgtaaataattacaacagatggcctactttaagaaatgccattgtcttacccttaagatggttaacttactataaactaaacacttatccttccttgttggaacttacagaaagagatttgattgttctatcaggactacgtttctatcgagagtttcggttgcctaaaaaagtggatcttgaaatgatcataaatgataaggctatatcacctcctaaaaatttaatatggactagtttccctagaaattatatgccgtcacacatacaaaattatatagaacatgaaaaattaaaattctctgatagtgataaatcaagaagagtattagagtattatttaagagataacaaattcaatgaatgtgatttacacaactgtgtagttaatcaaagttatcttaacaacccgaatcatgtggtatcattgacaggcaaagaaagagaactcagtgtaggtagaatgtttgcaatgcaaccaggaatgttcagacaagttcaaatattagcagagaaaatgatagcagaaaacatattacaatttttccctgaaagtcttacaagatatggtgatctagaactacagaaaatattagaattgaaagcaggaataagtaacaaatcaaatcgttacaatgataattacaacaattacattagtaagtgctctatcatcacagatctcagcaaattcaatcaagcatttcgatatgaaacatcatgtatttgtagtgatgtactggatgaactgcatggtgtacaatctctattttcctggttacatttaactattcctcatgtcacaataatatgcacatataggcatgcacccccctatataaaggatcatattgtagatcttaacaatgtagatgagcaaagtggactatatagatatcatatgggtggtatcgaagggtggtgtcaaaaactatggaccatagaagctatatcactattagatctaatatctctcaaagggaaattctcaattactgctttaattaatggtgacaatcaatcaatagatataagtaaaccagtcagactcatggaaggtcaaactcatgctcaagcagattatttgctagcattaaatagtctcaaattactgtataaagagtatgcaggaataggccacaaattaaaaggaactgagacttatatatcgagagatatgcaatttatgagtaaaacgatccaacataacggtgtatattacccagctagtataaagaaagtcctaagagtgggaccgtggataaacactatacttgatgacttcaaagtgagtctagaatctataggtagtttgacacaagaattagaatatagaggtgaaagtctattatgcagtttaatatttagaaatgtatggttatataatcaaattgcattacaacttaaaaatcatgcattatgtaacaacaaattatatttggatatattaaaagttctaaaacacttaaaaaccttttttaatcttgataacattgatacagcattaacattgtatatgaatttgcccatgttatttggtggtggtgatcccaacttgttatatcgaagtttctatagaagaactcctgatttcctcacagaggctatagttcactctgtgttcatacttagttattatacaaaccatgatttaaaagataaacttcaagatctgtcagatgatagattgaataagttcttaacatgcataatcacgtttgataaaaaccccaatgctgaattcgttacattgatgagagatcctcaagctttaggatctgagaggcaagctaaaattactagcgaaatcaatagactggcagttaccgaggttttgagcacagctccaaacaaaatattttccaaaagtgcacaacactataccactacagagatagatcttaatgatattatgcaaaatatagaacctacatatcctcacgggctaagagttgtttatgagagtttacccttttataaagcagagaaaatagtaaatcttatatccggtacaaaatctataactaacatactggaaaagacttctgccatagacttaacagatattgatagagccactgagatgatgaggaaaaacataactttgcttataaggatattaccattagattgtaacagagataaaagagaaatattgagtatggaaaacctaagtattactgaattaagcaaatacgttagagaaagatcttggtctttatccaatatagttggtgttacatcacccagtatcatgtatacaatggacataaaatatacaacaagcactatagctagtggcataatcatagagaaatataatgtcaacagtttaacacgtggtgagagaggacccactaaaccatgggttggttcatctacacaagagaaaaagacaatgccagtttataatagacaagttttaaccaaaaaacagagagatcaaatagatctattagcaaaattggattgggtgtatgcatctatagataacaaggatgaatttatggaggaacttagcataggaactcttgggttaacatatgagaaggccaaaaaattattcccacaatatttgagtgttaactatttgcatcgtcttacagtcagtagtagaccatgtgaattccctgcatctataccagcttatagaactacaaattatcactttgatactagccctattaatcgcatattaacagaaaagtatggtgatgaagatattgatatagtattccaaaactgtataagctttggccttagcttaatgtctgtagtagaacaatttactaatgtatgtcctaacagaattattctcatacccaagcttaatgagatacatttgatgaaacctcccatattcacaggcgatgttgatattcacaagttaaaacaagtgatacaaaaacaacatatgtttttaccagacaaaataagtttgactcaatatgtggaattattcttaagtaataaaacactcaaatctggatctaatgttaattctaatttaatattggcgcataagatatctgactattttcataatacttacattttgagtactaatttagctggacattggattcttattatacaacttatgaaagattctaagggtatttttgaaaaagattggggagagggatatataactgatcatatgttcattaatttgaaagttttcttcaatgcttataagacatatctcttgtgttttcataaaggttacggcagagcaaagctggagtgtgatatgaatacttcagatctcctatgtgtattggaattaatagacagtagttattggaagtctatgtctaaggtgtttttagaacaaaaagttatcaaatacattcttagccaggatgcaagtttacatagagtaaaaggatgtcatagcttcaaactatggtttcttaaacgtcttaatgtagcagaattcacagtttgcccttgggttgttaacatagattatcatccaacacatatgaaagcaatattaacttatattgatcttgttagaatgggattgataaatatagatagaatatacattaaaaataaacacaagttcaatgatgagttttatacttctaatctgttttacattaattataacttctcagataatactcatctattaactaaacatataaggattgctaattccgaattagaaagtaattacaacaaattatatcatcctacaccagaaaccctagaaaatatactaaccaatccggttaaaagtaatgagaaaaagacactgagtgactattgtataggtaaaaatgttgactcaataatgttaccatcgttatctaataagaagcttattaaatcgtctacaatgattagaaccaattacagcagacaagatttgtataatttatttcctacggttgtgattgataaaattatagatcattcaggtaatacagccaaatctaaccaactttacactactacttctcatcaaatatccttagtgcacaatagcacatcactttattgcatgcttccttggcatcatattaatagattcaattttgtatttagttctacaggttgtaaaattagtatagagtatattttaaaagatcttaaaattaaggatcctaattgtatagcattcataggtgaaggagcagggaatttattattgcgtacagtagtggaacttcatcctgatataagatatatttacagaagtctgaaagattgcaatgatcatagtttaccaattgagtttttaaggctgtacaatggacatatcaacattgattatggtgaaaatttgaccattcctgctacagatgcaaccaacaacattcattggtcttatttacatataaagtttgctgaacctatcagtctttttgtctgtgatgctgaattgcctgtaacagtcaactggagtaagattataatagagtggagcaagcatgtaagaaaatgcaagtactgttcttcagttaataaatgtacattgatagtaaaatatcatgctcaagatgatatcgatttcaaattagacaacataactatattaaaaacttatgtatgcttaggtagtaagttaaagggatctgaagtttacttagtccttacaataggtcctgcaaatgtgttcccagtatttaatgtagtacaaaatgctaaattgatactatcaagaactaaaaatttcatcatgcctaaaaaagctgataaagagtctattgatgcaaatattaagagtttgataccctttctttgttaccctataacaaaaaaaggaattaatactgcattgtctaaattaaagagtgttgttagtggagatatactatcatattctatagctggacgtaatgaagttttcagcaataaacttataaatcataagcatatgaacatcttaaagtggttcaatcatgttttaaatttcagatcaacagaattaaactataatcatttatatatggtagaatctacttatcctcatctaagtgaattgttaaacagcttgacaaccaatgaacttaaaaaactgattaaaatcacaggtagtttgttatacaacttttataatgaataatgagcaaaaatcttataacaaaaatagctacacactaacattgtattcaattatagttattgaaaattaataattatataatttttaataacttctagtgaactaatcctaaaattatcattttgatctaggaagaataagtttaaatccaaatctaattggtttatatgtatattaactaaattacgagatattagtttttgacactttttttctcgt

SEQ ID NO: 9 - DNA, 14589 bp, synthetic construct
  misc_feature 1..14589: note = Sequence in which the F gene is deleted in SEQ ID NO: 7
  source 1..14589: mol_type = other DNA
acgcgaaaaaatgcgtacaacaaacttgcgtaaaccaaaaaaatggggcaaataagaatttgataagtaccacttaaatttaactcctttggttagaggcgcgccatgggcagcaactcattgagtatgataaaagttagattgcaaaatctgtttgacaatgatgaagtagcattgttaaaaataacatgctatactgacaaattaatacagttaactaatgctttggctaaggcagttatacatacaatcaaattgaatggcattgtatttgtgcatgttattacaagtagtgatatttgccctaataataatattgtagtgaaatccaatttcacaacaatgccagtattacaaaatggaggttatatatgggaaatgatggaattaacacactgctctcaacctaatggcctaatagatgacaattgtgaaattaaattctccaaaaaactaagtgattcaacaatgaccaattatatgaatcaattatctgaattacttggatttgacctcaatccataaatcataataaatatcaactagcaaatcaatgtcactaacaccattagttaatataaaacttgacagaagataaaaatggggcaaataaatcaattcagccgacccaaccatggacacaacacacaatgataccacaccacaaagactgatgatcacagacatgaggccattatcgcttgagactataataacatctctaaccagagatatcataacacataaatttatatacttgataaatcatgaatgcatagtaagaaaacttgatgaaagacaggccacatttacatttctggtcaactatgaaatgaaactattgcacaaagtgggaagcactaaatataaaaaatatactgaatacaacacaaaatatggcactttccctatgccaatatttatcaatcatgatgggttcttagaatgcattggcattaagcctaccaagcacacacccataatatacaagtatgatctcaatccatgaatatcaaaccaagattcaaacaatccgaaataacaactttatgcataatcacactccatagtccaaatggagcctgaaaattatagttatttaaaattcctgcaggaaggagagacataagatgaaagatggggcaaatacaaaaatggctcttagcaaagtcaagttgaatgatacactcaacaaagatcaacttctatcatccagcaaatataccatccaacggagcacaggagacagcattgacactcctaattatgatgtgcagaaacacattaataagttatgtggcatgttattaatcacagaagatgctaatcataaattcactgggttaataggtatgttatatgctatgtctagattaggaagagaagacaccataaaaatactcaaagatgcgggatatcatgttaaggcaaatggagtggatgtaacaacacatcgtcaagacattaatgggaaagaaatgaaatttgaagtgttaacattagcaagcttaacaactgaaattcaaatcaacattgagatagaatctagaaaatcctacaaaaaaatgctaaaagaaatgggagaggtggctccagaatacaggcatgactctcctgattgtgggatgataatattatgtatagcggcattagtaataaccaaattagcagcaggagatagatcaggtcttacagctgtgattaggagagctaataatgtcctaaaaaatgaaatgaaacgttataaaggtttattacccaaggatatagccaacagcttctatgaagtgtttgaaaaatatcctcactttatagatgtttttgttcattttggtatagcacaatcttctaccagaggtggcagtagagttgaagggatttttgcaggattgtttatgaatgcctatggtgcagggcaagtgatgttacggtggggggtcttagcaaaatcagttaaaaacattatgttaggacacgctagtgtacaagcagaaatggaacaagttgtggaggtgtatgagtatgctcagaaattgggtggagaagcaggattctaccatatattgaacaacccaaaagcatcactattatctttgactcaatttcctcacttctctagtgtagtattgggcaatgctgctggcctaggcataatgggagaatacagaggtacaccaaggaatcaagatttatatgatgctgcaaaagcatatgctgaacaactcaaagaaaatggtgtgattaactacagtgtattagatttgacagcagaagaactagaggctatcaaacatcagcttaatccaaaagataatgatgtagagctttgagttaataaaaaagtggggcaaataaatcatcatggaaaagtttgctcctgaattccatggagaagatgcaaacaacagagccaccaaattcctagaatcaataaagggcaaattcacatcacccaaagatcccaagaaaaaagatagtatcatatctgtcaactcaatagatatagaagtaaccaaagaaagccctataacatcaaattcaaccattataaacccaataaatgagacagatgatactgtagggaacaagcccaattatcaaagaaagcctctagtaagtttcaaagaagaccctacgccaagtgataatcctttttcaaaactatacaaagaaaccatagaaacatttgataacaatgaagaagaatctagctattcatatgaagaaataaatgatcagacaaacgataatataacagcaagattagataggattgatgagaaattaagtgaaatactaggaatgcttcacacattagtagtagcgagtgcaggacccacatctgctcgggatggtataagagatgccatggttggtttaagagaagaaatgatagaaaaaatcagaactgaagcattaatgaccaatgacagactagaagctatggcaagactcaggaatgaagaaagtgaaaagatggcaaaagacacatcagatgaagtgtctctcaatccaacatcagagaaactgaacaacctgttggaagggaatgatagtgacaatgatctatcacttgaagatttctgattagctaccaaactgtacatcaaaacacaacaccaatagaaaaccaacaaacaaaccaactcacccatccaaccaaacatctatctgctgattagccaaccagccaaaaaacaaccagccaatctaaaactagccacccggaaaaaatcgatactatagttacaaaaaaagatggggcaaatatggaaacatacgtgaataaacttcacgagggctccacatacacagctgctgttcaatacaatgtcctagaaaaagacgatgatcctgcatcacttacaatatgggtgcccatgttccaatcatccatgccagcagatctactcataaaagaactagccaatgtcaatatactagtgaaacaaatatccacacccaagggaccctcattaagagtcatgataaactcaagaagtgcagtgctagcacaaatgcccagcaaatttaccatatgtgccaatgtgtccttggatgaaagaagcaagctggcatatgatgtaaccacaccctgtgaaattaaggcatgcagtctaacatgcctaaaatcaaaaaatatgttaactacagttaaagatctcactatgaaaacactcaacccaacacatgacatcattgctttatgtgaatttgaaaatatagtaacatcaaaaaaagtcataataccaacatacctaagatctatcagcgtcagaaataaagatctgaacacacttgaaaatataacaaccactgaattcaaaaatgccattacaaatgcaaaaatcatcccttactcaggattattgttagtcatcacagtgactgacaacaaaggagcattcaaatacataaagccacaaagtcaattcatagtagatcttggagcttacctagaaaaagaaagtatatattatgttacaacaaattggaagcacacagctacacgatttgcaatcaaacccatggaagattaacctttttcctctacatcaatgagtagattcatacaaactttctaactacattcttcacttcacaatcataatcaccaaccctctgtggttcaatcaatcaaacaaaactcatcaagagttccagatcatcccaagtcattgttcatcagatccagtactcaaataagttaataaaaaatcggtccgttgacagaagataaaaatggggcaaatgcaaacatgaagtgccttttgtacttagcctttttattcattggggtgaattgcaagttcaccatagtttttccacacaaccaaaaaggaaactggaaaaatgttccttctaattaccattattgcccgtcaagctcagatttaaattggcataatgacttaataggcacagccttacaagtcaaaatgcccaagagtcacaaggctattcaagcagacggttggatgtgtcatgcttccaaatgggtcactacttgtgatttccgctggtatggaccgaagtatataacacattccatccgatccttcactccatctgtagaacaatgcaaggaaagcattgaacaaacgaaacaaggaacttggctgaatccaggcttccctcctcaaagttgtggatatgcaactgtgacggatgccgaagcagtgattgtccaggtgactcctcaccatgtgctggttgatgaatacacaggagaatgggttgattcacagttcatcaacggaaaatgcagcaattacatatgccccactgtccataactctacaacctggcattctgactataaggtcaaagggctatgtgattctaacctcatttccatggacatcaccttcttctcagaggacggagagctatcatccctgggaaaggagggcacagggttcagaagtaactactttgcttatgaaactggaggcaaggcctgcaaaatgcaatactgcaagcattggggagtcagactcccatcaggtgtctggttcgagatggctgataaggatctctttgctgcagccagattccctgaatgcccagaagggtcaagtatctctgctccatctcagacctcagtggatgtaagtctaattcaggacgttgagaggatcttggattattccctctgccaagaaacctggagcaaaatcagagcgggtcttccaatctctccagtggatctcagctatcttgctcctaaaaacccaggaaccggtcctgctttcaccataatcaatggtaccctaaaatactttgagaccagatacatcagagtcgatattgctgctccaatcctctcaagaatggtcggaatgatcagtggaactaccacagaaagggaactgtgggatgactgggcaccatatgaagacgtggaaattggacccaatggagttctgaggaccagttcaggatataagtttcctttatacatgattggacatggtatgttggactccgatcttcatcttagctcaaaggctcaggtgttcgaacatcctcacattcaagacgctgcttcgcaacttcctgatgatgagagtttattttttggtgatactgggctatccaaaaatccaatcgagcttgtagaaggttggttcagtagttggaaaagctctattgcctcttttttctttatcatagggttaatcattggactattcttggttctccgagttggtatccatctttgcattaaagccagaagcacaccagtcacattaagtaaggatcaactgagtggtataaataatattgcatttagtaactaatagtcattaaaaagcggccggccagtcataacaatgaactaggatattaagaccaaaaacaacgctggggcaaatgcaaacatgtccaaaaccgaggaccaacgcaccgccaagacactagaaaggacctgggacacttttaatcatctattattcatatcatcgtgcttatacaagttaaatcttaaatctatagcacaaatcacattatctattttggcaattataatctcaacctcacttataattgcagccatcatattcatagcctcggcaaaccacaaagtcacactaacaactgcaatcatacaagatgcaacgaaccagatcaagaacacaaccccaacatacctcacccagaatccccagcatggaatcagcttctccaatctgtccggaactacatcacaatccaccaccatactagcttcaacaacaccaagtgctgattcaaccccacaatccacaacagtcaagatcaaaaacacaacaacaacccaaatattacctagcaaacccaccacaaaacaacgccaaaataaaccacaaaacaaacccaacaatgattttcactttgaagtgttcaattttgtaccctgcagcatatgcagcaacaatccaacctgctgggccatctgcaagagaataccaaacaaaaaacctggaaagaaaaccaccaccaagcccacaaaaaaaccaaccctcaagacaaccaaaaaagatcccaaatcccaaaccacaaaaccaaaggaagtactcactaccaagcctacaggaaagccaaccatcaacaccactaaaacaaacatcagaactacactgctcacctccaacaccaaaggaaatccagaacacacaagtcaagaggaaaccctccactcaaccacctccgaaggctatccaagcccatcacaagtccacacaacatccggtcaagaggaaaccctccactcaaccacctccgaaggctatccaagcccatcacaagtctacacaacatccgagtacctatcacaatctctatcttcatccaacacaacaaaatgatagtcattaaaaagcacgcgtgtattgttgcaaaaagccatgaccaaatcaaacagaatcaaaatcaactctgggcccattgaataccaaattaacttactatttgtaaaaatgagaattggggcaaatatgtcacgaaggaatccttgcaaattcgaaattcgaggtcattgcttgaatggtaaaaggtgtcattttagtcataattattttgaatggccaccccatgcactgcttgtaagacaaaactttatgttaaacagaatacttaagtctatggataaaagcatagatactttgtcagaaataagtggagctgcagagttggacagaacagaagagtatgccctcggtgtagttggagtgctagagagttatataggatcaataaataatataactaaacaatcagcatgtgttgccatgagcaaactccttactgaactcaacagcgatgacatcaaaaaactaagggacaatgaagagccaaactcacccaaagtaagagtgtacaatactgtcatatcatatattgaaagcaacaggaagaacaataaacaaactatccatctgttaaaaagattgccagcagacgtattgaagaaaaccatcaaaaacacattggatatccacaagagcataaccatcaataacccaaaagaatcaactgttagtgatacgaacgaccatgccaaaaataatgatactacctgacaaatatccttgtagtataaattccatactaataacaagtaattgtagagtcactatgtataatcaaaaaaacacactatatatcaatcaaaacaaccaaaatagccatatatacccaccggatcaaccattcaatgaaatccattggacctctcaagacttgattgatgcaactcaaaattttctacaacatctaggtattactgatgatatatacacaatatatatattagtgtcataatactcaatcctaatacttaccacatcatcaaattattaactcaaacaattcaagctatgggacaaaatggatcccattattagtggaaattctgctaatgtttatctaactgatagttatttaaaaggtgttatttctttctcagaatgtaacgctttaggaagttacatattcaatggtccttatctcaaaaatgattataccaacttaattagtagacaaaatccattaatagaacacataaatctaaagaaactaaatataacacagtccttaatatctaagtatcataaaggtgaaataaaaatagaagaacctacttactttcagtcattacttatgacatacaagagtatgacctcttcagaacagactactactactaatttacttaaaaagataataagaagagctatagaaatcagtgatgtcaaagtctatgctatattgaataaactggggctcaaagaaaaagacaagattaaatccaataatggacaagatgaagacaactcagtcattactaccataatcaaagatgatatacttttagctgtcaaggataatcaatctcatcttaaagcagacaaaaatcaatccacaaaacaaaaagatacaatcaaaacaacacttttgaagaaattaatgtgttcgatgcaacatcctccatcatggttaatacattggtttaatttatacacaaaattaaacagcatattaacacaatatcgatctagtgaggtaaaaaaccatggttttatattgatagataatcatactcttagtggattccaatttattttgaatcaatatggttgtatagtttatcataaggaactcaaaagaattactgtgacaacttataatcaattcttgacatggaaagatattagccttagtagattaaatgtttgtttgattacatggattagtaactgtttgaacacattaaacaaaagcttaggcttaagatgtggattcaataatgttatcttgacacaattattcctttatggagattgtatactaaaactattccacaatgaggggttctacataataaaagaggtagagggatttattatgtctctaattttaaatataacagaagaagatcaattcagaaaacggttttataatagtatgctcaacaacatcacagatgccgccaacaaagctcaaaaaaatctgctatcaagagtatgtcatacattattagataagacaatatcagataatataataaatggcagatggataattctattgagtaagttcctaaaattaattaagcttgcaggtgacaataacctcaacaatctgagtgaattatattttttgttcagaatatttggacacccaatggtagatgaaagacaagccatggatgctgttaaagttaattgcaacgagaccaaattttatttgttaagtagtttgagtatgttaagaggagcttttatatatagaattataaaagggtttgtaaataattacaacagatggcctactttaagaaatgccattgtcttacccttaagatggttaacttactataaactaaacacttatccttccttgttggaacttacagaaagagatttgattgttctatcaggactacgtttctatcgagagtttcggttgcctaaaaaagtggatcttgaaatgatcataaatgataaggctatatcacctcctaaaaatttaatatggactagtttccctagaaattatatgccgtcacacatacaaaattatatagaacatgaaaaattaaaattctctgatagtgataaatcaagaagagtattagagtattatttaagagataacaaattcaatgaatgtgatttacacaactgtgtagttaatcaaagttatcttaacaacccgaatcatgtggtatcattgacaggcaaagaaagagaactcagtgtaggtagaatgtttgcaatgcaaccaggaatgttcagacaagttcaaatattagcagagaaaatgatagcagaaaacatattacaatttttccctgaaagtcttacaagatatggtgatctagaactacagaaaatattagaattgaaagcaggaataagtaacaaatcaaatcgttacaatgataattacaacaattacattagtaagtgctctatcatcacagatctcagcaaattcaatcaagcatttcgatatgaaacatcatgtatttgtagtgatgtactggatgaactgcatggtgtacaatctctattttcctggttacatttaactattcctcatgtcacaataatatgcacatataggcatgcacccccctatataaaggatcatattgtagatcttaacaatgtagatgagcaaagtggactatatagatatcatatgggtggtatcgaagggtggtgtcaaaaactatggaccatagaagctatatcactattagatctaatatctctcaaagggaaattctcaattactgctttaattaatggtgacaatcaatcaatagatataagtaaaccagtcagactcatggaaggtcaaactcatgctcaagcagattatttgctagcattaaatagtctcaaattactgtataaagagtatgcaggaataggccacaaattaaaaggaactgagacttatatatcgagagatatgcaatttatgagtaaaacgatccaacataacggtgtatattacccagctagtataaagaaagtcctaagagtgggaccgtggataaacactatacttgatgacttcaaagtgagtctagaatctataggtagtttgacacaagaattagaatatagaggtgaaagtctattatgcagtttaatatttagaaatgtatggttatataatcaaattgcattacaacttaaaaatcatgcattatgtaacaacaaattatatttggatatattaaaagttctaaaacacttaaaaaccttttttaatcttgataacattgatacagcattaacattgtatatgaatttgcccatgttatttggtggtggtgatcccaacttgttatatcgaagtttctatagaagaactcctgatttcctcacagaggctatagttcactctgtgttcatacttagttattatacaaaccatgatttaaaagataaacttcaagatctgtcagatgatagattgaataagttcttaacatgcataatcacgtttgataaaaaccccaatgctgaattcgttacattgatgagagatcctcaagctttaggatctgagaggcaagctaaaattactagcgaaatcaatagactggcagttaccgaggttttgagcacagctccaaacaaaatattttccaaaagtgcacaacactataccactacagagatagatcttaatgatattatgcaaaatatagaacctacatatcctcacgggctaagagttgtttatgagagtttacccttttataaagcagagaaaatagtaaatcttatatccggtacaaaatctataactaacatactggaaaagacttctgccatagacttaacagatattgatagagccactgagatgatgaggaaaaacataactttgcttataaggatattaccattagattgtaacagagataaaagagaaatattgagtatggaaaacctaagtattactgaattaagcaaatacgttagagaaagatcttggtctttatccaatatagttggtgttacatcacccagtatcatgtatacaatggacataaaatatacaacaagcactatagctagtggcataatcatagagaaatataatgtcaacagtttaacacgtggtgagagaggacccactaaaccatgggttggttcatctacacaagagaaaaagacaatgccagtttataatagacaagttttaaccaaaaaacagagagatcaaatagatctattagcaaaattggattgggtgtatgcatctatagataacaaggatgaatttatggaggaacttagcataggaactcttgggttaacatatgagaaggccaaaaaattattcccacaatatttgagtgttaactatttgcatcgtcttacagtcagtagtagaccatgtgaattccctgcatctataccagcttatagaactacaaattatcactttgatactagccctattaatcgcatattaacagaaaagtatggtgatgaagatattgatatagtattccaaaactgtataagctttggccttagcttaatgtctgtagtagaacaatttactaatgtatgtcctaacagaattattctcatacccaagcttaatgagatacatttgatgaaacctcccatattcacaggcgatgttgatattcacaagttaaaacaagtgatacaaaaacaacatatgtttttaccagacaaaataagtttgactcaatatgtggaattattcttaagtaataaaacactcaaatctggatctaatgttaattctaatttaatattggcgcataagatatctgactattttcataatacttacattttgagtactaatttagctggacattggattcttattatacaacttatgaaagattctaagggtatttttgaaaaagattggggagagggatatataactgatcatatgttcattaatttgaaagttttcttcaatgcttataagacatatctcttgtgttttcataaaggttacggcagagcaaagctggagtgtgatatgaatacttcagatctcctatgtgtattggaattaatagacagtagttattggaagtctatgtctaaggtgtttttagaacaaaaagttatcaaatacattcttagccaggatgcaagtttacatagagtaaaaggatgtcatagcttcaaactatggtttcttaaacgtcttaatgtagcagaattcacagtttgcccttgggttgttaacatagattatcatccaacacatatgaaagcaatattaacttatattgatcttgttagaatgggattgataaatatagatagaatatacattaaaaataaacacaagttcaatgatgagttttatacttctaatctgttttacattaattataacttctcagataatactcatctattaactaaacatataaggattgctaattccgaattagaaagtaattacaacaaattatatcatcctacaccagaaaccctagaaaatatactaaccaatccggttaaaagtaatgagaaaaagacactgagtgactattgtataggtaaaaatgttgactcaataatgttaccatcgttatctaataagaagcttattaaatcgtctacaatgattagaaccaattacagcagacaagatttgtataatttatttcctacggttgtgattgataaaattatagatcattcaggtaatacagccaaatctaaccaactttacactactacttctcatcaaatatccttagtgcacaatagcacatcactttattgcatgcttccttggcatcatattaatagattcaattttgtatttagttctacaggttgtaaaattagtatagagtatattttaaaagatcttaaaattaaggatcctaattgtatagcattcataggtgaaggagcagggaatttattattgcgtacagtagtggaacttcatcctgatataagatatatttacagaagtctgaaagattgcaatgatcatagtttaccaattgagtttttaaggctgtacaatggacatatcaacattgattatggtgaaaatttgaccattcctgctacagatgcaaccaacaacattcattggtcttatttacatataaagtttgctgaacctatcagtctttttgtctgtgatgctgaattgcctgtaacagtcaactggagtaagattataatagagtggagcaagcatgtaagaaaatgcaagtactgttcttcagttaataaatgtacattgatagtaaaatatcatgctcaagatgatatcgatttcaaattagacaacataactatattaaaaacttatgtatgcttaggtagtaagttaaagggatctgaagtttacttagtccttacaataggtcctgcaaatgtgttcccagtatttaatgtagtacaaaatgctaaattgatactatcaagaactaaaaatttcatcatgcctaaaaaagctgataaagagtctattgatgcaaatattaagagtttgataccctttctttgttaccctataacaaaaaaaggaattaatactgcattgtctaaattaaagagtgttgttagtggagatatactatcatattctatagctggacgtaatgaagttttcagcaataaacttataaatcataagcatatgaacatcttaaagtggttcaatcatgttttaaatttcagatcaacagaattaaactataatcatttatatatggtagaatctacttatcctcatctaagtgaattgttaaacagcttgacaaccaatgaacttaaaaaactgattaaaatcacaggtagtttgttatacaacttttataatgaataatgagcaaaaatcttataacaaaaatagctacacactaacattgtattcaattatagttattgaaaattaataattatataatttttaataacttctagtgaactaatcctaaaattatcattttgatctaggaagaataagtttaaatccaaatctaattggtttatatgtatattaactaaattacgagatattagtttttgacactttttttctcgt

SEQ ID NO: 10 - DNA, 14948 bp, synthetic construct
  misc_feature 1..14948: note = The sequence in which the F gene of Backbone construct A wasreplaced with the VSV G gene.
  source 1..14948: mol_type = other DNA
acgcgaaaaaatgcgtacaacaaacttgcgtaaaccaaaaaaatggggcaaataagaatttgataagtaccacttaaatttaactcctttggttagaggcgcgccatgggcagcaactcattgagtatgataaaagttagattgcaaaatctgtttgacaatgatgaagtagcattgttaaaaataacatgctatactgacaaattaatacagttaactaatgctttggctaaggcagttatacatacaatcaaattgaatggcattgtatttgtgcatgttattacaagtagtgatatttgccctaataataatattgtagtgaaatccaatttcacaacaatgccagtattacaaaatggaggttatatatgggaaatgatggaattaacacactgctctcaacctaatggcctaatagatgacaattgtgaaattaaattctccaaaaaactaagtgattcaacaatgaccaattatatgaatcaattatctgaattacttggatttgacctcaatccataaatcataataaatatcaactagcaaatcaatgtcactaacaccattagttaatataaaacttgacagaagataaaaatggggcaaataaatcaattcagccgacccaaccatggacacaacacacaatgataccacaccacaaagactgatgatcacagacatgaggccattatcgcttgagactataataacatctctaaccagagatatcataacacataaatttatatacttgataaatcatgaatgcatagtaagaaaacttgatgaaagacaggccacatttacatttctggtcaactatgaaatgaaactattgcacaaagtgggaagcactaaatataaaaaatatactgaatacaacacaaaatatggcactttccctatgccaatatttatcaatcatgatgggttcttagaatgcattggcattaagcctaccaagcacacacccataatatacaagtatgatctcaatccatgaatatcaaaccaagattcaaacaatccgaaataacaactttatgcataatcacactccatagtccaaatggagcctgaaaattatagttatttaaaattcctgcaggaaggagagacataagatgaaagatggggcaaatacaaaaatggctcttagcaaagtcaagttgaatgatacactcaacaaagatcaacttctatcatccagcaaatataccatccaacggagcacaggagacagcattgacactcctaattatgatgtgcagaaacacattaataagttatgtggcatgttattaatcacagaagatgctaatcataaattcactgggttaataggtatgttatatgctatgtctagattaggaagagaagacaccataaaaatactcaaagatgcgggatatcatgttaaggcaaatggagtggatgtaacaacacatcgtcaagacattaatgggaaagaaatgaaatttgaagtgttaacattagcaagcttaacaactgaaattcaaatcaacattgagatagaatctagaaaatcctacaaaaaaatgctaaaagaaatgggagaggtggctccagaatacaggcatgactctcctgattgtgggatgataatattatgtatagcggcattagtaataaccaaattagcagcaggagatagatcaggtcttacagctgtgattaggagagctaataatgtcctaaaaaatgaaatgaaacgttataaaggtttattacccaaggatatagccaacagcttctatgaagtgtttgaaaaatatcctcactttatagatgtttttgttcattttggtatagcacaatcttctaccagaggtggcagtagagttgaagggatttttgcaggattgtttatgaatgcctatggtgcagggcaagtgatgttacggtggggggtcttagcaaaatcagttaaaaacattatgttaggacacgctagtgtacaagcagaaatggaacaagttgtggaggtgtatgagtatgctcagaaattgggtggagaagcaggattctaccatatattgaacaacccaaaagcatcactattatctttgactcaatttcctcacttctctagtgtagtattgggcaatgctgctggcctaggcataatgggagaatacagaggtacaccaaggaatcaagatttatatgatgctgcaaaagcatatgctgaacaactcaaagaaaatggtgtgattaactacagtgtattagatttgacagcagaagaactagaggctatcaaacatcagcttaatccaaaagataatgatgtagagctttgagttaataaaaaagtggggcaaataaatcatcatggaaaagtttgctcctgaattccatggagaagatgcaaacaacagagccaccaaattcctagaatcaataaagggcaaattcacatcacccaaagatcccaagaaaaaagatagtatcatatctgtcaactcaatagatatagaagtaaccaaagaaagccctataacatcaaattcaaccattataaacccaataaatgagacagatgatactgtagggaacaagcccaattatcaaagaaagcctctagtaagtttcaaagaagaccctacgccaagtgataatcctttttcaaaactatacaaagaaaccatagaaacatttgataacaatgaagaagaatctagctattcatatgaagaaataaatgatcagacaaacgataatataacagcaagattagataggattgatgagaaattaagtgaaatactaggaatgcttcacacattagtagtagcgagtgcaggacccacatctgctcgggatggtataagagatgccatggttggtttaagagaagaaatgatagaaaaaatcagaactgaagcattaatgaccaatgacagactagaagctatggcaagactcaggaatgaagaaagtgaaaagatggcaaaagacacatcagatgaagtgtctctcaatccaacatcagagaaactgaacaacctgttggaagggaatgatagtgacaatgatctatcacttgaagatttctgattagctaccaaactgtacatcaaaacacaacaccaatagaaaaccaacaaacaaaccaactcacccatccaaccaaacatctatctgctgattagccaaccagccaaaaaacaaccagccaatctaaaactagccacccggaaaaaatcgatactatagttacaaaaaaagatggggcaaatatggaaacatacgtgaataaacttcacgagggctccacatacacagctgctgttcaatacaatgtcctagaaaaagacgatgatcctgcatcacttacaatatgggtgcccatgttccaatcatccatgccagcagatctactcataaaagaactagccaatgtcaatatactagtgaaacaaatatccacacccaagggaccctcattaagagtcatgataaactcaagaagtgcagtgctagcacaaatgcccagcaaatttaccatatgtgccaatgtgtccttggatgaaagaagcaagctggcatatgatgtaaccacaccctgtgaaattaaggcatgcagtctaacatgcctaaaatcaaaaaatatgttaactacagttaaagatctcactatgaaaacactcaacccaacacatgacatcattgctttatgtgaatttgaaaatatagtaacatcaaaaaaagtcataataccaacatacctaagatctatcagcgtcagaaataaagatctgaacacacttgaaaatataacaaccactgaattcaaaaatgccattacaaatgcaaaaatcatcccttactcaggattattgttagtcatcacagtgactgacaacaaaggagcattcaaatacataaagccacaaagtcaattcatagtagatcttggagcttacctagaaaaagaaagtatatattatgttacaacaaattggaagcacacagctacacgatttgcaatcaaacccatggaagattaacctttttcctctacatcaatgagtagattcatacaaactttctaactacattcttcacttcacaatcataatcaccaaccctctgtggttcaatcaatcaaacaaaactcatcaagagttccagatcatcccaagtcattgttcatcagatccagtactcaaataagttaataaaaaatccacatggggcaaataatcattgagggaaatccaactaatcacaacatctgtcaacatagacaagtcaacacgctagataaaatcaaccaatggaaaatacatccataactatagaattctcaagcaaattctggccttactttacactaatacacatgataacaacaataatctctttgataatcataatctccatcatgattgcaatactaaacaaactctgcgaatataatgtattccataacaaaacctttgagctaccaagagctcgagtcaatacatagcattcaccaatctgatagctcaaaacagtaaccttgcatttgtaaatgaactaccctcacttcttcacaaaaccacatcaacatctcaccatgcaagccatcatctataccataaagtagttaattaaaaatggccggccagtcataacaatgaactaggatattaagaccaaaaacaacgctggggcaaatgcaaacatgtccaaaaccgaggaccaacgcaccgccaagacactagaaaggacctgggacacttttaatcatctattattcatatcatcgtgcttatacaagttaaatcttaaatctatagcacaaatcacattatctattttggcaattataatctcaacctcacttataattgcagccatcatattcatagcctcggcaaaccacaaagtcacactaacaactgcaatcatacaagatgcaacgaaccagatcaagaacacaaccccaacatacctcacccagaatccccagcatggaatcagcttctccaatctgtccggaactacatcacaatccaccaccatactagcttcaacaacaccaagtgctgattcaaccccacaatccacaacagtcaagatcaaaaacacaacaacaacccaaatattacctagcaaacccaccacaaaacaacgccaaaataaaccacaaaacaaacccaacaatgattttcactttgaagtgttcaattttgtaccctgcagcatatgcagcaacaatccaacctgctgggccatctgcaagagaataccaaacaaaaaacctggaaagaaaaccaccaccaagcccacaaaaaaaccaaccctcaagacaaccaaaaaagatcccaaatcccaaaccacaaaaccaaaggaagtactcactaccaagcctacaggaaagccaaccatcaacaccactaaaacaaacatcagaactacactgctcacctccaacaccaaaggaaatccagaacacacaagtcaagaggaaaccctccactcaaccacctccgaaggctatccaagcccatcacaagtccacacaacatccggtcaagaggaaaccctccactcaaccacctccgaaggctatccaagcccatcacaagtctacacaacatccgagtacctatcacaatctctatcttcatccaacacaacaaaatgatagtcattaaaaagcacgcgtttgacagaagataaaaatggggcaaatgcaaacatgaagtgccttttgtacttagcctttttattcattggggtgaattgcaagttcaccatagtttttccacacaaccaaaaaggaaactggaaaaatgttccttctaattaccattattgcccgtcaagctcagatttaaattggcataatgacttaataggcacagccttacaagtcaaaatgcccaagagtcacaaggctattcaagcagacggttggatgtgtcatgcttccaaatgggtcactacttgtgatttccgctggtatggaccgaagtatataacacattccatccgatccttcactccatctgtagaacaatgcaaggaaagcattgaacaaacgaaacaaggaacttggctgaatccaggcttccctcctcaaagttgtggatatgcaactgtgacggatgccgaagcagtgattgtccaggtgactcctcaccatgtgctggttgatgaatacacaggagaatgggttgattcacagttcatcaacggaaaatgcagcaattacatatgccccactgtccataactctacaacctggcattctgactataaggtcaaagggctatgtgattctaacctcatttccatggacatcaccttcttctcagaggacggagagctatcatccctgggaaaggagggcacagggttcagaagtaactactttgcttatgaaactggaggcaaggcctgcaaaatgcaatactgcaagcattggggagtcagactcccatcaggtgtctggttcgagatggctgataaggatctctttgctgcagccagattccctgaatgcccagaagggtcaagtatctctgctccatctcagacctcagtggatgtaagtctaattcaggacgttgagaggatcttggattattccctctgccaagaaacctggagcaaaatcagagcgggtcttccaatctctccagtggatctcagctatcttgctcctaaaaacccaggaaccggtcctgctttcaccataatcaatggtaccctaaaatactttgagaccagatacatcagagtcgatattgctgctccaatcctctcaagaatggtcggaatgatcagtggaactaccacagaaagggaactgtgggatgactgggcaccatatgaagacgtggaaattggacccaatggagttctgaggaccagttcaggatataagtttcctttatacatgattggacatggtatgttggactccgatcttcatcttagctcaaaggctcaggtgttcgaacatcctcacattcaagacgctgcttcgcaacttcctgatgatgagagtttattttttggtgatactgggctatccaaaaatccaatcgagcttgtagaaggttggttcagtagttggaaaagctctattgcctcttttttctttatcatagggttaatcattggactattcttggttctccgagttggtatccatctttgcattaaagccagaagcacaccagtcacattaagtaaggatcaactgagtggtataaataatattgcatttagtaactaatagtcattaaaaagcgggcccattgaataccaaattaacttactatttgtaaaaatgagaattggggcaaatatgtcacgaaggaatccttgcaaattcgaaattcgaggtcattgcttgaatggtaaaaggtgtcattttagtcataattattttgaatggccaccccatgcactgcttgtaagacaaaactttatgttaaacagaatacttaagtctatggataaaagcatagatactttgtcagaaataagtggagctgcagagttggacagaacagaagagtatgccctcggtgtagttggagtgctagagagttatataggatcaataaataatataactaaacaatcagcatgtgttgccatgagcaaactccttactgaactcaacagcgatgacatcaaaaaactaagggacaatgaagagccaaactcacccaaagtaagagtgtacaatactgtcatatcatatattgaaagcaacaggaagaacaataaacaaactatccatctgttaaaaagattgccagcagacgtattgaagaaaaccatcaaaaacacattggatatccacaagagcataaccatcaataacccaaaagaatcaactgttagtgatacgaacgaccatgccaaaaataatgatactacctgacaaatatccttgtagtataaattccatactaataacaagtaattgtagagtcactatgtataatcaaaaaaacacactatatatcaatcaaaacaaccaaaatagccatatatacccaccggatcaaccattcaatgaaatccattggacctctcaagacttgattgatgcaactcaaaattttctacaacatctaggtattactgatgatatatacacaatatatatattagtgtcataatactcaatcctaatacttaccacatcatcaaattattaactcaaacaattcaagctatgggacaaaatggatcccattattagtggaaattctgctaatgtttatctaactgatagttatttaaaaggtgttatttctttctcagaatgtaacgctttaggaagttacatattcaatggtccttatctcaaaaatgattataccaacttaattagtagacaaaatccattaatagaacacataaatctaaagaaactaaatataacacagtccttaatatctaagtatcataaaggtgaaataaaaatagaagaacctacttactttcagtcattacttatgacatacaagagtatgacctcttcagaacagactactactactaatttacttaaaaagataataagaagagctatagaaatcagtgatgtcaaagtctatgctatattgaataaactggggctcaaagaaaaagacaagattaaatccaataatggacaagatgaagacaactcagtcattactaccataatcaaagatgatatacttttagctgtcaaggataatcaatctcatcttaaagcagacaaaaatcaatccacaaaacaaaaagatacaatcaaaacaacacttttgaagaaattaatgtgttcgatgcaacatcctccatcatggttaatacattggtttaatttatacacaaaattaaacagcatattaacacaatatcgatctagtgaggtaaaaaaccatggttttatattgatagataatcatactcttagtggattccaatttattttgaatcaatatggttgtatagtttatcataaggaactcaaaagaattactgtgacaacttataatcaattcttgacatggaaagatattagccttagtagattaaatgtttgtttgattacatggattagtaactgtttgaacacattaaacaaaagcttaggcttaagatgtggattcaataatgttatcttgacacaattattcctttatggagattgtatactaaaactattccacaatgaggggttctacataataaaagaggtagagggatttattatgtctctaattttaaatataacagaagaagatcaattcagaaaacggttttataatagtatgctcaacaacatcacagatgccgccaacaaagctcaaaaaaatctgctatcaagagtatgtcatacattattagataagacaatatcagataatataataaatggcagatggataattctattgagtaagttcctaaaattaattaagcttgcaggtgacaataacctcaacaatctgagtgaattatattttttgttcagaatatttggacacccaatggtagatgaaagacaagccatggatgctgttaaagttaattgcaacgagaccaaattttatttgttaagtagtttgagtatgttaagaggagcttttatatatagaattataaaagggtttgtaaataattacaacagatggcctactttaagaaatgccattgtcttacccttaagatggttaacttactataaactaaacacttatccttccttgttggaacttacagaaagagatttgattgttctatcaggactacgtttctatcgagagtttcggttgcctaaaaaagtggatcttgaaatgatcataaatgataaggctatatcacctcctaaaaatttaatatggactagtttccctagaaattatatgccgtcacacatacaaaattatatagaacatgaaaaattaaaattctctgatagtgataaatcaagaagagtattagagtattatttaagagataacaaattcaatgaatgtgatttacacaactgtgtagttaatcaaagttatcttaacaacccgaatcatgtggtatcattgacaggcaaagaaagagaactcagtgtaggtagaatgtttgcaatgcaaccaggaatgttcagacaagttcaaatattagcagagaaaatgatagcagaaaacatattacaatttttccctgaaagtcttacaagatatggtgatctagaactacagaaaatattagaattgaaagcaggaataagtaacaaatcaaatcgttacaatgataattacaacaattacattagtaagtgctctatcatcacagatctcagcaaattcaatcaagcatttcgatatgaaacatcatgtatttgtagtgatgtactggatgaactgcatggtgtacaatctctattttcctggttacatttaactattcctcatgtcacaataatatgcacatataggcatgcacccccctatataaaggatcatattgtagatcttaacaatgtagatgagcaaagtggactatatagatatcatatgggtggtatcgaagggtggtgtcaaaaactatggaccatagaagctatatcactattagatctaatatctctcaaagggaaattctcaattactgctttaattaatggtgacaatcaatcaatagatataagtaaaccagtcagactcatggaaggtcaaactcatgctcaagcagattatttgctagcattaaatagtctcaaattactgtataaagagtatgcaggaataggccacaaattaaaaggaactgagacttatatatcgagagatatgcaatttatgagtaaaacgatccaacataacggtgtatattacccagctagtataaagaaagtcctaagagtgggaccgtggataaacactatacttgatgacttcaaagtgagtctagaatctataggtagtttgacacaagaattagaatatagaggtgaaagtctattatgcagtttaatatttagaaatgtatggttatataatcaaattgcattacaacttaaaaatcatgcattatgtaacaacaaattatatttggatatattaaaagttctaaaacacttaaaaaccttttttaatcttgataacattgatacagcattaacattgtatatgaatttgcccatgttatttggtggtggtgatcccaacttgttatatcgaagtttctatagaagaactcctgatttcctcacagaggctatagttcactctgtgttcatacttagttattatacaaaccatgatttaaaagataaacttcaagatctgtcagatgatagattgaataagttcttaacatgcataatcacgtttgataaaaaccccaatgctgaattcgttacattgatgagagatcctcaagctttaggatctgagaggcaagctaaaattactagcgaaatcaatagactggcagttaccgaggttttgagcacagctccaaacaaaatattttccaaaagtgcacaacactataccactacagagatagatcttaatgatattatgcaaaatatagaacctacatatcctcacgggctaagagttgtttatgagagtttacccttttataaagcagagaaaatagtaaatcttatatccggtacaaaatctataactaacatactggaaaagacttctgccatagacttaacagatattgatagagccactgagatgatgaggaaaaacataactttgcttataaggatattaccattagattgtaacagagataaaagagaaatattgagtatggaaaacctaagtattactgaattaagcaaatacgttagagaaagatcttggtctttatccaatatagttggtgttacatcacccagtatcatgtatacaatggacataaaatatacaacaagcactatagctagtggcataatcatagagaaatataatgtcaacagtttaacacgtggtgagagaggacccactaaaccatgggttggttcatctacacaagagaaaaagacaatgccagtttataatagacaagttttaaccaaaaaacagagagatcaaatagatctattagcaaaattggattgggtgtatgcatctatagataacaaggatgaatttatggaggaacttagcataggaactcttgggttaacatatgagaaggccaaaaaattattcccacaatatttgagtgttaactatttgcatcgtcttacagtcagtagtagaccatgtgaattccctgcatctataccagcttatagaactacaaattatcactttgatactagccctattaatcgcatattaacagaaaagtatggtgatgaagatattgatatagtattccaaaactgtataagctttggccttagcttaatgtctgtagtagaacaatttactaatgtatgtcctaacagaattattctcatacccaagcttaatgagatacatttgatgaaacctcccatattcacaggcgatgttgatattcacaagttaaaacaagtgatacaaaaacaacatatgtttttaccagacaaaataagtttgactcaatatgtggaattattcttaagtaataaaacactcaaatctggatctaatgttaattctaatttaatattggcgcataagatatctgactattttcataatacttacattttgagtactaatttagctggacattggattcttattatacaacttatgaaagattctaagggtatttttgaaaaagattggggagagggatatataactgatcatatgttcattaatttgaaagttttcttcaatgcttataagacatatctcttgtgttttcataaaggttacggcagagcaaagctggagtgtgatatgaatacttcagatctcctatgtgtattggaattaatagacagtagttattggaagtctatgtctaaggtgtttttagaacaaaaagttatcaaatacattcttagccaggatgcaagtttacatagagtaaaaggatgtcatagcttcaaactatggtttcttaaacgtcttaatgtagcagaattcacagtttgcccttgggttgttaacatagattatcatccaacacatatgaaagcaatattaacttatattgatcttgttagaatgggattgataaatatagatagaatatacattaaaaataaacacaagttcaatgatgagttttatacttctaatctgttttacattaattataacttctcagataatactcatctattaactaaacatataaggattgctaattccgaattagaaagtaattacaacaaattatatcatcctacaccagaaaccctagaaaatatactaaccaatccggttaaaagtaatgagaaaaagacactgagtgactattgtataggtaaaaatgttgactcaataatgttaccatcgttatctaataagaagcttattaaatcgtctacaatgattagaaccaattacagcagacaagatttgtataatttatttcctacggttgtgattgataaaattatagatcattcaggtaatacagccaaatctaaccaactttacactactacttctcatcaaatatccttagtgcacaatagcacatcactttattgcatgcttccttggcatcatattaatagattcaattttgtatttagttctacaggttgtaaaattagtatagagtatattttaaaagatcttaaaattaaggatcctaattgtatagcattcataggtgaaggagcagggaatttattattgcgtacagtagtggaacttcatcctgatataagatatatttacagaagtctgaaagattgcaatgatcatagtttaccaattgagtttttaaggctgtacaatggacatatcaacattgattatggtgaaaatttgaccattcctgctacagatgcaaccaacaacattcattggtcttatttacatataaagtttgctgaacctatcagtctttttgtctgtgatgctgaattgcctgtaacagtcaactggagtaagattataatagagtggagcaagcatgtaagaaaatgcaagtactgttcttcagttaataaatgtacattgatagtaaaatatcatgctcaagatgatatcgatttcaaattagacaacataactatattaaaaacttatgtatgcttaggtagtaagttaaagggatctgaagtttacttagtccttacaataggtcctgcaaatgtgttcccagtatttaatgtagtacaaaatgctaaattgatactatcaagaactaaaaatttcatcatgcctaaaaaagctgataaagagtctattgatgcaaatattaagagtttgataccctttctttgttaccctataacaaaaaaaggaattaatactgcattgtctaaattaaagagtgttgttagtggagatatactatcatattctatagctggacgtaatgaagttttcagcaataaacttataaatcataagcatatgaacatcttaaagtggttcaatcatgttttaaatttcagatcaacagaattaaactataatcatttatatatggtagaatctacttatcctcatctaagtgaattgttaaacagcttgacaaccaatgaacttaaaaaactgattaaaatcacaggtagtttgttatacaacttttataatgaataatgagcaaaaatcttataacaaaaatagctacacactaacattgtattcaattatagttattgaaaattaataattatataatttttaataacttctagtgaactaatcctaaaattatcattttgatctaggaagaataagtttaaatccaaatctaattggtttatatgtatattaactaaattacgagatattagtttttgacactttttttctcgt

SEQ ID NO: 11 - DNA, 16823 bp, synthetic construct
  misc_feature 1..16823: note = A sequence in which SEQ ID NO: 10 was digested with ApaI and SEQID NO: 4 was inserted.
  source 1..16823: mol_type = other DNA
acgcgaaaaaatgcgtacaacaaacttgcgtaaaccaaaaaaatggggcaaataagaatttgataagtaccacttaaatttaactcctttggttagaggcgcgccatgggcagcaactcattgagtatgataaaagttagattgcaaaatctgtttgacaatgatgaagtagcattgttaaaaataacatgctatactgacaaattaatacagttaactaatgctttggctaaggcagttatacatacaatcaaattgaatggcattgtatttgtgcatgttattacaagtagtgatatttgccctaataataatattgtagtgaaatccaatttcacaacaatgccagtattacaaaatggaggttatatatgggaaatgatggaattaacacactgctctcaacctaatggcctaatagatgacaattgtgaaattaaattctccaaaaaactaagtgattcaacaatgaccaattatatgaatcaattatctgaattacttggatttgacctcaatccataaatcataataaatatcaactagcaaatcaatgtcactaacaccattagttaatataaaacttgacagaagataaaaatggggcaaataaatcaattcagccgacccaaccatggacacaacacacaatgataccacaccacaaagactgatgatcacagacatgaggccattatcgcttgagactataataacatctctaaccagagatatcataacacataaatttatatacttgataaatcatgaatgcatagtaagaaaacttgatgaaagacaggccacatttacatttctggtcaactatgaaatgaaactattgcacaaagtgggaagcactaaatataaaaaatatactgaatacaacacaaaatatggcactttccctatgccaatatttatcaatcatgatgggttcttagaatgcattggcattaagcctaccaagcacacacccataatatacaagtatgatctcaatccatgaatatcaaaccaagattcaaacaatccgaaataacaactttatgcataatcacactccatagtccaaatggagcctgaaaattatagttatttaaaattcctgcaggaaggagagacataagatgaaagatggggcaaatacaaaaatggctcttagcaaagtcaagttgaatgatacactcaacaaagatcaacttctatcatccagcaaatataccatccaacggagcacaggagacagcattgacactcctaattatgatgtgcagaaacacattaataagttatgtggcatgttattaatcacagaagatgctaatcataaattcactgggttaataggtatgttatatgctatgtctagattaggaagagaagacaccataaaaatactcaaagatgcgggatatcatgttaaggcaaatggagtggatgtaacaacacatcgtcaagacattaatgggaaagaaatgaaatttgaagtgttaacattagcaagcttaacaactgaaattcaaatcaacattgagatagaatctagaaaatcctacaaaaaaatgctaaaagaaatgggagaggtggctccagaatacaggcatgactctcctgattgtgggatgataatattatgtatagcggcattagtaataaccaaattagcagcaggagatagatcaggtcttacagctgtgattaggagagctaataatgtcctaaaaaatgaaatgaaacgttataaaggtttattacccaaggatatagccaacagcttctatgaagtgtttgaaaaatatcctcactttatagatgtttttgttcattttggtatagcacaatcttctaccagaggtggcagtagagttgaagggatttttgcaggattgtttatgaatgcctatggtgcagggcaagtgatgttacggtggggggtcttagcaaaatcagttaaaaacattatgttaggacacgctagtgtacaagcagaaatggaacaagttgtggaggtgtatgagtatgctcagaaattgggtggagaagcaggattctaccatatattgaacaacccaaaagcatcactattatctttgactcaatttcctcacttctctagtgtagtattgggcaatgctgctggcctaggcataatgggagaatacagaggtacaccaaggaatcaagatttatatgatgctgcaaaagcatatgctgaacaactcaaagaaaatggtgtgattaactacagtgtattagatttgacagcagaagaactagaggctatcaaacatcagcttaatccaaaagataatgatgtagagctttgagttaataaaaaagtggggcaaataaatcatcatggaaaagtttgctcctgaattccatggagaagatgcaaacaacagagccaccaaattcctagaatcaataaagggcaaattcacatcacccaaagatcccaagaaaaaagatagtatcatatctgtcaactcaatagatatagaagtaaccaaagaaagccctataacatcaaattcaaccattataaacccaataaatgagacagatgatactgtagggaacaagcccaattatcaaagaaagcctctagtaagtttcaaagaagaccctacgccaagtgataatcctttttcaaaactatacaaagaaaccatagaaacatttgataacaatgaagaagaatctagctattcatatgaagaaataaatgatcagacaaacgataatataacagcaagattagataggattgatgagaaattaagtgaaatactaggaatgcttcacacattagtagtagcgagtgcaggacccacatctgctcgggatggtataagagatgccatggttggtttaagagaagaaatgatagaaaaaatcagaactgaagcattaatgaccaatgacagactagaagctatggcaagactcaggaatgaagaaagtgaaaagatggcaaaagacacatcagatgaagtgtctctcaatccaacatcagagaaactgaacaacctgttggaagggaatgatagtgacaatgatctatcacttgaagatttctgattagctaccaaactgtacatcaaaacacaacaccaatagaaaaccaacaaacaaaccaactcacccatccaaccaaacatctatctgctgattagccaaccagccaaaaaacaaccagccaatctaaaactagccacccggaaaaaatcgatactatagttacaaaaaaagatggggcaaatatggaaacatacgtgaataaacttcacgagggctccacatacacagctgctgttcaatacaatgtcctagaaaaagacgatgatcctgcatcacttacaatatgggtgcccatgttccaatcatccatgccagcagatctactcataaaagaactagccaatgtcaatatactagtgaaacaaatatccacacccaagggaccctcattaagagtcatgataaactcaagaagtgcagtgctagcacaaatgcccagcaaatttaccatatgtgccaatgtgtccttggatgaaagaagcaagctggcatatgatgtaaccacaccctgtgaaattaaggcatgcagtctaacatgcctaaaatcaaaaaatatgttaactacagttaaagatctcactatgaaaacactcaacccaacacatgacatcattgctttatgtgaatttgaaaatatagtaacatcaaaaaaagtcataataccaacatacctaagatctatcagcgtcagaaataaagatctgaacacacttgaaaatataacaaccactgaattcaaaaatgccattacaaatgcaaaaatcatcccttactcaggattattgttagtcatcacagtgactgacaacaaaggagcattcaaatacataaagccacaaagtcaattcatagtagatcttggagcttacctagaaaaagaaagtatatattatgttacaacaaattggaagcacacagctacacgatttgcaatcaaacccatggaagattaacctttttcctctacatcaatgagtagattcatacaaactttctaactacattcttcacttcacaatcataatcaccaaccctctgtggttcaatcaatcaaacaaaactcatcaagagttccagatcatcccaagtcattgttcatcagatccagtactcaaataagttaataaaaaatccacatggggcaaataatcattgagggaaatccaactaatcacaacatctgtcaacatagacaagtcaacacgctagataaaatcaaccaatggaaaatacatccataactatagaattctcaagcaaattctggccttactttacactaatacacatgataacaacaataatctctttgataatcataatctccatcatgattgcaatactaaacaaactctgcgaatataatgtattccataacaaaacctttgagctaccaagagctcgagtcaatacatagcattcaccaatctgatagctcaaaacagtaaccttgcatttgtaaatgaactaccctcacttcttcacaaaaccacatcaacatctcaccatgcaagccatcatctataccataaagtagttaattaaaaatggccggccagtcataacaatgaactaggatattaagaccaaaaacaacgctggggcaaatgcaaacatgtccaaaaccgaggaccaacgcaccgccaagacactagaaaggacctgggacacttttaatcatctattattcatatcatcgtgcttatacaagttaaatcttaaatctatagcacaaatcacattatctattttggcaattataatctcaacctcacttataattgcagccatcatattcatagcctcggcaaaccacaaagtcacactaacaactgcaatcatacaagatgcaacgaaccagatcaagaacacaaccccaacatacctcacccagaatccccagcatggaatcagcttctccaatctgtccggaactacatcacaatccaccaccatactagcttcaacaacaccaagtgctgattcaaccccacaatccacaacagtcaagatcaaaaacacaacaacaacccaaatattacctagcaaacccaccacaaaacaacgccaaaataaaccacaaaacaaacccaacaatgattttcactttgaagtgttcaattttgtaccctgcagcatatgcagcaacaatccaacctgctgggccatctgcaagagaataccaaacaaaaaacctggaaagaaaaccaccaccaagcccacaaaaaaaccaaccctcaagacaaccaaaaaagatcccaaatcccaaaccacaaaaccaaaggaagtactcactaccaagcctacaggaaagccaaccatcaacaccactaaaacaaacatcagaactacactgctcacctccaacaccaaaggaaatccagaacacacaagtcaagaggaaaccctccactcaaccacctccgaaggctatccaagcccatcacaagtccacacaacatccggtcaagaggaaaccctccactcaaccacctccgaaggctatccaagcccatcacaagtctacacaacatccgagtacctatcacaatctctatcttcatccaacacaacaaaatgatagtcattaaaaagcacgcgtttgacagaagataaaaatggggcaaatgcaaacatgaagtgccttttgtacttagcctttttattcattggggtgaattgcaagttcaccatagtttttccacacaaccaaaaaggaaactggaaaaatgttccttctaattaccattattgcccgtcaagctcagatttaaattggcataatgacttaataggcacagccttacaagtcaaaatgcccaagagtcacaaggctattcaagcagacggttggatgtgtcatgcttccaaatgggtcactacttgtgatttccgctggtatggaccgaagtatataacacattccatccgatccttcactccatctgtagaacaatgcaaggaaagcattgaacaaacgaaacaaggaacttggctgaatccaggcttccctcctcaaagttgtggatatgcaactgtgacggatgccgaagcagtgattgtccaggtgactcctcaccatgtgctggttgatgaatacacaggagaatgggttgattcacagttcatcaacggaaaatgcagcaattacatatgccccactgtccataactctacaacctggcattctgactataaggtcaaagggctatgtgattctaacctcatttccatggacatcaccttcttctcagaggacggagagctatcatccctgggaaaggagggcacagggttcagaagtaactactttgcttatgaaactggaggcaaggcctgcaaaatgcaatactgcaagcattggggagtcagactcccatcaggtgtctggttcgagatggctgataaggatctctttgctgcagccagattccctgaatgcccagaagggtcaagtatctctgctccatctcagacctcagtggatgtaagtctaattcaggacgttgagaggatcttggattattccctctgccaagaaacctggagcaaaatcagagcgggtcttccaatctctccagtggatctcagctatcttgctcctaaaaacccaggaaccggtcctgctttcaccataatcaatggtaccctaaaatactttgagaccagatacatcagagtcgatattgctgctccaatcctctcaagaatggtcggaatgatcagtggaactaccacagaaagggaactgtgggatgactgggcaccatatgaagacgtggaaattggacccaatggagttctgaggaccagttcaggatataagtttcctttatacatgattggacatggtatgttggactccgatcttcatcttagctcaaaggctcaggtgttcgaacatcctcacattcaagacgctgcttcgcaacttcctgatgatgagagtttattttttggtgatactgggctatccaaaaatccaatcgagcttgtagaaggttggttcagtagttggaaaagctctattgcctcttttttctttatcatagggttaatcattggactattcttggttctccgagttggtatccatctttgcattaaagccagaagcacaccagtcacattaagtaaggatcaactgagtggtataaataatattgcatttagtaactaatagtcattaaaaagcgggcccgtattgttgcaaaaagccatgaccaaatcaaacagaatcaaaatcaactctggggcaaataacaatggagttgccaatcctcaaaacaaatgctattaccacaatccttgctgcagtcacactctgtttcgcttccagtcaaaacatcactgaagaattttatcaatcaacatgcagtgcagtcagcaaaggctatcttagtgctctaagaactggttggtatactagtgttataactatagaattaagtaatatcaaggaaaataagtgtaatggtacagacgctaaggtaaaattaataaaacaagaattagataaatataaaaatgctgtaacagaattgcagttgctcatgcaaagcacaccagcagccaacaatcgagccagaagagaactaccaagatttatgaattatacactcaacaataccaaaaacaccaatgtaacattaagtaagaaaaggaaaagaagatttcttggatttttgttaggtgttggatctgcaatcgccagtggcattgccgtatccaaggtcctgcacctagaaggggaagtgaacaaaatcaaaagtgctctactatccacaaacaaggctgtagtcagcttatctaatggagtcagtgtcttaaccagcaaggtgttagacctcaaaaactatatagataaacagttgttacctattgttaacaagcaaagctgcagcatatcaaacattgaaactgtgatagagttccaacaaaagaacaacagactactagagattaccagagaatttagtgttaatgcaggtgtaactactcctgtaagcacttatatgttaactaatagtgagttattatcattaatcaatgatatgcctataacaaatgatcagaaaaagttaatgtccagcaatgttcaaatagttagacagcaaagttactctatcatgtcaataataaaagaggaagtcttggcatatgtagtacaattaccactatatggtgtaatagatactccttgttggaaactacacacatcccctttatgtacaaccaacacaaaggaaggatccaacatctgcttaacaagaaccgacagaggatggtactgtgacaatgcaggatcagtatcctttttcccacaagctgaaacatgtaaagttcaatcgaatcgggtgttttgtgacacaatgaacagtttaacattaccaagtgaggtaaatctctgcaacattgacatattcaaccccaaatatgattgcaaaattatgacttcaaaaacagatgtaagcagctccgttatcacatctctaggagccattgtgtcatgctatggcaaaaccaaatgtacagcatccaataaaaatcgtgggatcataaagacattctctaacgggtgtgattatgtatcaaataagggggtggatactgtgtctgtaggtaatacattatattatgtaaataagcaagaaggcaaaagtctctatgtaaaaggtgaaccaataataaatttctatgatccattagtgttcccctctctcctgtgggatgcatcaatatctcaagtcaatgagaaaattaatcagagtctagcatttatccgtaaatcagatgaattattaggctctggcggaagcggatacatccctgaggcaccaagggacggacaggcctacgtgcgcaaggatggcgagtgggtgctgctgtccacctttctgtgaataaaaatagcacctaatcatattcttacaatggttcgctatttgaccatagataacccatctatcattagattatcctaaaatttgaacttcatcacaactttcatctataaaccatctcacttacactttttaagtagatttctattttatagttatataaaacagggcccattgaataccaaattaacttactatttgtaaaaatgagaattggggcaaatatgtcacgaaggaatccttgcaaattcgaaattcgaggtcattgcttgaatggtaaaaggtgtcattttagtcataattattttgaatggccaccccatgcactgcttgtaagacaaaactttatgttaaacagaatacttaagtctatggataaaagcatagatactttgtcagaaataagtggagctgcagagttggacagaacagaagagtatgccctcggtgtagttggagtgctagagagttatataggatcaataaataatataactaaacaatcagcatgtgttgccatgagcaaactccttactgaactcaacagcgatgacatcaaaaaactaagggacaatgaagagccaaactcacccaaagtaagagtgtacaatactgtcatatcatatattgaaagcaacaggaagaacaataaacaaactatccatctgttaaaaagattgccagcagacgtattgaagaaaaccatcaaaaacacattggatatccacaagagcataaccatcaataacccaaaagaatcaactgttagtgatacgaacgaccatgccaaaaataatgatactacctgacaaatatccttgtagtataaattccatactaataacaagtaattgtagagtcactatgtataatcaaaaaaacacactatatatcaatcaaaacaaccaaaatagccatatatacccaccggatcaaccattcaatgaaatccattggacctctcaagacttgattgatgcaactcaaaattttctacaacatctaggtattactgatgatatatacacaatatatatattagtgtcataatactcaatcctaatacttaccacatcatcaaattattaactcaaacaattcaagctatgggacaaaatggatcccattattagtggaaattctgctaatgtttatctaactgatagttatttaaaaggtgttatttctttctcagaatgtaacgctttaggaagttacatattcaatggtccttatctcaaaaatgattataccaacttaattagtagacaaaatccattaatagaacacataaatctaaagaaactaaatataacacagtccttaatatctaagtatcataaaggtgaaataaaaatagaagaacctacttactttcagtcattacttatgacatacaagagtatgacctcttcagaacagactactactactaatttacttaaaaagataataagaagagctatagaaatcagtgatgtcaaagtctatgctatattgaataaactggggctcaaagaaaaagacaagattaaatccaataatggacaagatgaagacaactcagtcattactaccataatcaaagatgatatacttttagctgtcaaggataatcaatctcatcttaaagcagacaaaaatcaatccacaaaacaaaaagatacaatcaaaacaacacttttgaagaaattaatgtgttcgatgcaacatcctccatcatggttaatacattggtttaatttatacacaaaattaaacagcatattaacacaatatcgatctagtgaggtaaaaaaccatggttttatattgatagataatcatactcttagtggattccaatttattttgaatcaatatggttgtatagtttatcataaggaactcaaaagaattactgtgacaacttataatcaattcttgacatggaaagatattagccttagtagattaaatgtttgtttgattacatggattagtaactgtttgaacacattaaacaaaagcttaggcttaagatgtggattcaataatgttatcttgacacaattattcctttatggagattgtatactaaaactattccacaatgaggggttctacataataaaagaggtagagggatttattatgtctctaattttaaatataacagaagaagatcaattcagaaaacggttttataatagtatgctcaacaacatcacagatgccgccaacaaagctcaaaaaaatctgctatcaagagtatgtcatacattattagataagacaatatcagataatataataaatggcagatggataattctattgagtaagttcctaaaattaattaagcttgcaggtgacaataacctcaacaatctgagtgaattatattttttgttcagaatatttggacacccaatggtagatgaaagacaagccatggatgctgttaaagttaattgcaacgagaccaaattttatttgttaagtagtttgagtatgttaagaggagcttttatatatagaattataaaagggtttgtaaataattacaacagatggcctactttaagaaatgccattgtcttacccttaagatggttaacttactataaactaaacacttatccttccttgttggaacttacagaaagagatttgattgttctatcaggactacgtttctatcgagagtttcggttgcctaaaaaagtggatcttgaaatgatcataaatgataaggctatatcacctcctaaaaatttaatatggactagtttccctagaaattatatgccgtcacacatacaaaattatatagaacatgaaaaattaaaattctctgatagtgataaatcaagaagagtattagagtattatttaagagataacaaattcaatgaatgtgatttacacaactgtgtagttaatcaaagttatcttaacaacccgaatcatgtggtatcattgacaggcaaagaaagagaactcagtgtaggtagaatgtttgcaatgcaaccaggaatgttcagacaagttcaaatattagcagagaaaatgatagcagaaaacatattacaatttttccctgaaagtcttacaagatatggtgatctagaactacagaaaatattagaattgaaagcaggaataagtaacaaatcaaatcgttacaatgataattacaacaattacattagtaagtgctctatcatcacagatctcagcaaattcaatcaagcatttcgatatgaaacatcatgtatttgtagtgatgtactggatgaactgcatggtgtacaatctctattttcctggttacatttaactattcctcatgtcacaataatatgcacatataggcatgcacccccctatataaaggatcatattgtagatcttaacaatgtagatgagcaaagtggactatatagatatcatatgggtggtatcgaagggtggtgtcaaaaactatggaccatagaagctatatcactattagatctaatatctctcaaagggaaattctcaattactgctttaattaatggtgacaatcaatcaatagatataagtaaaccagtcagactcatggaaggtcaaactcatgctcaagcagattatttgctagcattaaatagtctcaaattactgtataaagagtatgcaggaataggccacaaattaaaaggaactgagacttatatatcgagagatatgcaatttatgagtaaaacgatccaacataacggtgtatattacccagctagtataaagaaagtcctaagagtgggaccgtggataaacactatacttgatgacttcaaagtgagtctagaatctataggtagtttgacacaagaattagaatatagaggtgaaagtctattatgcagtttaatatttagaaatgtatggttatataatcaaattgcattacaacttaaaaatcatgcattatgtaacaacaaattatatttggatatattaaaagttctaaaacacttaaaaaccttttttaatcttgataacattgatacagcattaacattgtatatgaatttgcccatgttatttggtggtggtgatcccaacttgttatatcgaagtttctatagaagaactcctgatttcctcacagaggctatagttcactctgtgttcatacttagttattatacaaaccatgatttaaaagataaacttcaagatctgtcagatgatagattgaataagttcttaacatgcataatcacgtttgataaaaaccccaatgctgaattcgttacattgatgagagatcctcaagctttaggatctgagaggcaagctaaaattactagcgaaatcaatagactggcagttaccgaggttttgagcacagctccaaacaaaatattttccaaaagtgcacaacactataccactacagagatagatcttaatgatattatgcaaaatatagaacctacatatcctcacgggctaagagttgtttatgagagtttacccttttataaagcagagaaaatagtaaatcttatatccggtacaaaatctataactaacatactggaaaagacttctgccatagacttaacagatattgatagagccactgagatgatgaggaaaaacataactttgcttataaggatattaccattagattgtaacagagataaaagagaaatattgagtatggaaaacctaagtattactgaattaagcaaatacgttagagaaagatcttggtctttatccaatatagttggtgttacatcacccagtatcatgtatacaatggacataaaatatacaacaagcactatagctagtggcataatcatagagaaatataatgtcaacagtttaacacgtggtgagagaggacccactaaaccatgggttggttcatctacacaagagaaaaagacaatgccagtttataatagacaagttttaaccaaaaaacagagagatcaaatagatctattagcaaaattggattgggtgtatgcatctatagataacaaggatgaatttatggaggaacttagcataggaactcttgggttaacatatgagaaggccaaaaaattattcccacaatatttgagtgttaactatttgcatcgtcttacagtcagtagtagaccatgtgaattccctgcatctataccagcttatagaactacaaattatcactttgatactagccctattaatcgcatattaacagaaaagtatggtgatgaagatattgatatagtattccaaaactgtataagctttggccttagcttaatgtctgtagtagaacaatttactaatgtatgtcctaacagaattattctcatacccaagcttaatgagatacatttgatgaaacctcccatattcacaggcgatgttgatattcacaagttaaaacaagtgatacaaaaacaacatatgtttttaccagacaaaataagtttgactcaatatgtggaattattcttaagtaataaaacactcaaatctggatctaatgttaattctaatttaatattggcgcataagatatctgactattttcataatacttacattttgagtactaatttagctggacattggattcttattatacaacttatgaaagattctaagggtatttttgaaaaagattggggagagggatatataactgatcatatgttcattaatttgaaagttttcttcaatgcttataagacatatctcttgtgttttcataaaggttacggcagagcaaagctggagtgtgatatgaatacttcagatctcctatgtgtattggaattaatagacagtagttattggaagtctatgtctaaggtgtttttagaacaaaaagttatcaaatacattcttagccaggatgcaagtttacatagagtaaaaggatgtcatagcttcaaactatggtttcttaaacgtcttaatgtagcagaattcacagtttgcccttgggttgttaacatagattatcatccaacacatatgaaagcaatattaacttatattgatcttgttagaatgggattgataaatatagatagaatatacattaaaaataaacacaagttcaatgatgagttttatacttctaatctgttttacattaattataacttctcagataatactcatctattaactaaacatataaggattgctaattccgaattagaaagtaattacaacaaattatatcatcctacaccagaaaccctagaaaatatactaaccaatccggttaaaagtaatgagaaaaagacactgagtgactattgtataggtaaaaatgttgactcaataatgttaccatcgttatctaataagaagcttattaaatcgtctacaatgattagaaccaattacagcagacaagatttgtataatttatttcctacggttgtgattgataaaattatagatcattcaggtaatacagccaaatctaaccaactttacactactacttctcatcaaatatccttagtgcacaatagcacatcactttattgcatgcttccttggcatcatattaatagattcaattttgtatttagttctacaggttgtaaaattagtatagagtatattttaaaagatcttaaaattaaggatcctaattgtatagcattcataggtgaaggagcagggaatttattattgcgtacagtagtggaacttcatcctgatataagatatatttacagaagtctgaaagattgcaatgatcatagtttaccaattgagtttttaaggctgtacaatggacatatcaacattgattatggtgaaaatttgaccattcctgctacagatgcaaccaacaacattcattggtcttatttacatataaagtttgctgaacctatcagtctttttgtctgtgatgctgaattgcctgtaacagtcaactggagtaagattataatagagtggagcaagcatgtaagaaaatgcaagtactgttcttcagttaataaatgtacattgatagtaaaatatcatgctcaagatgatatcgatttcaaattagacaacataactatattaaaaacttatgtatgcttaggtagtaagttaaagggatctgaagtttacttagtccttacaataggtcctgcaaatgtgttcccagtatttaatgtagtacaaaatgctaaattgatactatcaagaactaaaaatttcatcatgcctaaaaaagctgataaagagtctattgatgcaaatattaagagtttgataccctttctttgttaccctataacaaaaaaaggaattaatactgcattgtctaaattaaagagtgttgttagtggagatatactatcatattctatagctggacgtaatgaagttttcagcaataaacttataaatcataagcatatgaacatcttaaagtggttcaatcatgttttaaatttcagatcaacagaattaaactataatcatttatatatggtagaatctacttatcctcatctaagtgaattgttaaacagcttgacaaccaatgaacttaaaaaactgattaaaatcacaggtagtttgttatacaacttttataatgaataatgagcaaaaatcttataacaaaaatagctacacactaacattgtattcaattatagttattgaaaattaataattatataatttttaataacttctagtgaactaatcctaaaattatcattttgatctaggaagaataagtttaaatccaaatctaattggtttatatgtatattaactaaattacgagatattagtttttgacactttttttctcgt

SEQ ID NO: 12 - DNA, 15827 bp, synthetic construct
  misc_feature 1..15827: note = The sequence in which the G gene was removed from SEQ ID NO: 11.
  source 1..15827: mol_type = other DNA
acgcgaaaaaatgcgtacaacaaacttgcgtaaaccaaaaaaatggggcaaataagaatttgataagtaccacttaaatttaactcctttggttagaggcgcgccatgggcagcaactcattgagtatgataaaagttagattgcaaaatctgtttgacaatgatgaagtagcattgttaaaaataacatgctatactgacaaattaatacagttaactaatgctttggctaaggcagttatacatacaatcaaattgaatggcattgtatttgtgcatgttattacaagtagtgatatttgccctaataataatattgtagtgaaatccaatttcacaacaatgccagtattacaaaatggaggttatatatgggaaatgatggaattaacacactgctctcaacctaatggcctaatagatgacaattgtgaaattaaattctccaaaaaactaagtgattcaacaatgaccaattatatgaatcaattatctgaattacttggatttgacctcaatccataaatcataataaatatcaactagcaaatcaatgtcactaacaccattagttaatataaaacttgacagaagataaaaatggggcaaataaatcaattcagccgacccaaccatggacacaacacacaatgataccacaccacaaagactgatgatcacagacatgaggccattatcgcttgagactataataacatctctaaccagagatatcataacacataaatttatatacttgataaatcatgaatgcatagtaagaaaacttgatgaaagacaggccacatttacatttctggtcaactatgaaatgaaactattgcacaaagtgggaagcactaaatataaaaaatatactgaatacaacacaaaatatggcactttccctatgccaatatttatcaatcatgatgggttcttagaatgcattggcattaagcctaccaagcacacacccataatatacaagtatgatctcaatccatgaatatcaaaccaagattcaaacaatccgaaataacaactttatgcataatcacactccatagtccaaatggagcctgaaaattatagttatttaaaattcctgcaggaaggagagacataagatgaaagatggggcaaatacaaaaatggctcttagcaaagtcaagttgaatgatacactcaacaaagatcaacttctatcatccagcaaatataccatccaacggagcacaggagacagcattgacactcctaattatgatgtgcagaaacacattaataagttatgtggcatgttattaatcacagaagatgctaatcataaattcactgggttaataggtatgttatatgctatgtctagattaggaagagaagacaccataaaaatactcaaagatgcgggatatcatgttaaggcaaatggagtggatgtaacaacacatcgtcaagacattaatgggaaagaaatgaaatttgaagtgttaacattagcaagcttaacaactgaaattcaaatcaacattgagatagaatctagaaaatcctacaaaaaaatgctaaaagaaatgggagaggtggctccagaatacaggcatgactctcctgattgtgggatgataatattatgtatagcggcattagtaataaccaaattagcagcaggagatagatcaggtcttacagctgtgattaggagagctaataatgtcctaaaaaatgaaatgaaacgttataaaggtttattacccaaggatatagccaacagcttctatgaagtgtttgaaaaatatcctcactttatagatgtttttgttcattttggtatagcacaatcttctaccagaggtggcagtagagttgaagggatttttgcaggattgtttatgaatgcctatggtgcagggcaagtgatgttacggtggggggtcttagcaaaatcagttaaaaacattatgttaggacacgctagtgtacaagcagaaatggaacaagttgtggaggtgtatgagtatgctcagaaattgggtggagaagcaggattctaccatatattgaacaacccaaaagcatcactattatctttgactcaatttcctcacttctctagtgtagtattgggcaatgctgctggcctaggcataatgggagaatacagaggtacaccaaggaatcaagatttatatgatgctgcaaaagcatatgctgaacaactcaaagaaaatggtgtgattaactacagtgtattagatttgacagcagaagaactagaggctatcaaacatcagcttaatccaaaagataatgatgtagagctttgagttaataaaaaagtggggcaaataaatcatcatggaaaagtttgctcctgaattccatggagaagatgcaaacaacagagccaccaaattcctagaatcaataaagggcaaattcacatcacccaaagatcccaagaaaaaagatagtatcatatctgtcaactcaatagatatagaagtaaccaaagaaagccctataacatcaaattcaaccattataaacccaataaatgagacagatgatactgtagggaacaagcccaattatcaaagaaagcctctagtaagtttcaaagaagaccctacgccaagtgataatcctttttcaaaactatacaaagaaaccatagaaacatttgataacaatgaagaagaatctagctattcatatgaagaaataaatgatcagacaaacgataatataacagcaagattagataggattgatgagaaattaagtgaaatactaggaatgcttcacacattagtagtagcgagtgcaggacccacatctgctcgggatggtataagagatgccatggttggtttaagagaagaaatgatagaaaaaatcagaactgaagcattaatgaccaatgacagactagaagctatggcaagactcaggaatgaagaaagtgaaaagatggcaaaagacacatcagatgaagtgtctctcaatccaacatcagagaaactgaacaacctgttggaagggaatgatagtgacaatgatctatcacttgaagatttctgattagctaccaaactgtacatcaaaacacaacaccaatagaaaaccaacaaacaaaccaactcacccatccaaccaaacatctatctgctgattagccaaccagccaaaaaacaaccagccaatctaaaactagccacccggaaaaaatcgatactatagttacaaaaaaagatggggcaaatatggaaacatacgtgaataaacttcacgagggctccacatacacagctgctgttcaatacaatgtcctagaaaaagacgatgatcctgcatcacttacaatatgggtgcccatgttccaatcatccatgccagcagatctactcataaaagaactagccaatgtcaatatactagtgaaacaaatatccacacccaagggaccctcattaagagtcatgataaactcaagaagtgcagtgctagcacaaatgcccagcaaatttaccatatgtgccaatgtgtccttggatgaaagaagcaagctggcatatgatgtaaccacaccctgtgaaattaaggcatgcagtctaacatgcctaaaatcaaaaaatatgttaactacagttaaagatctcactatgaaaacactcaacccaacacatgacatcattgctttatgtgaatttgaaaatatagtaacatcaaaaaaagtcataataccaacatacctaagatctatcagcgtcagaaataaagatctgaacacacttgaaaatataacaaccactgaattcaaaaatgccattacaaatgcaaaaatcatcccttactcaggattattgttagtcatcacagtgactgacaacaaaggagcattcaaatacataaagccacaaagtcaattcatagtagatcttggagcttacctagaaaaagaaagtatatattatgttacaacaaattggaagcacacagctacacgatttgcaatcaaacccatggaagattaacctttttcctctacatcaatgagtagattcatacaaactttctaactacattcttcacttcacaatcataatcaccaaccctctgtggttcaatcaatcaaacaaaactcatcaagagttccagatcatcccaagtcattgttcatcagatccagtactcaaataagttaataaaaaatccacatggggcaaataatcattgagggaaatccaactaatcacaacatctgtcaacatagacaagtcaacacgctagataaaatcaaccaatggaaaatacatccataactatagaattctcaagcaaattctggccttactttacactaatacacatgataacaacaataatctctttgataatcataatctccatcatgattgcaatactaaacaaactctgcgaatataatgtattccataacaaaacctttgagctaccaagagctcgagtcaatacatagcattcaccaatctgatagctcaaaacagtaaccttgcatttgtaaatgaactaccctcacttcttcacaaaaccacatcaacatctcaccatgcaagccatcatctataccataaagtagttaattaaaaatggccggccagtcataacaatgaactaggatattaagaccaaaaacaacgctacgcgtttgacagaagataaaaatggggcaaatgcaaacatgaagtgccttttgtacttagcctttttattcattggggtgaattgcaagttcaccatagtttttccacacaaccaaaaaggaaactggaaaaatgttccttctaattaccattattgcccgtcaagctcagatttaaattggcataatgacttaataggcacagccttacaagtcaaaatgcccaagagtcacaaggctattcaagcagacggttggatgtgtcatgcttccaaatgggtcactacttgtgatttccgctggtatggaccgaagtatataacacattccatccgatccttcactccatctgtagaacaatgcaaggaaagcattgaacaaacgaaacaaggaacttggctgaatccaggcttccctcctcaaagttgtggatatgcaactgtgacggatgccgaagcagtgattgtccaggtgactcctcaccatgtgctggttgatgaatacacaggagaatgggttgattcacagttcatcaacggaaaatgcagcaattacatatgccccactgtccataactctacaacctggcattctgactataaggtcaaagggctatgtgattctaacctcatttccatggacatcaccttcttctcagaggacggagagctatcatccctgggaaaggagggcacagggttcagaagtaactactttgcttatgaaactggaggcaaggcctgcaaaatgcaatactgcaagcattggggagtcagactcccatcaggtgtctggttcgagatggctgataaggatctctttgctgcagccagattccctgaatgcccagaagggtcaagtatctctgctccatctcagacctcagtggatgtaagtctaattcaggacgttgagaggatcttggattattccctctgccaagaaacctggagcaaaatcagagcgggtcttccaatctctccagtggatctcagctatcttgctcctaaaaacccaggaaccggtcctgctttcaccataatcaatggtaccctaaaatactttgagaccagatacatcagagtcgatattgctgctccaatcctctcaagaatggtcggaatgatcagtggaactaccacagaaagggaactgtgggatgactgggcaccatatgaagacgtggaaattggacccaatggagttctgaggaccagttcaggatataagtttcctttatacatgattggacatggtatgttggactccgatcttcatcttagctcaaaggctcaggtgttcgaacatcctcacattcaagacgctgcttcgcaacttcctgatgatgagagtttattttttggtgatactgggctatccaaaaatccaatcgagcttgtagaaggttggttcagtagttggaaaagctctattgcctcttttttctttatcatagggttaatcattggactattcttggttctccgagttggtatccatctttgcattaaagccagaagcacaccagtcacattaagtaaggatcaactgagtggtataaataatattgcatttagtaactaatagtcattaaaaagcgggcccgtattgttgcaaaaagccatgaccaaatcaaacagaatcaaaatcaactctggggcaaataacaatggagttgccaatcctcaaaacaaatgctattaccacaatccttgctgcagtcacactctgtttcgcttccagtcaaaacatcactgaagaattttatcaatcaacatgcagtgcagtcagcaaaggctatcttagtgctctaagaactggttggtatactagtgttataactatagaattaagtaatatcaaggaaaataagtgtaatggtacagacgctaaggtaaaattaataaaacaagaattagataaatataaaaatgctgtaacagaattgcagttgctcatgcaaagcacaccagcagccaacaatcgagccagaagagaactaccaagatttatgaattatacactcaacaataccaaaaacaccaatgtaacattaagtaagaaaaggaaaagaagatttcttggatttttgttaggtgttggatctgcaatcgccagtggcattgccgtatccaaggtcctgcacctagaaggggaagtgaacaaaatcaaaagtgctctactatccacaaacaaggctgtagtcagcttatctaatggagtcagtgtcttaaccagcaaggtgttagacctcaaaaactatatagataaacagttgttacctattgttaacaagcaaagctgcagcatatcaaacattgaaactgtgatagagttccaacaaaagaacaacagactactagagattaccagagaatttagtgttaatgcaggtgtaactactcctgtaagcacttatatgttaactaatagtgagttattatcattaatcaatgatatgcctataacaaatgatcagaaaaagttaatgtccagcaatgttcaaatagttagacagcaaagttactctatcatgtcaataataaaagaggaagtcttggcatatgtagtacaattaccactatatggtgtaatagatactccttgttggaaactacacacatcccctttatgtacaaccaacacaaaggaaggatccaacatctgcttaacaagaaccgacagaggatggtactgtgacaatgcaggatcagtatcctttttcccacaagctgaaacatgtaaagttcaatcgaatcgggtgttttgtgacacaatgaacagtttaacattaccaagtgaggtaaatctctgcaacattgacatattcaaccccaaatatgattgcaaaattatgacttcaaaaacagatgtaagcagctccgttatcacatctctaggagccattgtgtcatgctatggcaaaaccaaatgtacagcatccaataaaaatcgtgggatcataaagacattctctaacgggtgtgattatgtatcaaataagggggtggatactgtgtctgtaggtaatacattatattatgtaaataagcaagaaggcaaaagtctctatgtaaaaggtgaaccaataataaatttctatgatccattagtgttcccctctctcctgtgggatgcatcaatatctcaagtcaatgagaaaattaatcagagtctagcatttatccgtaaatcagatgaattattaggctctggcggaagcggatacatccctgaggcaccaagggacggacaggcctacgtgcgcaaggatggcgagtgggtgctgctgtccacctttctgtgaataaaaatagcacctaatcatattcttacaatggttcgctatttgaccatagataacccatctatcattagattatcctaaaatttgaacttcatcacaactttcatctataaaccatctcacttacactttttaagtagatttctattttatagttatataaaacagggcccattgaataccaaattaacttactatttgtaaaaatgagaattggggcaaatatgtcacgaaggaatccttgcaaattcgaaattcgaggtcattgcttgaatggtaaaaggtgtcattttagtcataattattttgaatggccaccccatgcactgcttgtaagacaaaactttatgttaaacagaatacttaagtctatggataaaagcatagatactttgtcagaaataagtggagctgcagagttggacagaacagaagagtatgccctcggtgtagttggagtgctagagagttatataggatcaataaataatataactaaacaatcagcatgtgttgccatgagcaaactccttactgaactcaacagcgatgacatcaaaaaactaagggacaatgaagagccaaactcacccaaagtaagagtgtacaatactgtcatatcatatattgaaagcaacaggaagaacaataaacaaactatccatctgttaaaaagattgccagcagacgtattgaagaaaaccatcaaaaacacattggatatccacaagagcataaccatcaataacccaaaagaatcaactgttagtgatacgaacgaccatgccaaaaataatgatactacctgacaaatatccttgtagtataaattccatactaataacaagtaattgtagagtcactatgtataatcaaaaaaacacactatatatcaatcaaaacaaccaaaatagccatatatacccaccggatcaaccattcaatgaaatccattggacctctcaagacttgattgatgcaactcaaaattttctacaacatctaggtattactgatgatatatacacaatatatatattagtgtcataatactcaatcctaatacttaccacatcatcaaattattaactcaaacaattcaagctatgggacaaaatggatcccattattagtggaaattctgctaatgtttatctaactgatagttatttaaaaggtgttatttctttctcagaatgtaacgctttaggaagttacatattcaatggtccttatctcaaaaatgattataccaacttaattagtagacaaaatccattaatagaacacataaatctaaagaaactaaatataacacagtccttaatatctaagtatcataaaggtgaaataaaaatagaagaacctacttactttcagtcattacttatgacatacaagagtatgacctcttcagaacagactactactactaatttacttaaaaagataataagaagagctatagaaatcagtgatgtcaaagtctatgctatattgaataaactggggctcaaagaaaaagacaagattaaatccaataatggacaagatgaagacaactcagtcattactaccataatcaaagatgatatacttttagctgtcaaggataatcaatctcatcttaaagcagacaaaaatcaatccacaaaacaaaaagatacaatcaaaacaacacttttgaagaaattaatgtgttcgatgcaacatcctccatcatggttaatacattggtttaatttatacacaaaattaaacagcatattaacacaatatcgatctagtgaggtaaaaaaccatggttttatattgatagataatcatactcttagtggattccaatttattttgaatcaatatggttgtatagtttatcataaggaactcaaaagaattactgtgacaacttataatcaattcttgacatggaaagatattagccttagtagattaaatgtttgtttgattacatggattagtaactgtttgaacacattaaacaaaagcttaggcttaagatgtggattcaataatgttatcttgacacaattattcctttatggagattgtatactaaaactattccacaatgaggggttctacataataaaagaggtagagggatttattatgtctctaattttaaatataacagaagaagatcaattcagaaaacggttttataatagtatgctcaacaacatcacagatgccgccaacaaagctcaaaaaaatctgctatcaagagtatgtcatacattattagataagacaatatcagataatataataaatggcagatggataattctattgagtaagttcctaaaattaattaagcttgcaggtgacaataacctcaacaatctgagtgaattatattttttgttcagaatatttggacacccaatggtagatgaaagacaagccatggatgctgttaaagttaattgcaacgagaccaaattttatttgttaagtagtttgagtatgttaagaggagcttttatatatagaattataaaagggtttgtaaataattacaacagatggcctactttaagaaatgccattgtcttacccttaagatggttaacttactataaactaaacacttatccttccttgttggaacttacagaaagagatttgattgttctatcaggactacgtttctatcgagagtttcggttgcctaaaaaagtggatcttgaaatgatcataaatgataaggctatatcacctcctaaaaatttaatatggactagtttccctagaaattatatgccgtcacacatacaaaattatatagaacatgaaaaattaaaattctctgatagtgataaatcaagaagagtattagagtattatttaagagataacaaattcaatgaatgtgatttacacaactgtgtagttaatcaaagttatcttaacaacccgaatcatgtggtatcattgacaggcaaagaaagagaactcagtgtaggtagaatgtttgcaatgcaaccaggaatgttcagacaagttcaaatattagcagagaaaatgatagcagaaaacatattacaatttttccctgaaagtcttacaagatatggtgatctagaactacagaaaatattagaattgaaagcaggaataagtaacaaatcaaatcgttacaatgataattacaacaattacattagtaagtgctctatcatcacagatctcagcaaattcaatcaagcatttcgatatgaaacatcatgtatttgtagtgatgtactggatgaactgcatggtgtacaatctctattttcctggttacatttaactattcctcatgtcacaataatatgcacatataggcatgcacccccctatataaaggatcatattgtagatcttaacaatgtagatgagcaaagtggactatatagatatcatatgggtggtatcgaagggtggtgtcaaaaactatggaccatagaagctatatcactattagatctaatatctctcaaagggaaattctcaattactgctttaattaatggtgacaatcaatcaatagatataagtaaaccagtcagactcatggaaggtcaaactcatgctcaagcagattatttgctagcattaaatagtctcaaattactgtataaagagtatgcaggaataggccacaaattaaaaggaactgagacttatatatcgagagatatgcaatttatgagtaaaacgatccaacataacggtgtatattacccagctagtataaagaaagtcctaagagtgggaccgtggataaacactatacttgatgacttcaaagtgagtctagaatctataggtagtttgacacaagaattagaatatagaggtgaaagtctattatgcagtttaatatttagaaatgtatggttatataatcaaattgcattacaacttaaaaatcatgcattatgtaacaacaaattatatttggatatattaaaagttctaaaacacttaaaaaccttttttaatcttgataacattgatacagcattaacattgtatatgaatttgcccatgttatttggtggtggtgatcccaacttgttatatcgaagtttctatagaagaactcctgatttcctcacagaggctatagttcactctgtgttcatacttagttattatacaaaccatgatttaaaagataaacttcaagatctgtcagatgatagattgaataagttcttaacatgcataatcacgtttgataaaaaccccaatgctgaattcgttacattgatgagagatcctcaagctttaggatctgagaggcaagctaaaattactagcgaaatcaatagactggcagttaccgaggttttgagcacagctccaaacaaaatattttccaaaagtgcacaacactataccactacagagatagatcttaatgatattatgcaaaatatagaacctacatatcctcacgggctaagagttgtttatgagagtttacccttttataaagcagagaaaatagtaaatcttatatccggtacaaaatctataactaacatactggaaaagacttctgccatagacttaacagatattgatagagccactgagatgatgaggaaaaacataactttgcttataaggatattaccattagattgtaacagagataaaagagaaatattgagtatggaaaacctaagtattactgaattaagcaaatacgttagagaaagatcttggtctttatccaatatagttggtgttacatcacccagtatcatgtatacaatggacataaaatatacaacaagcactatagctagtggcataatcatagagaaatataatgtcaacagtttaacacgtggtgagagaggacccactaaaccatgggttggttcatctacacaagagaaaaagacaatgccagtttataatagacaagttttaaccaaaaaacagagagatcaaatagatctattagcaaaattggattgggtgtatgcatctatagataacaaggatgaatttatggaggaacttagcataggaactcttgggttaacatatgagaaggccaaaaaattattcccacaatatttgagtgttaactatttgcatcgtcttacagtcagtagtagaccatgtgaattccctgcatctataccagcttatagaactacaaattatcactttgatactagccctattaatcgcatattaacagaaaagtatggtgatgaagatattgatatagtattccaaaactgtataagctttggccttagcttaatgtctgtagtagaacaatttactaatgtatgtcctaacagaattattctcatacccaagcttaatgagatacatttgatgaaacctcccatattcacaggcgatgttgatattcacaagttaaaacaagtgatacaaaaacaacatatgtttttaccagacaaaataagtttgactcaatatgtggaattattcttaagtaataaaacactcaaatctggatctaatgttaattctaatttaatattggcgcataagatatctgactattttcataatacttacattttgagtactaatttagctggacattggattcttattatacaacttatgaaagattctaagggtatttttgaaaaagattggggagagggatatataactgatcatatgttcattaatttgaaagttttcttcaatgcttataagacatatctcttgtgttttcataaaggttacggcagagcaaagctggagtgtgatatgaatacttcagatctcctatgtgtattggaattaatagacagtagttattggaagtctatgtctaaggtgtttttagaacaaaaagttatcaaatacattcttagccaggatgcaagtttacatagagtaaaaggatgtcatagcttcaaactatggtttcttaaacgtcttaatgtagcagaattcacagtttgcccttgggttgttaacatagattatcatccaacacatatgaaagcaatattaacttatattgatcttgttagaatgggattgataaatatagatagaatatacattaaaaataaacacaagttcaatgatgagttttatacttctaatctgttttacattaattataacttctcagataatactcatctattaactaaacatataaggattgctaattccgaattagaaagtaattacaacaaattatatcatcctacaccagaaaccctagaaaatatactaaccaatccggttaaaagtaatgagaaaaagacactgagtgactattgtataggtaaaaatgttgactcaataatgttaccatcgttatctaataagaagcttattaaatcgtctacaatgattagaaccaattacagcagacaagatttgtataatttatttcctacggttgtgattgataaaattatagatcattcaggtaatacagccaaatctaaccaactttacactactacttctcatcaaatatccttagtgcacaatagcacatcactttattgcatgcttccttggcatcatattaatagattcaattttgtatttagttctacaggttgtaaaattagtatagagtatattttaaaagatcttaaaattaaggatcctaattgtatagcattcataggtgaaggagcagggaatttattattgcgtacagtagtggaacttcatcctgatataagatatatttacagaagtctgaaagattgcaatgatcatagtttaccaattgagtttttaaggctgtacaatggacatatcaacattgattatggtgaaaatttgaccattcctgctacagatgcaaccaacaacattcattggtcttatttacatataaagtttgctgaacctatcagtctttttgtctgtgatgctgaattgcctgtaacagtcaactggagtaagattataatagagtggagcaagcatgtaagaaaatgcaagtactgttcttcagttaataaatgtacattgatagtaaaatatcatgctcaagatgatatcgatttcaaattagacaacataactatattaaaaacttatgtatgcttaggtagtaagttaaagggatctgaagtttacttagtccttacaataggtcctgcaaatgtgttcccagtatttaatgtagtacaaaatgctaaattgatactatcaagaactaaaaatttcatcatgcctaaaaaagctgataaagagtctattgatgcaaatattaagagtttgataccctttctttgttaccctataacaaaaaaaggaattaatactgcattgtctaaattaaagagtgttgttagtggagatatactatcatattctatagctggacgtaatgaagttttcagcaataaacttataaatcataagcatatgaacatcttaaagtggttcaatcatgttttaaatttcagatcaacagaattaaactataatcatttatatatggtagaatctacttatcctcatctaagtgaattgttaaacagcttgacaaccaatgaacttaaaaaactgattaaaatcacaggtagtttgttatacaacttttataatgaataatgagcaaaaatcttataacaaaaatagctacacactaacattgtattcaattatagttattgaaaattaataattatataatttttaataacttctagtgaactaatcctaaaattatcattttgatctaggaagaataagtttaaatccaaatctaattggtttatatgtatattaactaaattacgagatattagtttttgacactttttttctcgt

SEQ ID NO: 13 - DNA, 15845 bp, synthetic construct
  misc_feature 1..15845: note = A sequence in which SEQ ID NO: 12 is cleaved with ApaI and SEQ IDNO: 5 is inserted.
  source 1..15845: mol_type = other DNA
acgcgaaaaaatgcgtacaacaaacttgcgtaaaccaaaaaaatggggcaaataagaatttgataagtaccacttaaatttaactcctttggttagaggcgcgccatgggcagcaactcattgagtatgataaaagttagattgcaaaatctgtttgacaatgatgaagtagcattgttaaaaataacatgctatactgacaaattaatacagttaactaatgctttggctaaggcagttatacatacaatcaaattgaatggcattgtatttgtgcatgttattacaagtagtgatatttgccctaataataatattgtagtgaaatccaatttcacaacaatgccagtattacaaaatggaggttatatatgggaaatgatggaattaacacactgctctcaacctaatggcctaatagatgacaattgtgaaattaaattctccaaaaaactaagtgattcaacaatgaccaattatatgaatcaattatctgaattacttggatttgacctcaatccataaatcataataaatatcaactagcaaatcaatgtcactaacaccattagttaatataaaacttgacagaagataaaaatggggcaaataaatcaattcagccgacccaaccatggacacaacacacaatgataccacaccacaaagactgatgatcacagacatgaggccattatcgcttgagactataataacatctctaaccagagatatcataacacataaatttatatacttgataaatcatgaatgcatagtaagaaaacttgatgaaagacaggccacatttacatttctggtcaactatgaaatgaaactattgcacaaagtgggaagcactaaatataaaaaatatactgaatacaacacaaaatatggcactttccctatgccaatatttatcaatcatgatgggttcttagaatgcattggcattaagcctaccaagcacacacccataatatacaagtatgatctcaatccatgaatatcaaaccaagattcaaacaatccgaaataacaactttatgcataatcacactccatagtccaaatggagcctgaaaattatagttatttaaaattcctgcaggaaggagagacataagatgaaagatggggcaaatacaaaaatggctcttagcaaagtcaagttgaatgatacactcaacaaagatcaacttctatcatccagcaaatataccatccaacggagcacaggagacagcattgacactcctaattatgatgtgcagaaacacattaataagttatgtggcatgttattaatcacagaagatgctaatcataaattcactgggttaataggtatgttatatgctatgtctagattaggaagagaagacaccataaaaatactcaaagatgcgggatatcatgttaaggcaaatggagtggatgtaacaacacatcgtcaagacattaatgggaaagaaatgaaatttgaagtgttaacattagcaagcttaacaactgaaattcaaatcaacattgagatagaatctagaaaatcctacaaaaaaatgctaaaagaaatgggagaggtggctccagaatacaggcatgactctcctgattgtgggatgataatattatgtatagcggcattagtaataaccaaattagcagcaggagatagatcaggtcttacagctgtgattaggagagctaataatgtcctaaaaaatgaaatgaaacgttataaaggtttattacccaaggatatagccaacagcttctatgaagtgtttgaaaaatatcctcactttatagatgtttttgttcattttggtatagcacaatcttctaccagaggtggcagtagagttgaagggatttttgcaggattgtttatgaatgcctatggtgcagggcaagtgatgttacggtggggggtcttagcaaaatcagttaaaaacattatgttaggacacgctagtgtacaagcagaaatggaacaagttgtggaggtgtatgagtatgctcagaaattgggtggagaagcaggattctaccatatattgaacaacccaaaagcatcactattatctttgactcaatttcctcacttctctagtgtagtattgggcaatgctgctggcctaggcataatgggagaatacagaggtacaccaaggaatcaagatttatatgatgctgcaaaagcatatgctgaacaactcaaagaaaatggtgtgattaactacagtgtattagatttgacagcagaagaactagaggctatcaaacatcagcttaatccaaaagataatgatgtagagctttgagttaataaaaaagtggggcaaataaatcatcatggaaaagtttgctcctgaattccatggagaagatgcaaacaacagagccaccaaattcctagaatcaataaagggcaaattcacatcacccaaagatcccaagaaaaaagatagtatcatatctgtcaactcaatagatatagaagtaaccaaagaaagccctataacatcaaattcaaccattataaacccaataaatgagacagatgatactgtagggaacaagcccaattatcaaagaaagcctctagtaagtttcaaagaagaccctacgccaagtgataatcctttttcaaaactatacaaagaaaccatagaaacatttgataacaatgaagaagaatctagctattcatatgaagaaataaatgatcagacaaacgataatataacagcaagattagataggattgatgagaaattaagtgaaatactaggaatgcttcacacattagtagtagcgagtgcaggacccacatctgctcgggatggtataagagatgccatggttggtttaagagaagaaatgatagaaaaaatcagaactgaagcattaatgaccaatgacagactagaagctatggcaagactcaggaatgaagaaagtgaaaagatggcaaaagacacatcagatgaagtgtctctcaatccaacatcagagaaactgaacaacctgttggaagggaatgatagtgacaatgatctatcacttgaagatttctgattagctaccaaactgtacatcaaaacacaacaccaatagaaaaccaacaaacaaaccaactcacccatccaaccaaacatctatctgctgattagccaaccagccaaaaaacaaccagccaatctaaaactagccacccggaaaaaatcgatactatagttacaaaaaaagatggggcaaatatggaaacatacgtgaataaacttcacgagggctccacatacacagctgctgttcaatacaatgtcctagaaaaagacgatgatcctgcatcacttacaatatgggtgcccatgttccaatcatccatgccagcagatctactcataaaagaactagccaatgtcaatatactagtgaaacaaatatccacacccaagggaccctcattaagagtcatgataaactcaagaagtgcagtgctagcacaaatgcccagcaaatttaccatatgtgccaatgtgtccttggatgaaagaagcaagctggcatatgatgtaaccacaccctgtgaaattaaggcatgcagtctaacatgcctaaaatcaaaaaatatgttaactacagttaaagatctcactatgaaaacactcaacccaacacatgacatcattgctttatgtgaatttgaaaatatagtaacatcaaaaaaagtcataataccaacatacctaagatctatcagcgtcagaaataaagatctgaacacacttgaaaatataacaaccactgaattcaaaaatgccattacaaatgcaaaaatcatcccttactcaggattattgttagtcatcacagtgactgacaacaaaggagcattcaaatacataaagccacaaagtcaattcatagtagatcttggagcttacctagaaaaagaaagtatatattatgttacaacaaattggaagcacacagctacacgatttgcaatcaaacccatggaagattaacctttttcctctacatcaatgagtagattcatacaaactttctaactacattcttcacttcacaatcataatcaccaaccctctgtggttcaatcaatcaaacaaaactcatcaagagttccagatcatcccaagtcattgttcatcagatccagtactcaaataagttaataaaaaatccacatggggcaaataatcattgagggaaatccaactaatcacaacatctgtcaacatagacaagtcaacacgctagataaaatcaaccaatggaaaatacatccataactatagaattctcaagcaaattctggccttactttacactaatacacatgataacaacaataatctctttgataatcataatctccatcatgattgcaatactaaacaaactctgcgaatataatgtattccataacaaaacctttgagctaccaagagctcgagtcaatacatagcattcaccaatctgatagctcaaaacagtaaccttgcatttgtaaatgaactaccctcacttcttcacaaaaccacatcaacatctcaccatgcaagccatcatctataccataaagtagttaattaaaaatggccggccagtcataacaatgaactaggatattaagaccaaaaacaacgctacgcgtttgacagaagataaaaatggggcaaatgcaaacatgaagtgccttttgtacttagcctttttattcattggggtgaattgcaagttcaccatagtttttccacacaaccaaaaaggaaactggaaaaatgttccttctaattaccattattgcccgtcaagctcagatttaaattggcataatgacttaataggcacagccttacaagtcaaaatgcccaagagtcacaaggctattcaagcagacggttggatgtgtcatgcttccaaatgggtcactacttgtgatttccgctggtatggaccgaagtatataacacattccatccgatccttcactccatctgtagaacaatgcaaggaaagcattgaacaaacgaaacaaggaacttggctgaatccaggcttccctcctcaaagttgtggatatgcaactgtgacggatgccgaagcagtgattgtccaggtgactcctcaccatgtgctggttgatgaatacacaggagaatgggttgattcacagttcatcaacggaaaatgcagcaattacatatgccccactgtccataactctacaacctggcattctgactataaggtcaaagggctatgtgattctaacctcatttccatggacatcaccttcttctcagaggacggagagctatcatccctgggaaaggagggcacagggttcagaagtaactactttgcttatgaaactggaggcaaggcctgcaaaatgcaatactgcaagcattggggagtcagactcccatcaggtgtctggttcgagatggctgataaggatctctttgctgcagccagattccctgaatgcccagaagggtcaagtatctctgctccatctcagacctcagtggatgtaagtctaattcaggacgttgagaggatcttggattattccctctgccaagaaacctggagcaaaatcagagcgggtcttccaatctctccagtggatctcagctatcttgctcctaaaaacccaggaaccggtcctgctttcaccataatcaatggtaccctaaaatactttgagaccagatacatcagagtcgatattgctgctccaatcctctcaagaatggtcggaatgatcagtggaactaccacagaaagggaactgtgggatgactgggcaccatatgaagacgtggaaattggacccaatggagttctgaggaccagttcaggatataagtttcctttatacatgattggacatggtatgttggactccgatcttcatcttagctcaaaggctcaggtgttcgaacatcctcacattcaagacgctgcttcgcaacttcctgatgatgagagtttattttttggtgatactgggctatccaaaaatccaatcgagcttgtagaaggttggttcagtagttggaaaagctctattgcctcttttttctttatcatagggttaatcattggactattcttggttctccgagttggtatccatctttgcattaaagccagaagcacaccagtcacattaagtaaggatcaactgagtggtataaataatattgcatttagtaactaatagtcattaaaaagcgggcccgtattgttgcaaaaagccatgaccaaatcaaacagaatcaaaatcaactctggggcaaataacaatggagttgccaatcctcaaaacaaatgctattaccacaatccttgctgcagtcacactctgtttcgcttccagtcaaaacatcactgaagaattttatcaatcaacatgcagtgcagtcagcaaaggctatcttagtgctctaagaactggttggtatactagtgttataactatagaattaagtaatatcaaggaaaataagtgtaatggtacagacgctaaggtaaaattaataaaacaagaattagataaatataaaaatgctgtaacagaattgcagttgctcatgcaaagcacaccagcagccaacaatggagccagaggctctggcggaagcggacttggatttttgttaggtgttggatctgcaatcgccagtggcattgccgtatccaaggtcctgcacctagaaggggaagtgaacaaaatcaaaagtgctctactatccacaaacaaggctgtagtcagcttatctaatggagtcagtgtcttaaccagcaaggtgttagacctcaaaaactatatagataaacagttgttacctattgttaacaagcaaagctgcagcatatcaaacattgaaactgtgatagagttccaacaaaagaacaacagactactagagattaccagagaatttagtgttaatgcaggtgtaactactcctgtaagcacttatatgttaactaatagtgagttattatcattaatcaatgatatgcctataacaaatgatcagaaaaagttaatgtccagcaatgttcaaatagttagacagcaaagttactctatcatgtcaataataaaagaggaagtcttggcatatgtagtacaattaccactatatggtgtaatagatactccttgttggaaactacacacatcccctttatgtacaaccaacacaaaggaaggatccaacatctgcttaacaagaaccgacagaggatggtactgtgacaatgcaggatcagtatcctttttcccacaagctgaaacatgtaaagttcaatcgaatcgggtgttttgtgacacaatgaacagtttaacattaccaagtgaggtaaatctctgcaacattgacatattcaaccccaaatatgattgcaaaattatgacttcaaaaacagatgtaagcagctccgttatcacatctctaggagccattgtgtcatgctatggcaaaaccaaatgtacagcatccaataaaaatcgtgggatcataaagacattctctaacgggtgtgattatgtatcaaataagggggtggatactgtgtctgtaggtaatacattatattatgtaaataagcaagaaggcaaaagtctctatgtaaaaggtgaaccaataataaatttctatgatccattagtgttcccctctgatgaatttgatgcatcaatatctcaagtcaatgagaaaattaatcagagtctagcatttatccgtaaatcagatgaattattacataatgtaaatgctggtaaatccaccacaaatatcatgataactaccataattatagtaattatagtaatattgttagcattaattgcagttggactgcttctatactgcaaggccagaagcacaccagtcacattaagtaaggatcaactgagtggtataaataatattgcatttagtaactgaataaaaatagcacctaatcatattcttacaatggttcgctatttgaccatagataacccatctatcattagattatcctaaaatttgaacttcatcacaactttcatctataaaccatctcacttacactttttaagtagatttctattttatagttatataaaacagggcccattgaataccaaattaacttactatttgtaaaaatgagaattggggcaaatatgtcacgaaggaatccttgcaaattcgaaattcgaggtcattgcttgaatggtaaaaggtgtcattttagtcataattattttgaatggccaccccatgcactgcttgtaagacaaaactttatgttaaacagaatacttaagtctatggataaaagcatagatactttgtcagaaataagtggagctgcagagttggacagaacagaagagtatgccctcggtgtagttggagtgctagagagttatataggatcaataaataatataactaaacaatcagcatgtgttgccatgagcaaactccttactgaactcaacagcgatgacatcaaaaaactaagggacaatgaagagccaaactcacccaaagtaagagtgtacaatactgtcatatcatatattgaaagcaacaggaagaacaataaacaaactatccatctgttaaaaagattgccagcagacgtattgaagaaaaccatcaaaaacacattggatatccacaagagcataaccatcaataacccaaaagaatcaactgttagtgatacgaacgaccatgccaaaaataatgatactacctgacaaatatccttgtagtataaattccatactaataacaagtaattgtagagtcactatgtataatcaaaaaaacacactatatatcaatcaaaacaaccaaaatagccatatatacccaccggatcaaccattcaatgaaatccattggacctctcaagacttgattgatgcaactcaaaattttctacaacatctaggtattactgatgatatatacacaatatatatattagtgtcataatactcaatcctaatacttaccacatcatcaaattattaactcaaacaattcaagctatgggacaaaatggatcccattattagtggaaattctgctaatgtttatctaactgatagttatttaaaaggtgttatttctttctcagaatgtaacgctttaggaagttacatattcaatggtccttatctcaaaaatgattataccaacttaattagtagacaaaatccattaatagaacacataaatctaaagaaactaaatataacacagtccttaatatctaagtatcataaaggtgaaataaaaatagaagaacctacttactttcagtcattacttatgacatacaagagtatgacctcttcagaacagactactactactaatttacttaaaaagataataagaagagctatagaaatcagtgatgtcaaagtctatgctatattgaataaactggggctcaaagaaaaagacaagattaaatccaataatggacaagatgaagacaactcagtcattactaccataatcaaagatgatatacttttagctgtcaaggataatcaatctcatcttaaagcagacaaaaatcaatccacaaaacaaaaagatacaatcaaaacaacacttttgaagaaattaatgtgttcgatgcaacatcctccatcatggttaatacattggtttaatttatacacaaaattaaacagcatattaacacaatatcgatctagtgaggtaaaaaaccatggttttatattgatagataatcatactcttagtggattccaatttattttgaatcaatatggttgtatagtttatcataaggaactcaaaagaattactgtgacaacttataatcaattcttgacatggaaagatattagccttagtagattaaatgtttgtttgattacatggattagtaactgtttgaacacattaaacaaaagcttaggcttaagatgtggattcaataatgttatcttgacacaattattcctttatggagattgtatactaaaactattccacaatgaggggttctacataataaaagaggtagagggatttattatgtctctaattttaaatataacagaagaagatcaattcagaaaacggttttataatagtatgctcaacaacatcacagatgccgccaacaaagctcaaaaaaatctgctatcaagagtatgtcatacattattagataagacaatatcagataatataataaatggcagatggataattctattgagtaagttcctaaaattaattaagcttgcaggtgacaataacctcaacaatctgagtgaattatattttttgttcagaatatttggacacccaatggtagatgaaagacaagccatggatgctgttaaagttaattgcaacgagaccaaattttatttgttaagtagtttgagtatgttaagaggagcttttatatatagaattataaaagggtttgtaaataattacaacagatggcctactttaagaaatgccattgtcttacccttaagatggttaacttactataaactaaacacttatccttccttgttggaacttacagaaagagatttgattgttctatcaggactacgtttctatcgagagtttcggttgcctaaaaaagtggatcttgaaatgatcataaatgataaggctatatcacctcctaaaaatttaatatggactagtttccctagaaattatatgccgtcacacatacaaaattatatagaacatgaaaaattaaaattctctgatagtgataaatcaagaagagtattagagtattatttaagagataacaaattcaatgaatgtgatttacacaactgtgtagttaatcaaagttatcttaacaacccgaatcatgtggtatcattgacaggcaaagaaagagaactcagtgtaggtagaatgtttgcaatgcaaccaggaatgttcagacaagttcaaatattagcagagaaaatgatagcagaaaacatattacaatttttccctgaaagtcttacaagatatggtgatctagaactacagaaaatattagaattgaaagcaggaataagtaacaaatcaaatcgttacaatgataattacaacaattacattagtaagtgctctatcatcacagatctcagcaaattcaatcaagcatttcgatatgaaacatcatgtatttgtagtgatgtactggatgaactgcatggtgtacaatctctattttcctggttacatttaactattcctcatgtcacaataatatgcacatataggcatgcacccccctatataaaggatcatattgtagatcttaacaatgtagatgagcaaagtggactatatagatatcatatgggtggtatcgaagggtggtgtcaaaaactatggaccatagaagctatatcactattagatctaatatctctcaaagggaaattctcaattactgctttaattaatggtgacaatcaatcaatagatataagtaaaccagtcagactcatggaaggtcaaactcatgctcaagcagattatttgctagcattaaatagtctcaaattactgtataaagagtatgcaggaataggccacaaattaaaaggaactgagacttatatatcgagagatatgcaatttatgagtaaaacgatccaacataacggtgtatattacccagctagtataaagaaagtcctaagagtgggaccgtggataaacactatacttgatgacttcaaagtgagtctagaatctataggtagtttgacacaagaattagaatatagaggtgaaagtctattatgcagtttaatatttagaaatgtatggttatataatcaaattgcattacaacttaaaaatcatgcattatgtaacaacaaattatatttggatatattaaaagttctaaaacacttaaaaaccttttttaatcttgataacattgatacagcattaacattgtatatgaatttgcccatgttatttggtggtggtgatcccaacttgttatatcgaagtttctatagaagaactcctgatttcctcacagaggctatagttcactctgtgttcatacttagttattatacaaaccatgatttaaaagataaacttcaagatctgtcagatgatagattgaataagttcttaacatgcataatcacgtttgataaaaaccccaatgctgaattcgttacattgatgagagatcctcaagctttaggatctgagaggcaagctaaaattactagcgaaatcaatagactggcagttaccgaggttttgagcacagctccaaacaaaatattttccaaaagtgcacaacactataccactacagagatagatcttaatgatattatgcaaaatatagaacctacatatcctcacgggctaagagttgtttatgagagtttacccttttataaagcagagaaaatagtaaatcttatatccggtacaaaatctataactaacatactggaaaagacttctgccatagacttaacagatattgatagagccactgagatgatgaggaaaaacataactttgcttataaggatattaccattagattgtaacagagataaaagagaaatattgagtatggaaaacctaagtattactgaattaagcaaatacgttagagaaagatcttggtctttatccaatatagttggtgttacatcacccagtatcatgtatacaatggacataaaatatacaacaagcactatagctagtggcataatcatagagaaatataatgtcaacagtttaacacgtggtgagagaggacccactaaaccatgggttggttcatctacacaagagaaaaagacaatgccagtttataatagacaagttttaaccaaaaaacagagagatcaaatagatctattagcaaaattggattgggtgtatgcatctatagataacaaggatgaatttatggaggaacttagcataggaactcttgggttaacatatgagaaggccaaaaaattattcccacaatatttgagtgttaactatttgcatcgtcttacagtcagtagtagaccatgtgaattccctgcatctataccagcttatagaactacaaattatcactttgatactagccctattaatcgcatattaacagaaaagtatggtgatgaagatattgatatagtattccaaaactgtataagctttggccttagcttaatgtctgtagtagaacaatttactaatgtatgtcctaacagaattattctcatacccaagcttaatgagatacatttgatgaaacctcccatattcacaggcgatgttgatattcacaagttaaaacaagtgatacaaaaacaacatatgtttttaccagacaaaataagtttgactcaatatgtggaattattcttaagtaataaaacactcaaatctggatctaatgttaattctaatttaatattggcgcataagatatctgactattttcataatacttacattttgagtactaatttagctggacattggattcttattatacaacttatgaaagattctaagggtatttttgaaaaagattggggagagggatatataactgatcatatgttcattaatttgaaagttttcttcaatgcttataagacatatctcttgtgttttcataaaggttacggcagagcaaagctggagtgtgatatgaatacttcagatctcctatgtgtattggaattaatagacagtagttattggaagtctatgtctaaggtgtttttagaacaaaaagttatcaaatacattcttagccaggatgcaagtttacatagagtaaaaggatgtcatagcttcaaactatggtttcttaaacgtcttaatgtagcagaattcacagtttgcccttgggttgttaacatagattatcatccaacacatatgaaagcaatattaacttatattgatcttgttagaatgggattgataaatatagatagaatatacattaaaaataaacacaagttcaatgatgagttttatacttctaatctgttttacattaattataacttctcagataatactcatctattaactaaacatataaggattgctaattccgaattagaaagtaattacaacaaattatatcatcctacaccagaaaccctagaaaatatactaaccaatccggttaaaagtaatgagaaaaagacactgagtgactattgtataggtaaaaatgttgactcaataatgttaccatcgttatctaataagaagcttattaaatcgtctacaatgattagaaccaattacagcagacaagatttgtataatttatttcctacggttgtgattgataaaattatagatcattcaggtaatacagccaaatctaaccaactttacactactacttctcatcaaatatccttagtgcacaatagcacatcactttattgcatgcttccttggcatcatattaatagattcaattttgtatttagttctacaggttgtaaaattagtatagagtatattttaaaagatcttaaaattaaggatcctaattgtatagcattcataggtgaaggagcagggaatttattattgcgtacagtagtggaacttcatcctgatataagatatatttacagaagtctgaaagattgcaatgatcatagtttaccaattgagtttttaaggctgtacaatggacatatcaacattgattatggtgaaaatttgaccattcctgctacagatgcaaccaacaacattcattggtcttatttacatataaagtttgctgaacctatcagtctttttgtctgtgatgctgaattgcctgtaacagtcaactggagtaagattataatagagtggagcaagcatgtaagaaaatgcaagtactgttcttcagttaataaatgtacattgatagtaaaatatcatgctcaagatgatatcgatttcaaattagacaacataactatattaaaaacttatgtatgcttaggtagtaagttaaagggatctgaagtttacttagtccttacaataggtcctgcaaatgtgttcccagtatttaatgtagtacaaaatgctaaattgatactatcaagaactaaaaatttcatcatgcctaaaaaagctgataaagagtctattgatgcaaatattaagagtttgataccctttctttgttaccctataacaaaaaaaggaattaatactgcattgtctaaattaaagagtgttgttagtggagatatactatcatattctatagctggacgtaatgaagttttcagcaataaacttataaatcataagcatatgaacatcttaaagtggttcaatcatgttttaaatttcagatcaacagaattaaactataatcatttatatatggtagaatctacttatcctcatctaagtgaattgttaaacagcttgacaaccaatgaacttaaaaaactgattaaaatcacaggtagtttgttatacaacttttataatgaataatgagcaaaaatcttataacaaaaatagctacacactaacattgtattcaattatagttattgaaaattaataattatataatttttaataacttctagtgaactaatcctaaaattatcattttgatctaggaagaataagtttaaatccaaatctaattggtttatatgtatattaactaaattacgagatattagtttttgacactttttttctcgt

SEQ ID NO: 14 - DNA, 16823 bp, synthetic construct
  misc_feature 1..16823: note = A sequence in which SEQ ID NO: 11 was digested with AscI and Sbfland replaced with deoptimized NS1 and NS2 coding regions.
  source 1..16823: mol_type = other DNA
acgcgaaaaaatgcgtacaacaaacttgcgtaaaccaaaaaaatggggcaaataagaatttgataagtaccacttaaatttaactcctttggttagaggcgcgccatgggttcgaattcgctatcgatgataaaagtacgtctacaaaatctatttgataatgatgaagtagcgctactaaaaataacgtgttatacggataaactaatacaactaacgaatgcgctagcgaaagcggtaatacatacgataaaactaaatggtatagtatttgtacatgtaataacgtcgtcggatatatgtccgaataataatatagtagtaaaatcgaattttacgacgatgccggtactacaaaatggtggttatatatgggaaatgatggaactaacgcattgttcgcaaccgaatggtctaatagatgataattgtgaaataaaattttcgaaaaaactatcggattcgacgatgacgaattatatgaatcaactatcggaactactaggttttgatctaaatccgtaaatcataataaatatcaactagcaaatcaatgtcactaacaccattagttaatataaaacttgacagaagataaaaatggggcaaataaatcaattcagccgacccaaccatggatacgacgcataatgatacgacgccgcaacgtctaatgataacggatatgcgtccgctatcgctagaaacgataataacgtcgctaacgcgagatataataacgcataaatttatatatctaataaatcatgaatgtatagtacgtaaactagatgaacgtcaagcgacgtttacgtttctagtaaattatgaaatgaaactactacataaagtaggttcgacgaaatataaaaaatatacggaatataatacgaaatatggtacgtttccgatgccgatatttataaatcatgatggttttctagaatgtataggtataaaaccgacgaaacatacgccgataatatataaatatgatctaaatccgtgaatatcaaaccaagattcaaacaatccgaaataacaactttatgcataatcacactccatagtccaaatggagcctgaaaattatagttatttaaaattcctgcaggaaggagagacataagatgaaagatggggcaaatacaaaaatggctcttagcaaagtcaagttgaatgatacactcaacaaagatcaacttctatcatccagcaaatataccatccaacggagcacaggagacagcattgacactcctaattatgatgtgcagaaacacattaataagttatgtggcatgttattaatcacagaagatgctaatcataaattcactgggttaataggtatgttatatgctatgtctagattaggaagagaagacaccataaaaatactcaaagatgcgggatatcatgttaaggcaaatggagtggatgtaacaacacatcgtcaagacattaatgggaaagaaatgaaatttgaagtgttaacattagcaagcttaacaactgaaattcaaatcaacattgagatagaatctagaaaatcctacaaaaaaatgctaaaagaaatgggagaggtggctccagaatacaggcatgactctcctgattgtgggatgataatattatgtatagcggcattagtaataaccaaattagcagcaggagatagatcaggtcttacagctgtgattaggagagctaataatgtcctaaaaaatgaaatgaaacgttataaaggtttattacccaaggatatagccaacagcttctatgaagtgtttgaaaaatatcctcactttatagatgtttttgttcattttggtatagcacaatcttctaccagaggtggcagtagagttgaagggatttttgcaggattgtttatgaatgcctatggtgcagggcaagtgatgttacggtggggggtcttagcaaaatcagttaaaaacattatgttaggacacgctagtgtacaagcagaaatggaacaagttgtggaggtgtatgagtatgctcagaaattgggtggagaagcaggattctaccatatattgaacaacccaaaagcatcactattatctttgactcaatttcctcacttctctagtgtagtattgggcaatgctgctggcctaggcataatgggagaatacagaggtacaccaaggaatcaagatttatatgatgctgcaaaagcatatgctgaacaactcaaagaaaatggtgtgattaactacagtgtattagatttgacagcagaagaactagaggctatcaaacatcagcttaatccaaaagataatgatgtagagctttgagttaataaaaaagtggggcaaataaatcatcatggaaaagtttgctcctgaattccatggagaagatgcaaacaacagagccaccaaattcctagaatcaataaagggcaaattcacatcacccaaagatcccaagaaaaaagatagtatcatatctgtcaactcaatagatatagaagtaaccaaagaaagccctataacatcaaattcaaccattataaacccaataaatgagacagatgatactgtagggaacaagcccaattatcaaagaaagcctctagtaagtttcaaagaagaccctacgccaagtgataatcctttttcaaaactatacaaagaaaccatagaaacatttgataacaatgaagaagaatctagctattcatatgaagaaataaatgatcagacaaacgataatataacagcaagattagataggattgatgagaaattaagtgaaatactaggaatgcttcacacattagtagtagcgagtgcaggacccacatctgctcgggatggtataagagatgccatggttggtttaagagaagaaatgatagaaaaaatcagaactgaagcattaatgaccaatgacagactagaagctatggcaagactcaggaatgaagaaagtgaaaagatggcaaaagacacatcagatgaagtgtctctcaatccaacatcagagaaactgaacaacctgttggaagggaatgatagtgacaatgatctatcacttgaagatttctgattagctaccaaactgtacatcaaaacacaacaccaatagaaaaccaacaaacaaaccaactcacccatccaaccaaacatctatctgctgattagccaaccagccaaaaaacaaccagccaatctaaaactagccacccggaaaaaatcgatactatagttacaaaaaaagatggggcaaatatggaaacatacgtgaataaacttcacgagggctccacatacacagctgctgttcaatacaatgtcctagaaaaagacgatgatcctgcatcacttacaatatgggtgcccatgttccaatcatccatgccagcagatctactcataaaagaactagccaatgtcaatatactagtgaaacaaatatccacacccaagggaccctcattaagagtcatgataaactcaagaagtgcagtgctagcacaaatgcccagcaaatttaccatatgtgccaatgtgtccttggatgaaagaagcaagctggcatatgatgtaaccacaccctgtgaaattaaggcatgcagtctaacatgcctaaaatcaaaaaatatgttaactacagttaaagatctcactatgaaaacactcaacccaacacatgacatcattgctttatgtgaatttgaaaatatagtaacatcaaaaaaagtcataataccaacatacctaagatctatcagcgtcagaaataaagatctgaacacacttgaaaatataacaaccactgaattcaaaaatgccattacaaatgcaaaaatcatcccttactcaggattattgttagtcatcacagtgactgacaacaaaggagcattcaaatacataaagccacaaagtcaattcatagtagatcttggagcttacctagaaaaagaaagtatatattatgttacaacaaattggaagcacacagctacacgatttgcaatcaaacccatggaagattaacctttttcctctacatcaatgagtagattcatacaaactttctaactacattcttcacttcacaatcataatcaccaaccctctgtggttcaatcaatcaaacaaaactcatcaagagttccagatcatcccaagtcattgttcatcagatccagtactcaaataagttaataaaaaatccacatggggcaaataatcattgagggaaatccaactaatcacaacatctgtcaacatagacaagtcaacacgctagataaaatcaaccaatggaaaatacatccataactatagaattctcaagcaaattctggccttactttacactaatacacatgataacaacaataatctctttgataatcataatctccatcatgattgcaatactaaacaaactctgcgaatataatgtattccataacaaaacctttgagctaccaagagctcgagtcaatacatagcattcaccaatctgatagctcaaaacagtaaccttgcatttgtaaatgaactaccctcacttcttcacaaaaccacatcaacatctcaccatgcaagccatcatctataccataaagtagttaattaaaaatggccggccagtcataacaatgaactaggatattaagaccaaaaacaacgctggggcaaatgcaaacatgtccaaaaccgaggaccaacgcaccgccaagacactagaaaggacctgggacacttttaatcatctattattcatatcatcgtgcttatacaagttaaatcttaaatctatagcacaaatcacattatctattttggcaattataatctcaacctcacttataattgcagccatcatattcatagcctcggcaaaccacaaagtcacactaacaactgcaatcatacaagatgcaacgaaccagatcaagaacacaaccccaacatacctcacccagaatccccagcatggaatcagcttctccaatctgtccggaactacatcacaatccaccaccatactagcttcaacaacaccaagtgctgattcaaccccacaatccacaacagtcaagatcaaaaacacaacaacaacccaaatattacctagcaaacccaccacaaaacaacgccaaaataaaccacaaaacaaacccaacaatgattttcactttgaagtgttcaattttgtaccctgcagcatatgcagcaacaatccaacctgctgggccatctgcaagagaataccaaacaaaaaacctggaaagaaaaccaccaccaagcccacaaaaaaaccaaccctcaagacaaccaaaaaagatcccaaatcccaaaccacaaaaccaaaggaagtactcactaccaagcctacaggaaagccaaccatcaacaccactaaaacaaacatcagaactacactgctcacctccaacaccaaaggaaatccagaacacacaagtcaagaggaaaccctccactcaaccacctccgaaggctatccaagcccatcacaagtccacacaacatccggtcaagaggaaaccctccactcaaccacctccgaaggctatccaagcccatcacaagtctacacaacatccgagtacctatcacaatctctatcttcatccaacacaacaaaatgatagtcattaaaaagcacgcgtttgacagaagataaaaatggggcaaatgcaaacatgaagtgccttttgtacttagcctttttattcattggggtgaattgcaagttcaccatagtttttccacacaaccaaaaaggaaactggaaaaatgttccttctaattaccattattgcccgtcaagctcagatttaaattggcataatgacttaataggcacagccttacaagtcaaaatgcccaagagtcacaaggctattcaagcagacggttggatgtgtcatgcttccaaatgggtcactacttgtgatttccgctggtatggaccgaagtatataacacattccatccgatccttcactccatctgtagaacaatgcaaggaaagcattgaacaaacgaaacaaggaacttggctgaatccaggcttccctcctcaaagttgtggatatgcaactgtgacggatgccgaagcagtgattgtccaggtgactcctcaccatgtgctggttgatgaatacacaggagaatgggttgattcacagttcatcaacggaaaatgcagcaattacatatgccccactgtccataactctacaacctggcattctgactataaggtcaaagggctatgtgattctaacctcatttccatggacatcaccttcttctcagaggacggagagctatcatccctgggaaaggagggcacagggttcagaagtaactactttgcttatgaaactggaggcaaggcctgcaaaatgcaatactgcaagcattggggagtcagactcccatcaggtgtctggttcgagatggctgataaggatctctttgctgcagccagattccctgaatgcccagaagggtcaagtatctctgctccatctcagacctcagtggatgtaagtctaattcaggacgttgagaggatcttggattattccctctgccaagaaacctggagcaaaatcagagcgggtcttccaatctctccagtggatctcagctatcttgctcctaaaaacccaggaaccggtcctgctttcaccataatcaatggtaccctaaaatactttgagaccagatacatcagagtcgatattgctgctccaatcctctcaagaatggtcggaatgatcagtggaactaccacagaaagggaactgtgggatgactgggcaccatatgaagacgtggaaattggacccaatggagttctgaggaccagttcaggatataagtttcctttatacatgattggacatggtatgttggactccgatcttcatcttagctcaaaggctcaggtgttcgaacatcctcacattcaagacgctgcttcgcaacttcctgatgatgagagtttattttttggtgatactgggctatccaaaaatccaatcgagcttgtagaaggttggttcagtagttggaaaagctctattgcctcttttttctttatcatagggttaatcattggactattcttggttctccgagttggtatccatctttgcattaaagccagaagcacaccagtcacattaagtaaggatcaactgagtggtataaataatattgcatttagtaactaatagtcattaaaaagcgggcccgtattgttgcaaaaagccatgaccaaatcaaacagaatcaaaatcaactctggggcaaataacaatggagttgccaatcctcaaaacaaatgctattaccacaatccttgctgcagtcacactctgtttcgcttccagtcaaaacatcactgaagaattttatcaatcaacatgcagtgcagtcagcaaaggctatcttagtgctctaagaactggttggtatactagtgttataactatagaattaagtaatatcaaggaaaataagtgtaatggtacagacgctaaggtaaaattaataaaacaagaattagataaatataaaaatgctgtaacagaattgcagttgctcatgcaaagcacaccagcagccaacaatcgagccagaagagaactaccaagatttatgaattatacactcaacaataccaaaaacaccaatgtaacattaagtaagaaaaggaaaagaagatttcttggatttttgttaggtgttggatctgcaatcgccagtggcattgccgtatccaaggtcctgcacctagaaggggaagtgaacaaaatcaaaagtgctctactatccacaaacaaggctgtagtcagcttatctaatggagtcagtgtcttaaccagcaaggtgttagacctcaaaaactatatagataaacagttgttacctattgttaacaagcaaagctgcagcatatcaaacattgaaactgtgatagagttccaacaaaagaacaacagactactagagattaccagagaatttagtgttaatgcaggtgtaactactcctgtaagcacttatatgttaactaatagtgagttattatcattaatcaatgatatgcctataacaaatgatcagaaaaagttaatgtccagcaatgttcaaatagttagacagcaaagttactctatcatgtcaataataaaagaggaagtcttggcatatgtagtacaattaccactatatggtgtaatagatactccttgttggaaactacacacatcccctttatgtacaaccaacacaaaggaaggatccaacatctgcttaacaagaaccgacagaggatggtactgtgacaatgcaggatcagtatcctttttcccacaagctgaaacatgtaaagttcaatcgaatcgggtgttttgtgacacaatgaacagtttaacattaccaagtgaggtaaatctctgcaacattgacatattcaaccccaaatatgattgcaaaattatgacttcaaaaacagatgtaagcagctccgttatcacatctctaggagccattgtgtcatgctatggcaaaaccaaatgtacagcatccaataaaaatcgtgggatcataaagacattctctaacgggtgtgattatgtatcaaataagggggtggatactgtgtctgtaggtaatacattatattatgtaaataagcaagaaggcaaaagtctctatgtaaaaggtgaaccaataataaatttctatgatccattagtgttcccctctctcctgtgggatgcatcaatatctcaagtcaatgagaaaattaatcagagtctagcatttatccgtaaatcagatgaattattaggctctggcggaagcggatacatccctgaggcaccaagggacggacaggcctacgtgcgcaaggatggcgagtgggtgctgctgtccacctttctgtgaataaaaatagcacctaatcatattcttacaatggttcgctatttgaccatagataacccatctatcattagattatcctaaaatttgaacttcatcacaactttcatctataaaccatctcacttacactttttaagtagatttctattttatagttatataaaacagggcccattgaataccaaattaacttactatttgtaaaaatgagaattggggcaaatatgtcacgaaggaatccttgcaaattcgaaattcgaggtcattgcttgaatggtaaaaggtgtcattttagtcataattattttgaatggccaccccatgcactgcttgtaagacaaaactttatgttaaacagaatacttaagtctatggataaaagcatagatactttgtcagaaataagtggagctgcagagttggacagaacagaagagtatgccctcggtgtagttggagtgctagagagttatataggatcaataaataatataactaaacaatcagcatgtgttgccatgagcaaactccttactgaactcaacagcgatgacatcaaaaaactaagggacaatgaagagccaaactcacccaaagtaagagtgtacaatactgtcatatcatatattgaaagcaacaggaagaacaataaacaaactatccatctgttaaaaagattgccagcagacgtattgaagaaaaccatcaaaaacacattggatatccacaagagcataaccatcaataacccaaaagaatcaactgttagtgatacgaacgaccatgccaaaaataatgatactacctgacaaatatccttgtagtataaattccatactaataacaagtaattgtagagtcactatgtataatcaaaaaaacacactatatatcaatcaaaacaaccaaaatagccatatatacccaccggatcaaccattcaatgaaatccattggacctctcaagacttgattgatgcaactcaaaattttctacaacatctaggtattactgatgatatatacacaatatatatattagtgtcataatactcaatcctaatacttaccacatcatcaaattattaactcaaacaattcaagctatgggacaaaatggatcccattattagtggaaattctgctaatgtttatctaactgatagttatttaaaaggtgttatttctttctcagaatgtaacgctttaggaagttacatattcaatggtccttatctcaaaaatgattataccaacttaattagtagacaaaatccattaatagaacacataaatctaaagaaactaaatataacacagtccttaatatctaagtatcataaaggtgaaataaaaatagaagaacctacttactttcagtcattacttatgacatacaagagtatgacctcttcagaacagactactactactaatttacttaaaaagataataagaagagctatagaaatcagtgatgtcaaagtctatgctatattgaataaactggggctcaaagaaaaagacaagattaaatccaataatggacaagatgaagacaactcagtcattactaccataatcaaagatgatatacttttagctgtcaaggataatcaatctcatcttaaagcagacaaaaatcaatccacaaaacaaaaagatacaatcaaaacaacacttttgaagaaattaatgtgttcgatgcaacatcctccatcatggttaatacattggtttaatttatacacaaaattaaacagcatattaacacaatatcgatctagtgaggtaaaaaaccatggttttatattgatagataatcatactcttagtggattccaatttattttgaatcaatatggttgtatagtttatcataaggaactcaaaagaattactgtgacaacttataatcaattcttgacatggaaagatattagccttagtagattaaatgtttgtttgattacatggattagtaactgtttgaacacattaaacaaaagcttaggcttaagatgtggattcaataatgttatcttgacacaattattcctttatggagattgtatactaaaactattccacaatgaggggttctacataataaaagaggtagagggatttattatgtctctaattttaaatataacagaagaagatcaattcagaaaacggttttataatagtatgctcaacaacatcacagatgccgccaacaaagctcaaaaaaatctgctatcaagagtatgtcatacattattagataagacaatatcagataatataataaatggcagatggataattctattgagtaagttcctaaaattaattaagcttgcaggtgacaataacctcaacaatctgagtgaattatattttttgttcagaatatttggacacccaatggtagatgaaagacaagccatggatgctgttaaagttaattgcaacgagaccaaattttatttgttaagtagtttgagtatgttaagaggagcttttatatatagaattataaaagggtttgtaaataattacaacagatggcctactttaagaaatgccattgtcttacccttaagatggttaacttactataaactaaacacttatccttccttgttggaacttacagaaagagatttgattgttctatcaggactacgtttctatcgagagtttcggttgcctaaaaaagtggatcttgaaatgatcataaatgataaggctatatcacctcctaaaaatttaatatggactagtttccctagaaattatatgccgtcacacatacaaaattatatagaacatgaaaaattaaaattctctgatagtgataaatcaagaagagtattagagtattatttaagagataacaaattcaatgaatgtgatttacacaactgtgtagttaatcaaagttatcttaacaacccgaatcatgtggtatcattgacaggcaaagaaagagaactcagtgtaggtagaatgtttgcaatgcaaccaggaatgttcagacaagttcaaatattagcagagaaaatgatagcagaaaacatattacaatttttccctgaaagtcttacaagatatggtgatctagaactacagaaaatattagaattgaaagcaggaataagtaacaaatcaaatcgttacaatgataattacaacaattacattagtaagtgctctatcatcacagatctcagcaaattcaatcaagcatttcgatatgaaacatcatgtatttgtagtgatgtactggatgaactgcatggtgtacaatctctattttcctggttacatttaactattcctcatgtcacaataatatgcacatataggcatgcacccccctatataaaggatcatattgtagatcttaacaatgtagatgagcaaagtggactatatagatatcatatgggtggtatcgaagggtggtgtcaaaaactatggaccatagaagctatatcactattagatctaatatctctcaaagggaaattctcaattactgctttaattaatggtgacaatcaatcaatagatataagtaaaccagtcagactcatggaaggtcaaactcatgctcaagcagattatttgctagcattaaatagtctcaaattactgtataaagagtatgcaggaataggccacaaattaaaaggaactgagacttatatatcgagagatatgcaatttatgagtaaaacgatccaacataacggtgtatattacccagctagtataaagaaagtcctaagagtgggaccgtggataaacactatacttgatgacttcaaagtgagtctagaatctataggtagtttgacacaagaattagaatatagaggtgaaagtctattatgcagtttaatatttagaaatgtatggttatataatcaaattgcattacaacttaaaaatcatgcattatgtaacaacaaattatatttggatatattaaaagttctaaaacacttaaaaaccttttttaatcttgataacattgatacagcattaacattgtatatgaatttgcccatgttatttggtggtggtgatcccaacttgttatatcgaagtttctatagaagaactcctgatttcctcacagaggctatagttcactctgtgttcatacttagttattatacaaaccatgatttaaaagataaacttcaagatctgtcagatgatagattgaataagttcttaacatgcataatcacgtttgataaaaaccccaatgctgaattcgttacattgatgagagatcctcaagctttaggatctgagaggcaagctaaaattactagcgaaatcaatagactggcagttaccgaggttttgagcacagctccaaacaaaatattttccaaaagtgcacaacactataccactacagagatagatcttaatgatattatgcaaaatatagaacctacatatcctcacgggctaagagttgtttatgagagtttacccttttataaagcagagaaaatagtaaatcttatatccggtacaaaatctataactaacatactggaaaagacttctgccatagacttaacagatattgatagagccactgagatgatgaggaaaaacataactttgcttataaggatattaccattagattgtaacagagataaaagagaaatattgagtatggaaaacctaagtattactgaattaagcaaatacgttagagaaagatcttggtctttatccaatatagttggtgttacatcacccagtatcatgtatacaatggacataaaatatacaacaagcactatagctagtggcataatcatagagaaatataatgtcaacagtttaacacgtggtgagagaggacccactaaaccatgggttggttcatctacacaagagaaaaagacaatgccagtttataatagacaagttttaaccaaaaaacagagagatcaaatagatctattagcaaaattggattgggtgtatgcatctatagataacaaggatgaatttatggaggaacttagcataggaactcttgggttaacatatgagaaggccaaaaaattattcccacaatatttgagtgttaactatttgcatcgtcttacagtcagtagtagaccatgtgaattccctgcatctataccagcttatagaactacaaattatcactttgatactagccctattaatcgcatattaacagaaaagtatggtgatgaagatattgatatagtattccaaaactgtataagctttggccttagcttaatgtctgtagtagaacaatttactaatgtatgtcctaacagaattattctcatacccaagcttaatgagatacatttgatgaaacctcccatattcacaggcgatgttgatattcacaagttaaaacaagtgatacaaaaacaacatatgtttttaccagacaaaataagtttgactcaatatgtggaattattcttaagtaataaaacactcaaatctggatctaatgttaattctaatttaatattggcgcataagatatctgactattttcataatacttacattttgagtactaatttagctggacattggattcttattatacaacttatgaaagattctaagggtatttttgaaaaagattggggagagggatatataactgatcatatgttcattaatttgaaagttttcttcaatgcttataagacatatctcttgtgttttcataaaggttacggcagagcaaagctggagtgtgatatgaatacttcagatctcctatgtgtattggaattaatagacagtagttattggaagtctatgtctaaggtgtttttagaacaaaaagttatcaaatacattcttagccaggatgcaagtttacatagagtaaaaggatgtcatagcttcaaactatggtttcttaaacgtcttaatgtagcagaattcacagtttgcccttgggttgttaacatagattatcatccaacacatatgaaagcaatattaacttatattgatcttgttagaatgggattgataaatatagatagaatatacattaaaaataaacacaagttcaatgatgagttttatacttctaatctgttttacattaattataacttctcagataatactcatctattaactaaacatataaggattgctaattccgaattagaaagtaattacaacaaattatatcatcctacaccagaaaccctagaaaatatactaaccaatccggttaaaagtaatgagaaaaagacactgagtgactattgtataggtaaaaatgttgactcaataatgttaccatcgttatctaataagaagcttattaaatcgtctacaatgattagaaccaattacagcagacaagatttgtataatttatttcctacggttgtgattgataaaattatagatcattcaggtaatacagccaaatctaaccaactttacactactacttctcatcaaatatccttagtgcacaatagcacatcactttattgcatgcttccttggcatcatattaatagattcaattttgtatttagttctacaggttgtaaaattagtatagagtatattttaaaagatcttaaaattaaggatcctaattgtatagcattcataggtgaaggagcagggaatttattattgcgtacagtagtggaacttcatcctgatataagatatatttacagaagtctgaaagattgcaatgatcatagtttaccaattgagtttttaaggctgtacaatggacatatcaacattgattatggtgaaaatttgaccattcctgctacagatgcaaccaacaacattcattggtcttatttacatataaagtttgctgaacctatcagtctttttgtctgtgatgctgaattgcctgtaacagtcaactggagtaagattataatagagtggagcaagcatgtaagaaaatgcaagtactgttcttcagttaataaatgtacattgatagtaaaatatcatgctcaagatgatatcgatttcaaattagacaacataactatattaaaaacttatgtatgcttaggtagtaagttaaagggatctgaagtttacttagtccttacaataggtcctgcaaatgtgttcccagtatttaatgtagtacaaaatgctaaattgatactatcaagaactaaaaatttcatcatgcctaaaaaagctgataaagagtctattgatgcaaatattaagagtttgataccctttctttgttaccctataacaaaaaaaggaattaatactgcattgtctaaattaaagagtgttgttagtggagatatactatcatattctatagctggacgtaatgaagttttcagcaataaacttataaatcataagcatatgaacatcttaaagtggttcaatcatgttttaaatttcagatcaacagaattaaactataatcatttatatatggtagaatctacttatcctcatctaagtgaattgttaaacagcttgacaaccaatgaacttaaaaaactgattaaaatcacaggtagtttgttatacaacttttataatgaataatgagcaaaaatcttataacaaaaatagctacacactaacattgtattcaattatagttattgaaaattaataattatataatttttaataacttctagtgaactaatcctaaaattatcattttgatctaggaagaataagtttaaatccaaatctaattggtttatatgtatattaactaaattacgagatattagtttttgacactttttttctcgt

SEQ ID NO: 15 - DNA, 15311 bp, synthetic construct
  misc_feature 1..15311: note = A sequence modifying the furin cleavage site II of the F geneincluded in SEQ ID NO: 1
  source 1..15311: mol_type = other DNA
acgcgaaaaaatgcgtacaacaaacttgcgtaaaccaaaaaaatggggcaaataagaatttgataagtaccacttaaatttaactcctttggttagaggcgcgccatgggcagcaactcattgagtatgataaaagttagattgcaaaatctgtttgacaatgatgaagtagcattgttaaaaataacatgctatactgacaaattaatacagttaactaatgctttggctaaggcagttatacatacaatcaaattgaatggcattgtatttgtgcatgttattacaagtagtgatatttgccctaataataatattgtagtgaaatccaatttcacaacaatgccagtattacaaaatggaggttatatatgggaaatgatggaattaacacactgctctcaacctaatggcctaatagatgacaattgtgaaattaaattctccaaaaaactaagtgattcaacaatgaccaattatatgaatcaattatctgaattacttggatttgacctcaatccataaatcataataaatatcaactagcaaatcaatgtcactaacaccattagttaatataaaacttgacagaagataaaaatggggcaaataaatcaattcagccgacccaaccatggacacaacacacaatgataccacaccacaaagactgatgatcacagacatgaggccattatcgcttgagactataataacatctctaaccagagatatcataacacataaatttatatacttgataaatcatgaatgcatagtaagaaaacttgatgaaagacaggccacatttacatttctggtcaactatgaaatgaaactattgcacaaagtgggaagcactaaatataaaaaatatactgaatacaacacaaaatatggcactttccctatgccaatatttatcaatcatgatgggttcttagaatgcattggcattaagcctaccaagcacacacccataatatacaagtatgatctcaatccatgaatatcaaaccaagattcaaacaatccgaaataacaactttatgcataatcacactccatagtccaaatggagcctgaaaattatagttatttaaaattcctgcaggaaggagagacataagatgaaagatggggcaaatacaaaaatggctcttagcaaagtcaagttgaatgatacactcaacaaagatcaacttctatcatccagcaaatataccatccaacggagcacaggagacagcattgacactcctaattatgatgtgcagaaacacattaataagttatgtggcatgttattaatcacagaagatgctaatcataaattcactgggttaataggtatgttatatgctatgtctagattaggaagagaagacaccataaaaatactcaaagatgcgggatatcatgttaaggcaaatggagtggatgtaacaacacatcgtcaagacattaatgggaaagaaatgaaatttgaagtgttaacattagcaagcttaacaactgaaattcaaatcaacattgagatagaatctagaaaatcctacaaaaaaatgctaaaagaaatgggagaggtggctccagaatacaggcatgactctcctgattgtgggatgataatattatgtatagcggcattagtaataaccaaattagcagcaggagatagatcaggtcttacagctgtgattaggagagctaataatgtcctaaaaaatgaaatgaaacgttataaaggtttattacccaaggatatagccaacagcttctatgaagtgtttgaaaaatatcctcactttatagatgtttttgttcattttggtatagcacaatcttctaccagaggtggcagtagagttgaagggatttttgcaggattgtttatgaatgcctatggtgcagggcaagtgatgttacggtggggggtcttagcaaaatcagttaaaaacattatgttaggacacgctagtgtacaagcagaaatggaacaagttgtggaggtgtatgagtatgctcagaaattgggtggagaagcaggattctaccatatattgaacaacccaaaagcatcactattatctttgactcaatttcctcacttctctagtgtagtattgggcaatgctgctggcctaggcataatgggagaatacagaggtacaccaaggaatcaagatttatatgatgctgcaaaagcatatgctgaacaactcaaagaaaatggtgtgattaactacagtgtattagatttgacagcagaagaactagaggctatcaaacatcagcttaatccaaaagataatgatgtagagctttgagttaataaaaaagtggggcaaataaatcatcatggaaaagtttgctcctgaattccatggagaagatgcaaacaacagagccaccaaattcctagaatcaataaagggcaaattcacatcacccaaagatcccaagaaaaaagatagtatcatatctgtcaactcaatagatatagaagtaaccaaagaaagccctataacatcaaattcaaccattataaacccaataaatgagacagatgatactgtagggaacaagcccaattatcaaagaaagcctctagtaagtttcaaagaagaccctacgccaagtgataatcctttttcaaaactatacaaagaaaccatagaaacatttgataacaatgaagaagaatctagctattcatatgaagaaataaatgatcagacaaacgataatataacagcaagattagataggattgatgagaaattaagtgaaatactaggaatgcttcacacattagtagtagcgagtgcaggacccacatctgctcgggatggtataagagatgccatggttggtttaagagaagaaatgatagaaaaaatcagaactgaagcattaatgaccaatgacagactagaagctatggcaagactcaggaatgaagaaagtgaaaagatggcaaaagacacatcagatgaagtgtctctcaatccaacatcagagaaactgaacaacctgttggaagggaatgatagtgacaatgatctatcacttgaagatttctgattagctaccaaactgtacatcaaaacacaacaccaatagaaaaccaacaaacaaaccaactcacccatccaaccaaacatctatctgctgattagccaaccagccaaaaaacaaccagccaatctaaaactagccacccggaaaaaatcgatactatagttacaaaaaaagatggggcaaatatggaaacatacgtgaataaacttcacgagggctccacatacacagctgctgttcaatacaatgtcctagaaaaagacgatgatcctgcatcacttacaatatgggtgcccatgttccaatcatccatgccagcagatctactcataaaagaactagccaatgtcaatatactagtgaaacaaatatccacacccaagggaccctcattaagagtcatgataaactcaagaagtgcagtgctagcacaaatgcccagcaaatttaccatatgtgccaatgtgtccttggatgaaagaagcaagctggcatatgatgtaaccacaccctgtgaaattaaggcatgcagtctaacatgcctaaaatcaaaaaatatgttaactacagttaaagatctcactatgaaaacactcaacccaacacatgacatcattgctttatgtgaatttgaaaatatagtaacatcaaaaaaagtcataataccaacatacctaagatctatcagcgtcagaaataaagatctgaacacacttgaaaatataacaaccactgaattcaaaaatgccattacaaatgcaaaaatcatcccttactcaggattattgttagtcatcacagtgactgacaacaaaggagcattcaaatacataaagccacaaagtcaattcatagtagatcttggagcttacctagaaaaagaaagtatatattatgttacaacaaattggaagcacacagctacacgatttgcaatcaaacccatggaagattaacctttttcctctacatcaatgagtagattcatacaaactttctaactacattcttcacttcacaatcataatcaccaaccctctgtggttcaatcaatcaaacaaaactcatcaagagttccagatcatcccaagtcattgttcatcagatccagtactcaaataagttaataaaaaatccacatggggcaaataatcattgagggaaatccaactaatcacaacatctgtcaacatagacaagtcaacacgctagataaaatcaaccaatggaaaatacatccataactatagaattctcaagcaaattctggccttactttacactaatacacatgataacaacaataatctctttgataatcataatctccatcatgattgcaatactaaacaaactctgcgaatataatgtattccataacaaaacctttgagctaccaagagctcgagtcaatacatagcattcaccaatctgatagctcaaaacagtaaccttgcatttgtaaatgaactaccctcacttcttcacaaaaccacatcaacatctcaccatgcaagccatcatctataccataaagtagttaattaaaaatggccggccagtcataacaatgaactaggatattaagaccaaaaacaacgctggggcaaatgcaaacatgtccaaaaccgaggaccaacgcaccgccaagacactagaaaggacctgggacacttttaatcatctattattcatatcatcgtgcttatacaagttaaatcttaaatctatagcacaaatcacattatctattttggcaattataatctcaacctcacttataattgcagccatcatattcatagcctcggcaaaccacaaagtcacactaacaactgcaatcatacaagatgcaacgaaccagatcaagaacacaaccccaacatacctcacccagaatccccagcatggaatcagcttctccaatctgtccggaactacatcacaatccaccaccatactagcttcaacaacaccaagtgctgattcaaccccacaatccacaacagtcaagatcaaaaacacaacaacaacccaaatattacctagcaaacccaccacaaaacaacgccaaaataaaccacaaaacaaacccaacaatgattttcactttgaagtgttcaattttgtaccctgcagcatatgcagcaacaatccaacctgctgggccatctgcaagagaataccaaacaaaaaacctggaaagaaaaccaccaccaagcccacaaaaaaaccaaccctcaagacaaccaaaaaagatcccaaatcccaaaccacaaaaccaaaggaagtactcactaccaagcctacaggaaagccaaccatcaacaccactaaaacaaacatcagaactacactgctcacctccaacaccaaaggaaatccagaacacacaagtcaagaggaaaccctccactcaaccacctccgaaggctatccaagcccatcacaagtccacacaacatccggtcaagaggaaaccctccactcaaccacctccgaaggctatccaagcccatcacaagtctacacaacatccgagtacctatcacaatctctatcttcatccaacacaacaaaatgatagtcattaaaaagcacgcgtgtattgttgcaaaaagccatgaccaaatcaaacagaatcaaaatcaactctggggcaaataacaatggagttgccaatcctcaaaacaaatgctattaccacaatccttgctgcagtcacactctgtttcgcttccagtcaaaacatcactgaagaattttatcaatcaacatgcagtgcagtcagcaaaggctatcttagtgctctaagaactggttggtatactagtgttataactatagaattaagtaatatcaaggaaaataagtgtaatggtacagacgctaaggtaaaattaataaaacaagaattagataaatataaaaatgctgtaacagaattgcagttgctcatgcaaagcacaccagcagccaacaatcgaccctccaaggaactaccaagatttatgaattatacactcaacaataccaaaaacaccaatgtaacattaagtaagaaaaggaaaagaagatttcttggatttttgttaggtgttggatctgcaatcgccagtggcattgccgtatccaaggtcctgcacctagaaggggaagtgaacaaaatcaaaagtgctctactatccacaaacaaggctgtagtcagcttatctaatggagtcagtgtcttaaccagcaaggtgttagacctcaaaaactatatagataaacagttgttacctattgttaacaagcaaagctgcagcatatcaaacattgaaactgtgatagagttccaacaaaagaacaacagactactagagattaccagagaatttagtgttaatgcaggtgtaactactcctgtaagcacttatatgttaactaatagtgagttattatcattaatcaatgatatgcctataacaaatgatcagaaaaagttaatgtccagcaatgttcaaatagttagacagcaaagttactctatcatgtcaataataaaagaggaagtcttggcatatgtagtacaattaccactatatggtgtaatagatactccttgttggaaactacacacatcccctttatgtacaaccaacacaaaggaaggatccaacatctgcttaacaagaaccgacagaggatggtactgtgacaatgcaggatcagtatcctttttcccacaagctgaaacatgtaaagttcaatcgaatcgggtgttttgtgacacaatgaacagtttaacattaccaagtgaggtaaatctctgcaacattgacatattcaaccccaaatatgattgcaaaattatgacttcaaaaacagatgtaagcagctccgttatcacatctctaggagccattgtgtcatgctatggcaaaaccaaatgtacagcatccaataaaaatcgtgggatcataaagacattctctaacgggtgtgattatgtatcaaataagggggtggatactgtgtctgtaggtaatacattatattatgtaaataagcaagaaggcaaaagtctctatgtaaaaggtgaaccaataataaatttctatgatccattagtgttcccctctgatgaatttgatgcatcaatatctcaagtcaatgagaaaattaatcagagtctagcatttatccgtaaatcagatgaattattacataatgtaaatgctggtaaatccaccacaaatatcatgataactaccataattatagtaattatagtaatattgttagcattaattgcagttggactgcttctatactgcaaggccagaagcacaccagtcacattaagtaaggatcaactgagtggtataaataatattgcatttagtaactgaataaaaatagcacctaatcatattcttacaatggttcgctatttgaccatagataacccatctatcattagattatcctaaaatttgaacttcatcacaactttcatctataaaccatctcacttacactttttaagtagatttctattttatagttatataaaacagggcccattgaataccaaattaacttactatttgtaaaaatgagaattggggcaaatatgtcacgaaggaatccttgcaaattcgaaattcgaggtcattgcttgaatggtaaaaggtgtcattttagtcataattattttgaatggccaccccatgcactgcttgtaagacaaaactttatgttaaacagaatacttaagtctatggataaaagcatagatactttgtcagaaataagtggagctgcagagttggacagaacagaagagtatgccctcggtgtagttggagtgctagagagttatataggatcaataaataatataactaaacaatcagcatgtgttgccatgagcaaactccttactgaactcaacagcgatgacatcaaaaaactaagggacaatgaagagccaaactcacccaaagtaagagtgtacaatactgtcatatcatatattgaaagcaacaggaagaacaataaacaaactatccatctgttaaaaagattgccagcagacgtattgaagaaaaccatcaaaaacacattggatatccacaagagcataaccatcaataacccaaaagaatcaactgttagtgatacgaacgaccatgccaaaaataatgatactacctgacaaatatccttgtagtataaattccatactaataacaagtaattgtagagtcactatgtataatcaaaaaaacacactatatatcaatcaaaacaaccaaaatagccatatatacccaccggatcaaccattcaatgaaatccattggacctctcaagacttgattgatgcaactcaaaattttctacaacatctaggtattactgatgatatatacacaatatatatattagtgtcataatactcaatcctaatacttaccacatcatcaaattattaactcaaacaattcaagctatgggacaaaatggatcccattattagtggaaattctgctaatgtttatctaactgatagttatttaaaaggtgttatttctttctcagaatgtaacgctttaggaagttacatattcaatggtccttatctcaaaaatgattataccaacttaattagtagacaaaatccattaatagaacacataaatctaaagaaactaaatataacacagtccttaatatctaagtatcataaaggtgaaataaaaatagaagaacctacttactttcagtcattacttatgacatacaagagtatgacctcttcagaacagactactactactaatttacttaaaaagataataagaagagctatagaaatcagtgatgtcaaagtctatgctatattgaataaactggggctcaaagaaaaagacaagattaaatccaataatggacaagatgaagacaactcagtcattactaccataatcaaagatgatatacttttagctgtcaaggataatcaatctcatcttaaagcagacaaaaatcaatccacaaaacaaaaagatacaatcaaaacaacacttttgaagaaattaatgtgttcgatgcaacatcctccatcatggttaatacattggtttaatttatacacaaaattaaacagcatattaacacaatatcgatctagtgaggtaaaaaaccatggttttatattgatagataatcatactcttagtggattccaatttattttgaatcaatatggttgtatagtttatcataaggaactcaaaagaattactgtgacaacttataatcaattcttgacatggaaagatattagccttagtagattaaatgtttgtttgattacatggattagtaactgtttgaacacattaaacaaaagcttaggcttaagatgtggattcaataatgttatcttgacacaattattcctttatggagattgtatactaaaactattccacaatgaggggttctacataataaaagaggtagagggatttattatgtctctaattttaaatataacagaagaagatcaattcagaaaacggttttataatagtatgctcaacaacatcacagatgccgccaacaaagctcaaaaaaatctgctatcaagagtatgtcatacattattagataagacaatatcagataatataataaatggcagatggataattctattgagtaagttcctaaaattaattaagcttgcaggtgacaataacctcaacaatctgagtgaattatattttttgttcagaatatttggacacccaatggtagatgaaagacaagccatggatgctgttaaagttaattgcaacgagaccaaattttatttgttaagtagtttgagtatgttaagaggagcttttatatatagaattataaaagggtttgtaaataattacaacagatggcctactttaagaaatgccattgtcttacccttaagatggttaacttactataaactaaacacttatccttccttgttggaacttacagaaagagatttgattgttctatcaggactacgtttctatcgagagtttcggttgcctaaaaaagtggatcttgaaatgatcataaatgataaggctatatcacctcctaaaaatttaatatggactagtttccctagaaattatatgccgtcacacatacaaaattatatagaacatgaaaaattaaaattctctgatagtgataaatcaagaagagtattagagtattatttaagagataacaaattcaatgaatgtgatttacacaactgtgtagttaatcaaagttatcttaacaacccgaatcatgtggtatcattgacaggcaaagaaagagaactcagtgtaggtagaatgtttgcaatgcaaccaggaatgttcagacaagttcaaatattagcagagaaaatgatagcagaaaacatattacaatttttccctgaaagtcttacaagatatggtgatctagaactacagaaaatattagaattgaaagcaggaataagtaacaaatcaaatcgttacaatgataattacaacaattacattagtaagtgctctatcatcacagatctcagcaaattcaatcaagcatttcgatatgaaacatcatgtatttgtagtgatgtactggatgaactgcatggtgtacaatctctattttcctggttacatttaactattcctcatgtcacaataatatgcacatataggcatgcacccccctatataaaggatcatattgtagatcttaacaatgtagatgagcaaagtggactatatagatatcatatgggtggtatcgaagggtggtgtcaaaaactatggaccatagaagctatatcactattagatctaatatctctcaaagggaaattctcaattactgctttaattaatggtgacaatcaatcaatagatataagtaaaccagtcagactcatggaaggtcaaactcatgctcaagcagattatttgctagcattaaatagtctcaaattactgtataaagagtatgcaggaataggccacaaattaaaaggaactgagacttatatatcgagagatatgcaatttatgagtaaaacgatccaacataacggtgtatattacccagctagtataaagaaagtcctaagagtgggaccgtggataaacactatacttgatgacttcaaagtgagtctagaatctataggtagtttgacacaagaattagaatatagaggtgaaagtctattatgcagtttaatatttagaaatgtatggttatataatcaaattgcattacaacttaaaaatcatgcattatgtaacaacaaattatatttggatatattaaaagttctaaaacacttaaaaaccttttttaatcttgataacattgatacagcattaacattgtatatgaatttgcccatgttatttggtggtggtgatcccaacttgttatatcgaagtttctatagaagaactcctgatttcctcacagaggctatagttcactctgtgttcatacttagttattatacaaaccatgatttaaaagataaacttcaagatctgtcagatgatagattgaataagttcttaacatgcataatcacgtttgataaaaaccccaatgctgaattcgttacattgatgagagatcctcaagctttaggatctgagaggcaagctaaaattactagcgaaatcaatagactggcagttaccgaggttttgagcacagctccaaacaaaatattttccaaaagtgcacaacactataccactacagagatagatcttaatgatattatgcaaaatatagaacctacatatcctcacgggctaagagttgtttatgagagtttacccttttataaagcagagaaaatagtaaatcttatatccggtacaaaatctataactaacatactggaaaagacttctgccatagacttaacagatattgatagagccactgagatgatgaggaaaaacataactttgcttataaggatattaccattagattgtaacagagataaaagagaaatattgagtatggaaaacctaagtattactgaattaagcaaatacgttagagaaagatcttggtctttatccaatatagttggtgttacatcacccagtatcatgtatacaatggacataaaatatacaacaagcactatagctagtggcataatcatagagaaatataatgtcaacagtttaacacgtggtgagagaggacccactaaaccatgggttggttcatctacacaagagaaaaagacaatgccagtttataatagacaagttttaaccaaaaaacagagagatcaaatagatctattagcaaaattggattgggtgtatgcatctatagataacaaggatgaatttatggaggaacttagcataggaactcttgggttaacatatgagaaggccaaaaaattattcccacaatatttgagtgttaactatttgcatcgtcttacagtcagtagtagaccatgtgaattccctgcatctataccagcttatagaactacaaattatcactttgatactagccctattaatcgcatattaacagaaaagtatggtgatgaagatattgatatagtattccaaaactgtataagctttggccttagcttaatgtctgtagtagaacaatttactaatgtatgtcctaacagaattattctcatacccaagcttaatgagatacatttgatgaaacctcccatattcacaggcgatgttgatattcacaagttaaaacaagtgatacaaaaacaacatatgtttttaccagacaaaataagtttgactcaatatgtggaattattcttaagtaataaaacactcaaatctggatctaatgttaattctaatttaatattggcgcataagatatctgactattttcataatacttacattttgagtactaatttagctggacattggattcttattatacaacttatgaaagattctaagggtatttttgaaaaagattggggagagggatatataactgatcatatgttcattaatttgaaagttttcttcaatgcttataagacatatctcttgtgttttcataaaggttacggcagagcaaagctggagtgtgatatgaatacttcagatctcctatgtgtattggaattaatagacagtagttattggaagtctatgtctaaggtgtttttagaacaaaaagttatcaaatacattcttagccaggatgcaagtttacatagagtaaaaggatgtcatagcttcaaactatggtttcttaaacgtcttaatgtagcagaattcacagtttgcccttgggttgttaacatagattatcatccaacacatatgaaagcaatattaacttatattgatcttgttagaatgggattgataaatatagatagaatatacattaaaaataaacacaagttcaatgatgagttttatacttctaatctgttttacattaattataacttctcagataatactcatctattaactaaacatataaggattgctaattccgaattagaaagtaattacaacaaattatatcatcctacaccagaaaccctagaaaatatactaaccaatccggttaaaagtaatgagaaaaagacactgagtgactattgtataggtaaaaatgttgactcaataatgttaccatcgttatctaataagaagcttattaaatcgtctacaatgattagaaccaattacagcagacaagatttgtataatttatttcctacggttgtgattgataaaattatagatcattcaggtaatacagccaaatctaaccaactttacactactacttctcatcaaatatccttagtgcacaatagcacatcactttattgcatgcttccttggcatcatattaatagattcaattttgtatttagttctacaggttgtaaaattagtatagagtatattttaaaagatcttaaaattaaggatcctaattgtatagcattcataggtgaaggagcagggaatttattattgcgtacagtagtggaacttcatcctgatataagatatatttacagaagtctgaaagattgcaatgatcatagtttaccaattgagtttttaaggctgtacaatggacatatcaacattgattatggtgaaaatttgaccattcctgctacagatgcaaccaacaacattcattggtcttatttacatataaagtttgctgaacctatcagtctttttgtctgtgatgctgaattgcctgtaacagtcaactggagtaagattataatagagtggagcaagcatgtaagaaaatgcaagtactgttcttcagttaataaatgtacattgatagtaaaatatcatgctcaagatgatatcgatttcaaattagacaacataactatattaaaaacttatgtatgcttaggtagtaagttaaagggatctgaagtttacttagtccttacaataggtcctgcaaatgtgttcccagtatttaatgtagtacaaaatgctaaattgatactatcaagaactaaaaatttcatcatgcctaaaaaagctgataaagagtctattgatgcaaatattaagagtttgataccctttctttgttaccctataacaaaaaaaggaattaatactgcattgtctaaattaaagagtgttgttagtggagatatactatcatattctatagctggacgtaatgaagttttcagcaataaacttataaatcataagcatatgaacatcttaaagtggttcaatcatgttttaaatttcagatcaacagaattaaactataatcatttatatatggtagaatctacttatcctcatctaagtgaattgttaaacagcttgacaaccaatgaacttaaaaaactgattaaaatcacaggtagtttgttatacaacttttataatgaataatgagcaaaaatcttataacaaaaatagctacacactaacattgtattcaattatagttattgaaaattaataattatataatttttaataacttctagtgaactaatcctaaaattatcattttgatctaggaagaataagtttaaatccaaatctaattggtttatatgtatattaactaaattacgagatattagtttttgacactttttttctcgt

SEQ ID NO: 16 - DNA, 15311 bp, synthetic construct
  misc_feature 1..15311: note = A sequence modifying the furin cleavage site I of the F geneincluded in SEQ ID NO: 1
  source 1..15311: mol_type = other DNA
acgcgaaaaaatgcgtacaacaaacttgcgtaaaccaaaaaaatggggcaaataagaatttgataagtaccacttaaatttaactcctttggttagaggcgcgccatgggcagcaactcattgagtatgataaaagttagattgcaaaatctgtttgacaatgatgaagtagcattgttaaaaataacatgctatactgacaaattaatacagttaactaatgctttggctaaggcagttatacatacaatcaaattgaatggcattgtatttgtgcatgttattacaagtagtgatatttgccctaataataatattgtagtgaaatccaatttcacaacaatgccagtattacaaaatggaggttatatatgggaaatgatggaattaacacactgctctcaacctaatggcctaatagatgacaattgtgaaattaaattctccaaaaaactaagtgattcaacaatgaccaattatatgaatcaattatctgaattacttggatttgacctcaatccataaatcataataaatatcaactagcaaatcaatgtcactaacaccattagttaatataaaacttgacagaagataaaaatggggcaaataaatcaattcagccgacccaaccatggacacaacacacaatgataccacaccacaaagactgatgatcacagacatgaggccattatcgcttgagactataataacatctctaaccagagatatcataacacataaatttatatacttgataaatcatgaatgcatagtaagaaaacttgatgaaagacaggccacatttacatttctggtcaactatgaaatgaaactattgcacaaagtgggaagcactaaatataaaaaatatactgaatacaacacaaaatatggcactttccctatgccaatatttatcaatcatgatgggttcttagaatgcattggcattaagcctaccaagcacacacccataatatacaagtatgatctcaatccatgaatatcaaaccaagattcaaacaatccgaaataacaactttatgcataatcacactccatagtccaaatggagcctgaaaattatagttatttaaaattcctgcaggaaggagagacataagatgaaagatggggcaaatacaaaaatggctcttagcaaagtcaagttgaatgatacactcaacaaagatcaacttctatcatccagcaaatataccatccaacggagcacaggagacagcattgacactcctaattatgatgtgcagaaacacattaataagttatgtggcatgttattaatcacagaagatgctaatcataaattcactgggttaataggtatgttatatgctatgtctagattaggaagagaagacaccataaaaatactcaaagatgcgggatatcatgttaaggcaaatggagtggatgtaacaacacatcgtcaagacattaatgggaaagaaatgaaatttgaagtgttaacattagcaagcttaacaactgaaattcaaatcaacattgagatagaatctagaaaatcctacaaaaaaatgctaaaagaaatgggagaggtggctccagaatacaggcatgactctcctgattgtgggatgataatattatgtatagcggcattagtaataaccaaattagcagcaggagatagatcaggtcttacagctgtgattaggagagctaataatgtcctaaaaaatgaaatgaaacgttataaaggtttattacccaaggatatagccaacagcttctatgaagtgtttgaaaaatatcctcactttatagatgtttttgttcattttggtatagcacaatcttctaccagaggtggcagtagagttgaagggatttttgcaggattgtttatgaatgcctatggtgcagggcaagtgatgttacggtggggggtcttagcaaaatcagttaaaaacattatgttaggacacgctagtgtacaagcagaaatggaacaagttgtggaggtgtatgagtatgctcagaaattgggtggagaagcaggattctaccatatattgaacaacccaaaagcatcactattatctttgactcaatttcctcacttctctagtgtagtattgggcaatgctgctggcctaggcataatgggagaatacagaggtacaccaaggaatcaagatttatatgatgctgcaaaagcatatgctgaacaactcaaagaaaatggtgtgattaactacagtgtattagatttgacagcagaagaactagaggctatcaaacatcagcttaatccaaaagataatgatgtagagctttgagttaataaaaaagtggggcaaataaatcatcatggaaaagtttgctcctgaattccatggagaagatgcaaacaacagagccaccaaattcctagaatcaataaagggcaaattcacatcacccaaagatcccaagaaaaaagatagtatcatatctgtcaactcaatagatatagaagtaaccaaagaaagccctataacatcaaattcaaccattataaacccaataaatgagacagatgatactgtagggaacaagcccaattatcaaagaaagcctctagtaagtttcaaagaagaccctacgccaagtgataatcctttttcaaaactatacaaagaaaccatagaaacatttgataacaatgaagaagaatctagctattcatatgaagaaataaatgatcagacaaacgataatataacagcaagattagataggattgatgagaaattaagtgaaatactaggaatgcttcacacattagtagtagcgagtgcaggacccacatctgctcgggatggtataagagatgccatggttggtttaagagaagaaatgatagaaaaaatcagaactgaagcattaatgaccaatgacagactagaagctatggcaagactcaggaatgaagaaagtgaaaagatggcaaaagacacatcagatgaagtgtctctcaatccaacatcagagaaactgaacaacctgttggaagggaatgatagtgacaatgatctatcacttgaagatttctgattagctaccaaactgtacatcaaaacacaacaccaatagaaaaccaacaaacaaaccaactcacccatccaaccaaacatctatctgctgattagccaaccagccaaaaaacaaccagccaatctaaaactagccacccggaaaaaatcgatactatagttacaaaaaaagatggggcaaatatggaaacatacgtgaataaacttcacgagggctccacatacacagctgctgttcaatacaatgtcctagaaaaagacgatgatcctgcatcacttacaatatgggtgcccatgttccaatcatccatgccagcagatctactcataaaagaactagccaatgtcaatatactagtgaaacaaatatccacacccaagggaccctcattaagagtcatgataaactcaagaagtgcagtgctagcacaaatgcccagcaaatttaccatatgtgccaatgtgtccttggatgaaagaagcaagctggcatatgatgtaaccacaccctgtgaaattaaggcatgcagtctaacatgcctaaaatcaaaaaatatgttaactacagttaaagatctcactatgaaaacactcaacccaacacatgacatcattgctttatgtgaatttgaaaatatagtaacatcaaaaaaagtcataataccaacatacctaagatctatcagcgtcagaaataaagatctgaacacacttgaaaatataacaaccactgaattcaaaaatgccattacaaatgcaaaaatcatcccttactcaggattattgttagtcatcacagtgactgacaacaaaggagcattcaaatacataaagccacaaagtcaattcatagtagatcttggagcttacctagaaaaagaaagtatatattatgttacaacaaattggaagcacacagctacacgatttgcaatcaaacccatggaagattaacctttttcctctacatcaatgagtagattcatacaaactttctaactacattcttcacttcacaatcataatcaccaaccctctgtggttcaatcaatcaaacaaaactcatcaagagttccagatcatcccaagtcattgttcatcagatccagtactcaaataagttaataaaaaatccacatggggcaaataatcattgagggaaatccaactaatcacaacatctgtcaacatagacaagtcaacacgctagataaaatcaaccaatggaaaatacatccataactatagaattctcaagcaaattctggccttactttacactaatacacatgataacaacaataatctctttgataatcataatctccatcatgattgcaatactaaacaaactctgcgaatataatgtattccataacaaaacctttgagctaccaagagctcgagtcaatacatagcattcaccaatctgatagctcaaaacagtaaccttgcatttgtaaatgaactaccctcacttcttcacaaaaccacatcaacatctcaccatgcaagccatcatctataccataaagtagttaattaaaaatggccggccagtcataacaatgaactaggatattaagaccaaaaacaacgctggggcaaatgcaaacatgtccaaaaccgaggaccaacgcaccgccaagacactagaaaggacctgggacacttttaatcatctattattcatatcatcgtgcttatacaagttaaatcttaaatctatagcacaaatcacattatctattttggcaattataatctcaacctcacttataattgcagccatcatattcatagcctcggcaaaccacaaagtcacactaacaactgcaatcatacaagatgcaacgaaccagatcaagaacacaaccccaacatacctcacccagaatccccagcatggaatcagcttctccaatctgtccggaactacatcacaatccaccaccatactagcttcaacaacaccaagtgctgattcaaccccacaatccacaacagtcaagatcaaaaacacaacaacaacccaaatattacctagcaaacccaccacaaaacaacgccaaaataaaccacaaaacaaacccaacaatgattttcactttgaagtgttcaattttgtaccctgcagcatatgcagcaacaatccaacctgctgggccatctgcaagagaataccaaacaaaaaacctggaaagaaaaccaccaccaagcccacaaaaaaaccaaccctcaagacaaccaaaaaagatcccaaatcccaaaccacaaaaccaaaggaagtactcactaccaagcctacaggaaagccaaccatcaacaccactaaaacaaacatcagaactacactgctcacctccaacaccaaaggaaatccagaacacacaagtcaagaggaaaccctccactcaaccacctccgaaggctatccaagcccatcacaagtccacacaacatccggtcaagaggaaaccctccactcaaccacctccgaaggctatccaagcccatcacaagtctacacaacatccgagtacctatcacaatctctatcttcatccaacacaacaaaatgatagtcattaaaaagcacgcgtgtattgttgcaaaaagccatgaccaaatcaaacagaatcaaaatcaactctggggcaaataacaatggagttgccaatcctcaaaacaaatgctattaccacaatccttgctgcagtcacactctgtttcgcttccagtcaaaacatcactgaagaattttatcaatcaacatgcagtgcagtcagcaaaggctatcttagtgctctaagaactggttggtatactagtgttataactatagaattaagtaatatcaaggaaaataagtgtaatggtacagacgctaaggtaaaattaataaaacaagaattagataaatataaaaatgctgtaacagaattgcagttgctcatgcaaagcacaccagcagccaacaatcgagccagaagagaactaccaagatttatgaattatacactcaacaataccaaaaacaccaatgtaacattaagtaagaaaaggaaaagaaagtttcttggatttttgttaggtgttggatctgcaatcgccagtggcattgccgtatccaaggtcctgcacctagaaggggaagtgaacaaaatcaaaagtgctctactatccacaaacaaggctgtagtcagcttatctaatggagtcagtgtcttaaccagcaaggtgttagacctcaaaaactatatagataaacagttgttacctattgttaacaagcaaagctgcagcatatcaaacattgaaactgtgatagagttccaacaaaagaacaacagactactagagattaccagagaatttagtgttaatgcaggtgtaactactcctgtaagcacttatatgttaactaatagtgagttattatcattaatcaatgatatgcctataacaaatgatcagaaaaagttaatgtccagcaatgttcaaatagttagacagcaaagttactctatcatgtcaataataaaagaggaagtcttggcatatgtagtacaattaccactatatggtgtaatagatactccttgttggaaactacacacatcccctttatgtacaaccaacacaaaggaaggatccaacatctgcttaacaagaaccgacagaggatggtactgtgacaatgcaggatcagtatcctttttcccacaagctgaaacatgtaaagttcaatcgaatcgggtgttttgtgacacaatgaacagtttaacattaccaagtgaggtaaatctctgcaacattgacatattcaaccccaaatatgattgcaaaattatgacttcaaaaacagatgtaagcagctccgttatcacatctctaggagccattgtgtcatgctatggcaaaaccaaatgtacagcatccaataaaaatcgtgggatcataaagacattctctaacgggtgtgattatgtatcaaataagggggtggatactgtgtctgtaggtaatacattatattatgtaaataagcaagaaggcaaaagtctctatgtaaaaggtgaaccaataataaatttctatgatccattagtgttcccctctgatgaatttgatgcatcaatatctcaagtcaatgagaaaattaatcagagtctagcatttatccgtaaatcagatgaattattacataatgtaaatgctggtaaatccaccacaaatatcatgataactaccataattatagtaattatagtaatattgttagcattaattgcagttggactgcttctatactgcaaggccagaagcacaccagtcacattaagtaaggatcaactgagtggtataaataatattgcatttagtaactgaataaaaatagcacctaatcatattcttacaatggttcgctatttgaccatagataacccatctatcattagattatcctaaaatttgaacttcatcacaactttcatctataaaccatctcacttacactttttaagtagatttctattttatagttatataaaacagggcccattgaataccaaattaacttactatttgtaaaaatgagaattggggcaaatatgtcacgaaggaatccttgcaaattcgaaattcgaggtcattgcttgaatggtaaaaggtgtcattttagtcataattattttgaatggccaccccatgcactgcttgtaagacaaaactttatgttaaacagaatacttaagtctatggataaaagcatagatactttgtcagaaataagtggagctgcagagttggacagaacagaagagtatgccctcggtgtagttggagtgctagagagttatataggatcaataaataatataactaaacaatcagcatgtgttgccatgagcaaactccttactgaactcaacagcgatgacatcaaaaaactaagggacaatgaagagccaaactcacccaaagtaagagtgtacaatactgtcatatcatatattgaaagcaacaggaagaacaataaacaaactatccatctgttaaaaagattgccagcagacgtattgaagaaaaccatcaaaaacacattggatatccacaagagcataaccatcaataacccaaaagaatcaactgttagtgatacgaacgaccatgccaaaaataatgatactacctgacaaatatccttgtagtataaattccatactaataacaagtaattgtagagtcactatgtataatcaaaaaaacacactatatatcaatcaaaacaaccaaaatagccatatatacccaccggatcaaccattcaatgaaatccattggacctctcaagacttgattgatgcaactcaaaattttctacaacatctaggtattactgatgatatatacacaatatatatattagtgtcataatactcaatcctaatacttaccacatcatcaaattattaactcaaacaattcaagctatgggacaaaatggatcccattattagtggaaattctgctaatgtttatctaactgatagttatttaaaaggtgttatttctttctcagaatgtaacgctttaggaagttacatattcaatggtccttatctcaaaaatgattataccaacttaattagtagacaaaatccattaatagaacacataaatctaaagaaactaaatataacacagtccttaatatctaagtatcataaaggtgaaataaaaatagaagaacctacttactttcagtcattacttatgacatacaagagtatgacctcttcagaacagactactactactaatttacttaaaaagataataagaagagctatagaaatcagtgatgtcaaagtctatgctatattgaataaactggggctcaaagaaaaagacaagattaaatccaataatggacaagatgaagacaactcagtcattactaccataatcaaagatgatatacttttagctgtcaaggataatcaatctcatcttaaagcagacaaaaatcaatccacaaaacaaaaagatacaatcaaaacaacacttttgaagaaattaatgtgttcgatgcaacatcctccatcatggttaatacattggtttaatttatacacaaaattaaacagcatattaacacaatatcgatctagtgaggtaaaaaaccatggttttatattgatagataatcatactcttagtggattccaatttattttgaatcaatatggttgtatagtttatcataaggaactcaaaagaattactgtgacaacttataatcaattcttgacatggaaagatattagccttagtagattaaatgtttgtttgattacatggattagtaactgtttgaacacattaaacaaaagcttaggcttaagatgtggattcaataatgttatcttgacacaattattcctttatggagattgtatactaaaactattccacaatgaggggttctacataataaaagaggtagagggatttattatgtctctaattttaaatataacagaagaagatcaattcagaaaacggttttataatagtatgctcaacaacatcacagatgccgccaacaaagctcaaaaaaatctgctatcaagagtatgtcatacattattagataagacaatatcagataatataataaatggcagatggataattctattgagtaagttcctaaaattaattaagcttgcaggtgacaataacctcaacaatctgagtgaattatattttttgttcagaatatttggacacccaatggtagatgaaagacaagccatggatgctgttaaagttaattgcaacgagaccaaattttatttgttaagtagtttgagtatgttaagaggagcttttatatatagaattataaaagggtttgtaaataattacaacagatggcctactttaagaaatgccattgtcttacccttaagatggttaacttactataaactaaacacttatccttccttgttggaacttacagaaagagatttgattgttctatcaggactacgtttctatcgagagtttcggttgcctaaaaaagtggatcttgaaatgatcataaatgataaggctatatcacctcctaaaaatttaatatggactagtttccctagaaattatatgccgtcacacatacaaaattatatagaacatgaaaaattaaaattctctgatagtgataaatcaagaagagtattagagtattatttaagagataacaaattcaatgaatgtgatttacacaactgtgtagttaatcaaagttatcttaacaacccgaatcatgtggtatcattgacaggcaaagaaagagaactcagtgtaggtagaatgtttgcaatgcaaccaggaatgttcagacaagttcaaatattagcagagaaaatgatagcagaaaacatattacaatttttccctgaaagtcttacaagatatggtgatctagaactacagaaaatattagaattgaaagcaggaataagtaacaaatcaaatcgttacaatgataattacaacaattacattagtaagtgctctatcatcacagatctcagcaaattcaatcaagcatttcgatatgaaacatcatgtatttgtagtgatgtactggatgaactgcatggtgtacaatctctattttcctggttacatttaactattcctcatgtcacaataatatgcacatataggcatgcacccccctatataaaggatcatattgtagatcttaacaatgtagatgagcaaagtggactatatagatatcatatgggtggtatcgaagggtggtgtcaaaaactatggaccatagaagctatatcactattagatctaatatctctcaaagggaaattctcaattactgctttaattaatggtgacaatcaatcaatagatataagtaaaccagtcagactcatggaaggtcaaactcatgctcaagcagattatttgctagcattaaatagtctcaaattactgtataaagagtatgcaggaataggccacaaattaaaaggaactgagacttatatatcgagagatatgcaatttatgagtaaaacgatccaacataacggtgtatattacccagctagtataaagaaagtcctaagagtgggaccgtggataaacactatacttgatgacttcaaagtgagtctagaatctataggtagtttgacacaagaattagaatatagaggtgaaagtctattatgcagtttaatatttagaaatgtatggttatataatcaaattgcattacaacttaaaaatcatgcattatgtaacaacaaattatatttggatatattaaaagttctaaaacacttaaaaaccttttttaatcttgataacattgatacagcattaacattgtatatgaatttgcccatgttatttggtggtggtgatcccaacttgttatatcgaagtttctatagaagaactcctgatttcctcacagaggctatagttcactctgtgttcatacttagttattatacaaaccatgatttaaaagataaacttcaagatctgtcagatgatagattgaataagttcttaacatgcataatcacgtttgataaaaaccccaatgctgaattcgttacattgatgagagatcctcaagctttaggatctgagaggcaagctaaaattactagcgaaatcaatagactggcagttaccgaggttttgagcacagctccaaacaaaatattttccaaaagtgcacaacactataccactacagagatagatcttaatgatattatgcaaaatatagaacctacatatcctcacgggctaagagttgtttatgagagtttacccttttataaagcagagaaaatagtaaatcttatatccggtacaaaatctataactaacatactggaaaagacttctgccatagacttaacagatattgatagagccactgagatgatgaggaaaaacataactttgcttataaggatattaccattagattgtaacagagataaaagagaaatattgagtatggaaaacctaagtattactgaattaagcaaatacgttagagaaagatcttggtctttatccaatatagttggtgttacatcacccagtatcatgtatacaatggacataaaatatacaacaagcactatagctagtggcataatcatagagaaatataatgtcaacagtttaacacgtggtgagagaggacccactaaaccatgggttggttcatctacacaagagaaaaagacaatgccagtttataatagacaagttttaaccaaaaaacagagagatcaaatagatctattagcaaaattggattgggtgtatgcatctatagataacaaggatgaatttatggaggaacttagcataggaactcttgggttaacatatgagaaggccaaaaaattattcccacaatatttgagtgttaactatttgcatcgtcttacagtcagtagtagaccatgtgaattccctgcatctataccagcttatagaactacaaattatcactttgatactagccctattaatcgcatattaacagaaaagtatggtgatgaagatattgatatagtattccaaaactgtataagctttggccttagcttaatgtctgtagtagaacaatttactaatgtatgtcctaacagaattattctcatacccaagcttaatgagatacatttgatgaaacctcccatattcacaggcgatgttgatattcacaagttaaaacaagtgatacaaaaacaacatatgtttttaccagacaaaataagtttgactcaatatgtggaattattcttaagtaataaaacactcaaatctggatctaatgttaattctaatttaatattggcgcataagatatctgactattttcataatacttacattttgagtactaatttagctggacattggattcttattatacaacttatgaaagattctaagggtatttttgaaaaagattggggagagggatatataactgatcatatgttcattaatttgaaagttttcttcaatgcttataagacatatctcttgtgttttcataaaggttacggcagagcaaagctggagtgtgatatgaatacttcagatctcctatgtgtattggaattaatagacagtagttattggaagtctatgtctaaggtgtttttagaacaaaaagttatcaaatacattcttagccaggatgcaagtttacatagagtaaaaggatgtcatagcttcaaactatggtttcttaaacgtcttaatgtagcagaattcacagtttgcccttgggttgttaacatagattatcatccaacacatatgaaagcaatattaacttatattgatcttgttagaatgggattgataaatatagatagaatatacattaaaaataaacacaagttcaatgatgagttttatacttctaatctgttttacattaattataacttctcagataatactcatctattaactaaacatataaggattgctaattccgaattagaaagtaattacaacaaattatatcatcctacaccagaaaccctagaaaatatactaaccaatccggttaaaagtaatgagaaaaagacactgagtgactattgtataggtaaaaatgttgactcaataatgttaccatcgttatctaataagaagcttattaaatcgtctacaatgattagaaccaattacagcagacaagatttgtataatttatttcctacggttgtgattgataaaattatagatcattcaggtaatacagccaaatctaaccaactttacactactacttctcatcaaatatccttagtgcacaatagcacatcactttattgcatgcttccttggcatcatattaatagattcaattttgtatttagttctacaggttgtaaaattagtatagagtatattttaaaagatcttaaaattaaggatcctaattgtatagcattcataggtgaaggagcagggaatttattattgcgtacagtagtggaacttcatcctgatataagatatatttacagaagtctgaaagattgcaatgatcatagtttaccaattgagtttttaaggctgtacaatggacatatcaacattgattatggtgaaaatttgaccattcctgctacagatgcaaccaacaacattcattggtcttatttacatataaagtttgctgaacctatcagtctttttgtctgtgatgctgaattgcctgtaacagtcaactggagtaagattataatagagtggagcaagcatgtaagaaaatgcaagtactgttcttcagttaataaatgtacattgatagtaaaatatcatgctcaagatgatatcgatttcaaattagacaacataactatattaaaaacttatgtatgcttaggtagtaagttaaagggatctgaagtttacttagtccttacaataggtcctgcaaatgtgttcccagtatttaatgtagtacaaaatgctaaattgatactatcaagaactaaaaatttcatcatgcctaaaaaagctgataaagagtctattgatgcaaatattaagagtttgataccctttctttgttaccctataacaaaaaaaggaattaatactgcattgtctaaattaaagagtgttgttagtggagatatactatcatattctatagctggacgtaatgaagttttcagcaataaacttataaatcataagcatatgaacatcttaaagtggttcaatcatgttttaaatttcagatcaacagaattaaactataatcatttatatatggtagaatctacttatcctcatctaagtgaattgttaaacagcttgacaaccaatgaacttaaaaaactgattaaaatcacaggtagtttgttatacaacttttataatgaataatgagcaaaaatcttataacaaaaatagctacacactaacattgtattcaattatagttattgaaaattaataattatataatttttaataacttctagtgaactaatcctaaaattatcattttgatctaggaagaataagtttaaatccaaatctaattggtttatatgtatattaactaaattacgagatattagtttttgacactttttttctcgt

SEQ ID NO: 17 - DNA, 17095 bp, synthetic construct
  misc_feature 1..17095: note = antigenic cDNA encoding the cRSVA_VSVG_A
  source 1..17095: mol_type = other DNA
taatacgactcactataggttttttcgcgtctgatgaggccgttaggccgaaactcctctccggagtcacgcgaaaaaatgcgtacaacaaacttgcgtaaaccaaaaaaatggggcaaataagaatttgataagtaccacttaaatttaactcctttggttagaggcgcgccatgggcagcaactcattgagtatgataaaagttagattgcaaaatctgtttgacaatgatgaagtagcattgttaaaaataacatgctatactgacaaattaatacagttaactaatgctttggctaaggcagttatacatacaatcaaattgaatggcattgtatttgtgcatgttattacaagtagtgatatttgccctaataataatattgtagtgaaatccaatttcacaacaatgccagtattacaaaatggaggttatatatgggaaatgatggaattaacacactgctctcaacctaatggcctaatagatgacaattgtgaaattaaattctccaaaaaactaagtgattcaacaatgaccaattatatgaatcaattatctgaattacttggatttgacctcaatccataaatcataataaatatcaactagcaaatcaatgtcactaacaccattagttaatataaaacttgacagaagataaaaatggggcaaataaatcaattcagccgacccaaccatggacacaacacacaatgataccacaccacaaagactgatgatcacagacatgaggccattatcgcttgagactataataacatctctaaccagagatatcataacacataaatttatatacttgataaatcatgaatgcatagtaagaaaacttgatgaaagacaggccacatttacatttctggtcaactatgaaatgaaactattgcacaaagtgggaagcactaaatataaaaaatatactgaatacaacacaaaatatggcactttccctatgccaatatttatcaatcatgatgggttcttagaatgcattggcattaagcctaccaagcacacacccataatatacaagtatgatctcaatccatgaatatcaaaccaagattcaaacaatccgaaataacaactttatgcataatcacactccatagtccaaatggagcctgaaaattatagttatttaaaattcctgcaggaaggagagacataagatgaaagatggggcaaatacaaaaatggctcttagcaaagtcaagttgaatgatacactcaacaaagatcaacttctatcatccagcaaatataccatccaacggagcacaggagacagcattgacactcctaattatgatgtgcagaaacacattaataagttatgtggcatgttattaatcacagaagatgctaatcataaattcactgggttaataggtatgttatatgctatgtctagattaggaagagaagacaccataaaaatactcaaagatgcgggatatcatgttaaggcaaatggagtggatgtaacaacacatcgtcaagacattaatgggaaagaaatgaaatttgaagtgttaacattagcaagcttaacaactgaaattcaaatcaacattgagatagaatctagaaaatcctacaaaaaaatgctaaaagaaatgggagaggtggctccagaatacaggcatgactctcctgattgtgggatgataatattatgtatagcggcattagtaataaccaaattagcagcaggagatagatcaggtcttacagctgtgattaggagagctaataatgtcctaaaaaatgaaatgaaacgttataaaggtttattacccaaggatatagccaacagcttctatgaagtgtttgaaaaatatcctcactttatagatgtttttgttcattttggtatagcacaatcttctaccagaggtggcagtagagttgaagggatttttgcaggattgtttatgaatgcctatggtgcagggcaagtgatgttacggtggggggtcttagcaaaatcagttaaaaacattatgttaggacacgctagtgtacaagcagaaatggaacaagttgtggaggtgtatgagtatgctcagaaattgggtggagaagcaggattctaccatatattgaacaacccaaaagcatcactattatctttgactcaatttcctcacttctctagtgtagtattgggcaatgctgctggcctaggcataatgggagaatacagaggtacaccaaggaatcaagatttatatgatgctgcaaaagcatatgctgaacaactcaaagaaaatggtgtgattaactacagtgtattagatttgacagcagaagaactagaggctatcaaacatcagcttaatccaaaagataatgatgtagagctttgagttaataaaaaagtggggcaaataaatcatcatggaaaagtttgctcctgaattccatggagaagatgcaaacaacagagccaccaaattcctagaatcaataaagggcaaattcacatcacccaaagatcccaagaaaaaagatagtatcatatctgtcaactcaatagatatagaagtaaccaaagaaagccctataacatcaaattcaaccattataaacccaataaatgagacagatgatactgtagggaacaagcccaattatcaaagaaagcctctagtaagtttcaaagaagaccctacgccaagtgataatcctttttcaaaactatacaaagaaaccatagaaacatttgataacaatgaagaagaatctagctattcatatgaagaaataaatgatcagacaaacgataatataacagcaagattagataggattgatgagaaattaagtgaaatactaggaatgcttcacacattagtagtagcgagtgcaggacccacatctgctcgggatggtataagagatgccatggttggtttaagagaagaaatgatagaaaaaatcagaactgaagcattaatgaccaatgacagactagaagctatggcaagactcaggaatgaagaaagtgaaaagatggcaaaagacacatcagatgaagtgtctctcaatccaacatcagagaaactgaacaacctgttggaagggaatgatagtgacaatgatctatcacttgaagatttctgattagctaccaaactgtacatcaaaacacaacaccaatagaaaaccaacaaacaaaccaactcacccatccaaccaaacatctatctgctgattagccaaccagccaaaaaacaaccagccaatctaaaactagccacccggaaaaaatcgatactatagttacaaaaaaagatggggcaaatatggaaacatacgtgaataaacttcacgagggctccacatacacagctgctgttcaatacaatgtcctagaaaaagacgatgatcctgcatcacttacaatatgggtgcccatgttccaatcatccatgccagcagatctactcataaaagaactagccaatgtcaatatactagtgaaacaaatatccacacccaagggaccctcattaagagtcatgataaactcaagaagtgcagtgctagcacaaatgcccagcaaatttaccatatgtgccaatgtgtccttggatgaaagaagcaagctggcatatgatgtaaccacaccctgtgaaattaaggcatgcagtctaacatgcctaaaatcaaaaaatatgttaactacagttaaagatctcactatgaaaacactcaacccaacacatgacatcattgctttatgtgaatttgaaaatatagtaacatcaaaaaaagtcataataccaacatacctaagatctatcagcgtcagaaataaagatctgaacacacttgaaaatataacaaccactgaattcaaaaatgccattacaaatgcaaaaatcatcccttactcaggattattgttagtcatcacagtgactgacaacaaaggagcattcaaatacataaagccacaaagtcaattcatagtagatcttggagcttacctagaaaaagaaagtatatattatgttacaacaaattggaagcacacagctacacgatttgcaatcaaacccatggaagattaacctttttcctctacatcaatgagtagattcatacaaactttctaactacattcttcacttcacaatcataatcaccaaccctctgtggttcaatcaatcaaacaaaactcatcaagagttccagatcatcccaagtcattgttcatcagatccagtactcaaataagttaataaaaaatccacatggggcaaataatcattgagggaaatccaactaatcacaacatctgtcaacatagacaagtcaacacgctagataaaatcaaccaatggaaaatacatccataactatagaattctcaagcaaattctggccttactttacactaatacacatgataacaacaataatctctttgataatcataatctccatcatgattgcaatactaaacaaactctgcgaatataatgtattccataacaaaacctttgagctaccaagagctcgagtcaatacatagcattcaccaatctgatagctcaaaacagtaaccttgcatttgtaaatgaactaccctcacttcttcacaaaaccacatcaacatctcaccatgcaagccatcatctataccataaagtagttaattaaaaatggccggccttgacagaagataaaaatggggcaaatgcaaacatgaagtgccttttgtacttagcctttttattcattggggtgaattgcaagttcaccatagtttttccacacaaccaaaaaggaaactggaaaaatgttccttctaattaccattattgcccgtcaagctcagatttaaattggcataatgacttaataggcacagccttacaagtcaaaatgcccaagagtcacaaggctattcaagcagacggttggatgtgtcatgcttccaaatgggtcactacttgtgatttccgctggtatggaccgaagtatataacacattccatccgatccttcactccatctgtagaacaatgcaaggaaagcattgaacaaacgaaacaaggaacttggctgaatccaggcttccctcctcaaagttgtggatatgcaactgtgacggatgccgaagcagtgattgtccaggtgactcctcaccatgtgctggttgatgaatacacaggagaatgggttgattcacagttcatcaacggaaaatgcagcaattacatatgccccactgtccataactctacaacctggcattctgactataaggtcaaagggctatgtgattctaacctcatttccatggacatcaccttcttctcagaggacggagagctatcatccctgggaaaggagggcacagggttcagaagtaactactttgcttatgaaactggaggcaaggcctgcaaaatgcaatactgcaagcattggggagtcagactcccatcaggtgtctggttcgagatggctgataaggatctctttgctgcagccagattccctgaatgcccagaagggtcaagtatctctgctccatctcagacctcagtggatgtaagtctaattcaggacgttgagaggatcttggattattccctctgccaagaaacctggagcaaaatcagagcgggtcttccaatctctccagtggatctcagctatcttgctcctaaaaacccaggaaccggtcctgctttcaccataatcaatggtaccctaaaatactttgagaccagatacatcagagtcgatattgctgctccaatcctctcaagaatggtcggaatgatcagtggaactaccacagaaagggaactgtgggatgactgggcaccatatgaagacgtggaaattggacccaatggagttctgaggaccagttcaggatataagtttcctttatacatgattggacatggtatgttggactccgatcttcatcttagctcaaaggctcaggtgttcgaacatcctcacattcaagacgctgcttcgcaacttcctgatgatgagagtttattttttggtgatactgggctatccaaaaatccaatcgagcttgtagaaggttggttcagtagttggaaaagctctattgcctcttttttctttatcatagggttaatcattggactattcttggttctccgagttggtatccatctttgcattaaagccagaagcacaccagtcacattaagtaaggatcaactgagtggtataaataatattgcatttagtaactaatagtcattaaaaagcggccggccagtcataacaatgaactaggatattaagaccaaaaacaacgctggggcaaatgcaaacatgtccaaaaccgaggaccaacgcaccgccaagacactagaaaggacctgggacacttttaatcatctattattcatatcatcgtgcttatacaagttaaatcttaaatctatagcacaaatcacattatctattttggcaattataatctcaacctcacttataattgcagccatcatattcatagcctcggcaaaccacaaagtcacactaacaactgcaatcatacaagatgcaacgaaccagatcaagaacacaaccccaacatacctcacccagaatccccagcatggaatcagcttctccaatctgtccggaactacatcacaatccaccaccatactagcttcaacaacaccaagtgctgattcaaccccacaatccacaacagtcaagatcaaaaacacaacaacaacccaaatattacctagcaaacccaccacaaaacaacgccaaaataaaccacaaaacaaacccaacaatgattttcactttgaagtgttcaattttgtaccctgcagcatatgcagcaacaatccaacctgctgggccatctgcaagagaataccaaacaaaaaacctggaaagaaaaccaccaccaagcccacaaaaaaaccaaccctcaagacaaccaaaaaagatcccaaatcccaaaccacaaaaccaaaggaagtactcactaccaagcctacaggaaagccaaccatcaacaccactaaaacaaacatcagaactacactgctcacctccaacaccaaaggaaatccagaacacacaagtcaagaggaaaccctccactcaaccacctccgaaggctatccaagcccatcacaagtccacacaacatccggtcaagaggaaaccctccactcaaccacctccgaaggctatccaagcccatcacaagtctacacaacatccgagtacctatcacaatctctatcttcatccaacacaacaaaatgatagtcattaaaaagcacgcgtgtattgttgcaaaaagccatgaccaaatcaaacagaatcaaaatcaactctggggcaaataacaatggagttgccaatcctcaaaacaaatgctattaccacaatccttgctgcagtcacactctgtttcgcttccagtcaaaacatcactgaagaattttatcaatcaacatgcagtgcagtcagcaaaggctatcttagtgctctaagaactggttggtatactagtgttataactatagaattaagtaatatcaaggaaaataagtgtaatggtacagacgctaaggtaaaattaataaaacaagaattagataaatataaaaatgctgtaacagaattgcagttgctcatgcaaagcacaccagcagccaacaatcgagccagaagagaactaccaagatttatgaattatacactcaacaataccaaaaacaccaatgtaacattaagtaagaaaaggaaaagaagatttcttggatttttgttaggtgttggatctgcaatcgccagtggcattgccgtatccaaggtcctgcacctagaaggggaagtgaacaaaatcaaaagtgctctactatccacaaacaaggctgtagtcagcttatctaatggagtcagtgtcttaaccagcaaggtgttagacctcaaaaactatatagataaacagttgttacctattgttaacaagcaaagctgcagcatatcaaacattgaaactgtgatagagttccaacaaaagaacaacagactactagagattaccagagaatttagtgttaatgcaggtgtaactactcctgtaagcacttatatgttaactaatagtgagttattatcattaatcaatgatatgcctataacaaatgatcagaaaaagttaatgtccagcaatgttcaaatagttagacagcaaagttactctatcatgtcaataataaaagaggaagtcttggcatatgtagtacaattaccactatatggtgtaatagatactccttgttggaaactacacacatcccctttatgtacaaccaacacaaaggaaggatccaacatctgcttaacaagaaccgacagaggatggtactgtgacaatgcaggatcagtatcctttttcccacaagctgaaacatgtaaagttcaatcgaatcgggtgttttgtgacacaatgaacagtttaacattaccaagtgaggtaaatctctgcaacattgacatattcaaccccaaatatgattgcaaaattatgacttcaaaaacagatgtaagcagctccgttatcacatctctaggagccattgtgtcatgctatggcaaaaccaaatgtacagcatccaataaaaatcgtgggatcataaagacattctctaacgggtgtgattatgtatcaaataagggggtggatactgtgtctgtaggtaatacattatattatgtaaataagcaagaaggcaaaagtctctatgtaaaaggtgaaccaataataaatttctatgatccattagtgttcccctctgatgaatttgatgcatcaatatctcaagtcaatgagaaaattaatcagagtctagcatttatccgtaaatcagatgaattattacataatgtaaatgctggtaaatccaccacaaatatcatgataactaccataattatagtaattatagtaatattgttagcattaattgcagttggactgcttctatactgcaaggccagaagcacaccagtcacattaagtaaggatcaactgagtggtataaataatattgcatttagtaactgaataaaaatagcacctaatcatattcttacaatggttcgctatttgaccatagataacccatctatcattagattatcctaaaatttgaacttcatcacaactttcatctataaaccatctcacttacactttttaagtagatttctattttatagttatataaaacagggcccattgaataccaaattaacttactatttgtaaaaatgagaattggggcaaatatgtcacgaaggaatccttgcaaattcgaaattcgaggtcattgcttgaatggtaaaaggtgtcattttagtcataattattttgaatggccaccccatgcactgcttgtaagacaaaactttatgttaaacagaatacttaagtctatggataaaagcatagatactttgtcagaaataagtggagctgcagagttggacagaacagaagagtatgccctcggtgtagttggagtgctagagagttatataggatcaataaataatataactaaacaatcagcatgtgttgccatgagcaaactccttactgaactcaacagcgatgacatcaaaaaactaagggacaatgaagagccaaactcacccaaagtaagagtgtacaatactgtcatatcatatattgaaagcaacaggaagaacaataaacaaactatccatctgttaaaaagattgccagcagacgtattgaagaaaaccatcaaaaacacattggatatccacaagagcataaccatcaataacccaaaagaatcaactgttagtgatacgaacgaccatgccaaaaataatgatactacctgacaaatatccttgtagtataaattccatactaataacaagtaattgtagagtcactatgtataatcaaaaaaacacactatatatcaatcaaaacaaccaaaatagccatatatacccaccggatcaaccattcaatgaaatccattggacctctcaagacttgattgatgcaactcaaaattttctacaacatctaggtattactgatgatatatacacaatatatatattagtgtcataatactcaatcctaatacttaccacatcatcaaattattaactcaaacaattcaagctatgggacaaaatggatcccattattagtggaaattctgctaatgtttatctaactgatagttatttaaaaggtgttatttctttctcagaatgtaacgctttaggaagttacatattcaatggtccttatctcaaaaatgattataccaacttaattagtagacaaaatccattaatagaacacataaatctaaagaaactaaatataacacagtccttaatatctaagtatcataaaggtgaaataaaaatagaagaacctacttactttcagtcattacttatgacatacaagagtatgacctcttcagaacagactactactactaatttacttaaaaagataataagaagagctatagaaatcagtgatgtcaaagtctatgctatattgaataaactggggctcaaagaaaaagacaagattaaatccaataatggacaagatgaagacaactcagtcattactaccataatcaaagatgatatacttttagctgtcaaggataatcaatctcatcttaaagcagacaaaaatcaatccacaaaacaaaaagatacaatcaaaacaacacttttgaagaaattaatgtgttcgatgcaacatcctccatcatggttaatacattggtttaatttatacacaaaattaaacagcatattaacacaatatcgatctagtgaggtaaaaaaccatggttttatattgatagataatcatactcttagtggattccaatttattttgaatcaatatggttgtatagtttatcataaggaactcaaaagaattactgtgacaacttataatcaattcttgacatggaaagatattagccttagtagattaaatgtttgtttgattacatggattagtaactgtttgaacacattaaacaaaagcttaggcttaagatgtggattcaataatgttatcttgacacaattattcctttatggagattgtatactaaaactattccacaatgaggggttctacataataaaagaggtagagggatttattatgtctctaattttaaatataacagaagaagatcaattcagaaaacggttttataatagtatgctcaacaacatcacagatgccgccaacaaagctcaaaaaaatctgctatcaagagtatgtcatacattattagataagacaatatcagataatataataaatggcagatggataattctattgagtaagttcctaaaattaattaagcttgcaggtgacaataacctcaacaatctgagtgaattatattttttgttcagaatatttggacacccaatggtagatgaaagacaagccatggatgctgttaaagttaattgcaacgagaccaaattttatttgttaagtagtttgagtatgttaagaggagcttttatatatagaattataaaagggtttgtaaataattacaacagatggcctactttaagaaatgccattgtcttacccttaagatggttaacttactataaactaaacacttatccttccttgttggaacttacagaaagagatttgattgttctatcaggactacgtttctatcgagagtttcggttgcctaaaaaagtggatcttgaaatgatcataaatgataaggctatatcacctcctaaaaatttaatatggactagtttccctagaaattatatgccgtcacacatacaaaattatatagaacatgaaaaattaaaattctctgatagtgataaatcaagaagagtattagagtattatttaagagataacaaattcaatgaatgtgatttacacaactgtgtagttaatcaaagttatcttaacaacccgaatcatgtggtatcattgacaggcaaagaaagagaactcagtgtaggtagaatgtttgcaatgcaaccaggaatgttcagacaagttcaaatattagcagagaaaatgatagcagaaaacatattacaatttttccctgaaagtcttacaagatatggtgatctagaactacagaaaatattagaattgaaagcaggaataagtaacaaatcaaatcgttacaatgataattacaacaattacattagtaagtgctctatcatcacagatctcagcaaattcaatcaagcatttcgatatgaaacatcatgtatttgtagtgatgtactggatgaactgcatggtgtacaatctctattttcctggttacatttaactattcctcatgtcacaataatatgcacatataggcatgcacccccctatataaaggatcatattgtagatcttaacaatgtagatgagcaaagtggactatatagatatcatatgggtggtatcgaagggtggtgtcaaaaactatggaccatagaagctatatcactattagatctaatatctctcaaagggaaattctcaattactgctttaattaatggtgacaatcaatcaatagatataagtaaaccagtcagactcatggaaggtcaaactcatgctcaagcagattatttgctagcattaaatagtctcaaattactgtataaagagtatgcaggaataggccacaaattaaaaggaactgagacttatatatcgagagatatgcaatttatgagtaaaacgatccaacataacggtgtatattacccagctagtataaagaaagtcctaagagtgggaccgtggataaacactatacttgatgacttcaaagtgagtctagaatctataggtagtttgacacaagaattagaatatagaggtgaaagtctattatgcagtttaatatttagaaatgtatggttatataatcaaattgcattacaacttaaaaatcatgcattatgtaacaacaaattatatttggatatattaaaagttctaaaacacttaaaaaccttttttaatcttgataacattgatacagcattaacattgtatatgaatttgcccatgttatttggtggtggtgatcccaacttgttatatcgaagtttctatagaagaactcctgatttcctcacagaggctatagttcactctgtgttcatacttagttattatacaaaccatgatttaaaagataaacttcaagatctgtcagatgatagattgaataagttcttaacatgcataatcacgtttgataaaaaccccaatgctgaattcgttacattgatgagagatcctcaagctttaggatctgagaggcaagctaaaattactagcgaaatcaatagactggcagttaccgaggttttgagcacagctccaaacaaaatattttccaaaagtgcacaacactataccactacagagatagatcttaatgatattatgcaaaatatagaacctacatatcctcacgggctaagagttgtttatgagagtttacccttttataaagcagagaaaatagtaaatcttatatccggtacaaaatctataactaacatactggaaaagacttctgccatagacttaacagatattgatagagccactgagatgatgaggaaaaacataactttgcttataaggatattaccattagattgtaacagagataaaagagaaatattgagtatggaaaacctaagtattactgaattaagcaaatacgttagagaaagatcttggtctttatccaatatagttggtgttacatcacccagtatcatgtatacaatggacataaaatatacaacaagcactatagctagtggcataatcatagagaaatataatgtcaacagtttaacacgtggtgagagaggacccactaaaccatgggttggttcatctacacaagagaaaaagacaatgccagtttataatagacaagttttaaccaaaaaacagagagatcaaatagatctattagcaaaattggattgggtgtatgcatctatagataacaaggatgaatttatggaggaacttagcataggaactcttgggttaacatatgagaaggccaaaaaattattcccacaatatttgagtgttaactatttgcatcgtcttacagtcagtagtagaccatgtgaattccctgcatctataccagcttatagaactacaaattatcactttgatactagccctattaatcgcatattaacagaaaagtatggtgatgaagatattgatatagtattccaaaactgtataagctttggccttagcttaatgtctgtagtagaacaatttactaatgtatgtcctaacagaattattctcatacccaagcttaatgagatacatttgatgaaacctcccatattcacaggcgatgttgatattcacaagttaaaacaagtgatacaaaaacaacatatgtttttaccagacaaaataagtttgactcaatatgtggaattattcttaagtaataaaacactcaaatctggatctaatgttaattctaatttaatattggcgcataagatatctgactattttcataatacttacattttgagtactaatttagctggacattggattcttattatacaacttatgaaagattctaagggtatttttgaaaaagattggggagagggatatataactgatcatatgttcattaatttgaaagttttcttcaatgcttataagacatatctcttgtgttttcataaaggttacggcagagcaaagctggagtgtgatatgaatacttcagatctcctatgtgtattggaattaatagacagtagttattggaagtctatgtctaaggtgtttttagaacaaaaagttatcaaatacattcttagccaggatgcaagtttacatagagtaaaaggatgtcatagcttcaaactatggtttcttaaacgtcttaatgtagcagaattcacagtttgcccttgggttgttaacatagattatcatccaacacatatgaaagcaatattaacttatattgatcttgttagaatgggattgataaatatagatagaatatacattaaaaataaacacaagttcaatgatgagttttatacttctaatctgttttacattaattataacttctcagataatactcatctattaactaaacatataaggattgctaattccgaattagaaagtaattacaacaaattatatcatcctacaccagaaaccctagaaaatatactaaccaatccggttaaaagtaatgagaaaaagacactgagtgactattgtataggtaaaaatgttgactcaataatgttaccatcgttatctaataagaagcttattaaatcgtctacaatgattagaaccaattacagcagacaagatttgtataatttatttcctacggttgtgattgataaaattatagatcattcaggtaatacagccaaatctaaccaactttacactactacttctcatcaaatatccttagtgcacaatagcacatcactttattgcatgcttccttggcatcatattaatagattcaattttgtatttagttctacaggttgtaaaattagtatagagtatattttaaaagatcttaaaattaaggatcctaattgtatagcattcataggtgaaggagcagggaatttattattgcgtacagtagtggaacttcatcctgatataagatatatttacagaagtctgaaagattgcaatgatcatagtttaccaattgagtttttaaggctgtacaatggacatatcaacattgattatggtgaaaatttgaccattcctgctacagatgcaaccaacaacattcattggtcttatttacatataaagtttgctgaacctatcagtctttttgtctgtgatgctgaattgcctgtaacagtcaactggagtaagattataatagagtggagcaagcatgtaagaaaatgcaagtactgttcttcagttaataaatgtacattgatagtaaaatatcatgctcaagatgatatcgatttcaaattagacaacataactatattaaaaacttatgtatgcttaggtagtaagttaaagggatctgaagtttacttagtccttacaataggtcctgcaaatgtgttcccagtatttaatgtagtacaaaatgctaaattgatactatcaagaactaaaaatttcatcatgcctaaaaaagctgataaagagtctattgatgcaaatattaagagtttgataccctttctttgttaccctataacaaaaaaaggaattaatactgcattgtctaaattaaagagtgttgttagtggagatatactatcatattctatagctggacgtaatgaagttttcagcaataaacttataaatcataagcatatgaacatcttaaagtggttcaatcatgttttaaatttcagatcaacagaattaaactataatcatttatatatggtagaatctacttatcctcatctaagtgaattgttaaacagcttgacaaccaatgaacttaaaaaactgattaaaatcacaggtagtttgttatacaacttttataatgaataatgagcaaaaatcttataacaaaaatagctacacactaacattgtattcaattatagttattgaaaattaataattatataatttttaataacttctagtgaactaatcctaaaattatcattttgatctaggaagaataagtttaaatccaaatctaattggtttatatgtatattaactaaattacgagatattagtttttgacactttttttctcgtggccggcatggtcccagcctcctcgctggcgccggctgggcaacatgcttcggcatggcgaatgggactagcataaccccttggggcctctaaacgggtcttgaggggttttttg

SEQ ID NO: 18 - DNA, 16677 bp, synthetic construct
  misc_feature 1..16677: note = antigenic cDNA encoding cRSVA_VSVG_A_SH deletion
  source 1..16677: mol_type = other DNA
taatacgactcactataggttttttcgcgtctgatgaggccgttaggccgaaactcctctccggagtcacgcgaaaaaatgcgtacaacaaacttgcgtaaaccaaaaaaatggggcaaataagaatttgataagtaccacttaaatttaactcctttggttagaggcgcgccatgggcagcaactcattgagtatgataaaagttagattgcaaaatctgtttgacaatgatgaagtagcattgttaaaaataacatgctatactgacaaattaatacagttaactaatgctttggctaaggcagttatacatacaatcaaattgaatggcattgtatttgtgcatgttattacaagtagtgatatttgccctaataataatattgtagtgaaatccaatttcacaacaatgccagtattacaaaatggaggttatatatgggaaatgatggaattaacacactgctctcaacctaatggcctaatagatgacaattgtgaaattaaattctccaaaaaactaagtgattcaacaatgaccaattatatgaatcaattatctgaattacttggatttgacctcaatccataaatcataataaatatcaactagcaaatcaatgtcactaacaccattagttaatataaaacttgacagaagataaaaatggggcaaataaatcaattcagccgacccaaccatggacacaacacacaatgataccacaccacaaagactgatgatcacagacatgaggccattatcgcttgagactataataacatctctaaccagagatatcataacacataaatttatatacttgataaatcatgaatgcatagtaagaaaacttgatgaaagacaggccacatttacatttctggtcaactatgaaatgaaactattgcacaaagtgggaagcactaaatataaaaaatatactgaatacaacacaaaatatggcactttccctatgccaatatttatcaatcatgatgggttcttagaatgcattggcattaagcctaccaagcacacacccataatatacaagtatgatctcaatccatgaatatcaaaccaagattcaaacaatccgaaataacaactttatgcataatcacactccatagtccaaatggagcctgaaaattatagttatttaaaattcctgcaggaaggagagacataagatgaaagatggggcaaatacaaaaatggctcttagcaaagtcaagttgaatgatacactcaacaaagatcaacttctatcatccagcaaatataccatccaacggagcacaggagacagcattgacactcctaattatgatgtgcagaaacacattaataagttatgtggcatgttattaatcacagaagatgctaatcataaattcactgggttaataggtatgttatatgctatgtctagattaggaagagaagacaccataaaaatactcaaagatgcgggatatcatgttaaggcaaatggagtggatgtaacaacacatcgtcaagacattaatgggaaagaaatgaaatttgaagtgttaacattagcaagcttaacaactgaaattcaaatcaacattgagatagaatctagaaaatcctacaaaaaaatgctaaaagaaatgggagaggtggctccagaatacaggcatgactctcctgattgtgggatgataatattatgtatagcggcattagtaataaccaaattagcagcaggagatagatcaggtcttacagctgtgattaggagagctaataatgtcctaaaaaatgaaatgaaacgttataaaggtttattacccaaggatatagccaacagcttctatgaagtgtttgaaaaatatcctcactttatagatgtttttgttcattttggtatagcacaatcttctaccagaggtggcagtagagttgaagggatttttgcaggattgtttatgaatgcctatggtgcagggcaagtgatgttacggtggggggtcttagcaaaatcagttaaaaacattatgttaggacacgctagtgtacaagcagaaatggaacaagttgtggaggtgtatgagtatgctcagaaattgggtggagaagcaggattctaccatatattgaacaacccaaaagcatcactattatctttgactcaatttcctcacttctctagtgtagtattgggcaatgctgctggcctaggcataatgggagaatacagaggtacaccaaggaatcaagatttatatgatgctgcaaaagcatatgctgaacaactcaaagaaaatggtgtgattaactacagtgtattagatttgacagcagaagaactagaggctatcaaacatcagcttaatccaaaagataatgatgtagagctttgagttaataaaaaagtggggcaaataaatcatcatggaaaagtttgctcctgaattccatggagaagatgcaaacaacagagccaccaaattcctagaatcaataaagggcaaattcacatcacccaaagatcccaagaaaaaagatagtatcatatctgtcaactcaatagatatagaagtaaccaaagaaagccctataacatcaaattcaaccattataaacccaataaatgagacagatgatactgtagggaacaagcccaattatcaaagaaagcctctagtaagtttcaaagaagaccctacgccaagtgataatcctttttcaaaactatacaaagaaaccatagaaacatttgataacaatgaagaagaatctagctattcatatgaagaaataaatgatcagacaaacgataatataacagcaagattagataggattgatgagaaattaagtgaaatactaggaatgcttcacacattagtagtagcgagtgcaggacccacatctgctcgggatggtataagagatgccatggttggtttaagagaagaaatgatagaaaaaatcagaactgaagcattaatgaccaatgacagactagaagctatggcaagactcaggaatgaagaaagtgaaaagatggcaaaagacacatcagatgaagtgtctctcaatccaacatcagagaaactgaacaacctgttggaagggaatgatagtgacaatgatctatcacttgaagatttctgattagctaccaaactgtacatcaaaacacaacaccaatagaaaaccaacaaacaaaccaactcacccatccaaccaaacatctatctgctgattagccaaccagccaaaaaacaaccagccaatctaaaactagccacccggaaaaaatcgatactatagttacaaaaaaagatggggcaaatatggaaacatacgtgaataaacttcacgagggctccacatacacagctgctgttcaatacaatgtcctagaaaaagacgatgatcctgcatcacttacaatatgggtgcccatgttccaatcatccatgccagcagatctactcataaaagaactagccaatgtcaatatactagtgaaacaaatatccacacccaagggaccctcattaagagtcatgataaactcaagaagtgcagtgctagcacaaatgcccagcaaatttaccatatgtgccaatgtgtccttggatgaaagaagcaagctggcatatgatgtaaccacaccctgtgaaattaaggcatgcagtctaacatgcctaaaatcaaaaaatatgttaactacagttaaagatctcactatgaaaacactcaacccaacacatgacatcattgctttatgtgaatttgaaaatatagtaacatcaaaaaaagtcataataccaacatacctaagatctatcagcgtcagaaataaagatctgaacacacttgaaaatataacaaccactgaattcaaaaatgccattacaaatgcaaaaatcatcccttactcaggattattgttagtcatcacagtgactgacaacaaaggagcattcaaatacataaagccacaaagtcaattcatagtagatcttggagcttacctagaaaaagaaagtatatattatgttacaacaaattggaagcacacagctacacgatttgcaatcaaacccatggaagattaacctttttcctctacatcaatgagtagattcatacaaactttctaactacattcttcacttcacaatcataatcaccaaccctctgtggttcaatcaatcaaacaaaactcatcaagagttccagatcatcccaagtcattgttcatcagatccagtactcaaataagttaataaaaaatcggtccgttgacagaagataaaaatggggcaaatgcaaacatgaagtgccttttgtacttagcctttttattcattggggtgaattgcaagttcaccatagtttttccacacaaccaaaaaggaaactggaaaaatgttccttctaattaccattattgcccgtcaagctcagatttaaattggcataatgacttaataggcacagccttacaagtcaaaatgcccaagagtcacaaggctattcaagcagacggttggatgtgtcatgcttccaaatgggtcactacttgtgatttccgctggtatggaccgaagtatataacacattccatccgatccttcactccatctgtagaacaatgcaaggaaagcattgaacaaacgaaacaaggaacttggctgaatccaggcttccctcctcaaagttgtggatatgcaactgtgacggatgccgaagcagtgattgtccaggtgactcctcaccatgtgctggttgatgaatacacaggagaatgggttgattcacagttcatcaacggaaaatgcagcaattacatatgccccactgtccataactctacaacctggcattctgactataaggtcaaagggctatgtgattctaacctcatttccatggacatcaccttcttctcagaggacggagagctatcatccctgggaaaggagggcacagggttcagaagtaactactttgcttatgaaactggaggcaaggcctgcaaaatgcaatactgcaagcattggggagtcagactcccatcaggtgtctggttcgagatggctgataaggatctctttgctgcagccagattccctgaatgcccagaagggtcaagtatctctgctccatctcagacctcagtggatgtaagtctaattcaggacgttgagaggatcttggattattccctctgccaagaaacctggagcaaaatcagagcgggtcttccaatctctccagtggatctcagctatcttgctcctaaaaacccaggaaccggtcctgctttcaccataatcaatggtaccctaaaatactttgagaccagatacatcagagtcgatattgctgctccaatcctctcaagaatggtcggaatgatcagtggaactaccacagaaagggaactgtgggatgactgggcaccatatgaagacgtggaaattggacccaatggagttctgaggaccagttcaggatataagtttcctttatacatgattggacatggtatgttggactccgatcttcatcttagctcaaaggctcaggtgttcgaacatcctcacattcaagacgctgcttcgcaacttcctgatgatgagagtttattttttggtgatactgggctatccaaaaatccaatcgagcttgtagaaggttggttcagtagttggaaaagctctattgcctcttttttctttatcatagggttaatcattggactattcttggttctccgagttggtatccatctttgcattaaagccagaagcacaccagtcacattaagtaaggatcaactgagtggtataaataatattgcatttagtaactaatagtcattaaaaagcggccggccagtcataacaatgaactaggatattaagaccaaaaacaacgctggggcaaatgcaaacatgtccaaaaccgaggaccaacgcaccgccaagacactagaaaggacctgggacacttttaatcatctattattcatatcatcgtgcttatacaagttaaatcttaaatctatagcacaaatcacattatctattttggcaattataatctcaacctcacttataattgcagccatcatattcatagcctcggcaaaccacaaagtcacactaacaactgcaatcatacaagatgcaacgaaccagatcaagaacacaaccccaacatacctcacccagaatccccagcatggaatcagcttctccaatctgtccggaactacatcacaatccaccaccatactagcttcaacaacaccaagtgctgattcaaccccacaatccacaacagtcaagatcaaaaacacaacaacaacccaaatattacctagcaaacccaccacaaaacaacgccaaaataaaccacaaaacaaacccaacaatgattttcactttgaagtgttcaattttgtaccctgcagcatatgcagcaacaatccaacctgctgggccatctgcaagagaataccaaacaaaaaacctggaaagaaaaccaccaccaagcccacaaaaaaaccaaccctcaagacaaccaaaaaagatcccaaatcccaaaccacaaaaccaaaggaagtactcactaccaagcctacaggaaagccaaccatcaacaccactaaaacaaacatcagaactacactgctcacctccaacaccaaaggaaatccagaacacacaagtcaagaggaaaccctccactcaaccacctccgaaggctatccaagcccatcacaagtccacacaacatccggtcaagaggaaaccctccactcaaccacctccgaaggctatccaagcccatcacaagtctacacaacatccgagtacctatcacaatctctatcttcatccaacacaacaaaatgatagtcattaaaaagcacgcgtgtattgttgcaaaaagccatgaccaaatcaaacagaatcaaaatcaactctggggcaaataacaatggagttgccaatcctcaaaacaaatgctattaccacaatccttgctgcagtcacactctgtttcgcttccagtcaaaacatcactgaagaattttatcaatcaacatgcagtgcagtcagcaaaggctatcttagtgctctaagaactggttggtatactagtgttataactatagaattaagtaatatcaaggaaaataagtgtaatggtacagacgctaaggtaaaattaataaaacaagaattagataaatataaaaatgctgtaacagaattgcagttgctcatgcaaagcacaccagcagccaacaatcgagccagaagagaactaccaagatttatgaattatacactcaacaataccaaaaacaccaatgtaacattaagtaagaaaaggaaaagaagatttcttggatttttgttaggtgttggatctgcaatcgccagtggcattgccgtatccaaggtcctgcacctagaaggggaagtgaacaaaatcaaaagtgctctactatccacaaacaaggctgtagtcagcttatctaatggagtcagtgtcttaaccagcaaggtgttagacctcaaaaactatatagataaacagttgttacctattgttaacaagcaaagctgcagcatatcaaacattgaaactgtgatagagttccaacaaaagaacaacagactactagagattaccagagaatttagtgttaatgcaggtgtaactactcctgtaagcacttatatgttaactaatagtgagttattatcattaatcaatgatatgcctataacaaatgatcagaaaaagttaatgtccagcaatgttcaaatagttagacagcaaagttactctatcatgtcaataataaaagaggaagtcttggcatatgtagtacaattaccactatatggtgtaatagatactccttgttggaaactacacacatcccctttatgtacaaccaacacaaaggaaggatccaacatctgcttaacaagaaccgacagaggatggtactgtgacaatgcaggatcagtatcctttttcccacaagctgaaacatgtaaagttcaatcgaatcgggtgttttgtgacacaatgaacagtttaacattaccaagtgaggtaaatctctgcaacattgacatattcaaccccaaatatgattgcaaaattatgacttcaaaaacagatgtaagcagctccgttatcacatctctaggagccattgtgtcatgctatggcaaaaccaaatgtacagcatccaataaaaatcgtgggatcataaagacattctctaacgggtgtgattatgtatcaaataagggggtggatactgtgtctgtaggtaatacattatattatgtaaataagcaagaaggcaaaagtctctatgtaaaaggtgaaccaataataaatttctatgatccattagtgttcccctctgatgaatttgatgcatcaatatctcaagtcaatgagaaaattaatcagagtctagcatttatccgtaaatcagatgaattattacataatgtaaatgctggtaaatccaccacaaatatcatgataactaccataattatagtaattatagtaatattgttagcattaattgcagttggactgcttctatactgcaaggccagaagcacaccagtcacattaagtaaggatcaactgagtggtataaataatattgcatttagtaactgaataaaaatagcacctaatcatattcttacaatggttcgctatttgaccatagataacccatctatcattagattatcctaaaatttgaacttcatcacaactttcatctataaaccatctcacttacactttttaagtagatttctattttatagttatataaaacagggcccattgaataccaaattaacttactatttgtaaaaatgagaattggggcaaatatgtcacgaaggaatccttgcaaattcgaaattcgaggtcattgcttgaatggtaaaaggtgtcattttagtcataattattttgaatggccaccccatgcactgcttgtaagacaaaactttatgttaaacagaatacttaagtctatggataaaagcatagatactttgtcagaaataagtggagctgcagagttggacagaacagaagagtatgccctcggtgtagttggagtgctagagagttatataggatcaataaataatataactaaacaatcagcatgtgttgccatgagcaaactccttactgaactcaacagcgatgacatcaaaaaactaagggacaatgaagagccaaactcacccaaagtaagagtgtacaatactgtcatatcatatattgaaagcaacaggaagaacaataaacaaactatccatctgttaaaaagattgccagcagacgtattgaagaaaaccatcaaaaacacattggatatccacaagagcataaccatcaataacccaaaagaatcaactgttagtgatacgaacgaccatgccaaaaataatgatactacctgacaaatatccttgtagtataaattccatactaataacaagtaattgtagagtcactatgtataatcaaaaaaacacactatatatcaatcaaaacaaccaaaatagccatatatacccaccggatcaaccattcaatgaaatccattggacctctcaagacttgattgatgcaactcaaaattttctacaacatctaggtattactgatgatatatacacaatatatatattagtgtcataatactcaatcctaatacttaccacatcatcaaattattaactcaaacaattcaagctatgggacaaaatggatcccattattagtggaaattctgctaatgtttatctaactgatagttatttaaaaggtgttatttctttctcagaatgtaacgctttaggaagttacatattcaatggtccttatctcaaaaatgattataccaacttaattagtagacaaaatccattaatagaacacataaatctaaagaaactaaatataacacagtccttaatatctaagtatcataaaggtgaaataaaaatagaagaacctacttactttcagtcattacttatgacatacaagagtatgacctcttcagaacagactactactactaatttacttaaaaagataataagaagagctatagaaatcagtgatgtcaaagtctatgctatattgaataaactggggctcaaagaaaaagacaagattaaatccaataatggacaagatgaagacaactcagtcattactaccataatcaaagatgatatacttttagctgtcaaggataatcaatctcatcttaaagcagacaaaaatcaatccacaaaacaaaaagatacaatcaaaacaacacttttgaagaaattaatgtgttcgatgcaacatcctccatcatggttaatacattggtttaatttatacacaaaattaaacagcatattaacacaatatcgatctagtgaggtaaaaaaccatggttttatattgatagataatcatactcttagtggattccaatttattttgaatcaatatggttgtatagtttatcataaggaactcaaaagaattactgtgacaacttataatcaattcttgacatggaaagatattagccttagtagattaaatgtttgtttgattacatggattagtaactgtttgaacacattaaacaaaagcttaggcttaagatgtggattcaataatgttatcttgacacaattattcctttatggagattgtatactaaaactattccacaatgaggggttctacataataaaagaggtagagggatttattatgtctctaattttaaatataacagaagaagatcaattcagaaaacggttttataatagtatgctcaacaacatcacagatgccgccaacaaagctcaaaaaaatctgctatcaagagtatgtcatacattattagataagacaatatcagataatataataaatggcagatggataattctattgagtaagttcctaaaattaattaagcttgcaggtgacaataacctcaacaatctgagtgaattatattttttgttcagaatatttggacacccaatggtagatgaaagacaagccatggatgctgttaaagttaattgcaacgagaccaaattttatttgttaagtagtttgagtatgttaagaggagcttttatatatagaattataaaagggtttgtaaataattacaacagatggcctactttaagaaatgccattgtcttacccttaagatggttaacttactataaactaaacacttatccttccttgttggaacttacagaaagagatttgattgttctatcaggactacgtttctatcgagagtttcggttgcctaaaaaagtggatcttgaaatgatcataaatgataaggctatatcacctcctaaaaatttaatatggactagtttccctagaaattatatgccgtcacacatacaaaattatatagaacatgaaaaattaaaattctctgatagtgataaatcaagaagagtattagagtattatttaagagataacaaattcaatgaatgtgatttacacaactgtgtagttaatcaaagttatcttaacaacccgaatcatgtggtatcattgacaggcaaagaaagagaactcagtgtaggtagaatgtttgcaatgcaaccaggaatgttcagacaagttcaaatattagcagagaaaatgatagcagaaaacatattacaatttttccctgaaagtcttacaagatatggtgatctagaactacagaaaatattagaattgaaagcaggaataagtaacaaatcaaatcgttacaatgataattacaacaattacattagtaagtgctctatcatcacagatctcagcaaattcaatcaagcatttcgatatgaaacatcatgtatttgtagtgatgtactggatgaactgcatggtgtacaatctctattttcctggttacatttaactattcctcatgtcacaataatatgcacatataggcatgcacccccctatataaaggatcatattgtagatcttaacaatgtagatgagcaaagtggactatatagatatcatatgggtggtatcgaagggtggtgtcaaaaactatggaccatagaagctatatcactattagatctaatatctctcaaagggaaattctcaattactgctttaattaatggtgacaatcaatcaatagatataagtaaaccagtcagactcatggaaggtcaaactcatgctcaagcagattatttgctagcattaaatagtctcaaattactgtataaagagtatgcaggaataggccacaaattaaaaggaactgagacttatatatcgagagatatgcaatttatgagtaaaacgatccaacataacggtgtatattacccagctagtataaagaaagtcctaagagtgggaccgtggataaacactatacttgatgacttcaaagtgagtctagaatctataggtagtttgacacaagaattagaatatagaggtgaaagtctattatgcagtttaatatttagaaatgtatggttatataatcaaattgcattacaacttaaaaatcatgcattatgtaacaacaaattatatttggatatattaaaagttctaaaacacttaaaaaccttttttaatcttgataacattgatacagcattaacattgtatatgaatttgcccatgttatttggtggtggtgatcccaacttgttatatcgaagtttctatagaagaactcctgatttcctcacagaggctatagttcactctgtgttcatacttagttattatacaaaccatgatttaaaagataaacttcaagatctgtcagatgatagattgaataagttcttaacatgcataatcacgtttgataaaaaccccaatgctgaattcgttacattgatgagagatcctcaagctttaggatctgagaggcaagctaaaattactagcgaaatcaatagactggcagttaccgaggttttgagcacagctccaaacaaaatattttccaaaagtgcacaacactataccactacagagatagatcttaatgatattatgcaaaatatagaacctacatatcctcacgggctaagagttgtttatgagagtttacccttttataaagcagagaaaatagtaaatcttatatccggtacaaaatctataactaacatactggaaaagacttctgccatagacttaacagatattgatagagccactgagatgatgaggaaaaacataactttgcttataaggatattaccattagattgtaacagagataaaagagaaatattgagtatggaaaacctaagtattactgaattaagcaaatacgttagagaaagatcttggtctttatccaatatagttggtgttacatcacccagtatcatgtatacaatggacataaaatatacaacaagcactatagctagtggcataatcatagagaaatataatgtcaacagtttaacacgtggtgagagaggacccactaaaccatgggttggttcatctacacaagagaaaaagacaatgccagtttataatagacaagttttaaccaaaaaacagagagatcaaatagatctattagcaaaattggattgggtgtatgcatctatagataacaaggatgaatttatggaggaacttagcataggaactcttgggttaacatatgagaaggccaaaaaattattcccacaatatttgagtgttaactatttgcatcgtcttacagtcagtagtagaccatgtgaattccctgcatctataccagcttatagaactacaaattatcactttgatactagccctattaatcgcatattaacagaaaagtatggtgatgaagatattgatatagtattccaaaactgtataagctttggccttagcttaatgtctgtagtagaacaatttactaatgtatgtcctaacagaattattctcatacccaagcttaatgagatacatttgatgaaacctcccatattcacaggcgatgttgatattcacaagttaaaacaagtgatacaaaaacaacatatgtttttaccagacaaaataagtttgactcaatatgtggaattattcttaagtaataaaacactcaaatctggatctaatgttaattctaatttaatattggcgcataagatatctgactattttcataatacttacattttgagtactaatttagctggacattggattcttattatacaacttatgaaagattctaagggtatttttgaaaaagattggggagagggatatataactgatcatatgttcattaatttgaaagttttcttcaatgcttataagacatatctcttgtgttttcataaaggttacggcagagcaaagctggagtgtgatatgaatacttcagatctcctatgtgtattggaattaatagacagtagttattggaagtctatgtctaaggtgtttttagaacaaaaagttatcaaatacattcttagccaggatgcaagtttacatagagtaaaaggatgtcatagcttcaaactatggtttcttaaacgtcttaatgtagcagaattcacagtttgcccttgggttgttaacatagattatcatccaacacatatgaaagcaatattaacttatattgatcttgttagaatgggattgataaatatagatagaatatacattaaaaataaacacaagttcaatgatgagttttatacttctaatctgttttacattaattataacttctcagataatactcatctattaactaaacatataaggattgctaattccgaattagaaagtaattacaacaaattatatcatcctacaccagaaaccctagaaaatatactaaccaatccggttaaaagtaatgagaaaaagacactgagtgactattgtataggtaaaaatgttgactcaataatgttaccatcgttatctaataagaagcttattaaatcgtctacaatgattagaaccaattacagcagacaagatttgtataatttatttcctacggttgtgattgataaaattatagatcattcaggtaatacagccaaatctaaccaactttacactactacttctcatcaaatatccttagtgcacaatagcacatcactttattgcatgcttccttggcatcatattaatagattcaattttgtatttagttctacaggttgtaaaattagtatagagtatattttaaaagatcttaaaattaaggatcctaattgtatagcattcataggtgaaggagcagggaatttattattgcgtacagtagtggaacttcatcctgatataagatatatttacagaagtctgaaagattgcaatgatcatagtttaccaattgagtttttaaggctgtacaatggacatatcaacattgattatggtgaaaatttgaccattcctgctacagatgcaaccaacaacattcattggtcttatttacatataaagtttgctgaacctatcagtctttttgtctgtgatgctgaattgcctgtaacagtcaactggagtaagattataatagagtggagcaagcatgtaagaaaatgcaagtactgttcttcagttaataaatgtacattgatagtaaaatatcatgctcaagatgatatcgatttcaaattagacaacataactatattaaaaacttatgtatgcttaggtagtaagttaaagggatctgaagtttacttagtccttacaataggtcctgcaaatgtgttcccagtatttaatgtagtacaaaatgctaaattgatactatcaagaactaaaaatttcatcatgcctaaaaaagctgataaagagtctattgatgcaaatattaagagtttgataccctttctttgttaccctataacaaaaaaaggaattaatactgcattgtctaaattaaagagtgttgttagtggagatatactatcatattctatagctggacgtaatgaagttttcagcaataaacttataaatcataagcatatgaacatcttaaagtggttcaatcatgttttaaatttcagatcaacagaattaaactataatcatttatatatggtagaatctacttatcctcatctaagtgaattgttaaacagcttgacaaccaatgaacttaaaaaactgattaaaatcacaggtagtttgttatacaacttttataatgaataatgagcaaaaatcttataacaaaaatagctacacactaacattgtattcaattatagttattgaaaattaataattatataatttttaataacttctagtgaactaatcctaaaattatcattttgatctaggaagaataagtttaaatccaaatctaattggtttatatgtatattaactaaattacgagatattagtttttgacactttttttctcgtggccggcatggtcccagcctcctcgctggcgccggctgggcaacatgcttcggcatggcgaatgggactagcataaccccttggggcctctaaacgggtcttgaggggttttttg

SEQ ID NO: 19 - DNA, 15689 bp, synthetic construct
  misc_feature 1..15689: note = antigenic cDNA encoding cRSVA_VSVG_A_SH deletion_G deletion
  source 1..15689: mol_type = other DNA
taatacgactcactataggttttttcgcgtctgatgaggccgttaggccgaaactcctctccggagtcacgcgaaaaaatgcgtacaacaaacttgcgtaaaccaaaaaaatggggcaaataagaatttgataagtaccacttaaatttaactcctttggttagaggcgcgccatgggcagcaactcattgagtatgataaaagttagattgcaaaatctgtttgacaatgatgaagtagcattgttaaaaataacatgctatactgacaaattaatacagttaactaatgctttggctaaggcagttatacatacaatcaaattgaatggcattgtatttgtgcatgttattacaagtagtgatatttgccctaataataatattgtagtgaaatccaatttcacaacaatgccagtattacaaaatggaggttatatatgggaaatgatggaattaacacactgctctcaacctaatggcctaatagatgacaattgtgaaattaaattctccaaaaaactaagtgattcaacaatgaccaattatatgaatcaattatctgaattacttggatttgacctcaatccataaatcataataaatatcaactagcaaatcaatgtcactaacaccattagttaatataaaacttgacagaagataaaaatggggcaaataaatcaattcagccgacccaaccatggacacaacacacaatgataccacaccacaaagactgatgatcacagacatgaggccattatcgcttgagactataataacatctctaaccagagatatcataacacataaatttatatacttgataaatcatgaatgcatagtaagaaaacttgatgaaagacaggccacatttacatttctggtcaactatgaaatgaaactattgcacaaagtgggaagcactaaatataaaaaatatactgaatacaacacaaaatatggcactttccctatgccaatatttatcaatcatgatgggttcttagaatgcattggcattaagcctaccaagcacacacccataatatacaagtatgatctcaatccatgaatatcaaaccaagattcaaacaatccgaaataacaactttatgcataatcacactccatagtccaaatggagcctgaaaattatagttatttaaaattcctgcaggaaggagagacataagatgaaagatggggcaaatacaaaaatggctcttagcaaagtcaagttgaatgatacactcaacaaagatcaacttctatcatccagcaaatataccatccaacggagcacaggagacagcattgacactcctaattatgatgtgcagaaacacattaataagttatgtggcatgttattaatcacagaagatgctaatcataaattcactgggttaataggtatgttatatgctatgtctagattaggaagagaagacaccataaaaatactcaaagatgcgggatatcatgttaaggcaaatggagtggatgtaacaacacatcgtcaagacattaatgggaaagaaatgaaatttgaagtgttaacattagcaagcttaacaactgaaattcaaatcaacattgagatagaatctagaaaatcctacaaaaaaatgctaaaagaaatgggagaggtggctccagaatacaggcatgactctcctgattgtgggatgataatattatgtatagcggcattagtaataaccaaattagcagcaggagatagatcaggtcttacagctgtgattaggagagctaataatgtcctaaaaaatgaaatgaaacgttataaaggtttattacccaaggatatagccaacagcttctatgaagtgtttgaaaaatatcctcactttatagatgtttttgttcattttggtatagcacaatcttctaccagaggtggcagtagagttgaagggatttttgcaggattgtttatgaatgcctatggtgcagggcaagtgatgttacggtggggggtcttagcaaaatcagttaaaaacattatgttaggacacgctagtgtacaagcagaaatggaacaagttgtggaggtgtatgagtatgctcagaaattgggtggagaagcaggattctaccatatattgaacaacccaaaagcatcactattatctttgactcaatttcctcacttctctagtgtagtattgggcaatgctgctggcctaggcataatgggagaatacagaggtacaccaaggaatcaagatttatatgatgctgcaaaagcatatgctgaacaactcaaagaaaatggtgtgattaactacagtgtattagatttgacagcagaagaactagaggctatcaaacatcagcttaatccaaaagataatgatgtagagctttgagttaataaaaaagtggggcaaataaatcatcatggaaaagtttgctcctgaattccatggagaagatgcaaacaacagagccaccaaattcctagaatcaataaagggcaaattcacatcacccaaagatcccaagaaaaaagatagtatcatatctgtcaactcaatagatatagaagtaaccaaagaaagccctataacatcaaattcaaccattataaacccaataaatgagacagatgatactgtagggaacaagcccaattatcaaagaaagcctctagtaagtttcaaagaagaccctacgccaagtgataatcctttttcaaaactatacaaagaaaccatagaaacatttgataacaatgaagaagaatctagctattcatatgaagaaataaatgatcagacaaacgataatataacagcaagattagataggattgatgagaaattaagtgaaatactaggaatgcttcacacattagtagtagcgagtgcaggacccacatctgctcgggatggtataagagatgccatggttggtttaagagaagaaatgatagaaaaaatcagaactgaagcattaatgaccaatgacagactagaagctatggcaagactcaggaatgaagaaagtgaaaagatggcaaaagacacatcagatgaagtgtctctcaatccaacatcagagaaactgaacaacctgttggaagggaatgatagtgacaatgatctatcacttgaagatttctgattagctaccaaactgtacatcaaaacacaacaccaatagaaaaccaacaaacaaaccaactcacccatccaaccaaacatctatctgctgattagccaaccagccaaaaaacaaccagccaatctaaaactagccacccggaaaaaatcgatactatagttacaaaaaaagatggggcaaatatggaaacatacgtgaataaacttcacgagggctccacatacacagctgctgttcaatacaatgtcctagaaaaagacgatgatcctgcatcacttacaatatgggtgcccatgttccaatcatccatgccagcagatctactcataaaagaactagccaatgtcaatatactagtgaaacaaatatccacacccaagggaccctcattaagagtcatgataaactcaagaagtgcagtgctagcacaaatgcccagcaaatttaccatatgtgccaatgtgtccttggatgaaagaagcaagctggcatatgatgtaaccacaccctgtgaaattaaggcatgcagtctaacatgcctaaaatcaaaaaatatgttaactacagttaaagatctcactatgaaaacactcaacccaacacatgacatcattgctttatgtgaatttgaaaatatagtaacatcaaaaaaagtcataataccaacatacctaagatctatcagcgtcagaaataaagatctgaacacacttgaaaatataacaaccactgaattcaaaaatgccattacaaatgcaaaaatcatcccttactcaggattattgttagtcatcacagtgactgacaacaaaggagcattcaaatacataaagccacaaagtcaattcatagtagatcttggagcttacctagaaaaagaaagtatatattatgttacaacaaattggaagcacacagctacacgatttgcaatcaaacccatggaagattaacctttttcctctacatcaatgagtagattcatacaaactttctaactacattcttcacttcacaatcataatcaccaaccctctgtggttcaatcaatcaaacaaaactcatcaagagttccagatcatcccaagtcattgttcatcagatccagtactcaaataagttaataaaaaatcggtccgttgacagaagataaaaatggggcaaatgcaaacatgaagtgccttttgtacttagcctttttattcattggggtgaattgcaagttcaccatagtttttccacacaaccaaaaaggaaactggaaaaatgttccttctaattaccattattgcccgtcaagctcagatttaaattggcataatgacttaataggcacagccttacaagtcaaaatgcccaagagtcacaaggctattcaagcagacggttggatgtgtcatgcttccaaatgggtcactacttgtgatttccgctggtatggaccgaagtatataacacattccatccgatccttcactccatctgtagaacaatgcaaggaaagcattgaacaaacgaaacaaggaacttggctgaatccaggcttccctcctcaaagttgtggatatgcaactgtgacggatgccgaagcagtgattgtccaggtgactcctcaccatgtgctggttgatgaatacacaggagaatgggttgattcacagttcatcaacggaaaatgcagcaattacatatgccccactgtccataactctacaacctggcattctgactataaggtcaaagggctatgtgattctaacctcatttccatggacatcaccttcttctcagaggacggagagctatcatccctgggaaaggagggcacagggttcagaagtaactactttgcttatgaaactggaggcaaggcctgcaaaatgcaatactgcaagcattggggagtcagactcccatcaggtgtctggttcgagatggctgataaggatctctttgctgcagccagattccctgaatgcccagaagggtcaagtatctctgctccatctcagacctcagtggatgtaagtctaattcaggacgttgagaggatcttggattattccctctgccaagaaacctggagcaaaatcagagcgggtcttccaatctctccagtggatctcagctatcttgctcctaaaaacccaggaaccggtcctgctttcaccataatcaatggtaccctaaaatactttgagaccagatacatcagagtcgatattgctgctccaatcctctcaagaatggtcggaatgatcagtggaactaccacagaaagggaactgtgggatgactgggcaccatatgaagacgtggaaattggacccaatggagttctgaggaccagttcaggatataagtttcctttatacatgattggacatggtatgttggactccgatcttcatcttagctcaaaggctcaggtgttcgaacatcctcacattcaagacgctgcttcgcaacttcctgatgatgagagtttattttttggtgatactgggctatccaaaaatccaatcgagcttgtagaaggttggttcagtagttggaaaagctctattgcctcttttttctttatcatagggttaatcattggactattcttggttctccgagttggtatccatctttgcattaaagccagaagcacaccagtcacattaagtaaggatcaactgagtggtataaataatattgcatttagtaactaatagtcattaaaaagcggccggccgtattgttgcaaaaagccatgaccaaatcaaacagaatcaaaatcaactctacgcgtgtattgttgcaaaaagccatgaccaaatcaaacagaatcaaaatcaactctggggcaaataacaatggagttgccaatcctcaaaacaaatgctattaccacaatccttgctgcagtcacactctgtttcgcttccagtcaaaacatcactgaagaattttatcaatcaacatgcagtgcagtcagcaaaggctatcttagtgctctaagaactggttggtatactagtgttataactatagaattaagtaatatcaaggaaaataagtgtaatggtacagacgctaaggtaaaattaataaaacaagaattagataaatataaaaatgctgtaacagaattgcagttgctcatgcaaagcacaccagcagccaacaatcgagccagaagagaactaccaagatttatgaattatacactcaacaataccaaaaacaccaatgtaacattaagtaagaaaaggaaaagaagatttcttggatttttgttaggtgttggatctgcaatcgccagtggcattgccgtatccaaggtcctgcacctagaaggggaagtgaacaaaatcaaaagtgctctactatccacaaacaaggctgtagtcagcttatctaatggagtcagtgtcttaaccagcaaggtgttagacctcaaaaactatatagataaacagttgttacctattgttaacaagcaaagctgcagcatatcaaacattgaaactgtgatagagttccaacaaaagaacaacagactactagagattaccagagaatttagtgttaatgcaggtgtaactactcctgtaagcacttatatgttaactaatagtgagttattatcattaatcaatgatatgcctataacaaatgatcagaaaaagttaatgtccagcaatgttcaaatagttagacagcaaagttactctatcatgtcaataataaaagaggaagtcttggcatatgtagtacaattaccactatatggtgtaatagatactccttgttggaaactacacacatcccctttatgtacaaccaacacaaaggaaggatccaacatctgcttaacaagaaccgacagaggatggtactgtgacaatgcaggatcagtatcctttttcccacaagctgaaacatgtaaagttcaatcgaatcgggtgttttgtgacacaatgaacagtttaacattaccaagtgaggtaaatctctgcaacattgacatattcaaccccaaatatgattgcaaaattatgacttcaaaaacagatgtaagcagctccgttatcacatctctaggagccattgtgtcatgctatggcaaaaccaaatgtacagcatccaataaaaatcgtgggatcataaagacattctctaacgggtgtgattatgtatcaaataagggggtggatactgtgtctgtaggtaatacattatattatgtaaataagcaagaaggcaaaagtctctatgtaaaaggtgaaccaataataaatttctatgatccattagtgttcccctctgatgaatttgatgcatcaatatctcaagtcaatgagaaaattaatcagagtctagcatttatccgtaaatcagatgaattattacataatgtaaatgctggtaaatccaccacaaatatcatgataactaccataattatagtaattatagtaatattgttagcattaattgcagttggactgcttctatactgcaaggccagaagcacaccagtcacattaagtaaggatcaactgagtggtataaataatattgcatttagtaactgaataaaaatagcacctaatcatattcttacaatggttcgctatttgaccatagataacccatctatcattagattatcctaaaatttgaacttcatcacaactttcatctataaaccatctcacttacactttttaagtagatttctattttatagttatataaaacagggcccattgaataccaaattaacttactatttgtaaaaatgagaattggggcaaatatgtcacgaaggaatccttgcaaattcgaaattcgaggtcattgcttgaatggtaaaaggtgtcattttagtcataattattttgaatggccaccccatgcactgcttgtaagacaaaactttatgttaaacagaatacttaagtctatggataaaagcatagatactttgtcagaaataagtggagctgcagagttggacagaacagaagagtatgccctcggtgtagttggagtgctagagagttatataggatcaataaataatataactaaacaatcagcatgtgttgccatgagcaaactccttactgaactcaacagcgatgacatcaaaaaactaagggacaatgaagagccaaactcacccaaagtaagagtgtacaatactgtcatatcatatattgaaagcaacaggaagaacaataaacaaactatccatctgttaaaaagattgccagcagacgtattgaagaaaaccatcaaaaacacattggatatccacaagagcataaccatcaataacccaaaagaatcaactgttagtgatacgaacgaccatgccaaaaataatgatactacctgacaaatatccttgtagtataaattccatactaataacaagtaattgtagagtcactatgtataatcaaaaaaacacactatatatcaatcaaaacaaccaaaatagccatatatacccaccggatcaaccattcaatgaaatccattggacctctcaagacttgattgatgcaactcaaaattttctacaacatctaggtattactgatgatatatacacaatatatatattagtgtcataatactcaatcctaatacttaccacatcatcaaattattaactcaaacaattcaagctatgggacaaaatggatcccattattagtggaaattctgctaatgtttatctaactgatagttatttaaaaggtgttatttctttctcagaatgtaacgctttaggaagttacatattcaatggtccttatctcaaaaatgattataccaacttaattagtagacaaaatccattaatagaacacataaatctaaagaaactaaatataacacagtccttaatatctaagtatcataaaggtgaaataaaaatagaagaacctacttactttcagtcattacttatgacatacaagagtatgacctcttcagaacagactactactactaatttacttaaaaagataataagaagagctatagaaatcagtgatgtcaaagtctatgctatattgaataaactggggctcaaagaaaaagacaagattaaatccaataatggacaagatgaagacaactcagtcattactaccataatcaaagatgatatacttttagctgtcaaggataatcaatctcatcttaaagcagacaaaaatcaatccacaaaacaaaaagatacaatcaaaacaacacttttgaagaaattaatgtgttcgatgcaacatcctccatcatggttaatacattggtttaatttatacacaaaattaaacagcatattaacacaatatcgatctagtgaggtaaaaaaccatggttttatattgatagataatcatactcttagtggattccaatttattttgaatcaatatggttgtatagtttatcataaggaactcaaaagaattactgtgacaacttataatcaattcttgacatggaaagatattagccttagtagattaaatgtttgtttgattacatggattagtaactgtttgaacacattaaacaaaagcttaggcttaagatgtggattcaataatgttatcttgacacaattattcctttatggagattgtatactaaaactattccacaatgaggggttctacataataaaagaggtagagggatttattatgtctctaattttaaatataacagaagaagatcaattcagaaaacggttttataatagtatgctcaacaacatcacagatgccgccaacaaagctcaaaaaaatctgctatcaagagtatgtcatacattattagataagacaatatcagataatataataaatggcagatggataattctattgagtaagttcctaaaattaattaagcttgcaggtgacaataacctcaacaatctgagtgaattatattttttgttcagaatatttggacacccaatggtagatgaaagacaagccatggatgctgttaaagttaattgcaacgagaccaaattttatttgttaagtagtttgagtatgttaagaggagcttttatatatagaattataaaagggtttgtaaataattacaacagatggcctactttaagaaatgccattgtcttacccttaagatggttaacttactataaactaaacacttatccttccttgttggaacttacagaaagagatttgattgttctatcaggactacgtttctatcgagagtttcggttgcctaaaaaagtggatcttgaaatgatcataaatgataaggctatatcacctcctaaaaatttaatatggactagtttccctagaaattatatgccgtcacacatacaaaattatatagaacatgaaaaattaaaattctctgatagtgataaatcaagaagagtattagagtattatttaagagataacaaattcaatgaatgtgatttacacaactgtgtagttaatcaaagttatcttaacaacccgaatcatgtggtatcattgacaggcaaagaaagagaactcagtgtaggtagaatgtttgcaatgcaaccaggaatgttcagacaagttcaaatattagcagagaaaatgatagcagaaaacatattacaatttttccctgaaagtcttacaagatatggtgatctagaactacagaaaatattagaattgaaagcaggaataagtaacaaatcaaatcgttacaatgataattacaacaattacattagtaagtgctctatcatcacagatctcagcaaattcaatcaagcatttcgatatgaaacatcatgtatttgtagtgatgtactggatgaactgcatggtgtacaatctctattttcctggttacatttaactattcctcatgtcacaataatatgcacatataggcatgcacccccctatataaaggatcatattgtagatcttaacaatgtagatgagcaaagtggactatatagatatcatatgggtggtatcgaagggtggtgtcaaaaactatggaccatagaagctatatcactattagatctaatatctctcaaagggaaattctcaattactgctttaattaatggtgacaatcaatcaatagatataagtaaaccagtcagactcatggaaggtcaaactcatgctcaagcagattatttgctagcattaaatagtctcaaattactgtataaagagtatgcaggaataggccacaaattaaaaggaactgagacttatatatcgagagatatgcaatttatgagtaaaacgatccaacataacggtgtatattacccagctagtataaagaaagtcctaagagtgggaccgtggataaacactatacttgatgacttcaaagtgagtctagaatctataggtagtttgacacaagaattagaatatagaggtgaaagtctattatgcagtttaatatttagaaatgtatggttatataatcaaattgcattacaacttaaaaatcatgcattatgtaacaacaaattatatttggatatattaaaagttctaaaacacttaaaaaccttttttaatcttgataacattgatacagcattaacattgtatatgaatttgcccatgttatttggtggtggtgatcccaacttgttatatcgaagtttctatagaagaactcctgatttcctcacagaggctatagttcactctgtgttcatacttagttattatacaaaccatgatttaaaagataaacttcaagatctgtcagatgatagattgaataagttcttaacatgcataatcacgtttgataaaaaccccaatgctgaattcgttacattgatgagagatcctcaagctttaggatctgagaggcaagctaaaattactagcgaaatcaatagactggcagttaccgaggttttgagcacagctccaaacaaaatattttccaaaagtgcacaacactataccactacagagatagatcttaatgatattatgcaaaatatagaacctacatatcctcacgggctaagagttgtttatgagagtttacccttttataaagcagagaaaatagtaaatcttatatccggtacaaaatctataactaacatactggaaaagacttctgccatagacttaacagatattgatagagccactgagatgatgaggaaaaacataactttgcttataaggatattaccattagattgtaacagagataaaagagaaatattgagtatggaaaacctaagtattactgaattaagcaaatacgttagagaaagatcttggtctttatccaatatagttggtgttacatcacccagtatcatgtatacaatggacataaaatatacaacaagcactatagctagtggcataatcatagagaaatataatgtcaacagtttaacacgtggtgagagaggacccactaaaccatgggttggttcatctacacaagagaaaaagacaatgccagtttataatagacaagttttaaccaaaaaacagagagatcaaatagatctattagcaaaattggattgggtgtatgcatctatagataacaaggatgaatttatggaggaacttagcataggaactcttgggttaacatatgagaaggccaaaaaattattcccacaatatttgagtgttaactatttgcatcgtcttacagtcagtagtagaccatgtgaattccctgcatctataccagcttatagaactacaaattatcactttgatactagccctattaatcgcatattaacagaaaagtatggtgatgaagatattgatatagtattccaaaactgtataagctttggccttagcttaatgtctgtagtagaacaatttactaatgtatgtcctaacagaattattctcatacccaagcttaatgagatacatttgatgaaacctcccatattcacaggcgatgttgatattcacaagttaaaacaagtgatacaaaaacaacatatgtttttaccagacaaaataagtttgactcaatatgtggaattattcttaagtaataaaacactcaaatctggatctaatgttaattctaatttaatattggcgcataagatatctgactattttcataatacttacattttgagtactaatttagctggacattggattcttattatacaacttatgaaagattctaagggtatttttgaaaaagattggggagagggatatataactgatcatatgttcattaatttgaaagttttcttcaatgcttataagacatatctcttgtgttttcataaaggttacggcagagcaaagctggagtgtgatatgaatacttcagatctcctatgtgtattggaattaatagacagtagttattggaagtctatgtctaaggtgtttttagaacaaaaagttatcaaatacattcttagccaggatgcaagtttacatagagtaaaaggatgtcatagcttcaaactatggtttcttaaacgtcttaatgtagcagaattcacagtttgcccttgggttgttaacatagattatcatccaacacatatgaaagcaatattaacttatattgatcttgttagaatgggattgataaatatagatagaatatacattaaaaataaacacaagttcaatgatgagttttatacttctaatctgttttacattaattataacttctcagataatactcatctattaactaaacatataaggattgctaattccgaattagaaagtaattacaacaaattatatcatcctacaccagaaaccctagaaaatatactaaccaatccggttaaaagtaatgagaaaaagacactgagtgactattgtataggtaaaaatgttgactcaataatgttaccatcgttatctaataagaagcttattaaatcgtctacaatgattagaaccaattacagcagacaagatttgtataatttatttcctacggttgtgattgataaaattatagatcattcaggtaatacagccaaatctaaccaactttacactactacttctcatcaaatatccttagtgcacaatagcacatcactttattgcatgcttccttggcatcatattaatagattcaattttgtatttagttctacaggttgtaaaattagtatagagtatattttaaaagatcttaaaattaaggatcctaattgtatagcattcataggtgaaggagcagggaatttattattgcgtacagtagtggaacttcatcctgatataagatatatttacagaagtctgaaagattgcaatgatcatagtttaccaattgagtttttaaggctgtacaatggacatatcaacattgattatggtgaaaatttgaccattcctgctacagatgcaaccaacaacattcattggtcttatttacatataaagtttgctgaacctatcagtctttttgtctgtgatgctgaattgcctgtaacagtcaactggagtaagattataatagagtggagcaagcatgtaagaaaatgcaagtactgttcttcagttaataaatgtacattgatagtaaaatatcatgctcaagatgatatcgatttcaaattagacaacataactatattaaaaacttatgtatgcttaggtagtaagttaaagggatctgaagtttacttagtccttacaataggtcctgcaaatgtgttcccagtatttaatgtagtacaaaatgctaaattgatactatcaagaactaaaaatttcatcatgcctaaaaaagctgataaagagtctattgatgcaaatattaagagtttgataccctttctttgttaccctataacaaaaaaaggaattaatactgcattgtctaaattaaagagtgttgttagtggagatatactatcatattctatagctggacgtaatgaagttttcagcaataaacttataaatcataagcatatgaacatcttaaagtggttcaatcatgttttaaatttcagatcaacagaattaaactataatcatttatatatggtagaatctacttatcctcatctaagtgaattgttaaacagcttgacaaccaatgaacttaaaaaactgattaaaatcacaggtagtttgttatacaacttttataatgaataatgagcaaaaatcttataacaaaaatagctacacactaacattgtattcaattatagttattgaaaattaataattatataatttttaataacttctagtgaactaatcctaaaattatcattttgatctaggaagaataagtttaaatccaaatctaattggtttatatgtatattaactaaattacgagatattagtttttgacactttttttctcgtggccggcatggtcccagcctcctcgctggcgccggctgggcaacatgcttcggcatggcgaatgggactagcataaccccttggggcctctaaacgggtcttgaggggttttttg

SEQ ID NO: 20 - DNA, 14772 bp, synthetic construct
  misc_feature 1..14772: note = antigenic cDNA encoding cRSVA_VSVG_A_SH deletion_F deletion
  source 1..14772: mol_type = other DNA
taatacgactcactataggttttttcgcgtctgatgaggccgttaggccgaaactcctctccggagtcacgcgaaaaaatgcgtacaacaaacttgcgtaaaccaaaaaaatggggcaaataagaatttgataagtaccacttaaatttaactcctttggttagaggcgcgccatgggcagcaactcattgagtatgataaaagttagattgcaaaatctgtttgacaatgatgaagtagcattgttaaaaataacatgctatactgacaaattaatacagttaactaatgctttggctaaggcagttatacatacaatcaaattgaatggcattgtatttgtgcatgttattacaagtagtgatatttgccctaataataatattgtagtgaaatccaatttcacaacaatgccagtattacaaaatggaggttatatatgggaaatgatggaattaacacactgctctcaacctaatggcctaatagatgacaattgtgaaattaaattctccaaaaaactaagtgattcaacaatgaccaattatatgaatcaattatctgaattacttggatttgacctcaatccataaatcataataaatatcaactagcaaatcaatgtcactaacaccattagttaatataaaacttgacagaagataaaaatggggcaaataaatcaattcagccgacccaaccatggacacaacacacaatgataccacaccacaaagactgatgatcacagacatgaggccattatcgcttgagactataataacatctctaaccagagatatcataacacataaatttatatacttgataaatcatgaatgcatagtaagaaaacttgatgaaagacaggccacatttacatttctggtcaactatgaaatgaaactattgcacaaagtgggaagcactaaatataaaaaatatactgaatacaacacaaaatatggcactttccctatgccaatatttatcaatcatgatgggttcttagaatgcattggcattaagcctaccaagcacacacccataatatacaagtatgatctcaatccatgaatatcaaaccaagattcaaacaatccgaaataacaactttatgcataatcacactccatagtccaaatggagcctgaaaattatagttatttaaaattcctgcaggaaggagagacataagatgaaagatggggcaaatacaaaaatggctcttagcaaagtcaagttgaatgatacactcaacaaagatcaacttctatcatccagcaaatataccatccaacggagcacaggagacagcattgacactcctaattatgatgtgcagaaacacattaataagttatgtggcatgttattaatcacagaagatgctaatcataaattcactgggttaataggtatgttatatgctatgtctagattaggaagagaagacaccataaaaatactcaaagatgcgggatatcatgttaaggcaaatggagtggatgtaacaacacatcgtcaagacattaatgggaaagaaatgaaatttgaagtgttaacattagcaagcttaacaactgaaattcaaatcaacattgagatagaatctagaaaatcctacaaaaaaatgctaaaagaaatgggagaggtggctccagaatacaggcatgactctcctgattgtgggatgataatattatgtatagcggcattagtaataaccaaattagcagcaggagatagatcaggtcttacagctgtgattaggagagctaataatgtcctaaaaaatgaaatgaaacgttataaaggtttattacccaaggatatagccaacagcttctatgaagtgtttgaaaaatatcctcactttatagatgtttttgttcattttggtatagcacaatcttctaccagaggtggcagtagagttgaagggatttttgcaggattgtttatgaatgcctatggtgcagggcaagtgatgttacggtggggggtcttagcaaaatcagttaaaaacattatgttaggacacgctagtgtacaagcagaaatggaacaagttgtggaggtgtatgagtatgctcagaaattgggtggagaagcaggattctaccatatattgaacaacccaaaagcatcactattatctttgactcaatttcctcacttctctagtgtagtattgggcaatgctgctggcctaggcataatgggagaatacagaggtacaccaaggaatcaagatttatatgatgctgcaaaagcatatgctgaacaactcaaagaaaatggtgtgattaactacagtgtattagatttgacagcagaagaactagaggctatcaaacatcagcttaatccaaaagataatgatgtagagctttgagttaataaaaaagtggggcaaataaatcatcatggaaaagtttgctcctgaattccatggagaagatgcaaacaacagagccaccaaattcctagaatcaataaagggcaaattcacatcacccaaagatcccaagaaaaaagatagtatcatatctgtcaactcaatagatatagaagtaaccaaagaaagccctataacatcaaattcaaccattataaacccaataaatgagacagatgatactgtagggaacaagcccaattatcaaagaaagcctctagtaagtttcaaagaagaccctacgccaagtgataatcctttttcaaaactatacaaagaaaccatagaaacatttgataacaatgaagaagaatctagctattcatatgaagaaataaatgatcagacaaacgataatataacagcaagattagataggattgatgagaaattaagtgaaatactaggaatgcttcacacattagtagtagcgagtgcaggacccacatctgctcgggatggtataagagatgccatggttggtttaagagaagaaatgatagaaaaaatcagaactgaagcattaatgaccaatgacagactagaagctatggcaagactcaggaatgaagaaagtgaaaagatggcaaaagacacatcagatgaagtgtctctcaatccaacatcagagaaactgaacaacctgttggaagggaatgatagtgacaatgatctatcacttgaagatttctgattagctaccaaactgtacatcaaaacacaacaccaatagaaaaccaacaaacaaaccaactcacccatccaaccaaacatctatctgctgattagccaaccagccaaaaaacaaccagccaatctaaaactagccacccggaaaaaatcgatactatagttacaaaaaaagatggggcaaatatggaaacatacgtgaataaacttcacgagggctccacatacacagctgctgttcaatacaatgtcctagaaaaagacgatgatcctgcatcacttacaatatgggtgcccatgttccaatcatccatgccagcagatctactcataaaagaactagccaatgtcaatatactagtgaaacaaatatccacacccaagggaccctcattaagagtcatgataaactcaagaagtgcagtgctagcacaaatgcccagcaaatttaccatatgtgccaatgtgtccttggatgaaagaagcaagctggcatatgatgtaaccacaccctgtgaaattaaggcatgcagtctaacatgcctaaaatcaaaaaatatgttaactacagttaaagatctcactatgaaaacactcaacccaacacatgacatcattgctttatgtgaatttgaaaatatagtaacatcaaaaaaagtcataataccaacatacctaagatctatcagcgtcagaaataaagatctgaacacacttgaaaatataacaaccactgaattcaaaaatgccattacaaatgcaaaaatcatcccttactcaggattattgttagtcatcacagtgactgacaacaaaggagcattcaaatacataaagccacaaagtcaattcatagtagatcttggagcttacctagaaaaagaaagtatatattatgttacaacaaattggaagcacacagctacacgatttgcaatcaaacccatggaagattaacctttttcctctacatcaatgagtagattcatacaaactttctaactacattcttcacttcacaatcataatcaccaaccctctgtggttcaatcaatcaaacaaaactcatcaagagttccagatcatcccaagtcattgttcatcagatccagtactcaaataagttaataaaaaatcggtccgttgacagaagataaaaatggggcaaatgcaaacatgaagtgccttttgtacttagcctttttattcattggggtgaattgcaagttcaccatagtttttccacacaaccaaaaaggaaactggaaaaatgttccttctaattaccattattgcccgtcaagctcagatttaaattggcataatgacttaataggcacagccttacaagtcaaaatgcccaagagtcacaaggctattcaagcagacggttggatgtgtcatgcttccaaatgggtcactacttgtgatttccgctggtatggaccgaagtatataacacattccatccgatccttcactccatctgtagaacaatgcaaggaaagcattgaacaaacgaaacaaggaacttggctgaatccaggcttccctcctcaaagttgtggatatgcaactgtgacggatgccgaagcagtgattgtccaggtgactcctcaccatgtgctggttgatgaatacacaggagaatgggttgattcacagttcatcaacggaaaatgcagcaattacatatgccccactgtccataactctacaacctggcattctgactataaggtcaaagggctatgtgattctaacctcatttccatggacatcaccttcttctcagaggacggagagctatcatccctgggaaaggagggcacagggttcagaagtaactactttgcttatgaaactggaggcaaggcctgcaaaatgcaatactgcaagcattggggagtcagactcccatcaggtgtctggttcgagatggctgataaggatctctttgctgcagccagattccctgaatgcccagaagggtcaagtatctctgctccatctcagacctcagtggatgtaagtctaattcaggacgttgagaggatcttggattattccctctgccaagaaacctggagcaaaatcagagcgggtcttccaatctctccagtggatctcagctatcttgctcctaaaaacccaggaaccggtcctgctttcaccataatcaatggtaccctaaaatactttgagaccagatacatcagagtcgatattgctgctccaatcctctcaagaatggtcggaatgatcagtggaactaccacagaaagggaactgtgggatgactgggcaccatatgaagacgtggaaattggacccaatggagttctgaggaccagttcaggatataagtttcctttatacatgattggacatggtatgttggactccgatcttcatcttagctcaaaggctcaggtgttcgaacatcctcacattcaagacgctgcttcgcaacttcctgatgatgagagtttattttttggtgatactgggctatccaaaaatccaatcgagcttgtagaaggttggttcagtagttggaaaagctctattgcctcttttttctttatcatagggttaatcattggactattcttggttctccgagttggtatccatctttgcattaaagccagaagcacaccagtcacattaagtaaggatcaactgagtggtataaataatattgcatttagtaactaatagtcattaaaaagcggccggccagtcataacaatgaactaggatattaagaccaaaaacaacgctggggcaaatgcaaacatgtccaaaaccgaggaccaacgcaccgccaagacactagaaaggacctgggacacttttaatcatctattattcatatcatcgtgcttatacaagttaaatcttaaatctatagcacaaatcacattatctattttggcaattataatctcaacctcacttataattgcagccatcatattcatagcctcggcaaaccacaaagtcacactaacaactgcaatcatacaagatgcaacgaaccagatcaagaacacaaccccaacatacctcacccagaatccccagcatggaatcagcttctccaatctgtccggaactacatcacaatccaccaccatactagcttcaacaacaccaagtgctgattcaaccccacaatccacaacagtcaagatcaaaaacacaacaacaacccaaatattacctagcaaacccaccacaaaacaacgccaaaataaaccacaaaacaaacccaacaatgattttcactttgaagtgttcaattttgtaccctgcagcatatgcagcaacaatccaacctgctgggccatctgcaagagaataccaaacaaaaaacctggaaagaaaaccaccaccaagcccacaaaaaaaccaaccctcaagacaaccaaaaaagatcccaaatcccaaaccacaaaaccaaaggaagtactcactaccaagcctacaggaaagccaaccatcaacaccactaaaacaaacatcagaactacactgctcacctccaacaccaaaggaaatccagaacacacaagtcaagaggaaaccctccactcaaccacctccgaaggctatccaagcccatcacaagtccacacaacatccggtcaagaggaaaccctccactcaaccacctccgaaggctatccaagcccatcacaagtctacacaacatccgagtacctatcacaatctctatcttcatccaacacaacaaaatgatagtcattaaaaagcacgcgtgtattgttgcaaaaagccatgaccaaatcaaacagaatcaaaatcaactctgggcccattgaataccaaattaacttactatttgtaaaaatgagaattggggcaaatatgtcacgaaggaatccttgcaaattcgaaattcgaggtcattgcttgaatggtaaaaggtgtcattttagtcataattattttgaatggccaccccatgcactgcttgtaagacaaaactttatgttaaacagaatacttaagtctatggataaaagcatagatactttgtcagaaataagtggagctgcagagttggacagaacagaagagtatgccctcggtgtagttggagtgctagagagttatataggatcaataaataatataactaaacaatcagcatgtgttgccatgagcaaactccttactgaactcaacagcgatgacatcaaaaaactaagggacaatgaagagccaaactcacccaaagtaagagtgtacaatactgtcatatcatatattgaaagcaacaggaagaacaataaacaaactatccatctgttaaaaagattgccagcagacgtattgaagaaaaccatcaaaaacacattggatatccacaagagcataaccatcaataacccaaaagaatcaactgttagtgatacgaacgaccatgccaaaaataatgatactacctgacaaatatccttgtagtataaattccatactaataacaagtaattgtagagtcactatgtataatcaaaaaaacacactatatatcaatcaaaacaaccaaaatagccatatatacccaccggatcaaccattcaatgaaatccattggacctctcaagacttgattgatgcaactcaaaattttctacaacatctaggtattactgatgatatatacacaatatatatattagtgtcataatactcaatcctaatacttaccacatcatcaaattattaactcaaacaattcaagctatgggacaaaatggatcccattattagtggaaattctgctaatgtttatctaactgatagttatttaaaaggtgttatttctttctcagaatgtaacgctttaggaagttacatattcaatggtccttatctcaaaaatgattataccaacttaattagtagacaaaatccattaatagaacacataaatctaaagaaactaaatataacacagtccttaatatctaagtatcataaaggtgaaataaaaatagaagaacctacttactttcagtcattacttatgacatacaagagtatgacctcttcagaacagactactactactaatttacttaaaaagataataagaagagctatagaaatcagtgatgtcaaagtctatgctatattgaataaactggggctcaaagaaaaagacaagattaaatccaataatggacaagatgaagacaactcagtcattactaccataatcaaagatgatatacttttagctgtcaaggataatcaatctcatcttaaagcagacaaaaatcaatccacaaaacaaaaagatacaatcaaaacaacacttttgaagaaattaatgtgttcgatgcaacatcctccatcatggttaatacattggtttaatttatacacaaaattaaacagcatattaacacaatatcgatctagtgaggtaaaaaaccatggttttatattgatagataatcatactcttagtggattccaatttattttgaatcaatatggttgtatagtttatcataaggaactcaaaagaattactgtgacaacttataatcaattcttgacatggaaagatattagccttagtagattaaatgtttgtttgattacatggattagtaactgtttgaacacattaaacaaaagcttaggcttaagatgtggattcaataatgttatcttgacacaattattcctttatggagattgtatactaaaactattccacaatgaggggttctacataataaaagaggtagagggatttattatgtctctaattttaaatataacagaagaagatcaattcagaaaacggttttataatagtatgctcaacaacatcacagatgccgccaacaaagctcaaaaaaatctgctatcaagagtatgtcatacattattagataagacaatatcagataatataataaatggcagatggataattctattgagtaagttcctaaaattaattaagcttgcaggtgacaataacctcaacaatctgagtgaattatattttttgttcagaatatttggacacccaatggtagatgaaagacaagccatggatgctgttaaagttaattgcaacgagaccaaattttatttgttaagtagtttgagtatgttaagaggagcttttatatatagaattataaaagggtttgtaaataattacaacagatggcctactttaagaaatgccattgtcttacccttaagatggttaacttactataaactaaacacttatccttccttgttggaacttacagaaagagatttgattgttctatcaggactacgtttctatcgagagtttcggttgcctaaaaaagtggatcttgaaatgatcataaatgataaggctatatcacctcctaaaaatttaatatggactagtttccctagaaattatatgccgtcacacatacaaaattatatagaacatgaaaaattaaaattctctgatagtgataaatcaagaagagtattagagtattatttaagagataacaaattcaatgaatgtgatttacacaactgtgtagttaatcaaagttatcttaacaacccgaatcatgtggtatcattgacaggcaaagaaagagaactcagtgtaggtagaatgtttgcaatgcaaccaggaatgttcagacaagttcaaatattagcagagaaaatgatagcagaaaacatattacaatttttccctgaaagtcttacaagatatggtgatctagaactacagaaaatattagaattgaaagcaggaataagtaacaaatcaaatcgttacaatgataattacaacaattacattagtaagtgctctatcatcacagatctcagcaaattcaatcaagcatttcgatatgaaacatcatgtatttgtagtgatgtactggatgaactgcatggtgtacaatctctattttcctggttacatttaactattcctcatgtcacaataatatgcacatataggcatgcacccccctatataaaggatcatattgtagatcttaacaatgtagatgagcaaagtggactatatagatatcatatgggtggtatcgaagggtggtgtcaaaaactatggaccatagaagctatatcactattagatctaatatctctcaaagggaaattctcaattactgctttaattaatggtgacaatcaatcaatagatataagtaaaccagtcagactcatggaaggtcaaactcatgctcaagcagattatttgctagcattaaatagtctcaaattactgtataaagagtatgcaggaataggccacaaattaaaaggaactgagacttatatatcgagagatatgcaatttatgagtaaaacgatccaacataacggtgtatattacccagctagtataaagaaagtcctaagagtgggaccgtggataaacactatacttgatgacttcaaagtgagtctagaatctataggtagtttgacacaagaattagaatatagaggtgaaagtctattatgcagtttaatatttagaaatgtatggttatataatcaaattgcattacaacttaaaaatcatgcattatgtaacaacaaattatatttggatatattaaaagttctaaaacacttaaaaaccttttttaatcttgataacattgatacagcattaacattgtatatgaatttgcccatgttatttggtggtggtgatcccaacttgttatatcgaagtttctatagaagaactcctgatttcctcacagaggctatagttcactctgtgttcatacttagttattatacaaaccatgatttaaaagataaacttcaagatctgtcagatgatagattgaataagttcttaacatgcataatcacgtttgataaaaaccccaatgctgaattcgttacattgatgagagatcctcaagctttaggatctgagaggcaagctaaaattactagcgaaatcaatagactggcagttaccgaggttttgagcacagctccaaacaaaatattttccaaaagtgcacaacactataccactacagagatagatcttaatgatattatgcaaaatatagaacctacatatcctcacgggctaagagttgtttatgagagtttacccttttataaagcagagaaaatagtaaatcttatatccggtacaaaatctataactaacatactggaaaagacttctgccatagacttaacagatattgatagagccactgagatgatgaggaaaaacataactttgcttataaggatattaccattagattgtaacagagataaaagagaaatattgagtatggaaaacctaagtattactgaattaagcaaatacgttagagaaagatcttggtctttatccaatatagttggtgttacatcacccagtatcatgtatacaatggacataaaatatacaacaagcactatagctagtggcataatcatagagaaatataatgtcaacagtttaacacgtggtgagagaggacccactaaaccatgggttggttcatctacacaagagaaaaagacaatgccagtttataatagacaagttttaaccaaaaaacagagagatcaaatagatctattagcaaaattggattgggtgtatgcatctatagataacaaggatgaatttatggaggaacttagcataggaactcttgggttaacatatgagaaggccaaaaaattattcccacaatatttgagtgttaactatttgcatcgtcttacagtcagtagtagaccatgtgaattccctgcatctataccagcttatagaactacaaattatcactttgatactagccctattaatcgcatattaacagaaaagtatggtgatgaagatattgatatagtattccaaaactgtataagctttggccttagcttaatgtctgtagtagaacaatttactaatgtatgtcctaacagaattattctcatacccaagcttaatgagatacatttgatgaaacctcccatattcacaggcgatgttgatattcacaagttaaaacaagtgatacaaaaacaacatatgtttttaccagacaaaataagtttgactcaatatgtggaattattcttaagtaataaaacactcaaatctggatctaatgttaattctaatttaatattggcgcataagatatctgactattttcataatacttacattttgagtactaatttagctggacattggattcttattatacaacttatgaaagattctaagggtatttttgaaaaagattggggagagggatatataactgatcatatgttcattaatttgaaagttttcttcaatgcttataagacatatctcttgtgttttcataaaggttacggcagagcaaagctggagtgtgatatgaatacttcagatctcctatgtgtattggaattaatagacagtagttattggaagtctatgtctaaggtgtttttagaacaaaaagttatcaaatacattcttagccaggatgcaagtttacatagagtaaaaggatgtcatagcttcaaactatggtttcttaaacgtcttaatgtagcagaattcacagtttgcccttgggttgttaacatagattatcatccaacacatatgaaagcaatattaacttatattgatcttgttagaatgggattgataaatatagatagaatatacattaaaaataaacacaagttcaatgatgagttttatacttctaatctgttttacattaattataacttctcagataatactcatctattaactaaacatataaggattgctaattccgaattagaaagtaattacaacaaattatatcatcctacaccagaaaccctagaaaatatactaaccaatccggttaaaagtaatgagaaaaagacactgagtgactattgtataggtaaaaatgttgactcaataatgttaccatcgttatctaataagaagcttattaaatcgtctacaatgattagaaccaattacagcagacaagatttgtataatttatttcctacggttgtgattgataaaattatagatcattcaggtaatacagccaaatctaaccaactttacactactacttctcatcaaatatccttagtgcacaatagcacatcactttattgcatgcttccttggcatcatattaatagattcaattttgtatttagttctacaggttgtaaaattagtatagagtatattttaaaagatcttaaaattaaggatcctaattgtatagcattcataggtgaaggagcagggaatttattattgcgtacagtagtggaacttcatcctgatataagatatatttacagaagtctgaaagattgcaatgatcatagtttaccaattgagtttttaaggctgtacaatggacatatcaacattgattatggtgaaaatttgaccattcctgctacagatgcaaccaacaacattcattggtcttatttacatataaagtttgctgaacctatcagtctttttgtctgtgatgctgaattgcctgtaacagtcaactggagtaagattataatagagtggagcaagcatgtaagaaaatgcaagtactgttcttcagttaataaatgtacattgatagtaaaatatcatgctcaagatgatatcgatttcaaattagacaacataactatattaaaaacttatgtatgcttaggtagtaagttaaagggatctgaagtttacttagtccttacaataggtcctgcaaatgtgttcccagtatttaatgtagtacaaaatgctaaattgatactatcaagaactaaaaatttcatcatgcctaaaaaagctgataaagagtctattgatgcaaatattaagagtttgataccctttctttgttaccctataacaaaaaaaggaattaatactgcattgtctaaattaaagagtgttgttagtggagatatactatcatattctatagctggacgtaatgaagttttcagcaataaacttataaatcataagcatatgaacatcttaaagtggttcaatcatgttttaaatttcagatcaacagaattaaactataatcatttatatatggtagaatctacttatcctcatctaagtgaattgttaaacagcttgacaaccaatgaacttaaaaaactgattaaaatcacaggtagtttgttatacaacttttataatgaataatgagcaaaaatcttataacaaaaatagctacacactaacattgtattcaattatagttattgaaaattaataattatataatttttaataacttctagtgaactaatcctaaaattatcattttgatctaggaagaataagtttaaatccaaatctaattggtttatatgtatattaactaaattacgagatattagtttttgacactttttttctcgtggccggcatggtcccagcctcctcgctggcgccggctgggcaacatgcttcggcatggcgaatgggactagcataaccccttggggcctctaaacgggtcttgaggggttttttg

SEQ ID NO: 21 - DNA, 15131 bp, synthetic construct
  misc_feature 1..15131: note = antigenic cDNA encoding cRSVA_VSVG_S
  source 1..15131: mol_type = other DNA
taatacgactcactataggttttttcgcgtctgatgaggccgttaggccgaaactcctctccggagtcacgcgaaaaaatgcgtacaacaaacttgcgtaaaccaaaaaaatggggcaaataagaatttgataagtaccacttaaatttaactcctttggttagaggcgcgccatgggcagcaactcattgagtatgataaaagttagattgcaaaatctgtttgacaatgatgaagtagcattgttaaaaataacatgctatactgacaaattaatacagttaactaatgctttggctaaggcagttatacatacaatcaaattgaatggcattgtatttgtgcatgttattacaagtagtgatatttgccctaataataatattgtagtgaaatccaatttcacaacaatgccagtattacaaaatggaggttatatatgggaaatgatggaattaacacactgctctcaacctaatggcctaatagatgacaattgtgaaattaaattctccaaaaaactaagtgattcaacaatgaccaattatatgaatcaattatctgaattacttggatttgacctcaatccataaatcataataaatatcaactagcaaatcaatgtcactaacaccattagttaatataaaacttgacagaagataaaaatggggcaaataaatcaattcagccgacccaaccatggacacaacacacaatgataccacaccacaaagactgatgatcacagacatgaggccattatcgcttgagactataataacatctctaaccagagatatcataacacataaatttatatacttgataaatcatgaatgcatagtaagaaaacttgatgaaagacaggccacatttacatttctggtcaactatgaaatgaaactattgcacaaagtgggaagcactaaatataaaaaatatactgaatacaacacaaaatatggcactttccctatgccaatatttatcaatcatgatgggttcttagaatgcattggcattaagcctaccaagcacacacccataatatacaagtatgatctcaatccatgaatatcaaaccaagattcaaacaatccgaaataacaactttatgcataatcacactccatagtccaaatggagcctgaaaattatagttatttaaaattcctgcaggaaggagagacataagatgaaagatggggcaaatacaaaaatggctcttagcaaagtcaagttgaatgatacactcaacaaagatcaacttctatcatccagcaaatataccatccaacggagcacaggagacagcattgacactcctaattatgatgtgcagaaacacattaataagttatgtggcatgttattaatcacagaagatgctaatcataaattcactgggttaataggtatgttatatgctatgtctagattaggaagagaagacaccataaaaatactcaaagatgcgggatatcatgttaaggcaaatggagtggatgtaacaacacatcgtcaagacattaatgggaaagaaatgaaatttgaagtgttaacattagcaagcttaacaactgaaattcaaatcaacattgagatagaatctagaaaatcctacaaaaaaatgctaaaagaaatgggagaggtggctccagaatacaggcatgactctcctgattgtgggatgataatattatgtatagcggcattagtaataaccaaattagcagcaggagatagatcaggtcttacagctgtgattaggagagctaataatgtcctaaaaaatgaaatgaaacgttataaaggtttattacccaaggatatagccaacagcttctatgaagtgtttgaaaaatatcctcactttatagatgtttttgttcattttggtatagcacaatcttctaccagaggtggcagtagagttgaagggatttttgcaggattgtttatgaatgcctatggtgcagggcaagtgatgttacggtggggggtcttagcaaaatcagttaaaaacattatgttaggacacgctagtgtacaagcagaaatggaacaagttgtggaggtgtatgagtatgctcagaaattgggtggagaagcaggattctaccatatattgaacaacccaaaagcatcactattatctttgactcaatttcctcacttctctagtgtagtattgggcaatgctgctggcctaggcataatgggagaatacagaggtacaccaaggaatcaagatttatatgatgctgcaaaagcatatgctgaacaactcaaagaaaatggtgtgattaactacagtgtattagatttgacagcagaagaactagaggctatcaaacatcagcttaatccaaaagataatgatgtagagctttgagttaataaaaaagtggggcaaataaatcatcatggaaaagtttgctcctgaattccatggagaagatgcaaacaacagagccaccaaattcctagaatcaataaagggcaaattcacatcacccaaagatcccaagaaaaaagatagtatcatatctgtcaactcaatagatatagaagtaaccaaagaaagccctataacatcaaattcaaccattataaacccaataaatgagacagatgatactgtagggaacaagcccaattatcaaagaaagcctctagtaagtttcaaagaagaccctacgccaagtgataatcctttttcaaaactatacaaagaaaccatagaaacatttgataacaatgaagaagaatctagctattcatatgaagaaataaatgatcagacaaacgataatataacagcaagattagataggattgatgagaaattaagtgaaatactaggaatgcttcacacattagtagtagcgagtgcaggacccacatctgctcgggatggtataagagatgccatggttggtttaagagaagaaatgatagaaaaaatcagaactgaagcattaatgaccaatgacagactagaagctatggcaagactcaggaatgaagaaagtgaaaagatggcaaaagacacatcagatgaagtgtctctcaatccaacatcagagaaactgaacaacctgttggaagggaatgatagtgacaatgatctatcacttgaagatttctgattagctaccaaactgtacatcaaaacacaacaccaatagaaaaccaacaaacaaaccaactcacccatccaaccaaacatctatctgctgattagccaaccagccaaaaaacaaccagccaatctaaaactagccacccggaaaaaatcgatactatagttacaaaaaaagatggggcaaatatggaaacatacgtgaataaacttcacgagggctccacatacacagctgctgttcaatacaatgtcctagaaaaagacgatgatcctgcatcacttacaatatgggtgcccatgttccaatcatccatgccagcagatctactcataaaagaactagccaatgtcaatatactagtgaaacaaatatccacacccaagggaccctcattaagagtcatgataaactcaagaagtgcagtgctagcacaaatgcccagcaaatttaccatatgtgccaatgtgtccttggatgaaagaagcaagctggcatatgatgtaaccacaccctgtgaaattaaggcatgcagtctaacatgcctaaaatcaaaaaatatgttaactacagttaaagatctcactatgaaaacactcaacccaacacatgacatcattgctttatgtgaatttgaaaatatagtaacatcaaaaaaagtcataataccaacatacctaagatctatcagcgtcagaaataaagatctgaacacacttgaaaatataacaaccactgaattcaaaaatgccattacaaatgcaaaaatcatcccttactcaggattattgttagtcatcacagtgactgacaacaaaggagcattcaaatacataaagccacaaagtcaattcatagtagatcttggagcttacctagaaaaagaaagtatatattatgttacaacaaattggaagcacacagctacacgatttgcaatcaaacccatggaagattaacctttttcctctacatcaatgagtagattcatacaaactttctaactacattcttcacttcacaatcataatcaccaaccctctgtggttcaatcaatcaaacaaaactcatcaagagttccagatcatcccaagtcattgttcatcagatccagtactcaaataagttaataaaaaatccacatggggcaaataatcattgagggaaatccaactaatcacaacatctgtcaacatagacaagtcaacacgctagataaaatcaaccaatggaaaatacatccataactatagaattctcaagcaaattctggccttactttacactaatacacatgataacaacaataatctctttgataatcataatctccatcatgattgcaatactaaacaaactctgcgaatataatgtattccataacaaaacctttgagctaccaagagctcgagtcaatacatagcattcaccaatctgatagctcaaaacagtaaccttgcatttgtaaatgaactaccctcacttcttcacaaaaccacatcaacatctcaccatgcaagccatcatctataccataaagtagttaattaaaaatggccggccagtcataacaatgaactaggatattaagaccaaaaacaacgctggggcaaatgcaaacatgtccaaaaccgaggaccaacgcaccgccaagacactagaaaggacctgggacacttttaatcatctattattcatatcatcgtgcttatacaagttaaatcttaaatctatagcacaaatcacattatctattttggcaattataatctcaacctcacttataattgcagccatcatattcatagcctcggcaaaccacaaagtcacactaacaactgcaatcatacaagatgcaacgaaccagatcaagaacacaaccccaacatacctcacccagaatccccagcatggaatcagcttctccaatctgtccggaactacatcacaatccaccaccatactagcttcaacaacaccaagtgctgattcaaccccacaatccacaacagtcaagatcaaaaacacaacaacaacccaaatattacctagcaaacccaccacaaaacaacgccaaaataaaccacaaaacaaacccaacaatgattttcactttgaagtgttcaattttgtaccctgcagcatatgcagcaacaatccaacctgctgggccatctgcaagagaataccaaacaaaaaacctggaaagaaaaccaccaccaagcccacaaaaaaaccaaccctcaagacaaccaaaaaagatcccaaatcccaaaccacaaaaccaaaggaagtactcactaccaagcctacaggaaagccaaccatcaacaccactaaaacaaacatcagaactacactgctcacctccaacaccaaaggaaatccagaacacacaagtcaagaggaaaccctccactcaaccacctccgaaggctatccaagcccatcacaagtccacacaacatccggtcaagaggaaaccctccactcaaccacctccgaaggctatccaagcccatcacaagtctacacaacatccgagtacctatcacaatctctatcttcatccaacacaacaaaatgatagtcattaaaaagcacgcgtttgacagaagataaaaatggggcaaatgcaaacatgaagtgccttttgtacttagcctttttattcattggggtgaattgcaagttcaccatagtttttccacacaaccaaaaaggaaactggaaaaatgttccttctaattaccattattgcccgtcaagctcagatttaaattggcataatgacttaataggcacagccttacaagtcaaaatgcccaagagtcacaaggctattcaagcagacggttggatgtgtcatgcttccaaatgggtcactacttgtgatttccgctggtatggaccgaagtatataacacattccatccgatccttcactccatctgtagaacaatgcaaggaaagcattgaacaaacgaaacaaggaacttggctgaatccaggcttccctcctcaaagttgtggatatgcaactgtgacggatgccgaagcagtgattgtccaggtgactcctcaccatgtgctggttgatgaatacacaggagaatgggttgattcacagttcatcaacggaaaatgcagcaattacatatgccccactgtccataactctacaacctggcattctgactataaggtcaaagggctatgtgattctaacctcatttccatggacatcaccttcttctcagaggacggagagctatcatccctgggaaaggagggcacagggttcagaagtaactactttgcttatgaaactggaggcaaggcctgcaaaatgcaatactgcaagcattggggagtcagactcccatcaggtgtctggttcgagatggctgataaggatctctttgctgcagccagattccctgaatgcccagaagggtcaagtatctctgctccatctcagacctcagtggatgtaagtctaattcaggacgttgagaggatcttggattattccctctgccaagaaacctggagcaaaatcagagcgggtcttccaatctctccagtggatctcagctatcttgctcctaaaaacccaggaaccggtcctgctttcaccataatcaatggtaccctaaaatactttgagaccagatacatcagagtcgatattgctgctccaatcctctcaagaatggtcggaatgatcagtggaactaccacagaaagggaactgtgggatgactgggcaccatatgaagacgtggaaattggacccaatggagttctgaggaccagttcaggatataagtttcctttatacatgattggacatggtatgttggactccgatcttcatcttagctcaaaggctcaggtgttcgaacatcctcacattcaagacgctgcttcgcaacttcctgatgatgagagtttattttttggtgatactgggctatccaaaaatccaatcgagcttgtagaaggttggttcagtagttggaaaagctctattgcctcttttttctttatcatagggttaatcattggactattcttggttctccgagttggtatccatctttgcattaaagccagaagcacaccagtcacattaagtaaggatcaactgagtggtataaataatattgcatttagtaactaatagtcattaaaaagcgggcccattgaataccaaattaacttactatttgtaaaaatgagaattggggcaaatatgtcacgaaggaatccttgcaaattcgaaattcgaggtcattgcttgaatggtaaaaggtgtcattttagtcataattattttgaatggccaccccatgcactgcttgtaagacaaaactttatgttaaacagaatacttaagtctatggataaaagcatagatactttgtcagaaataagtggagctgcagagttggacagaacagaagagtatgccctcggtgtagttggagtgctagagagttatataggatcaataaataatataactaaacaatcagcatgtgttgccatgagcaaactccttactgaactcaacagcgatgacatcaaaaaactaagggacaatgaagagccaaactcacccaaagtaagagtgtacaatactgtcatatcatatattgaaagcaacaggaagaacaataaacaaactatccatctgttaaaaagattgccagcagacgtattgaagaaaaccatcaaaaacacattggatatccacaagagcataaccatcaataacccaaaagaatcaactgttagtgatacgaacgaccatgccaaaaataatgatactacctgacaaatatccttgtagtataaattccatactaataacaagtaattgtagagtcactatgtataatcaaaaaaacacactatatatcaatcaaaacaaccaaaatagccatatatacccaccggatcaaccattcaatgaaatccattggacctctcaagacttgattgatgcaactcaaaattttctacaacatctaggtattactgatgatatatacacaatatatatattagtgtcataatactcaatcctaatacttaccacatcatcaaattattaactcaaacaattcaagctatgggacaaaatggatcccattattagtggaaattctgctaatgtttatctaactgatagttatttaaaaggtgttatttctttctcagaatgtaacgctttaggaagttacatattcaatggtccttatctcaaaaatgattataccaacttaattagtagacaaaatccattaatagaacacataaatctaaagaaactaaatataacacagtccttaatatctaagtatcataaaggtgaaataaaaatagaagaacctacttactttcagtcattacttatgacatacaagagtatgacctcttcagaacagactactactactaatttacttaaaaagataataagaagagctatagaaatcagtgatgtcaaagtctatgctatattgaataaactggggctcaaagaaaaagacaagattaaatccaataatggacaagatgaagacaactcagtcattactaccataatcaaagatgatatacttttagctgtcaaggataatcaatctcatcttaaagcagacaaaaatcaatccacaaaacaaaaagatacaatcaaaacaacacttttgaagaaattaatgtgttcgatgcaacatcctccatcatggttaatacattggtttaatttatacacaaaattaaacagcatattaacacaatatcgatctagtgaggtaaaaaaccatggttttatattgatagataatcatactcttagtggattccaatttattttgaatcaatatggttgtatagtttatcataaggaactcaaaagaattactgtgacaacttataatcaattcttgacatggaaagatattagccttagtagattaaatgtttgtttgattacatggattagtaactgtttgaacacattaaacaaaagcttaggcttaagatgtggattcaataatgttatcttgacacaattattcctttatggagattgtatactaaaactattccacaatgaggggttctacataataaaagaggtagagggatttattatgtctctaattttaaatataacagaagaagatcaattcagaaaacggttttataatagtatgctcaacaacatcacagatgccgccaacaaagctcaaaaaaatctgctatcaagagtatgtcatacattattagataagacaatatcagataatataataaatggcagatggataattctattgagtaagttcctaaaattaattaagcttgcaggtgacaataacctcaacaatctgagtgaattatattttttgttcagaatatttggacacccaatggtagatgaaagacaagccatggatgctgttaaagttaattgcaacgagaccaaattttatttgttaagtagtttgagtatgttaagaggagcttttatatatagaattataaaagggtttgtaaataattacaacagatggcctactttaagaaatgccattgtcttacccttaagatggttaacttactataaactaaacacttatccttccttgttggaacttacagaaagagatttgattgttctatcaggactacgtttctatcgagagtttcggttgcctaaaaaagtggatcttgaaatgatcataaatgataaggctatatcacctcctaaaaatttaatatggactagtttccctagaaattatatgccgtcacacatacaaaattatatagaacatgaaaaattaaaattctctgatagtgataaatcaagaagagtattagagtattatttaagagataacaaattcaatgaatgtgatttacacaactgtgtagttaatcaaagttatcttaacaacccgaatcatgtggtatcattgacaggcaaagaaagagaactcagtgtaggtagaatgtttgcaatgcaaccaggaatgttcagacaagttcaaatattagcagagaaaatgatagcagaaaacatattacaatttttccctgaaagtcttacaagatatggtgatctagaactacagaaaatattagaattgaaagcaggaataagtaacaaatcaaatcgttacaatgataattacaacaattacattagtaagtgctctatcatcacagatctcagcaaattcaatcaagcatttcgatatgaaacatcatgtatttgtagtgatgtactggatgaactgcatggtgtacaatctctattttcctggttacatttaactattcctcatgtcacaataatatgcacatataggcatgcacccccctatataaaggatcatattgtagatcttaacaatgtagatgagcaaagtggactatatagatatcatatgggtggtatcgaagggtggtgtcaaaaactatggaccatagaagctatatcactattagatctaatatctctcaaagggaaattctcaattactgctttaattaatggtgacaatcaatcaatagatataagtaaaccagtcagactcatggaaggtcaaactcatgctcaagcagattatttgctagcattaaatagtctcaaattactgtataaagagtatgcaggaataggccacaaattaaaaggaactgagacttatatatcgagagatatgcaatttatgagtaaaacgatccaacataacggtgtatattacccagctagtataaagaaagtcctaagagtgggaccgtggataaacactatacttgatgacttcaaagtgagtctagaatctataggtagtttgacacaagaattagaatatagaggtgaaagtctattatgcagtttaatatttagaaatgtatggttatataatcaaattgcattacaacttaaaaatcatgcattatgtaacaacaaattatatttggatatattaaaagttctaaaacacttaaaaaccttttttaatcttgataacattgatacagcattaacattgtatatgaatttgcccatgttatttggtggtggtgatcccaacttgttatatcgaagtttctatagaagaactcctgatttcctcacagaggctatagttcactctgtgttcatacttagttattatacaaaccatgatttaaaagataaacttcaagatctgtcagatgatagattgaataagttcttaacatgcataatcacgtttgataaaaaccccaatgctgaattcgttacattgatgagagatcctcaagctttaggatctgagaggcaagctaaaattactagcgaaatcaatagactggcagttaccgaggttttgagcacagctccaaacaaaatattttccaaaagtgcacaacactataccactacagagatagatcttaatgatattatgcaaaatatagaacctacatatcctcacgggctaagagttgtttatgagagtttacccttttataaagcagagaaaatagtaaatcttatatccggtacaaaatctataactaacatactggaaaagacttctgccatagacttaacagatattgatagagccactgagatgatgaggaaaaacataactttgcttataaggatattaccattagattgtaacagagataaaagagaaatattgagtatggaaaacctaagtattactgaattaagcaaatacgttagagaaagatcttggtctttatccaatatagttggtgttacatcacccagtatcatgtatacaatggacataaaatatacaacaagcactatagctagtggcataatcatagagaaatataatgtcaacagtttaacacgtggtgagagaggacccactaaaccatgggttggttcatctacacaagagaaaaagacaatgccagtttataatagacaagttttaaccaaaaaacagagagatcaaatagatctattagcaaaattggattgggtgtatgcatctatagataacaaggatgaatttatggaggaacttagcataggaactcttgggttaacatatgagaaggccaaaaaattattcccacaatatttgagtgttaactatttgcatcgtcttacagtcagtagtagaccatgtgaattccctgcatctataccagcttatagaactacaaattatcactttgatactagccctattaatcgcatattaacagaaaagtatggtgatgaagatattgatatagtattccaaaactgtataagctttggccttagcttaatgtctgtagtagaacaatttactaatgtatgtcctaacagaattattctcatacccaagcttaatgagatacatttgatgaaacctcccatattcacaggcgatgttgatattcacaagttaaaacaagtgatacaaaaacaacatatgtttttaccagacaaaataagtttgactcaatatgtggaattattcttaagtaataaaacactcaaatctggatctaatgttaattctaatttaatattggcgcataagatatctgactattttcataatacttacattttgagtactaatttagctggacattggattcttattatacaacttatgaaagattctaagggtatttttgaaaaagattggggagagggatatataactgatcatatgttcattaatttgaaagttttcttcaatgcttataagacatatctcttgtgttttcataaaggttacggcagagcaaagctggagtgtgatatgaatacttcagatctcctatgtgtattggaattaatagacagtagttattggaagtctatgtctaaggtgtttttagaacaaaaagttatcaaatacattcttagccaggatgcaagtttacatagagtaaaaggatgtcatagcttcaaactatggtttcttaaacgtcttaatgtagcagaattcacagtttgcccttgggttgttaacatagattatcatccaacacatatgaaagcaatattaacttatattgatcttgttagaatgggattgataaatatagatagaatatacattaaaaataaacacaagttcaatgatgagttttatacttctaatctgttttacattaattataacttctcagataatactcatctattaactaaacatataaggattgctaattccgaattagaaagtaattacaacaaattatatcatcctacaccagaaaccctagaaaatatactaaccaatccggttaaaagtaatgagaaaaagacactgagtgactattgtataggtaaaaatgttgactcaataatgttaccatcgttatctaataagaagcttattaaatcgtctacaatgattagaaccaattacagcagacaagatttgtataatttatttcctacggttgtgattgataaaattatagatcattcaggtaatacagccaaatctaaccaactttacactactacttctcatcaaatatccttagtgcacaatagcacatcactttattgcatgcttccttggcatcatattaatagattcaattttgtatttagttctacaggttgtaaaattagtatagagtatattttaaaagatcttaaaattaaggatcctaattgtatagcattcataggtgaaggagcagggaatttattattgcgtacagtagtggaacttcatcctgatataagatatatttacagaagtctgaaagattgcaatgatcatagtttaccaattgagtttttaaggctgtacaatggacatatcaacattgattatggtgaaaatttgaccattcctgctacagatgcaaccaacaacattcattggtcttatttacatataaagtttgctgaacctatcagtctttttgtctgtgatgctgaattgcctgtaacagtcaactggagtaagattataatagagtggagcaagcatgtaagaaaatgcaagtactgttcttcagttaataaatgtacattgatagtaaaatatcatgctcaagatgatatcgatttcaaattagacaacataactatattaaaaacttatgtatgcttaggtagtaagttaaagggatctgaagtttacttagtccttacaataggtcctgcaaatgtgttcccagtatttaatgtagtacaaaatgctaaattgatactatcaagaactaaaaatttcatcatgcctaaaaaagctgataaagagtctattgatgcaaatattaagagtttgataccctttctttgttaccctataacaaaaaaaggaattaatactgcattgtctaaattaaagagtgttgttagtggagatatactatcatattctatagctggacgtaatgaagttttcagcaataaacttataaatcataagcatatgaacatcttaaagtggttcaatcatgttttaaatttcagatcaacagaattaaactataatcatttatatatggtagaatctacttatcctcatctaagtgaattgttaaacagcttgacaaccaatgaacttaaaaaactgattaaaatcacaggtagtttgttatacaacttttataatgaataatgagcaaaaatcttataacaaaaatagctacacactaacattgtattcaattatagttattgaaaattaataattatataatttttaataacttctagtgaactaatcctaaaattatcattttgatctaggaagaataagtttaaatccaaatctaattggtttatatgtatattaactaaattacgagatattagtttttgacactttttttctcgtggccggcatggtcccagcctcctcgctggcgccggctgggcaacatgcttcggcatggcgaatgggactagcataaccccttggggcctctaaacgggtcttgaggggttttttg

SEQ ID NO: 22 - DNA, 17006 bp, synthetic construct
  misc_feature 1..17006: note = antigenic cDNA encoding cRSVA_VSVG_A_preF_ef
  source 1..17006: mol_type = other DNA
taatacgactcactataggttttttcgcgtctgatgaggccgttaggccgaaactcctctccggagtcacgcgaaaaaatgcgtacaacaaacttgcgtaaaccaaaaaaatggggcaaataagaatttgataagtaccacttaaatttaactcctttggttagaggcgcgccatgggcagcaactcattgagtatgataaaagttagattgcaaaatctgtttgacaatgatgaagtagcattgttaaaaataacatgctatactgacaaattaatacagttaactaatgctttggctaaggcagttatacatacaatcaaattgaatggcattgtatttgtgcatgttattacaagtagtgatatttgccctaataataatattgtagtgaaatccaatttcacaacaatgccagtattacaaaatggaggttatatatgggaaatgatggaattaacacactgctctcaacctaatggcctaatagatgacaattgtgaaattaaattctccaaaaaactaagtgattcaacaatgaccaattatatgaatcaattatctgaattacttggatttgacctcaatccataaatcataataaatatcaactagcaaatcaatgtcactaacaccattagttaatataaaacttgacagaagataaaaatggggcaaataaatcaattcagccgacccaaccatggacacaacacacaatgataccacaccacaaagactgatgatcacagacatgaggccattatcgcttgagactataataacatctctaaccagagatatcataacacataaatttatatacttgataaatcatgaatgcatagtaagaaaacttgatgaaagacaggccacatttacatttctggtcaactatgaaatgaaactattgcacaaagtgggaagcactaaatataaaaaatatactgaatacaacacaaaatatggcactttccctatgccaatatttatcaatcatgatgggttcttagaatgcattggcattaagcctaccaagcacacacccataatatacaagtatgatctcaatccatgaatatcaaaccaagattcaaacaatccgaaataacaactttatgcataatcacactccatagtccaaatggagcctgaaaattatagttatttaaaattcctgcaggaaggagagacataagatgaaagatggggcaaatacaaaaatggctcttagcaaagtcaagttgaatgatacactcaacaaagatcaacttctatcatccagcaaatataccatccaacggagcacaggagacagcattgacactcctaattatgatgtgcagaaacacattaataagttatgtggcatgttattaatcacagaagatgctaatcataaattcactgggttaataggtatgttatatgctatgtctagattaggaagagaagacaccataaaaatactcaaagatgcgggatatcatgttaaggcaaatggagtggatgtaacaacacatcgtcaagacattaatgggaaagaaatgaaatttgaagtgttaacattagcaagcttaacaactgaaattcaaatcaacattgagatagaatctagaaaatcctacaaaaaaatgctaaaagaaatgggagaggtggctccagaatacaggcatgactctcctgattgtgggatgataatattatgtatagcggcattagtaataaccaaattagcagcaggagatagatcaggtcttacagctgtgattaggagagctaataatgtcctaaaaaatgaaatgaaacgttataaaggtttattacccaaggatatagccaacagcttctatgaagtgtttgaaaaatatcctcactttatagatgtttttgttcattttggtatagcacaatcttctaccagaggtggcagtagagttgaagggatttttgcaggattgtttatgaatgcctatggtgcagggcaagtgatgttacggtggggggtcttagcaaaatcagttaaaaacattatgttaggacacgctagtgtacaagcagaaatggaacaagttgtggaggtgtatgagtatgctcagaaattgggtggagaagcaggattctaccatatattgaacaacccaaaagcatcactattatctttgactcaatttcctcacttctctagtgtagtattgggcaatgctgctggcctaggcataatgggagaatacagaggtacaccaaggaatcaagatttatatgatgctgcaaaagcatatgctgaacaactcaaagaaaatggtgtgattaactacagtgtattagatttgacagcagaagaactagaggctatcaaacatcagcttaatccaaaagataatgatgtagagctttgagttaataaaaaagtggggcaaataaatcatcatggaaaagtttgctcctgaattccatggagaagatgcaaacaacagagccaccaaattcctagaatcaataaagggcaaattcacatcacccaaagatcccaagaaaaaagatagtatcatatctgtcaactcaatagatatagaagtaaccaaagaaagccctataacatcaaattcaaccattataaacccaataaatgagacagatgatactgtagggaacaagcccaattatcaaagaaagcctctagtaagtttcaaagaagaccctacgccaagtgataatcctttttcaaaactatacaaagaaaccatagaaacatttgataacaatgaagaagaatctagctattcatatgaagaaataaatgatcagacaaacgataatataacagcaagattagataggattgatgagaaattaagtgaaatactaggaatgcttcacacattagtagtagcgagtgcaggacccacatctgctcgggatggtataagagatgccatggttggtttaagagaagaaatgatagaaaaaatcagaactgaagcattaatgaccaatgacagactagaagctatggcaagactcaggaatgaagaaagtgaaaagatggcaaaagacacatcagatgaagtgtctctcaatccaacatcagagaaactgaacaacctgttggaagggaatgatagtgacaatgatctatcacttgaagatttctgattagctaccaaactgtacatcaaaacacaacaccaatagaaaaccaacaaacaaaccaactcacccatccaaccaaacatctatctgctgattagccaaccagccaaaaaacaaccagccaatctaaaactagccacccggaaaaaatcgatactatagttacaaaaaaagatggggcaaatatggaaacatacgtgaataaacttcacgagggctccacatacacagctgctgttcaatacaatgtcctagaaaaagacgatgatcctgcatcacttacaatatgggtgcccatgttccaatcatccatgccagcagatctactcataaaagaactagccaatgtcaatatactagtgaaacaaatatccacacccaagggaccctcattaagagtcatgataaactcaagaagtgcagtgctagcacaaatgcccagcaaatttaccatatgtgccaatgtgtccttggatgaaagaagcaagctggcatatgatgtaaccacaccctgtgaaattaaggcatgcagtctaacatgcctaaaatcaaaaaatatgttaactacagttaaagatctcactatgaaaacactcaacccaacacatgacatcattgctttatgtgaatttgaaaatatagtaacatcaaaaaaagtcataataccaacatacctaagatctatcagcgtcagaaataaagatctgaacacacttgaaaatataacaaccactgaattcaaaaatgccattacaaatgcaaaaatcatcccttactcaggattattgttagtcatcacagtgactgacaacaaaggagcattcaaatacataaagccacaaagtcaattcatagtagatcttggagcttacctagaaaaagaaagtatatattatgttacaacaaattggaagcacacagctacacgatttgcaatcaaacccatggaagattaacctttttcctctacatcaatgagtagattcatacaaactttctaactacattcttcacttcacaatcataatcaccaaccctctgtggttcaatcaatcaaacaaaactcatcaagagttccagatcatcccaagtcattgttcatcagatccagtactcaaataagttaataaaaaatccacatggggcaaataatcattgagggaaatccaactaatcacaacatctgtcaacatagacaagtcaacacgctagataaaatcaaccaatggaaaatacatccataactatagaattctcaagcaaattctggccttactttacactaatacacatgataacaacaataatctctttgataatcataatctccatcatgattgcaatactaaacaaactctgcgaatataatgtattccataacaaaacctttgagctaccaagagctcgagtcaatacatagcattcaccaatctgatagctcaaaacagtaaccttgcatttgtaaatgaactaccctcacttcttcacaaaaccacatcaacatctcaccatgcaagccatcatctataccataaagtagttaattaaaaatggccggccagtcataacaatgaactaggatattaagaccaaaaacaacgctggggcaaatgcaaacatgtccaaaaccgaggaccaacgcaccgccaagacactagaaaggacctgggacacttttaatcatctattattcatatcatcgtgcttatacaagttaaatcttaaatctatagcacaaatcacattatctattttggcaattataatctcaacctcacttataattgcagccatcatattcatagcctcggcaaaccacaaagtcacactaacaactgcaatcatacaagatgcaacgaaccagatcaagaacacaaccccaacatacctcacccagaatccccagcatggaatcagcttctccaatctgtccggaactacatcacaatccaccaccatactagcttcaacaacaccaagtgctgattcaaccccacaatccacaacagtcaagatcaaaaacacaacaacaacccaaatattacctagcaaacccaccacaaaacaacgccaaaataaaccacaaaacaaacccaacaatgattttcactttgaagtgttcaattttgtaccctgcagcatatgcagcaacaatccaacctgctgggccatctgcaagagaataccaaacaaaaaacctggaaagaaaaccaccaccaagcccacaaaaaaaccaaccctcaagacaaccaaaaaagatcccaaatcccaaaccacaaaaccaaaggaagtactcactaccaagcctacaggaaagccaaccatcaacaccactaaaacaaacatcagaactacactgctcacctccaacaccaaaggaaatccagaacacacaagtcaagaggaaaccctccactcaaccacctccgaaggctatccaagcccatcacaagtccacacaacatccggtcaagaggaaaccctccactcaaccacctccgaaggctatccaagcccatcacaagtctacacaacatccgagtacctatcacaatctctatcttcatccaacacaacaaaatgatagtcattaaaaagcacgcgtttgacagaagataaaaatggggcaaatgcaaacatgaagtgccttttgtacttagcctttttattcattggggtgaattgcaagttcaccatagtttttccacacaaccaaaaaggaaactggaaaaatgttccttctaattaccattattgcccgtcaagctcagatttaaattggcataatgacttaataggcacagccttacaagtcaaaatgcccaagagtcacaaggctattcaagcagacggttggatgtgtcatgcttccaaatgggtcactacttgtgatttccgctggtatggaccgaagtatataacacattccatccgatccttcactccatctgtagaacaatgcaaggaaagcattgaacaaacgaaacaaggaacttggctgaatccaggcttccctcctcaaagttgtggatatgcaactgtgacggatgccgaagcagtgattgtccaggtgactcctcaccatgtgctggttgatgaatacacaggagaatgggttgattcacagttcatcaacggaaaatgcagcaattacatatgccccactgtccataactctacaacctggcattctgactataaggtcaaagggctatgtgattctaacctcatttccatggacatcaccttcttctcagaggacggagagctatcatccctgggaaaggagggcacagggttcagaagtaactactttgcttatgaaactggaggcaaggcctgcaaaatgcaatactgcaagcattggggagtcagactcccatcaggtgtctggttcgagatggctgataaggatctctttgctgcagccagattccctgaatgcccagaagggtcaagtatctctgctccatctcagacctcagtggatgtaagtctaattcaggacgttgagaggatcttggattattccctctgccaagaaacctggagcaaaatcagagcgggtcttccaatctctccagtggatctcagctatcttgctcctaaaaacccaggaaccggtcctgctttcaccataatcaatggtaccctaaaatactttgagaccagatacatcagagtcgatattgctgctccaatcctctcaagaatggtcggaatgatcagtggaactaccacagaaagggaactgtgggatgactgggcaccatatgaagacgtggaaattggacccaatggagttctgaggaccagttcaggatataagtttcctttatacatgattggacatggtatgttggactccgatcttcatcttagctcaaaggctcaggtgttcgaacatcctcacattcaagacgctgcttcgcaacttcctgatgatgagagtttattttttggtgatactgggctatccaaaaatccaatcgagcttgtagaaggttggttcagtagttggaaaagctctattgcctcttttttctttatcatagggttaatcattggactattcttggttctccgagttggtatccatctttgcattaaagccagaagcacaccagtcacattaagtaaggatcaactgagtggtataaataatattgcatttagtaactaatagtcattaaaaagcgggcccgtattgttgcaaaaagccatgaccaaatcaaacagaatcaaaatcaactctggggcaaataacaatggagttgccaatcctcaaaacaaatgctattaccacaatccttgctgcagtcacactctgtttcgcttccagtcaaaacatcactgaagaattttatcaatcaacatgcagtgcagtcagcaaaggctatcttagtgctctaagaactggttggtatactagtgttataactatagaattaagtaatatcaaggaaaataagtgtaatggtacagacgctaaggtaaaattaataaaacaagaattagataaatataaaaatgctgtaacagaattgcagttgctcatgcaaagcacaccagcagccaacaatcgagccagaagagaactaccaagatttatgaattatacactcaacaataccaaaaacaccaatgtaacattaagtaagaaaaggaaaagaagatttcttggatttttgttaggtgttggatctgcaatcgccagtggcattgccgtatccaaggtcctgcacctagaaggggaagtgaacaaaatcaaaagtgctctactatccacaaacaaggctgtagtcagcttatctaatggagtcagtgtcttaaccagcaaggtgttagacctcaaaaactatatagataaacagttgttacctattgttaacaagcaaagctgcagcatatcaaacattgaaactgtgatagagttccaacaaaagaacaacagactactagagattaccagagaatttagtgttaatgcaggtgtaactactcctgtaagcacttatatgttaactaatagtgagttattatcattaatcaatgatatgcctataacaaatgatcagaaaaagttaatgtccagcaatgttcaaatagttagacagcaaagttactctatcatgtcaataataaaagaggaagtcttggcatatgtagtacaattaccactatatggtgtaatagatactccttgttggaaactacacacatcccctttatgtacaaccaacacaaaggaaggatccaacatctgcttaacaagaaccgacagaggatggtactgtgacaatgcaggatcagtatcctttttcccacaagctgaaacatgtaaagttcaatcgaatcgggtgttttgtgacacaatgaacagtttaacattaccaagtgaggtaaatctctgcaacattgacatattcaaccccaaatatgattgcaaaattatgacttcaaaaacagatgtaagcagctccgttatcacatctctaggagccattgtgtcatgctatggcaaaaccaaatgtacagcatccaataaaaatcgtgggatcataaagacattctctaacgggtgtgattatgtatcaaataagggggtggatactgtgtctgtaggtaatacattatattatgtaaataagcaagaaggcaaaagtctctatgtaaaaggtgaaccaataataaatttctatgatccattagtgttcccctctctcctgtgggatgcatcaatatctcaagtcaatgagaaaattaatcagagtctagcatttatccgtaaatcagatgaattattaggctctggcggaagcggatacatccctgaggcaccaagggacggacaggcctacgtgcgcaaggatggcgagtgggtgctgctgtccacctttctgtgaataaaaatagcacctaatcatattcttacaatggttcgctatttgaccatagataacccatctatcattagattatcctaaaatttgaacttcatcacaactttcatctataaaccatctcacttacactttttaagtagatttctattttatagttatataaaacagggcccattgaataccaaattaacttactatttgtaaaaatgagaattggggcaaatatgtcacgaaggaatccttgcaaattcgaaattcgaggtcattgcttgaatggtaaaaggtgtcattttagtcataattattttgaatggccaccccatgcactgcttgtaagacaaaactttatgttaaacagaatacttaagtctatggataaaagcatagatactttgtcagaaataagtggagctgcagagttggacagaacagaagagtatgccctcggtgtagttggagtgctagagagttatataggatcaataaataatataactaaacaatcagcatgtgttgccatgagcaaactccttactgaactcaacagcgatgacatcaaaaaactaagggacaatgaagagccaaactcacccaaagtaagagtgtacaatactgtcatatcatatattgaaagcaacaggaagaacaataaacaaactatccatctgttaaaaagattgccagcagacgtattgaagaaaaccatcaaaaacacattggatatccacaagagcataaccatcaataacccaaaagaatcaactgttagtgatacgaacgaccatgccaaaaataatgatactacctgacaaatatccttgtagtataaattccatactaataacaagtaattgtagagtcactatgtataatcaaaaaaacacactatatatcaatcaaaacaaccaaaatagccatatatacccaccggatcaaccattcaatgaaatccattggacctctcaagacttgattgatgcaactcaaaattttctacaacatctaggtattactgatgatatatacacaatatatatattagtgtcataatactcaatcctaatacttaccacatcatcaaattattaactcaaacaattcaagctatgggacaaaatggatcccattattagtggaaattctgctaatgtttatctaactgatagttatttaaaaggtgttatttctttctcagaatgtaacgctttaggaagttacatattcaatggtccttatctcaaaaatgattataccaacttaattagtagacaaaatccattaatagaacacataaatctaaagaaactaaatataacacagtccttaatatctaagtatcataaaggtgaaataaaaatagaagaacctacttactttcagtcattacttatgacatacaagagtatgacctcttcagaacagactactactactaatttacttaaaaagataataagaagagctatagaaatcagtgatgtcaaagtctatgctatattgaataaactggggctcaaagaaaaagacaagattaaatccaataatggacaagatgaagacaactcagtcattactaccataatcaaagatgatatacttttagctgtcaaggataatcaatctcatcttaaagcagacaaaaatcaatccacaaaacaaaaagatacaatcaaaacaacacttttgaagaaattaatgtgttcgatgcaacatcctccatcatggttaatacattggtttaatttatacacaaaattaaacagcatattaacacaatatcgatctagtgaggtaaaaaaccatggttttatattgatagataatcatactcttagtggattccaatttattttgaatcaatatggttgtatagtttatcataaggaactcaaaagaattactgtgacaacttataatcaattcttgacatggaaagatattagccttagtagattaaatgtttgtttgattacatggattagtaactgtttgaacacattaaacaaaagcttaggcttaagatgtggattcaataatgttatcttgacacaattattcctttatggagattgtatactaaaactattccacaatgaggggttctacataataaaagaggtagagggatttattatgtctctaattttaaatataacagaagaagatcaattcagaaaacggttttataatagtatgctcaacaacatcacagatgccgccaacaaagctcaaaaaaatctgctatcaagagtatgtcatacattattagataagacaatatcagataatataataaatggcagatggataattctattgagtaagttcctaaaattaattaagcttgcaggtgacaataacctcaacaatctgagtgaattatattttttgttcagaatatttggacacccaatggtagatgaaagacaagccatggatgctgttaaagttaattgcaacgagaccaaattttatttgttaagtagtttgagtatgttaagaggagcttttatatatagaattataaaagggtttgtaaataattacaacagatggcctactttaagaaatgccattgtcttacccttaagatggttaacttactataaactaaacacttatccttccttgttggaacttacagaaagagatttgattgttctatcaggactacgtttctatcgagagtttcggttgcctaaaaaagtggatcttgaaatgatcataaatgataaggctatatcacctcctaaaaatttaatatggactagtttccctagaaattatatgccgtcacacatacaaaattatatagaacatgaaaaattaaaattctctgatagtgataaatcaagaagagtattagagtattatttaagagataacaaattcaatgaatgtgatttacacaactgtgtagttaatcaaagttatcttaacaacccgaatcatgtggtatcattgacaggcaaagaaagagaactcagtgtaggtagaatgtttgcaatgcaaccaggaatgttcagacaagttcaaatattagcagagaaaatgatagcagaaaacatattacaatttttccctgaaagtcttacaagatatggtgatctagaactacagaaaatattagaattgaaagcaggaataagtaacaaatcaaatcgttacaatgataattacaacaattacattagtaagtgctctatcatcacagatctcagcaaattcaatcaagcatttcgatatgaaacatcatgtatttgtagtgatgtactggatgaactgcatggtgtacaatctctattttcctggttacatttaactattcctcatgtcacaataatatgcacatataggcatgcacccccctatataaaggatcatattgtagatcttaacaatgtagatgagcaaagtggactatatagatatcatatgggtggtatcgaagggtggtgtcaaaaactatggaccatagaagctatatcactattagatctaatatctctcaaagggaaattctcaattactgctttaattaatggtgacaatcaatcaatagatataagtaaaccagtcagactcatggaaggtcaaactcatgctcaagcagattatttgctagcattaaatagtctcaaattactgtataaagagtatgcaggaataggccacaaattaaaaggaactgagacttatatatcgagagatatgcaatttatgagtaaaacgatccaacataacggtgtatattacccagctagtataaagaaagtcctaagagtgggaccgtggataaacactatacttgatgacttcaaagtgagtctagaatctataggtagtttgacacaagaattagaatatagaggtgaaagtctattatgcagtttaatatttagaaatgtatggttatataatcaaattgcattacaacttaaaaatcatgcattatgtaacaacaaattatatttggatatattaaaagttctaaaacacttaaaaaccttttttaatcttgataacattgatacagcattaacattgtatatgaatttgcccatgttatttggtggtggtgatcccaacttgttatatcgaagtttctatagaagaactcctgatttcctcacagaggctatagttcactctgtgttcatacttagttattatacaaaccatgatttaaaagataaacttcaagatctgtcagatgatagattgaataagttcttaacatgcataatcacgtttgataaaaaccccaatgctgaattcgttacattgatgagagatcctcaagctttaggatctgagaggcaagctaaaattactagcgaaatcaatagactggcagttaccgaggttttgagcacagctccaaacaaaatattttccaaaagtgcacaacactataccactacagagatagatcttaatgatattatgcaaaatatagaacctacatatcctcacgggctaagagttgtttatgagagtttacccttttataaagcagagaaaatagtaaatcttatatccggtacaaaatctataactaacatactggaaaagacttctgccatagacttaacagatattgatagagccactgagatgatgaggaaaaacataactttgcttataaggatattaccattagattgtaacagagataaaagagaaatattgagtatggaaaacctaagtattactgaattaagcaaatacgttagagaaagatcttggtctttatccaatatagttggtgttacatcacccagtatcatgtatacaatggacataaaatatacaacaagcactatagctagtggcataatcatagagaaatataatgtcaacagtttaacacgtggtgagagaggacccactaaaccatgggttggttcatctacacaagagaaaaagacaatgccagtttataatagacaagttttaaccaaaaaacagagagatcaaatagatctattagcaaaattggattgggtgtatgcatctatagataacaaggatgaatttatggaggaacttagcataggaactcttgggttaacatatgagaaggccaaaaaattattcccacaatatttgagtgttaactatttgcatcgtcttacagtcagtagtagaccatgtgaattccctgcatctataccagcttatagaactacaaattatcactttgatactagccctattaatcgcatattaacagaaaagtatggtgatgaagatattgatatagtattccaaaactgtataagctttggccttagcttaatgtctgtagtagaacaatttactaatgtatgtcctaacagaattattctcatacccaagcttaatgagatacatttgatgaaacctcccatattcacaggcgatgttgatattcacaagttaaaacaagtgatacaaaaacaacatatgtttttaccagacaaaataagtttgactcaatatgtggaattattcttaagtaataaaacactcaaatctggatctaatgttaattctaatttaatattggcgcataagatatctgactattttcataatacttacattttgagtactaatttagctggacattggattcttattatacaacttatgaaagattctaagggtatttttgaaaaagattggggagagggatatataactgatcatatgttcattaatttgaaagttttcttcaatgcttataagacatatctcttgtgttttcataaaggttacggcagagcaaagctggagtgtgatatgaatacttcagatctcctatgtgtattggaattaatagacagtagttattggaagtctatgtctaaggtgtttttagaacaaaaagttatcaaatacattcttagccaggatgcaagtttacatagagtaaaaggatgtcatagcttcaaactatggtttcttaaacgtcttaatgtagcagaattcacagtttgcccttgggttgttaacatagattatcatccaacacatatgaaagcaatattaacttatattgatcttgttagaatgggattgataaatatagatagaatatacattaaaaataaacacaagttcaatgatgagttttatacttctaatctgttttacattaattataacttctcagataatactcatctattaactaaacatataaggattgctaattccgaattagaaagtaattacaacaaattatatcatcctacaccagaaaccctagaaaatatactaaccaatccggttaaaagtaatgagaaaaagacactgagtgactattgtataggtaaaaatgttgactcaataatgttaccatcgttatctaataagaagcttattaaatcgtctacaatgattagaaccaattacagcagacaagatttgtataatttatttcctacggttgtgattgataaaattatagatcattcaggtaatacagccaaatctaaccaactttacactactacttctcatcaaatatccttagtgcacaatagcacatcactttattgcatgcttccttggcatcatattaatagattcaattttgtatttagttctacaggttgtaaaattagtatagagtatattttaaaagatcttaaaattaaggatcctaattgtatagcattcataggtgaaggagcagggaatttattattgcgtacagtagtggaacttcatcctgatataagatatatttacagaagtctgaaagattgcaatgatcatagtttaccaattgagtttttaaggctgtacaatggacatatcaacattgattatggtgaaaatttgaccattcctgctacagatgcaaccaacaacattcattggtcttatttacatataaagtttgctgaacctatcagtctttttgtctgtgatgctgaattgcctgtaacagtcaactggagtaagattataatagagtggagcaagcatgtaagaaaatgcaagtactgttcttcagttaataaatgtacattgatagtaaaatatcatgctcaagatgatatcgatttcaaattagacaacataactatattaaaaacttatgtatgcttaggtagtaagttaaagggatctgaagtttacttagtccttacaataggtcctgcaaatgtgttcccagtatttaatgtagtacaaaatgctaaattgatactatcaagaactaaaaatttcatcatgcctaaaaaagctgataaagagtctattgatgcaaatattaagagtttgataccctttctttgttaccctataacaaaaaaaggaattaatactgcattgtctaaattaaagagtgttgttagtggagatatactatcatattctatagctggacgtaatgaagttttcagcaataaacttataaatcataagcatatgaacatcttaaagtggttcaatcatgttttaaatttcagatcaacagaattaaactataatcatttatatatggtagaatctacttatcctcatctaagtgaattgttaaacagcttgacaaccaatgaacttaaaaaactgattaaaatcacaggtagtttgttatacaacttttataatgaataatgagcaaaaatcttataacaaaaatagctacacactaacattgtattcaattatagttattgaaaattaataattatataatttttaataacttctagtgaactaatcctaaaattatcattttgatctaggaagaataagtttaaatccaaatctaattggtttatatgtatattaactaaattacgagatattagtttttgacactttttttctcgtggccggcatggtcccagcctcctcgctggcgccggctgggcaacatgcttcggcatggcgaatgggactagcataaccccttggggcctctaaacgggtcttgaggggttttttg

SEQ ID NO: 23 - DNA, 16010 bp, synthetic construct
  misc_feature 1..16010: note = antigenic cDNA encoding cRSVA_VSVG_S_preF_ef
  source 1..16010: mol_type = other DNA
taatacgactcactataggttttttcgcgtctgatgaggccgttaggccgaaactcctctccggagtcacgcgaaaaaatgcgtacaacaaacttgcgtaaaccaaaaaaatggggcaaataagaatttgataagtaccacttaaatttaactcctttggttagaggcgcgccatgggcagcaactcattgagtatgataaaagttagattgcaaaatctgtttgacaatgatgaagtagcattgttaaaaataacatgctatactgacaaattaatacagttaactaatgctttggctaaggcagttatacatacaatcaaattgaatggcattgtatttgtgcatgttattacaagtagtgatatttgccctaataataatattgtagtgaaatccaatttcacaacaatgccagtattacaaaatggaggttatatatgggaaatgatggaattaacacactgctctcaacctaatggcctaatagatgacaattgtgaaattaaattctccaaaaaactaagtgattcaacaatgaccaattatatgaatcaattatctgaattacttggatttgacctcaatccataaatcataataaatatcaactagcaaatcaatgtcactaacaccattagttaatataaaacttgacagaagataaaaatggggcaaataaatcaattcagccgacccaaccatggacacaacacacaatgataccacaccacaaagactgatgatcacagacatgaggccattatcgcttgagactataataacatctctaaccagagatatcataacacataaatttatatacttgataaatcatgaatgcatagtaagaaaacttgatgaaagacaggccacatttacatttctggtcaactatgaaatgaaactattgcacaaagtgggaagcactaaatataaaaaatatactgaatacaacacaaaatatggcactttccctatgccaatatttatcaatcatgatgggttcttagaatgcattggcattaagcctaccaagcacacacccataatatacaagtatgatctcaatccatgaatatcaaaccaagattcaaacaatccgaaataacaactttatgcataatcacactccatagtccaaatggagcctgaaaattatagttatttaaaattcctgcaggaaggagagacataagatgaaagatggggcaaatacaaaaatggctcttagcaaagtcaagttgaatgatacactcaacaaagatcaacttctatcatccagcaaatataccatccaacggagcacaggagacagcattgacactcctaattatgatgtgcagaaacacattaataagttatgtggcatgttattaatcacagaagatgctaatcataaattcactgggttaataggtatgttatatgctatgtctagattaggaagagaagacaccataaaaatactcaaagatgcgggatatcatgttaaggcaaatggagtggatgtaacaacacatcgtcaagacattaatgggaaagaaatgaaatttgaagtgttaacattagcaagcttaacaactgaaattcaaatcaacattgagatagaatctagaaaatcctacaaaaaaatgctaaaagaaatgggagaggtggctccagaatacaggcatgactctcctgattgtgggatgataatattatgtatagcggcattagtaataaccaaattagcagcaggagatagatcaggtcttacagctgtgattaggagagctaataatgtcctaaaaaatgaaatgaaacgttataaaggtttattacccaaggatatagccaacagcttctatgaagtgtttgaaaaatatcctcactttatagatgtttttgttcattttggtatagcacaatcttctaccagaggtggcagtagagttgaagggatttttgcaggattgtttatgaatgcctatggtgcagggcaagtgatgttacggtggggggtcttagcaaaatcagttaaaaacattatgttaggacacgctagtgtacaagcagaaatggaacaagttgtggaggtgtatgagtatgctcagaaattgggtggagaagcaggattctaccatatattgaacaacccaaaagcatcactattatctttgactcaatttcctcacttctctagtgtagtattgggcaatgctgctggcctaggcataatgggagaatacagaggtacaccaaggaatcaagatttatatgatgctgcaaaagcatatgctgaacaactcaaagaaaatggtgtgattaactacagtgtattagatttgacagcagaagaactagaggctatcaaacatcagcttaatccaaaagataatgatgtagagctttgagttaataaaaaagtggggcaaataaatcatcatggaaaagtttgctcctgaattccatggagaagatgcaaacaacagagccaccaaattcctagaatcaataaagggcaaattcacatcacccaaagatcccaagaaaaaagatagtatcatatctgtcaactcaatagatatagaagtaaccaaagaaagccctataacatcaaattcaaccattataaacccaataaatgagacagatgatactgtagggaacaagcccaattatcaaagaaagcctctagtaagtttcaaagaagaccctacgccaagtgataatcctttttcaaaactatacaaagaaaccatagaaacatttgataacaatgaagaagaatctagctattcatatgaagaaataaatgatcagacaaacgataatataacagcaagattagataggattgatgagaaattaagtgaaatactaggaatgcttcacacattagtagtagcgagtgcaggacccacatctgctcgggatggtataagagatgccatggttggtttaagagaagaaatgatagaaaaaatcagaactgaagcattaatgaccaatgacagactagaagctatggcaagactcaggaatgaagaaagtgaaaagatggcaaaagacacatcagatgaagtgtctctcaatccaacatcagagaaactgaacaacctgttggaagggaatgatagtgacaatgatctatcacttgaagatttctgattagctaccaaactgtacatcaaaacacaacaccaatagaaaaccaacaaacaaaccaactcacccatccaaccaaacatctatctgctgattagccaaccagccaaaaaacaaccagccaatctaaaactagccacccggaaaaaatcgatactatagttacaaaaaaagatggggcaaatatggaaacatacgtgaataaacttcacgagggctccacatacacagctgctgttcaatacaatgtcctagaaaaagacgatgatcctgcatcacttacaatatgggtgcccatgttccaatcatccatgccagcagatctactcataaaagaactagccaatgtcaatatactagtgaaacaaatatccacacccaagggaccctcattaagagtcatgataaactcaagaagtgcagtgctagcacaaatgcccagcaaatttaccatatgtgccaatgtgtccttggatgaaagaagcaagctggcatatgatgtaaccacaccctgtgaaattaaggcatgcagtctaacatgcctaaaatcaaaaaatatgttaactacagttaaagatctcactatgaaaacactcaacccaacacatgacatcattgctttatgtgaatttgaaaatatagtaacatcaaaaaaagtcataataccaacatacctaagatctatcagcgtcagaaataaagatctgaacacacttgaaaatataacaaccactgaattcaaaaatgccattacaaatgcaaaaatcatcccttactcaggattattgttagtcatcacagtgactgacaacaaaggagcattcaaatacataaagccacaaagtcaattcatagtagatcttggagcttacctagaaaaagaaagtatatattatgttacaacaaattggaagcacacagctacacgatttgcaatcaaacccatggaagattaacctttttcctctacatcaatgagtagattcatacaaactttctaactacattcttcacttcacaatcataatcaccaaccctctgtggttcaatcaatcaaacaaaactcatcaagagttccagatcatcccaagtcattgttcatcagatccagtactcaaataagttaataaaaaatccacatggggcaaataatcattgagggaaatccaactaatcacaacatctgtcaacatagacaagtcaacacgctagataaaatcaaccaatggaaaatacatccataactatagaattctcaagcaaattctggccttactttacactaatacacatgataacaacaataatctctttgataatcataatctccatcatgattgcaatactaaacaaactctgcgaatataatgtattccataacaaaacctttgagctaccaagagctcgagtcaatacatagcattcaccaatctgatagctcaaaacagtaaccttgcatttgtaaatgaactaccctcacttcttcacaaaaccacatcaacatctcaccatgcaagccatcatctataccataaagtagttaattaaaaatggccggccagtcataacaatgaactaggatattaagaccaaaaacaacgctacgcgtttgacagaagataaaaatggggcaaatgcaaacatgaagtgccttttgtacttagcctttttattcattggggtgaattgcaagttcaccatagtttttccacacaaccaaaaaggaaactggaaaaatgttccttctaattaccattattgcccgtcaagctcagatttaaattggcataatgacttaataggcacagccttacaagtcaaaatgcccaagagtcacaaggctattcaagcagacggttggatgtgtcatgcttccaaatgggtcactacttgtgatttccgctggtatggaccgaagtatataacacattccatccgatccttcactccatctgtagaacaatgcaaggaaagcattgaacaaacgaaacaaggaacttggctgaatccaggcttccctcctcaaagttgtggatatgcaactgtgacggatgccgaagcagtgattgtccaggtgactcctcaccatgtgctggttgatgaatacacaggagaatgggttgattcacagttcatcaacggaaaatgcagcaattacatatgccccactgtccataactctacaacctggcattctgactataaggtcaaagggctatgtgattctaacctcatttccatggacatcaccttcttctcagaggacggagagctatcatccctgggaaaggagggcacagggttcagaagtaactactttgcttatgaaactggaggcaaggcctgcaaaatgcaatactgcaagcattggggagtcagactcccatcaggtgtctggttcgagatggctgataaggatctctttgctgcagccagattccctgaatgcccagaagggtcaagtatctctgctccatctcagacctcagtggatgtaagtctaattcaggacgttgagaggatcttggattattccctctgccaagaaacctggagcaaaatcagagcgggtcttccaatctctccagtggatctcagctatcttgctcctaaaaacccaggaaccggtcctgctttcaccataatcaatggtaccctaaaatactttgagaccagatacatcagagtcgatattgctgctccaatcctctcaagaatggtcggaatgatcagtggaactaccacagaaagggaactgtgggatgactgggcaccatatgaagacgtggaaattggacccaatggagttctgaggaccagttcaggatataagtttcctttatacatgattggacatggtatgttggactccgatcttcatcttagctcaaaggctcaggtgttcgaacatcctcacattcaagacgctgcttcgcaacttcctgatgatgagagtttattttttggtgatactgggctatccaaaaatccaatcgagcttgtagaaggttggttcagtagttggaaaagctctattgcctcttttttctttatcatagggttaatcattggactattcttggttctccgagttggtatccatctttgcattaaagccagaagcacaccagtcacattaagtaaggatcaactgagtggtataaataatattgcatttagtaactaatagtcattaaaaagcgggcccgtattgttgcaaaaagccatgaccaaatcaaacagaatcaaaatcaactctggggcaaataacaatggagttgccaatcctcaaaacaaatgctattaccacaatccttgctgcagtcacactctgtttcgcttccagtcaaaacatcactgaagaattttatcaatcaacatgcagtgcagtcagcaaaggctatcttagtgctctaagaactggttggtatactagtgttataactatagaattaagtaatatcaaggaaaataagtgtaatggtacagacgctaaggtaaaattaataaaacaagaattagataaatataaaaatgctgtaacagaattgcagttgctcatgcaaagcacaccagcagccaacaatcgagccagaagagaactaccaagatttatgaattatacactcaacaataccaaaaacaccaatgtaacattaagtaagaaaaggaaaagaagatttcttggatttttgttaggtgttggatctgcaatcgccagtggcattgccgtatccaaggtcctgcacctagaaggggaagtgaacaaaatcaaaagtgctctactatccacaaacaaggctgtagtcagcttatctaatggagtcagtgtcttaaccagcaaggtgttagacctcaaaaactatatagataaacagttgttacctattgttaacaagcaaagctgcagcatatcaaacattgaaactgtgatagagttccaacaaaagaacaacagactactagagattaccagagaatttagtgttaatgcaggtgtaactactcctgtaagcacttatatgttaactaatagtgagttattatcattaatcaatgatatgcctataacaaatgatcagaaaaagttaatgtccagcaatgttcaaatagttagacagcaaagttactctatcatgtcaataataaaagaggaagtcttggcatatgtagtacaattaccactatatggtgtaatagatactccttgttggaaactacacacatcccctttatgtacaaccaacacaaaggaaggatccaacatctgcttaacaagaaccgacagaggatggtactgtgacaatgcaggatcagtatcctttttcccacaagctgaaacatgtaaagttcaatcgaatcgggtgttttgtgacacaatgaacagtttaacattaccaagtgaggtaaatctctgcaacattgacatattcaaccccaaatatgattgcaaaattatgacttcaaaaacagatgtaagcagctccgttatcacatctctaggagccattgtgtcatgctatggcaaaaccaaatgtacagcatccaataaaaatcgtgggatcataaagacattctctaacgggtgtgattatgtatcaaataagggggtggatactgtgtctgtaggtaatacattatattatgtaaataagcaagaaggcaaaagtctctatgtaaaaggtgaaccaataataaatttctatgatccattagtgttcccctctctcctgtgggatgcatcaatatctcaagtcaatgagaaaattaatcagagtctagcatttatccgtaaatcagatgaattattaggctctggcggaagcggatacatccctgaggcaccaagggacggacaggcctacgtgcgcaaggatggcgagtgggtgctgctgtccacctttctgtgaataaaaatagcacctaatcatattcttacaatggttcgctatttgaccatagataacccatctatcattagattatcctaaaatttgaacttcatcacaactttcatctataaaccatctcacttacactttttaagtagatttctattttatagttatataaaacagggcccattgaataccaaattaacttactatttgtaaaaatgagaattggggcaaatatgtcacgaaggaatccttgcaaattcgaaattcgaggtcattgcttgaatggtaaaaggtgtcattttagtcataattattttgaatggccaccccatgcactgcttgtaagacaaaactttatgttaaacagaatacttaagtctatggataaaagcatagatactttgtcagaaataagtggagctgcagagttggacagaacagaagagtatgccctcggtgtagttggagtgctagagagttatataggatcaataaataatataactaaacaatcagcatgtgttgccatgagcaaactccttactgaactcaacagcgatgacatcaaaaaactaagggacaatgaagagccaaactcacccaaagtaagagtgtacaatactgtcatatcatatattgaaagcaacaggaagaacaataaacaaactatccatctgttaaaaagattgccagcagacgtattgaagaaaaccatcaaaaacacattggatatccacaagagcataaccatcaataacccaaaagaatcaactgttagtgatacgaacgaccatgccaaaaataatgatactacctgacaaatatccttgtagtataaattccatactaataacaagtaattgtagagtcactatgtataatcaaaaaaacacactatatatcaatcaaaacaaccaaaatagccatatatacccaccggatcaaccattcaatgaaatccattggacctctcaagacttgattgatgcaactcaaaattttctacaacatctaggtattactgatgatatatacacaatatatatattagtgtcataatactcaatcctaatacttaccacatcatcaaattattaactcaaacaattcaagctatgggacaaaatggatcccattattagtggaaattctgctaatgtttatctaactgatagttatttaaaaggtgttatttctttctcagaatgtaacgctttaggaagttacatattcaatggtccttatctcaaaaatgattataccaacttaattagtagacaaaatccattaatagaacacataaatctaaagaaactaaatataacacagtccttaatatctaagtatcataaaggtgaaataaaaatagaagaacctacttactttcagtcattacttatgacatacaagagtatgacctcttcagaacagactactactactaatttacttaaaaagataataagaagagctatagaaatcagtgatgtcaaagtctatgctatattgaataaactggggctcaaagaaaaagacaagattaaatccaataatggacaagatgaagacaactcagtcattactaccataatcaaagatgatatacttttagctgtcaaggataatcaatctcatcttaaagcagacaaaaatcaatccacaaaacaaaaagatacaatcaaaacaacacttttgaagaaattaatgtgttcgatgcaacatcctccatcatggttaatacattggtttaatttatacacaaaattaaacagcatattaacacaatatcgatctagtgaggtaaaaaaccatggttttatattgatagataatcatactcttagtggattccaatttattttgaatcaatatggttgtatagtttatcataaggaactcaaaagaattactgtgacaacttataatcaattcttgacatggaaagatattagccttagtagattaaatgtttgtttgattacatggattagtaactgtttgaacacattaaacaaaagcttaggcttaagatgtggattcaataatgttatcttgacacaattattcctttatggagattgtatactaaaactattccacaatgaggggttctacataataaaagaggtagagggatttattatgtctctaattttaaatataacagaagaagatcaattcagaaaacggttttataatagtatgctcaacaacatcacagatgccgccaacaaagctcaaaaaaatctgctatcaagagtatgtcatacattattagataagacaatatcagataatataataaatggcagatggataattctattgagtaagttcctaaaattaattaagcttgcaggtgacaataacctcaacaatctgagtgaattatattttttgttcagaatatttggacacccaatggtagatgaaagacaagccatggatgctgttaaagttaattgcaacgagaccaaattttatttgttaagtagtttgagtatgttaagaggagcttttatatatagaattataaaagggtttgtaaataattacaacagatggcctactttaagaaatgccattgtcttacccttaagatggttaacttactataaactaaacacttatccttccttgttggaacttacagaaagagatttgattgttctatcaggactacgtttctatcgagagtttcggttgcctaaaaaagtggatcttgaaatgatcataaatgataaggctatatcacctcctaaaaatttaatatggactagtttccctagaaattatatgccgtcacacatacaaaattatatagaacatgaaaaattaaaattctctgatagtgataaatcaagaagagtattagagtattatttaagagataacaaattcaatgaatgtgatttacacaactgtgtagttaatcaaagttatcttaacaacccgaatcatgtggtatcattgacaggcaaagaaagagaactcagtgtaggtagaatgtttgcaatgcaaccaggaatgttcagacaagttcaaatattagcagagaaaatgatagcagaaaacatattacaatttttccctgaaagtcttacaagatatggtgatctagaactacagaaaatattagaattgaaagcaggaataagtaacaaatcaaatcgttacaatgataattacaacaattacattagtaagtgctctatcatcacagatctcagcaaattcaatcaagcatttcgatatgaaacatcatgtatttgtagtgatgtactggatgaactgcatggtgtacaatctctattttcctggttacatttaactattcctcatgtcacaataatatgcacatataggcatgcacccccctatataaaggatcatattgtagatcttaacaatgtagatgagcaaagtggactatatagatatcatatgggtggtatcgaagggtggtgtcaaaaactatggaccatagaagctatatcactattagatctaatatctctcaaagggaaattctcaattactgctttaattaatggtgacaatcaatcaatagatataagtaaaccagtcagactcatggaaggtcaaactcatgctcaagcagattatttgctagcattaaatagtctcaaattactgtataaagagtatgcaggaataggccacaaattaaaaggaactgagacttatatatcgagagatatgcaatttatgagtaaaacgatccaacataacggtgtatattacccagctagtataaagaaagtcctaagagtgggaccgtggataaacactatacttgatgacttcaaagtgagtctagaatctataggtagtttgacacaagaattagaatatagaggtgaaagtctattatgcagtttaatatttagaaatgtatggttatataatcaaattgcattacaacttaaaaatcatgcattatgtaacaacaaattatatttggatatattaaaagttctaaaacacttaaaaaccttttttaatcttgataacattgatacagcattaacattgtatatgaatttgcccatgttatttggtggtggtgatcccaacttgttatatcgaagtttctatagaagaactcctgatttcctcacagaggctatagttcactctgtgttcatacttagttattatacaaaccatgatttaaaagataaacttcaagatctgtcagatgatagattgaataagttcttaacatgcataatcacgtttgataaaaaccccaatgctgaattcgttacattgatgagagatcctcaagctttaggatctgagaggcaagctaaaattactagcgaaatcaatagactggcagttaccgaggttttgagcacagctccaaacaaaatattttccaaaagtgcacaacactataccactacagagatagatcttaatgatattatgcaaaatatagaacctacatatcctcacgggctaagagttgtttatgagagtttacccttttataaagcagagaaaatagtaaatcttatatccggtacaaaatctataactaacatactggaaaagacttctgccatagacttaacagatattgatagagccactgagatgatgaggaaaaacataactttgcttataaggatattaccattagattgtaacagagataaaagagaaatattgagtatggaaaacctaagtattactgaattaagcaaatacgttagagaaagatcttggtctttatccaatatagttggtgttacatcacccagtatcatgtatacaatggacataaaatatacaacaagcactatagctagtggcataatcatagagaaatataatgtcaacagtttaacacgtggtgagagaggacccactaaaccatgggttggttcatctacacaagagaaaaagacaatgccagtttataatagacaagttttaaccaaaaaacagagagatcaaatagatctattagcaaaattggattgggtgtatgcatctatagataacaaggatgaatttatggaggaacttagcataggaactcttgggttaacatatgagaaggccaaaaaattattcccacaatatttgagtgttaactatttgcatcgtcttacagtcagtagtagaccatgtgaattccctgcatctataccagcttatagaactacaaattatcactttgatactagccctattaatcgcatattaacagaaaagtatggtgatgaagatattgatatagtattccaaaactgtataagctttggccttagcttaatgtctgtagtagaacaatttactaatgtatgtcctaacagaattattctcatacccaagcttaatgagatacatttgatgaaacctcccatattcacaggcgatgttgatattcacaagttaaaacaagtgatacaaaaacaacatatgtttttaccagacaaaataagtttgactcaatatgtggaattattcttaagtaataaaacactcaaatctggatctaatgttaattctaatttaatattggcgcataagatatctgactattttcataatacttacattttgagtactaatttagctggacattggattcttattatacaacttatgaaagattctaagggtatttttgaaaaagattggggagagggatatataactgatcatatgttcattaatttgaaagttttcttcaatgcttataagacatatctcttgtgttttcataaaggttacggcagagcaaagctggagtgtgatatgaatacttcagatctcctatgtgtattggaattaatagacagtagttattggaagtctatgtctaaggtgtttttagaacaaaaagttatcaaatacattcttagccaggatgcaagtttacatagagtaaaaggatgtcatagcttcaaactatggtttcttaaacgtcttaatgtagcagaattcacagtttgcccttgggttgttaacatagattatcatccaacacatatgaaagcaatattaacttatattgatcttgttagaatgggattgataaatatagatagaatatacattaaaaataaacacaagttcaatgatgagttttatacttctaatctgttttacattaattataacttctcagataatactcatctattaactaaacatataaggattgctaattccgaattagaaagtaattacaacaaattatatcatcctacaccagaaaccctagaaaatatactaaccaatccggttaaaagtaatgagaaaaagacactgagtgactattgtataggtaaaaatgttgactcaataatgttaccatcgttatctaataagaagcttattaaatcgtctacaatgattagaaccaattacagcagacaagatttgtataatttatttcctacggttgtgattgataaaattatagatcattcaggtaatacagccaaatctaaccaactttacactactacttctcatcaaatatccttagtgcacaatagcacatcactttattgcatgcttccttggcatcatattaatagattcaattttgtatttagttctacaggttgtaaaattagtatagagtatattttaaaagatcttaaaattaaggatcctaattgtatagcattcataggtgaaggagcagggaatttattattgcgtacagtagtggaacttcatcctgatataagatatatttacagaagtctgaaagattgcaatgatcatagtttaccaattgagtttttaaggctgtacaatggacatatcaacattgattatggtgaaaatttgaccattcctgctacagatgcaaccaacaacattcattggtcttatttacatataaagtttgctgaacctatcagtctttttgtctgtgatgctgaattgcctgtaacagtcaactggagtaagattataatagagtggagcaagcatgtaagaaaatgcaagtactgttcttcagttaataaatgtacattgatagtaaaatatcatgctcaagatgatatcgatttcaaattagacaacataactatattaaaaacttatgtatgcttaggtagtaagttaaagggatctgaagtttacttagtccttacaataggtcctgcaaatgtgttcccagtatttaatgtagtacaaaatgctaaattgatactatcaagaactaaaaatttcatcatgcctaaaaaagctgataaagagtctattgatgcaaatattaagagtttgataccctttctttgttaccctataacaaaaaaaggaattaatactgcattgtctaaattaaagagtgttgttagtggagatatactatcatattctatagctggacgtaatgaagttttcagcaataaacttataaatcataagcatatgaacatcttaaagtggttcaatcatgttttaaatttcagatcaacagaattaaactataatcatttatatatggtagaatctacttatcctcatctaagtgaattgttaaacagcttgacaaccaatgaacttaaaaaactgattaaaatcacaggtagtttgttatacaacttttataatgaataatgagcaaaaatcttataacaaaaatagctacacactaacattgtattcaattatagttattgaaaattaataattatataatttttaataacttctagtgaactaatcctaaaattatcattttgatctaggaagaataagtttaaatccaaatctaattggtttatatgtatattaactaaattacgagatattagtttttgacactttttttctcgtggccggcatggtcccagcctcctcgctggcgccggctgggcaacatgcttcggcatggcgaatgggactagcataaccccttggggcctctaaacgggtcttgaggggttttttg

SEQ ID NO: 24 - DNA, 16028 bp, synthetic construct
  misc_feature 1..16028: note = antigenic cDNA encoding cRSVA_VSVG_S_preF_sc
  source 1..16028: mol_type = other DNA
taatacgactcactataggttttttcgcgtctgatgaggccgttaggccgaaactcctctccggagtcacgcgaaaaaatgcgtacaacaaacttgcgtaaaccaaaaaaatggggcaaataagaatttgataagtaccacttaaatttaactcctttggttagaggcgcgccatgggcagcaactcattgagtatgataaaagttagattgcaaaatctgtttgacaatgatgaagtagcattgttaaaaataacatgctatactgacaaattaatacagttaactaatgctttggctaaggcagttatacatacaatcaaattgaatggcattgtatttgtgcatgttattacaagtagtgatatttgccctaataataatattgtagtgaaatccaatttcacaacaatgccagtattacaaaatggaggttatatatgggaaatgatggaattaacacactgctctcaacctaatggcctaatagatgacaattgtgaaattaaattctccaaaaaactaagtgattcaacaatgaccaattatatgaatcaattatctgaattacttggatttgacctcaatccataaatcataataaatatcaactagcaaatcaatgtcactaacaccattagttaatataaaacttgacagaagataaaaatggggcaaataaatcaattcagccgacccaaccatggacacaacacacaatgataccacaccacaaagactgatgatcacagacatgaggccattatcgcttgagactataataacatctctaaccagagatatcataacacataaatttatatacttgataaatcatgaatgcatagtaagaaaacttgatgaaagacaggccacatttacatttctggtcaactatgaaatgaaactattgcacaaagtgggaagcactaaatataaaaaatatactgaatacaacacaaaatatggcactttccctatgccaatatttatcaatcatgatgggttcttagaatgcattggcattaagcctaccaagcacacacccataatatacaagtatgatctcaatccatgaatatcaaaccaagattcaaacaatccgaaataacaactttatgcataatcacactccatagtccaaatggagcctgaaaattatagttatttaaaattcctgcaggaaggagagacataagatgaaagatggggcaaatacaaaaatggctcttagcaaagtcaagttgaatgatacactcaacaaagatcaacttctatcatccagcaaatataccatccaacggagcacaggagacagcattgacactcctaattatgatgtgcagaaacacattaataagttatgtggcatgttattaatcacagaagatgctaatcataaattcactgggttaataggtatgttatatgctatgtctagattaggaagagaagacaccataaaaatactcaaagatgcgggatatcatgttaaggcaaatggagtggatgtaacaacacatcgtcaagacattaatgggaaagaaatgaaatttgaagtgttaacattagcaagcttaacaactgaaattcaaatcaacattgagatagaatctagaaaatcctacaaaaaaatgctaaaagaaatgggagaggtggctccagaatacaggcatgactctcctgattgtgggatgataatattatgtatagcggcattagtaataaccaaattagcagcaggagatagatcaggtcttacagctgtgattaggagagctaataatgtcctaaaaaatgaaatgaaacgttataaaggtttattacccaaggatatagccaacagcttctatgaagtgtttgaaaaatatcctcactttatagatgtttttgttcattttggtatagcacaatcttctaccagaggtggcagtagagttgaagggatttttgcaggattgtttatgaatgcctatggtgcagggcaagtgatgttacggtggggggtcttagcaaaatcagttaaaaacattatgttaggacacgctagtgtacaagcagaaatggaacaagttgtggaggtgtatgagtatgctcagaaattgggtggagaagcaggattctaccatatattgaacaacccaaaagcatcactattatctttgactcaatttcctcacttctctagtgtagtattgggcaatgctgctggcctaggcataatgggagaatacagaggtacaccaaggaatcaagatttatatgatgctgcaaaagcatatgctgaacaactcaaagaaaatggtgtgattaactacagtgtattagatttgacagcagaagaactagaggctatcaaacatcagcttaatccaaaagataatgatgtagagctttgagttaataaaaaagtggggcaaataaatcatcatggaaaagtttgctcctgaattccatggagaagatgcaaacaacagagccaccaaattcctagaatcaataaagggcaaattcacatcacccaaagatcccaagaaaaaagatagtatcatatctgtcaactcaatagatatagaagtaaccaaagaaagccctataacatcaaattcaaccattataaacccaataaatgagacagatgatactgtagggaacaagcccaattatcaaagaaagcctctagtaagtttcaaagaagaccctacgccaagtgataatcctttttcaaaactatacaaagaaaccatagaaacatttgataacaatgaagaagaatctagctattcatatgaagaaataaatgatcagacaaacgataatataacagcaagattagataggattgatgagaaattaagtgaaatactaggaatgcttcacacattagtagtagcgagtgcaggacccacatctgctcgggatggtataagagatgccatggttggtttaagagaagaaatgatagaaaaaatcagaactgaagcattaatgaccaatgacagactagaagctatggcaagactcaggaatgaagaaagtgaaaagatggcaaaagacacatcagatgaagtgtctctcaatccaacatcagagaaactgaacaacctgttggaagggaatgatagtgacaatgatctatcacttgaagatttctgattagctaccaaactgtacatcaaaacacaacaccaatagaaaaccaacaaacaaaccaactcacccatccaaccaaacatctatctgctgattagccaaccagccaaaaaacaaccagccaatctaaaactagccacccggaaaaaatcgatactatagttacaaaaaaagatggggcaaatatggaaacatacgtgaataaacttcacgagggctccacatacacagctgctgttcaatacaatgtcctagaaaaagacgatgatcctgcatcacttacaatatgggtgcccatgttccaatcatccatgccagcagatctactcataaaagaactagccaatgtcaatatactagtgaaacaaatatccacacccaagggaccctcattaagagtcatgataaactcaagaagtgcagtgctagcacaaatgcccagcaaatttaccatatgtgccaatgtgtccttggatgaaagaagcaagctggcatatgatgtaaccacaccctgtgaaattaaggcatgcagtctaacatgcctaaaatcaaaaaatatgttaactacagttaaagatctcactatgaaaacactcaacccaacacatgacatcattgctttatgtgaatttgaaaatatagtaacatcaaaaaaagtcataataccaacatacctaagatctatcagcgtcagaaataaagatctgaacacacttgaaaatataacaaccactgaattcaaaaatgccattacaaatgcaaaaatcatcccttactcaggattattgttagtcatcacagtgactgacaacaaaggagcattcaaatacataaagccacaaagtcaattcatagtagatcttggagcttacctagaaaaagaaagtatatattatgttacaacaaattggaagcacacagctacacgatttgcaatcaaacccatggaagattaacctttttcctctacatcaatgagtagattcatacaaactttctaactacattcttcacttcacaatcataatcaccaaccctctgtggttcaatcaatcaaacaaaactcatcaagagttccagatcatcccaagtcattgttcatcagatccagtactcaaataagttaataaaaaatccacatggggcaaataatcattgagggaaatccaactaatcacaacatctgtcaacatagacaagtcaacacgctagataaaatcaaccaatggaaaatacatccataactatagaattctcaagcaaattctggccttactttacactaatacacatgataacaacaataatctctttgataatcataatctccatcatgattgcaatactaaacaaactctgcgaatataatgtattccataacaaaacctttgagctaccaagagctcgagtcaatacatagcattcaccaatctgatagctcaaaacagtaaccttgcatttgtaaatgaactaccctcacttcttcacaaaaccacatcaacatctcaccatgcaagccatcatctataccataaagtagttaattaaaaatggccggccagtcataacaatgaactaggatattaagaccaaaaacaacgctacgcgtttgacagaagataaaaatggggcaaatgcaaacatgaagtgccttttgtacttagcctttttattcattggggtgaattgcaagttcaccatagtttttccacacaaccaaaaaggaaactggaaaaatgttccttctaattaccattattgcccgtcaagctcagatttaaattggcataatgacttaataggcacagccttacaagtcaaaatgcccaagagtcacaaggctattcaagcagacggttggatgtgtcatgcttccaaatgggtcactacttgtgatttccgctggtatggaccgaagtatataacacattccatccgatccttcactccatctgtagaacaatgcaaggaaagcattgaacaaacgaaacaaggaacttggctgaatccaggcttccctcctcaaagttgtggatatgcaactgtgacggatgccgaagcagtgattgtccaggtgactcctcaccatgtgctggttgatgaatacacaggagaatgggttgattcacagttcatcaacggaaaatgcagcaattacatatgccccactgtccataactctacaacctggcattctgactataaggtcaaagggctatgtgattctaacctcatttccatggacatcaccttcttctcagaggacggagagctatcatccctgggaaaggagggcacagggttcagaagtaactactttgcttatgaaactggaggcaaggcctgcaaaatgcaatactgcaagcattggggagtcagactcccatcaggtgtctggttcgagatggctgataaggatctctttgctgcagccagattccctgaatgcccagaagggtcaagtatctctgctccatctcagacctcagtggatgtaagtctaattcaggacgttgagaggatcttggattattccctctgccaagaaacctggagcaaaatcagagcgggtcttccaatctctccagtggatctcagctatcttgctcctaaaaacccaggaaccggtcctgctttcaccataatcaatggtaccctaaaatactttgagaccagatacatcagagtcgatattgctgctccaatcctctcaagaatggtcggaatgatcagtggaactaccacagaaagggaactgtgggatgactgggcaccatatgaagacgtggaaattggacccaatggagttctgaggaccagttcaggatataagtttcctttatacatgattggacatggtatgttggactccgatcttcatcttagctcaaaggctcaggtgttcgaacatcctcacattcaagacgctgcttcgcaacttcctgatgatgagagtttattttttggtgatactgggctatccaaaaatccaatcgagcttgtagaaggttggttcagtagttggaaaagctctattgcctcttttttctttatcatagggttaatcattggactattcttggttctccgagttggtatccatctttgcattaaagccagaagcacaccagtcacattaagtaaggatcaactgagtggtataaataatattgcatttagtaactaatagtcattaaaaagcgggcccgtattgttgcaaaaagccatgaccaaatcaaacagaatcaaaatcaactctggggcaaataacaatggagttgccaatcctcaaaacaaatgctattaccacaatccttgctgcagtcacactctgtttcgcttccagtcaaaacatcactgaagaattttatcaatcaacatgcagtgcagtcagcaaaggctatcttagtgctctaagaactggttggtatactagtgttataactatagaattaagtaatatcaaggaaaataagtgtaatggtacagacgctaaggtaaaattaataaaacaagaattagataaatataaaaatgctgtaacagaattgcagttgctcatgcaaagcacaccagcagccaacaatggagccagaggctctggcggaagcggacttggatttttgttaggtgttggatctgcaatcgccagtggcattgccgtatccaaggtcctgcacctagaaggggaagtgaacaaaatcaaaagtgctctactatccacaaacaaggctgtagtcagcttatctaatggagtcagtgtcttaaccagcaaggtgttagacctcaaaaactatatagataaacagttgttacctattgttaacaagcaaagctgcagcatatcaaacattgaaactgtgatagagttccaacaaaagaacaacagactactagagattaccagagaatttagtgttaatgcaggtgtaactactcctgtaagcacttatatgttaactaatagtgagttattatcattaatcaatgatatgcctataacaaatgatcagaaaaagttaatgtccagcaatgttcaaatagttagacagcaaagttactctatcatgtcaataataaaagaggaagtcttggcatatgtagtacaattaccactatatggtgtaatagatactccttgttggaaactacacacatcccctttatgtacaaccaacacaaaggaaggatccaacatctgcttaacaagaaccgacagaggatggtactgtgacaatgcaggatcagtatcctttttcccacaagctgaaacatgtaaagttcaatcgaatcgggtgttttgtgacacaatgaacagtttaacattaccaagtgaggtaaatctctgcaacattgacatattcaaccccaaatatgattgcaaaattatgacttcaaaaacagatgtaagcagctccgttatcacatctctaggagccattgtgtcatgctatggcaaaaccaaatgtacagcatccaataaaaatcgtgggatcataaagacattctctaacgggtgtgattatgtatcaaataagggggtggatactgtgtctgtaggtaatacattatattatgtaaataagcaagaaggcaaaagtctctatgtaaaaggtgaaccaataataaatttctatgatccattagtgttcccctctgatgaatttgatgcatcaatatctcaagtcaatgagaaaattaatcagagtctagcatttatccgtaaatcagatgaattattacataatgtaaatgctggtaaatccaccacaaatatcatgataactaccataattatagtaattatagtaatattgttagcattaattgcagttggactgcttctatactgcaaggccagaagcacaccagtcacattaagtaaggatcaactgagtggtataaataatattgcatttagtaactgaataaaaatagcacctaatcatattcttacaatggttcgctatttgaccatagataacccatctatcattagattatcctaaaatttgaacttcatcacaactttcatctataaaccatctcacttacactttttaagtagatttctattttatagttatataaaacagggcccattgaataccaaattaacttactatttgtaaaaatgagaattggggcaaatatgtcacgaaggaatccttgcaaattcgaaattcgaggtcattgcttgaatggtaaaaggtgtcattttagtcataattattttgaatggccaccccatgcactgcttgtaagacaaaactttatgttaaacagaatacttaagtctatggataaaagcatagatactttgtcagaaataagtggagctgcagagttggacagaacagaagagtatgccctcggtgtagttggagtgctagagagttatataggatcaataaataatataactaaacaatcagcatgtgttgccatgagcaaactccttactgaactcaacagcgatgacatcaaaaaactaagggacaatgaagagccaaactcacccaaagtaagagtgtacaatactgtcatatcatatattgaaagcaacaggaagaacaataaacaaactatccatctgttaaaaagattgccagcagacgtattgaagaaaaccatcaaaaacacattggatatccacaagagcataaccatcaataacccaaaagaatcaactgttagtgatacgaacgaccatgccaaaaataatgatactacctgacaaatatccttgtagtataaattccatactaataacaagtaattgtagagtcactatgtataatcaaaaaaacacactatatatcaatcaaaacaaccaaaatagccatatatacccaccggatcaaccattcaatgaaatccattggacctctcaagacttgattgatgcaactcaaaattttctacaacatctaggtattactgatgatatatacacaatatatatattagtgtcataatactcaatcctaatacttaccacatcatcaaattattaactcaaacaattcaagctatgggacaaaatggatcccattattagtggaaattctgctaatgtttatctaactgatagttatttaaaaggtgttatttctttctcagaatgtaacgctttaggaagttacatattcaatggtccttatctcaaaaatgattataccaacttaattagtagacaaaatccattaatagaacacataaatctaaagaaactaaatataacacagtccttaatatctaagtatcataaaggtgaaataaaaatagaagaacctacttactttcagtcattacttatgacatacaagagtatgacctcttcagaacagactactactactaatttacttaaaaagataataagaagagctatagaaatcagtgatgtcaaagtctatgctatattgaataaactggggctcaaagaaaaagacaagattaaatccaataatggacaagatgaagacaactcagtcattactaccataatcaaagatgatatacttttagctgtcaaggataatcaatctcatcttaaagcagacaaaaatcaatccacaaaacaaaaagatacaatcaaaacaacacttttgaagaaattaatgtgttcgatgcaacatcctccatcatggttaatacattggtttaatttatacacaaaattaaacagcatattaacacaatatcgatctagtgaggtaaaaaaccatggttttatattgatagataatcatactcttagtggattccaatttattttgaatcaatatggttgtatagtttatcataaggaactcaaaagaattactgtgacaacttataatcaattcttgacatggaaagatattagccttagtagattaaatgtttgtttgattacatggattagtaactgtttgaacacattaaacaaaagcttaggcttaagatgtggattcaataatgttatcttgacacaattattcctttatggagattgtatactaaaactattccacaatgaggggttctacataataaaagaggtagagggatttattatgtctctaattttaaatataacagaagaagatcaattcagaaaacggttttataatagtatgctcaacaacatcacagatgccgccaacaaagctcaaaaaaatctgctatcaagagtatgtcatacattattagataagacaatatcagataatataataaatggcagatggataattctattgagtaagttcctaaaattaattaagcttgcaggtgacaataacctcaacaatctgagtgaattatattttttgttcagaatatttggacacccaatggtagatgaaagacaagccatggatgctgttaaagttaattgcaacgagaccaaattttatttgttaagtagtttgagtatgttaagaggagcttttatatatagaattataaaagggtttgtaaataattacaacagatggcctactttaagaaatgccattgtcttacccttaagatggttaacttactataaactaaacacttatccttccttgttggaacttacagaaagagatttgattgttctatcaggactacgtttctatcgagagtttcggttgcctaaaaaagtggatcttgaaatgatcataaatgataaggctatatcacctcctaaaaatttaatatggactagtttccctagaaattatatgccgtcacacatacaaaattatatagaacatgaaaaattaaaattctctgatagtgataaatcaagaagagtattagagtattatttaagagataacaaattcaatgaatgtgatttacacaactgtgtagttaatcaaagttatcttaacaacccgaatcatgtggtatcattgacaggcaaagaaagagaactcagtgtaggtagaatgtttgcaatgcaaccaggaatgttcagacaagttcaaatattagcagagaaaatgatagcagaaaacatattacaatttttccctgaaagtcttacaagatatggtgatctagaactacagaaaatattagaattgaaagcaggaataagtaacaaatcaaatcgttacaatgataattacaacaattacattagtaagtgctctatcatcacagatctcagcaaattcaatcaagcatttcgatatgaaacatcatgtatttgtagtgatgtactggatgaactgcatggtgtacaatctctattttcctggttacatttaactattcctcatgtcacaataatatgcacatataggcatgcacccccctatataaaggatcatattgtagatcttaacaatgtagatgagcaaagtggactatatagatatcatatgggtggtatcgaagggtggtgtcaaaaactatggaccatagaagctatatcactattagatctaatatctctcaaagggaaattctcaattactgctttaattaatggtgacaatcaatcaatagatataagtaaaccagtcagactcatggaaggtcaaactcatgctcaagcagattatttgctagcattaaatagtctcaaattactgtataaagagtatgcaggaataggccacaaattaaaaggaactgagacttatatatcgagagatatgcaatttatgagtaaaacgatccaacataacggtgtatattacccagctagtataaagaaagtcctaagagtgggaccgtggataaacactatacttgatgacttcaaagtgagtctagaatctataggtagtttgacacaagaattagaatatagaggtgaaagtctattatgcagtttaatatttagaaatgtatggttatataatcaaattgcattacaacttaaaaatcatgcattatgtaacaacaaattatatttggatatattaaaagttctaaaacacttaaaaaccttttttaatcttgataacattgatacagcattaacattgtatatgaatttgcccatgttatttggtggtggtgatcccaacttgttatatcgaagtttctatagaagaactcctgatttcctcacagaggctatagttcactctgtgttcatacttagttattatacaaaccatgatttaaaagataaacttcaagatctgtcagatgatagattgaataagttcttaacatgcataatcacgtttgataaaaaccccaatgctgaattcgttacattgatgagagatcctcaagctttaggatctgagaggcaagctaaaattactagcgaaatcaatagactggcagttaccgaggttttgagcacagctccaaacaaaatattttccaaaagtgcacaacactataccactacagagatagatcttaatgatattatgcaaaatatagaacctacatatcctcacgggctaagagttgtttatgagagtttacccttttataaagcagagaaaatagtaaatcttatatccggtacaaaatctataactaacatactggaaaagacttctgccatagacttaacagatattgatagagccactgagatgatgaggaaaaacataactttgcttataaggatattaccattagattgtaacagagataaaagagaaatattgagtatggaaaacctaagtattactgaattaagcaaatacgttagagaaagatcttggtctttatccaatatagttggtgttacatcacccagtatcatgtatacaatggacataaaatatacaacaagcactatagctagtggcataatcatagagaaatataatgtcaacagtttaacacgtggtgagagaggacccactaaaccatgggttggttcatctacacaagagaaaaagacaatgccagtttataatagacaagttttaaccaaaaaacagagagatcaaatagatctattagcaaaattggattgggtgtatgcatctatagataacaaggatgaatttatggaggaacttagcataggaactcttgggttaacatatgagaaggccaaaaaattattcccacaatatttgagtgttaactatttgcatcgtcttacagtcagtagtagaccatgtgaattccctgcatctataccagcttatagaactacaaattatcactttgatactagccctattaatcgcatattaacagaaaagtatggtgatgaagatattgatatagtattccaaaactgtataagctttggccttagcttaatgtctgtagtagaacaatttactaatgtatgtcctaacagaattattctcatacccaagcttaatgagatacatttgatgaaacctcccatattcacaggcgatgttgatattcacaagttaaaacaagtgatacaaaaacaacatatgtttttaccagacaaaataagtttgactcaatatgtggaattattcttaagtaataaaacactcaaatctggatctaatgttaattctaatttaatattggcgcataagatatctgactattttcataatacttacattttgagtactaatttagctggacattggattcttattatacaacttatgaaagattctaagggtatttttgaaaaagattggggagagggatatataactgatcatatgttcattaatttgaaagttttcttcaatgcttataagacatatctcttgtgttttcataaaggttacggcagagcaaagctggagtgtgatatgaatacttcagatctcctatgtgtattggaattaatagacagtagttattggaagtctatgtctaaggtgtttttagaacaaaaagttatcaaatacattcttagccaggatgcaagtttacatagagtaaaaggatgtcatagcttcaaactatggtttcttaaacgtcttaatgtagcagaattcacagtttgcccttgggttgttaacatagattatcatccaacacatatgaaagcaatattaacttatattgatcttgttagaatgggattgataaatatagatagaatatacattaaaaataaacacaagttcaatgatgagttttatacttctaatctgttttacattaattataacttctcagataatactcatctattaactaaacatataaggattgctaattccgaattagaaagtaattacaacaaattatatcatcctacaccagaaaccctagaaaatatactaaccaatccggttaaaagtaatgagaaaaagacactgagtgactattgtataggtaaaaatgttgactcaataatgttaccatcgttatctaataagaagcttattaaatcgtctacaatgattagaaccaattacagcagacaagatttgtataatttatttcctacggttgtgattgataaaattatagatcattcaggtaatacagccaaatctaaccaactttacactactacttctcatcaaatatccttagtgcacaatagcacatcactttattgcatgcttccttggcatcatattaatagattcaattttgtatttagttctacaggttgtaaaattagtatagagtatattttaaaagatcttaaaattaaggatcctaattgtatagcattcataggtgaaggagcagggaatttattattgcgtacagtagtggaacttcatcctgatataagatatatttacagaagtctgaaagattgcaatgatcatagtttaccaattgagtttttaaggctgtacaatggacatatcaacattgattatggtgaaaatttgaccattcctgctacagatgcaaccaacaacattcattggtcttatttacatataaagtttgctgaacctatcagtctttttgtctgtgatgctgaattgcctgtaacagtcaactggagtaagattataatagagtggagcaagcatgtaagaaaatgcaagtactgttcttcagttaataaatgtacattgatagtaaaatatcatgctcaagatgatatcgatttcaaattagacaacataactatattaaaaacttatgtatgcttaggtagtaagttaaagggatctgaagtttacttagtccttacaataggtcctgcaaatgtgttcccagtatttaatgtagtacaaaatgctaaattgatactatcaagaactaaaaatttcatcatgcctaaaaaagctgataaagagtctattgatgcaaatattaagagtttgataccctttctttgttaccctataacaaaaaaaggaattaatactgcattgtctaaattaaagagtgttgttagtggagatatactatcatattctatagctggacgtaatgaagttttcagcaataaacttataaatcataagcatatgaacatcttaaagtggttcaatcatgttttaaatttcagatcaacagaattaaactataatcatttatatatggtagaatctacttatcctcatctaagtgaattgttaaacagcttgacaaccaatgaacttaaaaaactgattaaaatcacaggtagtttgttatacaacttttataatgaataatgagcaaaaatcttataacaaaaatagctacacactaacattgtattcaattatagttattgaaaattaataattatataatttttaataacttctagtgaactaatcctaaaattatcattttgatctaggaagaataagtttaaatccaaatctaattggtttatatgtatattaactaaattacgagatattagtttttgacactttttttctcgtggccggcatggtcccagcctcctcgctggcgccggctgggcaacatgcttcggcatggcgaatgggactagcataaccccttggggcctctaaacgggtcttgaggggttttttg

SEQ ID NO: 25 - DNA, 17006 bp, synthetic construct
  misc_feature 1..17006: note = antigenic cDNA encoding cRSVA_VSVG_A_preF_ef_NS1/NS2deop
  source 1..17006: mol_type = other DNA
taatacgactcactataggttttttcgcgtctgatgaggccgttaggccgaaactcctctccggagtcacgcgaaaaaatgcgtacaacaaacttgcgtaaaccaaaaaaatggggcaaataagaatttgataagtaccacttaaatttaactcctttggttagaggcgcgccatgggttcgaattcgctatcgatgataaaagtacgtctacaaaatctatttgataatgatgaagtagcgctactaaaaataacgtgttatacggataaactaatacaactaacgaatgcgctagcgaaagcggtaatacatacgataaaactaaatggtatagtatttgtacatgtaataacgtcgtcggatatatgtccgaataataatatagtagtaaaatcgaattttacgacgatgccggtactacaaaatggtggttatatatgggaaatgatggaactaacgcattgttcgcaaccgaatggtctaatagatgataattgtgaaataaaattttcgaaaaaactatcggattcgacgatgacgaattatatgaatcaactatcggaactactaggttttgatctaaatccgtaaatcataataaatatcaactagcaaatcaatgtcactaacaccattagttaatataaaacttgacagaagataaaaatggggcaaataaatcaattcagccgacccaaccatggatacgacgcataatgatacgacgccgcaacgtctaatgataacggatatgcgtccgctatcgctagaaacgataataacgtcgctaacgcgagatataataacgcataaatttatatatctaataaatcatgaatgtatagtacgtaaactagatgaacgtcaagcgacgtttacgtttctagtaaattatgaaatgaaactactacataaagtaggttcgacgaaatataaaaaatatacggaatataatacgaaatatggtacgtttccgatgccgatatttataaatcatgatggttttctagaatgtataggtataaaaccgacgaaacatacgccgataatatataaatatgatctaaatccgtgaatatcaaaccaagattcaaacaatccgaaataacaactttatgcataatcacactccatagtccaaatggagcctgaaaattatagttatttaaaattcctgcaggaaggagagacataagatgaaagatggggcaaatacaaaaatggctcttagcaaagtcaagttgaatgatacactcaacaaagatcaacttctatcatccagcaaatataccatccaacggagcacaggagacagcattgacactcctaattatgatgtgcagaaacacattaataagttatgtggcatgttattaatcacagaagatgctaatcataaattcactgggttaataggtatgttatatgctatgtctagattaggaagagaagacaccataaaaatactcaaagatgcgggatatcatgttaaggcaaatggagtggatgtaacaacacatcgtcaagacattaatgggaaagaaatgaaatttgaagtgttaacattagcaagcttaacaactgaaattcaaatcaacattgagatagaatctagaaaatcctacaaaaaaatgctaaaagaaatgggagaggtggctccagaatacaggcatgactctcctgattgtgggatgataatattatgtatagcggcattagtaataaccaaattagcagcaggagatagatcaggtcttacagctgtgattaggagagctaataatgtcctaaaaaatgaaatgaaacgttataaaggtttattacccaaggatatagccaacagcttctatgaagtgtttgaaaaatatcctcactttatagatgtttttgttcattttggtatagcacaatcttctaccagaggtggcagtagagttgaagggatttttgcaggattgtttatgaatgcctatggtgcagggcaagtgatgttacggtggggggtcttagcaaaatcagttaaaaacattatgttaggacacgctagtgtacaagcagaaatggaacaagttgtggaggtgtatgagtatgctcagaaattgggtggagaagcaggattctaccatatattgaacaacccaaaagcatcactattatctttgactcaatttcctcacttctctagtgtagtattgggcaatgctgctggcctaggcataatgggagaatacagaggtacaccaaggaatcaagatttatatgatgctgcaaaagcatatgctgaacaactcaaagaaaatggtgtgattaactacagtgtattagatttgacagcagaagaactagaggctatcaaacatcagcttaatccaaaagataatgatgtagagctttgagttaataaaaaagtggggcaaataaatcatcatggaaaagtttgctcctgaattccatggagaagatgcaaacaacagagccaccaaattcctagaatcaataaagggcaaattcacatcacccaaagatcccaagaaaaaagatagtatcatatctgtcaactcaatagatatagaagtaaccaaagaaagccctataacatcaaattcaaccattataaacccaataaatgagacagatgatactgtagggaacaagcccaattatcaaagaaagcctctagtaagtttcaaagaagaccctacgccaagtgataatcctttttcaaaactatacaaagaaaccatagaaacatttgataacaatgaagaagaatctagctattcatatgaagaaataaatgatcagacaaacgataatataacagcaagattagataggattgatgagaaattaagtgaaatactaggaatgcttcacacattagtagtagcgagtgcaggacccacatctgctcgggatggtataagagatgccatggttggtttaagagaagaaatgatagaaaaaatcagaactgaagcattaatgaccaatgacagactagaagctatggcaagactcaggaatgaagaaagtgaaaagatggcaaaagacacatcagatgaagtgtctctcaatccaacatcagagaaactgaacaacctgttggaagggaatgatagtgacaatgatctatcacttgaagatttctgattagctaccaaactgtacatcaaaacacaacaccaatagaaaaccaacaaacaaaccaactcacccatccaaccaaacatctatctgctgattagccaaccagccaaaaaacaaccagccaatctaaaactagccacccggaaaaaatcgatactatagttacaaaaaaagatggggcaaatatggaaacatacgtgaataaacttcacgagggctccacatacacagctgctgttcaatacaatgtcctagaaaaagacgatgatcctgcatcacttacaatatgggtgcccatgttccaatcatccatgccagcagatctactcataaaagaactagccaatgtcaatatactagtgaaacaaatatccacacccaagggaccctcattaagagtcatgataaactcaagaagtgcagtgctagcacaaatgcccagcaaatttaccatatgtgccaatgtgtccttggatgaaagaagcaagctggcatatgatgtaaccacaccctgtgaaattaaggcatgcagtctaacatgcctaaaatcaaaaaatatgttaactacagttaaagatctcactatgaaaacactcaacccaacacatgacatcattgctttatgtgaatttgaaaatatagtaacatcaaaaaaagtcataataccaacatacctaagatctatcagcgtcagaaataaagatctgaacacacttgaaaatataacaaccactgaattcaaaaatgccattacaaatgcaaaaatcatcccttactcaggattattgttagtcatcacagtgactgacaacaaaggagcattcaaatacataaagccacaaagtcaattcatagtagatcttggagcttacctagaaaaagaaagtatatattatgttacaacaaattggaagcacacagctacacgatttgcaatcaaacccatggaagattaacctttttcctctacatcaatgagtagattcatacaaactttctaactacattcttcacttcacaatcataatcaccaaccctctgtggttcaatcaatcaaacaaaactcatcaagagttccagatcatcccaagtcattgttcatcagatccagtactcaaataagttaataaaaaatccacatggggcaaataatcattgagggaaatccaactaatcacaacatctgtcaacatagacaagtcaacacgctagataaaatcaaccaatggaaaatacatccataactatagaattctcaagcaaattctggccttactttacactaatacacatgataacaacaataatctctttgataatcataatctccatcatgattgcaatactaaacaaactctgcgaatataatgtattccataacaaaacctttgagctaccaagagctcgagtcaatacatagcattcaccaatctgatagctcaaaacagtaaccttgcatttgtaaatgaactaccctcacttcttcacaaaaccacatcaacatctcaccatgcaagccatcatctataccataaagtagttaattaaaaatggccggccagtcataacaatgaactaggatattaagaccaaaaacaacgctggggcaaatgcaaacatgtccaaaaccgaggaccaacgcaccgccaagacactagaaaggacctgggacacttttaatcatctattattcatatcatcgtgcttatacaagttaaatcttaaatctatagcacaaatcacattatctattttggcaattataatctcaacctcacttataattgcagccatcatattcatagcctcggcaaaccacaaagtcacactaacaactgcaatcatacaagatgcaacgaaccagatcaagaacacaaccccaacatacctcacccagaatccccagcatggaatcagcttctccaatctgtccggaactacatcacaatccaccaccatactagcttcaacaacaccaagtgctgattcaaccccacaatccacaacagtcaagatcaaaaacacaacaacaacccaaatattacctagcaaacccaccacaaaacaacgccaaaataaaccacaaaacaaacccaacaatgattttcactttgaagtgttcaattttgtaccctgcagcatatgcagcaacaatccaacctgctgggccatctgcaagagaataccaaacaaaaaacctggaaagaaaaccaccaccaagcccacaaaaaaaccaaccctcaagacaaccaaaaaagatcccaaatcccaaaccacaaaaccaaaggaagtactcactaccaagcctacaggaaagccaaccatcaacaccactaaaacaaacatcagaactacactgctcacctccaacaccaaaggaaatccagaacacacaagtcaagaggaaaccctccactcaaccacctccgaaggctatccaagcccatcacaagtccacacaacatccggtcaagaggaaaccctccactcaaccacctccgaaggctatccaagcccatcacaagtctacacaacatccgagtacctatcacaatctctatcttcatccaacacaacaaaatgatagtcattaaaaagcacgcgtttgacagaagataaaaatggggcaaatgcaaacatgaagtgccttttgtacttagcctttttattcattggggtgaattgcaagttcaccatagtttttccacacaaccaaaaaggaaactggaaaaatgttccttctaattaccattattgcccgtcaagctcagatttaaattggcataatgacttaataggcacagccttacaagtcaaaatgcccaagagtcacaaggctattcaagcagacggttggatgtgtcatgcttccaaatgggtcactacttgtgatttccgctggtatggaccgaagtatataacacattccatccgatccttcactccatctgtagaacaatgcaaggaaagcattgaacaaacgaaacaaggaacttggctgaatccaggcttccctcctcaaagttgtggatatgcaactgtgacggatgccgaagcagtgattgtccaggtgactcctcaccatgtgctggttgatgaatacacaggagaatgggttgattcacagttcatcaacggaaaatgcagcaattacatatgccccactgtccataactctacaacctggcattctgactataaggtcaaagggctatgtgattctaacctcatttccatggacatcaccttcttctcagaggacggagagctatcatccctgggaaaggagggcacagggttcagaagtaactactttgcttatgaaactggaggcaaggcctgcaaaatgcaatactgcaagcattggggagtcagactcccatcaggtgtctggttcgagatggctgataaggatctctttgctgcagccagattccctgaatgcccagaagggtcaagtatctctgctccatctcagacctcagtggatgtaagtctaattcaggacgttgagaggatcttggattattccctctgccaagaaacctggagcaaaatcagagcgggtcttccaatctctccagtggatctcagctatcttgctcctaaaaacccaggaaccggtcctgctttcaccataatcaatggtaccctaaaatactttgagaccagatacatcagagtcgatattgctgctccaatcctctcaagaatggtcggaatgatcagtggaactaccacagaaagggaactgtgggatgactgggcaccatatgaagacgtggaaattggacccaatggagttctgaggaccagttcaggatataagtttcctttatacatgattggacatggtatgttggactccgatcttcatcttagctcaaaggctcaggtgttcgaacatcctcacattcaagacgctgcttcgcaacttcctgatgatgagagtttattttttggtgatactgggctatccaaaaatccaatcgagcttgtagaaggttggttcagtagttggaaaagctctattgcctcttttttctttatcatagggttaatcattggactattcttggttctccgagttggtatccatctttgcattaaagccagaagcacaccagtcacattaagtaaggatcaactgagtggtataaataatattgcatttagtaactaatagtcattaaaaagcgggcccgtattgttgcaaaaagccatgaccaaatcaaacagaatcaaaatcaactctggggcaaataacaatggagttgccaatcctcaaaacaaatgctattaccacaatccttgctgcagtcacactctgtttcgcttccagtcaaaacatcactgaagaattttatcaatcaacatgcagtgcagtcagcaaaggctatcttagtgctctaagaactggttggtatactagtgttataactatagaattaagtaatatcaaggaaaataagtgtaatggtacagacgctaaggtaaaattaataaaacaagaattagataaatataaaaatgctgtaacagaattgcagttgctcatgcaaagcacaccagcagccaacaatcgagccagaagagaactaccaagatttatgaattatacactcaacaataccaaaaacaccaatgtaacattaagtaagaaaaggaaaagaagatttcttggatttttgttaggtgttggatctgcaatcgccagtggcattgccgtatccaaggtcctgcacctagaaggggaagtgaacaaaatcaaaagtgctctactatccacaaacaaggctgtagtcagcttatctaatggagtcagtgtcttaaccagcaaggtgttagacctcaaaaactatatagataaacagttgttacctattgttaacaagcaaagctgcagcatatcaaacattgaaactgtgatagagttccaacaaaagaacaacagactactagagattaccagagaatttagtgttaatgcaggtgtaactactcctgtaagcacttatatgttaactaatagtgagttattatcattaatcaatgatatgcctataacaaatgatcagaaaaagttaatgtccagcaatgttcaaatagttagacagcaaagttactctatcatgtcaataataaaagaggaagtcttggcatatgtagtacaattaccactatatggtgtaatagatactccttgttggaaactacacacatcccctttatgtacaaccaacacaaaggaaggatccaacatctgcttaacaagaaccgacagaggatggtactgtgacaatgcaggatcagtatcctttttcccacaagctgaaacatgtaaagttcaatcgaatcgggtgttttgtgacacaatgaacagtttaacattaccaagtgaggtaaatctctgcaacattgacatattcaaccccaaatatgattgcaaaattatgacttcaaaaacagatgtaagcagctccgttatcacatctctaggagccattgtgtcatgctatggcaaaaccaaatgtacagcatccaataaaaatcgtgggatcataaagacattctctaacgggtgtgattatgtatcaaataagggggtggatactgtgtctgtaggtaatacattatattatgtaaataagcaagaaggcaaaagtctctatgtaaaaggtgaaccaataataaatttctatgatccattagtgttcccctctctcctgtgggatgcatcaatatctcaagtcaatgagaaaattaatcagagtctagcatttatccgtaaatcagatgaattattaggctctggcggaagcggatacatccctgaggcaccaagggacggacaggcctacgtgcgcaaggatggcgagtgggtgctgctgtccacctttctgtgaataaaaatagcacctaatcatattcttacaatggttcgctatttgaccatagataacccatctatcattagattatcctaaaatttgaacttcatcacaactttcatctataaaccatctcacttacactttttaagtagatttctattttatagttatataaaacagggcccattgaataccaaattaacttactatttgtaaaaatgagaattggggcaaatatgtcacgaaggaatccttgcaaattcgaaattcgaggtcattgcttgaatggtaaaaggtgtcattttagtcataattattttgaatggccaccccatgcactgcttgtaagacaaaactttatgttaaacagaatacttaagtctatggataaaagcatagatactttgtcagaaataagtggagctgcagagttggacagaacagaagagtatgccctcggtgtagttggagtgctagagagttatataggatcaataaataatataactaaacaatcagcatgtgttgccatgagcaaactccttactgaactcaacagcgatgacatcaaaaaactaagggacaatgaagagccaaactcacccaaagtaagagtgtacaatactgtcatatcatatattgaaagcaacaggaagaacaataaacaaactatccatctgttaaaaagattgccagcagacgtattgaagaaaaccatcaaaaacacattggatatccacaagagcataaccatcaataacccaaaagaatcaactgttagtgatacgaacgaccatgccaaaaataatgatactacctgacaaatatccttgtagtataaattccatactaataacaagtaattgtagagtcactatgtataatcaaaaaaacacactatatatcaatcaaaacaaccaaaatagccatatatacccaccggatcaaccattcaatgaaatccattggacctctcaagacttgattgatgcaactcaaaattttctacaacatctaggtattactgatgatatatacacaatatatatattagtgtcataatactcaatcctaatacttaccacatcatcaaattattaactcaaacaattcaagctatgggacaaaatggatcccattattagtggaaattctgctaatgtttatctaactgatagttatttaaaaggtgttatttctttctcagaatgtaacgctttaggaagttacatattcaatggtccttatctcaaaaatgattataccaacttaattagtagacaaaatccattaatagaacacataaatctaaagaaactaaatataacacagtccttaatatctaagtatcataaaggtgaaataaaaatagaagaacctacttactttcagtcattacttatgacatacaagagtatgacctcttcagaacagactactactactaatttacttaaaaagataataagaagagctatagaaatcagtgatgtcaaagtctatgctatattgaataaactggggctcaaagaaaaagacaagattaaatccaataatggacaagatgaagacaactcagtcattactaccataatcaaagatgatatacttttagctgtcaaggataatcaatctcatcttaaagcagacaaaaatcaatccacaaaacaaaaagatacaatcaaaacaacacttttgaagaaattaatgtgttcgatgcaacatcctccatcatggttaatacattggtttaatttatacacaaaattaaacagcatattaacacaatatcgatctagtgaggtaaaaaaccatggttttatattgatagataatcatactcttagtggattccaatttattttgaatcaatatggttgtatagtttatcataaggaactcaaaagaattactgtgacaacttataatcaattcttgacatggaaagatattagccttagtagattaaatgtttgtttgattacatggattagtaactgtttgaacacattaaacaaaagcttaggcttaagatgtggattcaataatgttatcttgacacaattattcctttatggagattgtatactaaaactattccacaatgaggggttctacataataaaagaggtagagggatttattatgtctctaattttaaatataacagaagaagatcaattcagaaaacggttttataatagtatgctcaacaacatcacagatgccgccaacaaagctcaaaaaaatctgctatcaagagtatgtcatacattattagataagacaatatcagataatataataaatggcagatggataattctattgagtaagttcctaaaattaattaagcttgcaggtgacaataacctcaacaatctgagtgaattatattttttgttcagaatatttggacacccaatggtagatgaaagacaagccatggatgctgttaaagttaattgcaacgagaccaaattttatttgttaagtagtttgagtatgttaagaggagcttttatatatagaattataaaagggtttgtaaataattacaacagatggcctactttaagaaatgccattgtcttacccttaagatggttaacttactataaactaaacacttatccttccttgttggaacttacagaaagagatttgattgttctatcaggactacgtttctatcgagagtttcggttgcctaaaaaagtggatcttgaaatgatcataaatgataaggctatatcacctcctaaaaatttaatatggactagtttccctagaaattatatgccgtcacacatacaaaattatatagaacatgaaaaattaaaattctctgatagtgataaatcaagaagagtattagagtattatttaagagataacaaattcaatgaatgtgatttacacaactgtgtagttaatcaaagttatcttaacaacccgaatcatgtggtatcattgacaggcaaagaaagagaactcagtgtaggtagaatgtttgcaatgcaaccaggaatgttcagacaagttcaaatattagcagagaaaatgatagcagaaaacatattacaatttttccctgaaagtcttacaagatatggtgatctagaactacagaaaatattagaattgaaagcaggaataagtaacaaatcaaatcgttacaatgataattacaacaattacattagtaagtgctctatcatcacagatctcagcaaattcaatcaagcatttcgatatgaaacatcatgtatttgtagtgatgtactggatgaactgcatggtgtacaatctctattttcctggttacatttaactattcctcatgtcacaataatatgcacatataggcatgcacccccctatataaaggatcatattgtagatcttaacaatgtagatgagcaaagtggactatatagatatcatatgggtggtatcgaagggtggtgtcaaaaactatggaccatagaagctatatcactattagatctaatatctctcaaagggaaattctcaattactgctttaattaatggtgacaatcaatcaatagatataagtaaaccagtcagactcatggaaggtcaaactcatgctcaagcagattatttgctagcattaaatagtctcaaattactgtataaagagtatgcaggaataggccacaaattaaaaggaactgagacttatatatcgagagatatgcaatttatgagtaaaacgatccaacataacggtgtatattacccagctagtataaagaaagtcctaagagtgggaccgtggataaacactatacttgatgacttcaaagtgagtctagaatctataggtagtttgacacaagaattagaatatagaggtgaaagtctattatgcagtttaatatttagaaatgtatggttatataatcaaattgcattacaacttaaaaatcatgcattatgtaacaacaaattatatttggatatattaaaagttctaaaacacttaaaaaccttttttaatcttgataacattgatacagcattaacattgtatatgaatttgcccatgttatttggtggtggtgatcccaacttgttatatcgaagtttctatagaagaactcctgatttcctcacagaggctatagttcactctgtgttcatacttagttattatacaaaccatgatttaaaagataaacttcaagatctgtcagatgatagattgaataagttcttaacatgcataatcacgtttgataaaaaccccaatgctgaattcgttacattgatgagagatcctcaagctttaggatctgagaggcaagctaaaattactagcgaaatcaatagactggcagttaccgaggttttgagcacagctccaaacaaaatattttccaaaagtgcacaacactataccactacagagatagatcttaatgatattatgcaaaatatagaacctacatatcctcacgggctaagagttgtttatgagagtttacccttttataaagcagagaaaatagtaaatcttatatccggtacaaaatctataactaacatactggaaaagacttctgccatagacttaacagatattgatagagccactgagatgatgaggaaaaacataactttgcttataaggatattaccattagattgtaacagagataaaagagaaatattgagtatggaaaacctaagtattactgaattaagcaaatacgttagagaaagatcttggtctttatccaatatagttggtgttacatcacccagtatcatgtatacaatggacataaaatatacaacaagcactatagctagtggcataatcatagagaaatataatgtcaacagtttaacacgtggtgagagaggacccactaaaccatgggttggttcatctacacaagagaaaaagacaatgccagtttataatagacaagttttaaccaaaaaacagagagatcaaatagatctattagcaaaattggattgggtgtatgcatctatagataacaaggatgaatttatggaggaacttagcataggaactcttgggttaacatatgagaaggccaaaaaattattcccacaatatttgagtgttaactatttgcatcgtcttacagtcagtagtagaccatgtgaattccctgcatctataccagcttatagaactacaaattatcactttgatactagccctattaatcgcatattaacagaaaagtatggtgatgaagatattgatatagtattccaaaactgtataagctttggccttagcttaatgtctgtagtagaacaatttactaatgtatgtcctaacagaattattctcatacccaagcttaatgagatacatttgatgaaacctcccatattcacaggcgatgttgatattcacaagttaaaacaagtgatacaaaaacaacatatgtttttaccagacaaaataagtttgactcaatatgtggaattattcttaagtaataaaacactcaaatctggatctaatgttaattctaatttaatattggcgcataagatatctgactattttcataatacttacattttgagtactaatttagctggacattggattcttattatacaacttatgaaagattctaagggtatttttgaaaaagattggggagagggatatataactgatcatatgttcattaatttgaaagttttcttcaatgcttataagacatatctcttgtgttttcataaaggttacggcagagcaaagctggagtgtgatatgaatacttcagatctcctatgtgtattggaattaatagacagtagttattggaagtctatgtctaaggtgtttttagaacaaaaagttatcaaatacattcttagccaggatgcaagtttacatagagtaaaaggatgtcatagcttcaaactatggtttcttaaacgtcttaatgtagcagaattcacagtttgcccttgggttgttaacatagattatcatccaacacatatgaaagcaatattaacttatattgatcttgttagaatgggattgataaatatagatagaatatacattaaaaataaacacaagttcaatgatgagttttatacttctaatctgttttacattaattataacttctcagataatactcatctattaactaaacatataaggattgctaattccgaattagaaagtaattacaacaaattatatcatcctacaccagaaaccctagaaaatatactaaccaatccggttaaaagtaatgagaaaaagacactgagtgactattgtataggtaaaaatgttgactcaataatgttaccatcgttatctaataagaagcttattaaatcgtctacaatgattagaaccaattacagcagacaagatttgtataatttatttcctacggttgtgattgataaaattatagatcattcaggtaatacagccaaatctaaccaactttacactactacttctcatcaaatatccttagtgcacaatagcacatcactttattgcatgcttccttggcatcatattaatagattcaattttgtatttagttctacaggttgtaaaattagtatagagtatattttaaaagatcttaaaattaaggatcctaattgtatagcattcataggtgaaggagcagggaatttattattgcgtacagtagtggaacttcatcctgatataagatatatttacagaagtctgaaagattgcaatgatcatagtttaccaattgagtttttaaggctgtacaatggacatatcaacattgattatggtgaaaatttgaccattcctgctacagatgcaaccaacaacattcattggtcttatttacatataaagtttgctgaacctatcagtctttttgtctgtgatgctgaattgcctgtaacagtcaactggagtaagattataatagagtggagcaagcatgtaagaaaatgcaagtactgttcttcagttaataaatgtacattgatagtaaaatatcatgctcaagatgatatcgatttcaaattagacaacataactatattaaaaacttatgtatgcttaggtagtaagttaaagggatctgaagtttacttagtccttacaataggtcctgcaaatgtgttcccagtatttaatgtagtacaaaatgctaaattgatactatcaagaactaaaaatttcatcatgcctaaaaaagctgataaagagtctattgatgcaaatattaagagtttgataccctttctttgttaccctataacaaaaaaaggaattaatactgcattgtctaaattaaagagtgttgttagtggagatatactatcatattctatagctggacgtaatgaagttttcagcaataaacttataaatcataagcatatgaacatcttaaagtggttcaatcatgttttaaatttcagatcaacagaattaaactataatcatttatatatggtagaatctacttatcctcatctaagtgaattgttaaacagcttgacaaccaatgaacttaaaaaactgattaaaatcacaggtagtttgttatacaacttttataatgaataatgagcaaaaatcttataacaaaaatagctacacactaacattgtattcaattatagttattgaaaattaataattatataatttttaataacttctagtgaactaatcctaaaattatcattttgatctaggaagaataagtttaaatccaaatctaattggtttatatgtatattaactaaattacgagatattagtttttgacactttttttctcgtggccggcatggtcccagcctcctcgctggcgccggctgggcaacatgcttcggcatggcgaatgggactagcataaccccttggggcctctaaacgggtcttgaggggttttttg

SEQ ID NO: 26 - DNA, 15494 bp, synthetic construct
  misc_feature 1..15494: note = antigenic cDNA encoding cRSVA_ mF1
  source 1..15494: mol_type = other DNA
taatacgactcactataggttttttcgcgtctgatgaggccgttaggccgaaactcctctccggagtcacgcgaaaaaatgcgtacaacaaacttgcgtaaaccaaaaaaatggggcaaataagaatttgataagtaccacttaaatttaactcctttggttagaggcgcgccatgggcagcaactcattgagtatgataaaagttagattgcaaaatctgtttgacaatgatgaagtagcattgttaaaaataacatgctatactgacaaattaatacagttaactaatgctttggctaaggcagttatacatacaatcaaattgaatggcattgtatttgtgcatgttattacaagtagtgatatttgccctaataataatattgtagtgaaatccaatttcacaacaatgccagtattacaaaatggaggttatatatgggaaatgatggaattaacacactgctctcaacctaatggcctaatagatgacaattgtgaaattaaattctccaaaaaactaagtgattcaacaatgaccaattatatgaatcaattatctgaattacttggatttgacctcaatccataaatcataataaatatcaactagcaaatcaatgtcactaacaccattagttaatataaaacttgacagaagataaaaatggggcaaataaatcaattcagccgacccaaccatggacacaacacacaatgataccacaccacaaagactgatgatcacagacatgaggccattatcgcttgagactataataacatctctaaccagagatatcataacacataaatttatatacttgataaatcatgaatgcatagtaagaaaacttgatgaaagacaggccacatttacatttctggtcaactatgaaatgaaactattgcacaaagtgggaagcactaaatataaaaaatatactgaatacaacacaaaatatggcactttccctatgccaatatttatcaatcatgatgggttcttagaatgcattggcattaagcctaccaagcacacacccataatatacaagtatgatctcaatccatgaatatcaaaccaagattcaaacaatccgaaataacaactttatgcataatcacactccatagtccaaatggagcctgaaaattatagttatttaaaattcctgcaggaaggagagacataagatgaaagatggggcaaatacaaaaatggctcttagcaaagtcaagttgaatgatacactcaacaaagatcaacttctatcatccagcaaatataccatccaacggagcacaggagacagcattgacactcctaattatgatgtgcagaaacacattaataagttatgtggcatgttattaatcacagaagatgctaatcataaattcactgggttaataggtatgttatatgctatgtctagattaggaagagaagacaccataaaaatactcaaagatgcgggatatcatgttaaggcaaatggagtggatgtaacaacacatcgtcaagacattaatgggaaagaaatgaaatttgaagtgttaacattagcaagcttaacaactgaaattcaaatcaacattgagatagaatctagaaaatcctacaaaaaaatgctaaaagaaatgggagaggtggctccagaatacaggcatgactctcctgattgtgggatgataatattatgtatagcggcattagtaataaccaaattagcagcaggagatagatcaggtcttacagctgtgattaggagagctaataatgtcctaaaaaatgaaatgaaacgttataaaggtttattacccaaggatatagccaacagcttctatgaagtgtttgaaaaatatcctcactttatagatgtttttgttcattttggtatagcacaatcttctaccagaggtggcagtagagttgaagggatttttgcaggattgtttatgaatgcctatggtgcagggcaagtgatgttacggtggggggtcttagcaaaatcagttaaaaacattatgttaggacacgctagtgtacaagcagaaatggaacaagttgtggaggtgtatgagtatgctcagaaattgggtggagaagcaggattctaccatatattgaacaacccaaaagcatcactattatctttgactcaatttcctcacttctctagtgtagtattgggcaatgctgctggcctaggcataatgggagaatacagaggtacaccaaggaatcaagatttatatgatgctgcaaaagcatatgctgaacaactcaaagaaaatggtgtgattaactacagtgtattagatttgacagcagaagaactagaggctatcaaacatcagcttaatccaaaagataatgatgtagagctttgagttaataaaaaagtggggcaaataaatcatcatggaaaagtttgctcctgaattccatggagaagatgcaaacaacagagccaccaaattcctagaatcaataaagggcaaattcacatcacccaaagatcccaagaaaaaagatagtatcatatctgtcaactcaatagatatagaagtaaccaaagaaagccctataacatcaaattcaaccattataaacccaataaatgagacagatgatactgtagggaacaagcccaattatcaaagaaagcctctagtaagtttcaaagaagaccctacgccaagtgataatcctttttcaaaactatacaaagaaaccatagaaacatttgataacaatgaagaagaatctagctattcatatgaagaaataaatgatcagacaaacgataatataacagcaagattagataggattgatgagaaattaagtgaaatactaggaatgcttcacacattagtagtagcgagtgcaggacccacatctgctcgggatggtataagagatgccatggttggtttaagagaagaaatgatagaaaaaatcagaactgaagcattaatgaccaatgacagactagaagctatggcaagactcaggaatgaagaaagtgaaaagatggcaaaagacacatcagatgaagtgtctctcaatccaacatcagagaaactgaacaacctgttggaagggaatgatagtgacaatgatctatcacttgaagatttctgattagctaccaaactgtacatcaaaacacaacaccaatagaaaaccaacaaacaaaccaactcacccatccaaccaaacatctatctgctgattagccaaccagccaaaaaacaaccagccaatctaaaactagccacccggaaaaaatcgatactatagttacaaaaaaagatggggcaaatatggaaacatacgtgaataaacttcacgagggctccacatacacagctgctgttcaatacaatgtcctagaaaaagacgatgatcctgcatcacttacaatatgggtgcccatgttccaatcatccatgccagcagatctactcataaaagaactagccaatgtcaatatactagtgaaacaaatatccacacccaagggaccctcattaagagtcatgataaactcaagaagtgcagtgctagcacaaatgcccagcaaatttaccatatgtgccaatgtgtccttggatgaaagaagcaagctggcatatgatgtaaccacaccctgtgaaattaaggcatgcagtctaacatgcctaaaatcaaaaaatatgttaactacagttaaagatctcactatgaaaacactcaacccaacacatgacatcattgctttatgtgaatttgaaaatatagtaacatcaaaaaaagtcataataccaacatacctaagatctatcagcgtcagaaataaagatctgaacacacttgaaaatataacaaccactgaattcaaaaatgccattacaaatgcaaaaatcatcccttactcaggattattgttagtcatcacagtgactgacaacaaaggagcattcaaatacataaagccacaaagtcaattcatagtagatcttggagcttacctagaaaaagaaagtatatattatgttacaacaaattggaagcacacagctacacgatttgcaatcaaacccatggaagattaacctttttcctctacatcaatgagtagattcatacaaactttctaactacattcttcacttcacaatcataatcaccaaccctctgtggttcaatcaatcaaacaaaactcatcaagagttccagatcatcccaagtcattgttcatcagatccagtactcaaataagttaataaaaaatccacatggggcaaataatcattgagggaaatccaactaatcacaacatctgtcaacatagacaagtcaacacgctagataaaatcaaccaatggaaaatacatccataactatagaattctcaagcaaattctggccttactttacactaatacacatgataacaacaataatctctttgataatcataatctccatcatgattgcaatactaaacaaactctgcgaatataatgtattccataacaaaacctttgagctaccaagagctcgagtcaatacatagcattcaccaatctgatagctcaaaacagtaaccttgcatttgtaaatgaactaccctcacttcttcacaaaaccacatcaacatctcaccatgcaagccatcatctataccataaagtagttaattaaaaatggccggccagtcataacaatgaactaggatattaagaccaaaaacaacgctggggcaaatgcaaacatgtccaaaaccgaggaccaacgcaccgccaagacactagaaaggacctgggacacttttaatcatctattattcatatcatcgtgcttatacaagttaaatcttaaatctatagcacaaatcacattatctattttggcaattataatctcaacctcacttataattgcagccatcatattcatagcctcggcaaaccacaaagtcacactaacaactgcaatcatacaagatgcaacgaaccagatcaagaacacaaccccaacatacctcacccagaatccccagcatggaatcagcttctccaatctgtccggaactacatcacaatccaccaccatactagcttcaacaacaccaagtgctgattcaaccccacaatccacaacagtcaagatcaaaaacacaacaacaacccaaatattacctagcaaacccaccacaaaacaacgccaaaataaaccacaaaacaaacccaacaatgattttcactttgaagtgttcaattttgtaccctgcagcatatgcagcaacaatccaacctgctgggccatctgcaagagaataccaaacaaaaaacctggaaagaaaaccaccaccaagcccacaaaaaaaccaaccctcaagacaaccaaaaaagatcccaaatcccaaaccacaaaaccaaaggaagtactcactaccaagcctacaggaaagccaaccatcaacaccactaaaacaaacatcagaactacactgctcacctccaacaccaaaggaaatccagaacacacaagtcaagaggaaaccctccactcaaccacctccgaaggctatccaagcccatcacaagtccacacaacatccggtcaagaggaaaccctccactcaaccacctccgaaggctatccaagcccatcacaagtctacacaacatccgagtacctatcacaatctctatcttcatccaacacaacaaaatgatagtcattaaaaagcacgcgtgtattgttgcaaaaagccatgaccaaatcaaacagaatcaaaatcaactctggggcaaataacaatggagttgccaatcctcaaaacaaatgctattaccacaatccttgctgcagtcacactctgtttcgcttccagtcaaaacatcactgaagaattttatcaatcaacatgcagtgcagtcagcaaaggctatcttagtgctctaagaactggttggtatactagtgttataactatagaattaagtaatatcaaggaaaataagtgtaatggtacagacgctaaggtaaaattaataaaacaagaattagataaatataaaaatgctgtaacagaattgcagttgctcatgcaaagcacaccagcagccaacaatcgaccctccaaggaactaccaagatttatgaattatacactcaacaataccaaaaacaccaatgtaacattaagtaagaaaaggaaaagaagatttcttggatttttgttaggtgttggatctgcaatcgccagtggcattgccgtatccaaggtcctgcacctagaaggggaagtgaacaaaatcaaaagtgctctactatccacaaacaaggctgtagtcagcttatctaatggagtcagtgtcttaaccagcaaggtgttagacctcaaaaactatatagataaacagttgttacctattgttaacaagcaaagctgcagcatatcaaacattgaaactgtgatagagttccaacaaaagaacaacagactactagagattaccagagaatttagtgttaatgcaggtgtaactactcctgtaagcacttatatgttaactaatagtgagttattatcattaatcaatgatatgcctataacaaatgatcagaaaaagttaatgtccagcaatgttcaaatagttagacagcaaagttactctatcatgtcaataataaaagaggaagtcttggcatatgtagtacaattaccactatatggtgtaatagatactccttgttggaaactacacacatcccctttatgtacaaccaacacaaaggaaggatccaacatctgcttaacaagaaccgacagaggatggtactgtgacaatgcaggatcagtatcctttttcccacaagctgaaacatgtaaagttcaatcgaatcgggtgttttgtgacacaatgaacagtttaacattaccaagtgaggtaaatctctgcaacattgacatattcaaccccaaatatgattgcaaaattatgacttcaaaaacagatgtaagcagctccgttatcacatctctaggagccattgtgtcatgctatggcaaaaccaaatgtacagcatccaataaaaatcgtgggatcataaagacattctctaacgggtgtgattatgtatcaaataagggggtggatactgtgtctgtaggtaatacattatattatgtaaataagcaagaaggcaaaagtctctatgtaaaaggtgaaccaataataaatttctatgatccattagtgttcccctctgatgaatttgatgcatcaatatctcaagtcaatgagaaaattaatcagagtctagcatttatccgtaaatcagatgaattattacataatgtaaatgctggtaaatccaccacaaatatcatgataactaccataattatagtaattatagtaatattgttagcattaattgcagttggactgcttctatactgcaaggccagaagcacaccagtcacattaagtaaggatcaactgagtggtataaataatattgcatttagtaactgaataaaaatagcacctaatcatattcttacaatggttcgctatttgaccatagataacccatctatcattagattatcctaaaatttgaacttcatcacaactttcatctataaaccatctcacttacactttttaagtagatttctattttatagttatataaaacagggcccattgaataccaaattaacttactatttgtaaaaatgagaattggggcaaatatgtcacgaaggaatccttgcaaattcgaaattcgaggtcattgcttgaatggtaaaaggtgtcattttagtcataattattttgaatggccaccccatgcactgcttgtaagacaaaactttatgttaaacagaatacttaagtctatggataaaagcatagatactttgtcagaaataagtggagctgcagagttggacagaacagaagagtatgccctcggtgtagttggagtgctagagagttatataggatcaataaataatataactaaacaatcagcatgtgttgccatgagcaaactccttactgaactcaacagcgatgacatcaaaaaactaagggacaatgaagagccaaactcacccaaagtaagagtgtacaatactgtcatatcatatattgaaagcaacaggaagaacaataaacaaactatccatctgttaaaaagattgccagcagacgtattgaagaaaaccatcaaaaacacattggatatccacaagagcataaccatcaataacccaaaagaatcaactgttagtgatacgaacgaccatgccaaaaataatgatactacctgacaaatatccttgtagtataaattccatactaataacaagtaattgtagagtcactatgtataatcaaaaaaacacactatatatcaatcaaaacaaccaaaatagccatatatacccaccggatcaaccattcaatgaaatccattggacctctcaagacttgattgatgcaactcaaaattttctacaacatctaggtattactgatgatatatacacaatatatatattagtgtcataatactcaatcctaatacttaccacatcatcaaattattaactcaaacaattcaagctatgggacaaaatggatcccattattagtggaaattctgctaatgtttatctaactgatagttatttaaaaggtgttatttctttctcagaatgtaacgctttaggaagttacatattcaatggtccttatctcaaaaatgattataccaacttaattagtagacaaaatccattaatagaacacataaatctaaagaaactaaatataacacagtccttaatatctaagtatcataaaggtgaaataaaaatagaagaacctacttactttcagtcattacttatgacatacaagagtatgacctcttcagaacagactactactactaatttacttaaaaagataataagaagagctatagaaatcagtgatgtcaaagtctatgctatattgaataaactggggctcaaagaaaaagacaagattaaatccaataatggacaagatgaagacaactcagtcattactaccataatcaaagatgatatacttttagctgtcaaggataatcaatctcatcttaaagcagacaaaaatcaatccacaaaacaaaaagatacaatcaaaacaacacttttgaagaaattaatgtgttcgatgcaacatcctccatcatggttaatacattggtttaatttatacacaaaattaaacagcatattaacacaatatcgatctagtgaggtaaaaaaccatggttttatattgatagataatcatactcttagtggattccaatttattttgaatcaatatggttgtatagtttatcataaggaactcaaaagaattactgtgacaacttataatcaattcttgacatggaaagatattagccttagtagattaaatgtttgtttgattacatggattagtaactgtttgaacacattaaacaaaagcttaggcttaagatgtggattcaataatgttatcttgacacaattattcctttatggagattgtatactaaaactattccacaatgaggggttctacataataaaagaggtagagggatttattatgtctctaattttaaatataacagaagaagatcaattcagaaaacggttttataatagtatgctcaacaacatcacagatgccgccaacaaagctcaaaaaaatctgctatcaagagtatgtcatacattattagataagacaatatcagataatataataaatggcagatggataattctattgagtaagttcctaaaattaattaagcttgcaggtgacaataacctcaacaatctgagtgaattatattttttgttcagaatatttggacacccaatggtagatgaaagacaagccatggatgctgttaaagttaattgcaacgagaccaaattttatttgttaagtagtttgagtatgttaagaggagcttttatatatagaattataaaagggtttgtaaataattacaacagatggcctactttaagaaatgccattgtcttacccttaagatggttaacttactataaactaaacacttatccttccttgttggaacttacagaaagagatttgattgttctatcaggactacgtttctatcgagagtttcggttgcctaaaaaagtggatcttgaaatgatcataaatgataaggctatatcacctcctaaaaatttaatatggactagtttccctagaaattatatgccgtcacacatacaaaattatatagaacatgaaaaattaaaattctctgatagtgataaatcaagaagagtattagagtattatttaagagataacaaattcaatgaatgtgatttacacaactgtgtagttaatcaaagttatcttaacaacccgaatcatgtggtatcattgacaggcaaagaaagagaactcagtgtaggtagaatgtttgcaatgcaaccaggaatgttcagacaagttcaaatattagcagagaaaatgatagcagaaaacatattacaatttttccctgaaagtcttacaagatatggtgatctagaactacagaaaatattagaattgaaagcaggaataagtaacaaatcaaatcgttacaatgataattacaacaattacattagtaagtgctctatcatcacagatctcagcaaattcaatcaagcatttcgatatgaaacatcatgtatttgtagtgatgtactggatgaactgcatggtgtacaatctctattttcctggttacatttaactattcctcatgtcacaataatatgcacatataggcatgcacccccctatataaaggatcatattgtagatcttaacaatgtagatgagcaaagtggactatatagatatcatatgggtggtatcgaagggtggtgtcaaaaactatggaccatagaagctatatcactattagatctaatatctctcaaagggaaattctcaattactgctttaattaatggtgacaatcaatcaatagatataagtaaaccagtcagactcatggaaggtcaaactcatgctcaagcagattatttgctagcattaaatagtctcaaattactgtataaagagtatgcaggaataggccacaaattaaaaggaactgagacttatatatcgagagatatgcaatttatgagtaaaacgatccaacataacggtgtatattacccagctagtataaagaaagtcctaagagtgggaccgtggataaacactatacttgatgacttcaaagtgagtctagaatctataggtagtttgacacaagaattagaatatagaggtgaaagtctattatgcagtttaatatttagaaatgtatggttatataatcaaattgcattacaacttaaaaatcatgcattatgtaacaacaaattatatttggatatattaaaagttctaaaacacttaaaaaccttttttaatcttgataacattgatacagcattaacattgtatatgaatttgcccatgttatttggtggtggtgatcccaacttgttatatcgaagtttctatagaagaactcctgatttcctcacagaggctatagttcactctgtgttcatacttagttattatacaaaccatgatttaaaagataaacttcaagatctgtcagatgatagattgaataagttcttaacatgcataatcacgtttgataaaaaccccaatgctgaattcgttacattgatgagagatcctcaagctttaggatctgagaggcaagctaaaattactagcgaaatcaatagactggcagttaccgaggttttgagcacagctccaaacaaaatattttccaaaagtgcacaacactataccactacagagatagatcttaatgatattatgcaaaatatagaacctacatatcctcacgggctaagagttgtttatgagagtttacccttttataaagcagagaaaatagtaaatcttatatccggtacaaaatctataactaacatactggaaaagacttctgccatagacttaacagatattgatagagccactgagatgatgaggaaaaacataactttgcttataaggatattaccattagattgtaacagagataaaagagaaatattgagtatggaaaacctaagtattactgaattaagcaaatacgttagagaaagatcttggtctttatccaatatagttggtgttacatcacccagtatcatgtatacaatggacataaaatatacaacaagcactatagctagtggcataatcatagagaaatataatgtcaacagtttaacacgtggtgagagaggacccactaaaccatgggttggttcatctacacaagagaaaaagacaatgccagtttataatagacaagttttaaccaaaaaacagagagatcaaatagatctattagcaaaattggattgggtgtatgcatctatagataacaaggatgaatttatggaggaacttagcataggaactcttgggttaacatatgagaaggccaaaaaattattcccacaatatttgagtgttaactatttgcatcgtcttacagtcagtagtagaccatgtgaattccctgcatctataccagcttatagaactacaaattatcactttgatactagccctattaatcgcatattaacagaaaagtatggtgatgaagatattgatatagtattccaaaactgtataagctttggccttagcttaatgtctgtagtagaacaatttactaatgtatgtcctaacagaattattctcatacccaagcttaatgagatacatttgatgaaacctcccatattcacaggcgatgttgatattcacaagttaaaacaagtgatacaaaaacaacatatgtttttaccagacaaaataagtttgactcaatatgtggaattattcttaagtaataaaacactcaaatctggatctaatgttaattctaatttaatattggcgcataagatatctgactattttcataatacttacattttgagtactaatttagctggacattggattcttattatacaacttatgaaagattctaagggtatttttgaaaaagattggggagagggatatataactgatcatatgttcattaatttgaaagttttcttcaatgcttataagacatatctcttgtgttttcataaaggttacggcagagcaaagctggagtgtgatatgaatacttcagatctcctatgtgtattggaattaatagacagtagttattggaagtctatgtctaaggtgtttttagaacaaaaagttatcaaatacattcttagccaggatgcaagtttacatagagtaaaaggatgtcatagcttcaaactatggtttcttaaacgtcttaatgtagcagaattcacagtttgcccttgggttgttaacatagattatcatccaacacatatgaaagcaatattaacttatattgatcttgttagaatgggattgataaatatagatagaatatacattaaaaataaacacaagttcaatgatgagttttatacttctaatctgttttacattaattataacttctcagataatactcatctattaactaaacatataaggattgctaattccgaattagaaagtaattacaacaaattatatcatcctacaccagaaaccctagaaaatatactaaccaatccggttaaaagtaatgagaaaaagacactgagtgactattgtataggtaaaaatgttgactcaataatgttaccatcgttatctaataagaagcttattaaatcgtctacaatgattagaaccaattacagcagacaagatttgtataatttatttcctacggttgtgattgataaaattatagatcattcaggtaatacagccaaatctaaccaactttacactactacttctcatcaaatatccttagtgcacaatagcacatcactttattgcatgcttccttggcatcatattaatagattcaattttgtatttagttctacaggttgtaaaattagtatagagtatattttaaaagatcttaaaattaaggatcctaattgtatagcattcataggtgaaggagcagggaatttattattgcgtacagtagtggaacttcatcctgatataagatatatttacagaagtctgaaagattgcaatgatcatagtttaccaattgagtttttaaggctgtacaatggacatatcaacattgattatggtgaaaatttgaccattcctgctacagatgcaaccaacaacattcattggtcttatttacatataaagtttgctgaacctatcagtctttttgtctgtgatgctgaattgcctgtaacagtcaactggagtaagattataatagagtggagcaagcatgtaagaaaatgcaagtactgttcttcagttaataaatgtacattgatagtaaaatatcatgctcaagatgatatcgatttcaaattagacaacataactatattaaaaacttatgtatgcttaggtagtaagttaaagggatctgaagtttacttagtccttacaataggtcctgcaaatgtgttcccagtatttaatgtagtacaaaatgctaaattgatactatcaagaactaaaaatttcatcatgcctaaaaaagctgataaagagtctattgatgcaaatattaagagtttgataccctttctttgttaccctataacaaaaaaaggaattaatactgcattgtctaaattaaagagtgttgttagtggagatatactatcatattctatagctggacgtaatgaagttttcagcaataaacttataaatcataagcatatgaacatcttaaagtggttcaatcatgttttaaatttcagatcaacagaattaaactataatcatttatatatggtagaatctacttatcctcatctaagtgaattgttaaacagcttgacaaccaatgaacttaaaaaactgattaaaatcacaggtagtttgttatacaacttttataatgaataatgagcaaaaatcttataacaaaaatagctacacactaacattgtattcaattatagttattgaaaattaataattatataatttttaataacttctagtgaactaatcctaaaattatcattttgatctaggaagaataagtttaaatccaaatctaattggtttatatgtatattaactaaattacgagatattagtttttgacactttttttctcgtggccggcatggtcccagcctcctcgctggcgccggctgggcaacatgcttcggcatggcgaatgggactagcataaccccttggggcctctaaacgggtcttgaggggttttttg

SEQ ID NO: 27 - DNA, 15494 bp, synthetic construct
  misc_feature 1..15494: note = antigenic cDNA encoding cRSVA_ mF2
  source 1..15494: mol_type = other DNA
taatacgactcactataggttttttcgcgtctgatgaggccgttaggccgaaactcctctccggagtcacgcgaaaaaatgcgtacaacaaacttgcgtaaaccaaaaaaatggggcaaataagaatttgataagtaccacttaaatttaactcctttggttagaggcgcgccatgggcagcaactcattgagtatgataaaagttagattgcaaaatctgtttgacaatgatgaagtagcattgttaaaaataacatgctatactgacaaattaatacagttaactaatgctttggctaaggcagttatacatacaatcaaattgaatggcattgtatttgtgcatgttattacaagtagtgatatttgccctaataataatattgtagtgaaatccaatttcacaacaatgccagtattacaaaatggaggttatatatgggaaatgatggaattaacacactgctctcaacctaatggcctaatagatgacaattgtgaaattaaattctccaaaaaactaagtgattcaacaatgaccaattatatgaatcaattatctgaattacttggatttgacctcaatccataaatcataataaatatcaactagcaaatcaatgtcactaacaccattagttaatataaaacttgacagaagataaaaatggggcaaataaatcaattcagccgacccaaccatggacacaacacacaatgataccacaccacaaagactgatgatcacagacatgaggccattatcgcttgagactataataacatctctaaccagagatatcataacacataaatttatatacttgataaatcatgaatgcatagtaagaaaacttgatgaaagacaggccacatttacatttctggtcaactatgaaatgaaactattgcacaaagtgggaagcactaaatataaaaaatatactgaatacaacacaaaatatggcactttccctatgccaatatttatcaatcatgatgggttcttagaatgcattggcattaagcctaccaagcacacacccataatatacaagtatgatctcaatccatgaatatcaaaccaagattcaaacaatccgaaataacaactttatgcataatcacactccatagtccaaatggagcctgaaaattatagttatttaaaattcctgcaggaaggagagacataagatgaaagatggggcaaatacaaaaatggctcttagcaaagtcaagttgaatgatacactcaacaaagatcaacttctatcatccagcaaatataccatccaacggagcacaggagacagcattgacactcctaattatgatgtgcagaaacacattaataagttatgtggcatgttattaatcacagaagatgctaatcataaattcactgggttaataggtatgttatatgctatgtctagattaggaagagaagacaccataaaaatactcaaagatgcgggatatcatgttaaggcaaatggagtggatgtaacaacacatcgtcaagacattaatgggaaagaaatgaaatttgaagtgttaacattagcaagcttaacaactgaaattcaaatcaacattgagatagaatctagaaaatcctacaaaaaaatgctaaaagaaatgggagaggtggctccagaatacaggcatgactctcctgattgtgggatgataatattatgtatagcggcattagtaataaccaaattagcagcaggagatagatcaggtcttacagctgtgattaggagagctaataatgtcctaaaaaatgaaatgaaacgttataaaggtttattacccaaggatatagccaacagcttctatgaagtgtttgaaaaatatcctcactttatagatgtttttgttcattttggtatagcacaatcttctaccagaggtggcagtagagttgaagggatttttgcaggattgtttatgaatgcctatggtgcagggcaagtgatgttacggtggggggtcttagcaaaatcagttaaaaacattatgttaggacacgctagtgtacaagcagaaatggaacaagttgtggaggtgtatgagtatgctcagaaattgggtggagaagcaggattctaccatatattgaacaacccaaaagcatcactattatctttgactcaatttcctcacttctctagtgtagtattgggcaatgctgctggcctaggcataatgggagaatacagaggtacaccaaggaatcaagatttatatgatgctgcaaaagcatatgctgaacaactcaaagaaaatggtgtgattaactacagtgtattagatttgacagcagaagaactagaggctatcaaacatcagcttaatccaaaagataatgatgtagagctttgagttaataaaaaagtggggcaaataaatcatcatggaaaagtttgctcctgaattccatggagaagatgcaaacaacagagccaccaaattcctagaatcaataaagggcaaattcacatcacccaaagatcccaagaaaaaagatagtatcatatctgtcaactcaatagatatagaagtaaccaaagaaagccctataacatcaaattcaaccattataaacccaataaatgagacagatgatactgtagggaacaagcccaattatcaaagaaagcctctagtaagtttcaaagaagaccctacgccaagtgataatcctttttcaaaactatacaaagaaaccatagaaacatttgataacaatgaagaagaatctagctattcatatgaagaaataaatgatcagacaaacgataatataacagcaagattagataggattgatgagaaattaagtgaaatactaggaatgcttcacacattagtagtagcgagtgcaggacccacatctgctcgggatggtataagagatgccatggttggtttaagagaagaaatgatagaaaaaatcagaactgaagcattaatgaccaatgacagactagaagctatggcaagactcaggaatgaagaaagtgaaaagatggcaaaagacacatcagatgaagtgtctctcaatccaacatcagagaaactgaacaacctgttggaagggaatgatagtgacaatgatctatcacttgaagatttctgattagctaccaaactgtacatcaaaacacaacaccaatagaaaaccaacaaacaaaccaactcacccatccaaccaaacatctatctgctgattagccaaccagccaaaaaacaaccagccaatctaaaactagccacccggaaaaaatcgatactatagttacaaaaaaagatggggcaaatatggaaacatacgtgaataaacttcacgagggctccacatacacagctgctgttcaatacaatgtcctagaaaaagacgatgatcctgcatcacttacaatatgggtgcccatgttccaatcatccatgccagcagatctactcataaaagaactagccaatgtcaatatactagtgaaacaaatatccacacccaagggaccctcattaagagtcatgataaactcaagaagtgcagtgctagcacaaatgcccagcaaatttaccatatgtgccaatgtgtccttggatgaaagaagcaagctggcatatgatgtaaccacaccctgtgaaattaaggcatgcagtctaacatgcctaaaatcaaaaaatatgttaactacagttaaagatctcactatgaaaacactcaacccaacacatgacatcattgctttatgtgaatttgaaaatatagtaacatcaaaaaaagtcataataccaacatacctaagatctatcagcgtcagaaataaagatctgaacacacttgaaaatataacaaccactgaattcaaaaatgccattacaaatgcaaaaatcatcccttactcaggattattgttagtcatcacagtgactgacaacaaaggagcattcaaatacataaagccacaaagtcaattcatagtagatcttggagcttacctagaaaaagaaagtatatattatgttacaacaaattggaagcacacagctacacgatttgcaatcaaacccatggaagattaacctttttcctctacatcaatgagtagattcatacaaactttctaactacattcttcacttcacaatcataatcaccaaccctctgtggttcaatcaatcaaacaaaactcatcaagagttccagatcatcccaagtcattgttcatcagatccagtactcaaataagttaataaaaaatccacatggggcaaataatcattgagggaaatccaactaatcacaacatctgtcaacatagacaagtcaacacgctagataaaatcaaccaatggaaaatacatccataactatagaattctcaagcaaattctggccttactttacactaatacacatgataacaacaataatctctttgataatcataatctccatcatgattgcaatactaaacaaactctgcgaatataatgtattccataacaaaacctttgagctaccaagagctcgagtcaatacatagcattcaccaatctgatagctcaaaacagtaaccttgcatttgtaaatgaactaccctcacttcttcacaaaaccacatcaacatctcaccatgcaagccatcatctataccataaagtagttaattaaaaatggccggccagtcataacaatgaactaggatattaagaccaaaaacaacgctggggcaaatgcaaacatgtccaaaaccgaggaccaacgcaccgccaagacactagaaaggacctgggacacttttaatcatctattattcatatcatcgtgcttatacaagttaaatcttaaatctatagcacaaatcacattatctattttggcaattataatctcaacctcacttataattgcagccatcatattcatagcctcggcaaaccacaaagtcacactaacaactgcaatcatacaagatgcaacgaaccagatcaagaacacaaccccaacatacctcacccagaatccccagcatggaatcagcttctccaatctgtccggaactacatcacaatccaccaccatactagcttcaacaacaccaagtgctgattcaaccccacaatccacaacagtcaagatcaaaaacacaacaacaacccaaatattacctagcaaacccaccacaaaacaacgccaaaataaaccacaaaacaaacccaacaatgattttcactttgaagtgttcaattttgtaccctgcagcatatgcagcaacaatccaacctgctgggccatctgcaagagaataccaaacaaaaaacctggaaagaaaaccaccaccaagcccacaaaaaaaccaaccctcaagacaaccaaaaaagatcccaaatcccaaaccacaaaaccaaaggaagtactcactaccaagcctacaggaaagccaaccatcaacaccactaaaacaaacatcagaactacactgctcacctccaacaccaaaggaaatccagaacacacaagtcaagaggaaaccctccactcaaccacctccgaaggctatccaagcccatcacaagtccacacaacatccggtcaagaggaaaccctccactcaaccacctccgaaggctatccaagcccatcacaagtctacacaacatccgagtacctatcacaatctctatcttcatccaacacaacaaaatgatagtcattaaaaagcacgcgtgtattgttgcaaaaagccatgaccaaatcaaacagaatcaaaatcaactctggggcaaataacaatggagttgccaatcctcaaaacaaatgctattaccacaatccttgctgcagtcacactctgtttcgcttccagtcaaaacatcactgaagaattttatcaatcaacatgcagtgcagtcagcaaaggctatcttagtgctctaagaactggttggtatactagtgttataactatagaattaagtaatatcaaggaaaataagtgtaatggtacagacgctaaggtaaaattaataaaacaagaattagataaatataaaaatgctgtaacagaattgcagttgctcatgcaaagcacaccagcagccaacaatcgagccagaagagaactaccaagatttatgaattatacactcaacaataccaaaaacaccaatgtaacattaagtaagaaaaggaaaagaaagtttcttggatttttgttaggtgttggatctgcaatcgccagtggcattgccgtatccaaggtcctgcacctagaaggggaagtgaacaaaatcaaaagtgctctactatccacaaacaaggctgtagtcagcttatctaatggagtcagtgtcttaaccagcaaggtgttagacctcaaaaactatatagataaacagttgttacctattgttaacaagcaaagctgcagcatatcaaacattgaaactgtgatagagttccaacaaaagaacaacagactactagagattaccagagaatttagtgttaatgcaggtgtaactactcctgtaagcacttatatgttaactaatagtgagttattatcattaatcaatgatatgcctataacaaatgatcagaaaaagttaatgtccagcaatgttcaaatagttagacagcaaagttactctatcatgtcaataataaaagaggaagtcttggcatatgtagtacaattaccactatatggtgtaatagatactccttgttggaaactacacacatcccctttatgtacaaccaacacaaaggaaggatccaacatctgcttaacaagaaccgacagaggatggtactgtgacaatgcaggatcagtatcctttttcccacaagctgaaacatgtaaagttcaatcgaatcgggtgttttgtgacacaatgaacagtttaacattaccaagtgaggtaaatctctgcaacattgacatattcaaccccaaatatgattgcaaaattatgacttcaaaaacagatgtaagcagctccgttatcacatctctaggagccattgtgtcatgctatggcaaaaccaaatgtacagcatccaataaaaatcgtgggatcataaagacattctctaacgggtgtgattatgtatcaaataagggggtggatactgtgtctgtaggtaatacattatattatgtaaataagcaagaaggcaaaagtctctatgtaaaaggtgaaccaataataaatttctatgatccattagtgttcccctctgatgaatttgatgcatcaatatctcaagtcaatgagaaaattaatcagagtctagcatttatccgtaaatcagatgaattattacataatgtaaatgctggtaaatccaccacaaatatcatgataactaccataattatagtaattatagtaatattgttagcattaattgcagttggactgcttctatactgcaaggccagaagcacaccagtcacattaagtaaggatcaactgagtggtataaataatattgcatttagtaactgaataaaaatagcacctaatcatattcttacaatggttcgctatttgaccatagataacccatctatcattagattatcctaaaatttgaacttcatcacaactttcatctataaaccatctcacttacactttttaagtagatttctattttatagttatataaaacagggcccattgaataccaaattaacttactatttgtaaaaatgagaattggggcaaatatgtcacgaaggaatccttgcaaattcgaaattcgaggtcattgcttgaatggtaaaaggtgtcattttagtcataattattttgaatggccaccccatgcactgcttgtaagacaaaactttatgttaaacagaatacttaagtctatggataaaagcatagatactttgtcagaaataagtggagctgcagagttggacagaacagaagagtatgccctcggtgtagttggagtgctagagagttatataggatcaataaataatataactaaacaatcagcatgtgttgccatgagcaaactccttactgaactcaacagcgatgacatcaaaaaactaagggacaatgaagagccaaactcacccaaagtaagagtgtacaatactgtcatatcatatattgaaagcaacaggaagaacaataaacaaactatccatctgttaaaaagattgccagcagacgtattgaagaaaaccatcaaaaacacattggatatccacaagagcataaccatcaataacccaaaagaatcaactgttagtgatacgaacgaccatgccaaaaataatgatactacctgacaaatatccttgtagtataaattccatactaataacaagtaattgtagagtcactatgtataatcaaaaaaacacactatatatcaatcaaaacaaccaaaatagccatatatacccaccggatcaaccattcaatgaaatccattggacctctcaagacttgattgatgcaactcaaaattttctacaacatctaggtattactgatgatatatacacaatatatatattagtgtcataatactcaatcctaatacttaccacatcatcaaattattaactcaaacaattcaagctatgggacaaaatggatcccattattagtggaaattctgctaatgtttatctaactgatagttatttaaaaggtgttatttctttctcagaatgtaacgctttaggaagttacatattcaatggtccttatctcaaaaatgattataccaacttaattagtagacaaaatccattaatagaacacataaatctaaagaaactaaatataacacagtccttaatatctaagtatcataaaggtgaaataaaaatagaagaacctacttactttcagtcattacttatgacatacaagagtatgacctcttcagaacagactactactactaatttacttaaaaagataataagaagagctatagaaatcagtgatgtcaaagtctatgctatattgaataaactggggctcaaagaaaaagacaagattaaatccaataatggacaagatgaagacaactcagtcattactaccataatcaaagatgatatacttttagctgtcaaggataatcaatctcatcttaaagcagacaaaaatcaatccacaaaacaaaaagatacaatcaaaacaacacttttgaagaaattaatgtgttcgatgcaacatcctccatcatggttaatacattggtttaatttatacacaaaattaaacagcatattaacacaatatcgatctagtgaggtaaaaaaccatggttttatattgatagataatcatactcttagtggattccaatttattttgaatcaatatggttgtatagtttatcataaggaactcaaaagaattactgtgacaacttataatcaattcttgacatggaaagatattagccttagtagattaaatgtttgtttgattacatggattagtaactgtttgaacacattaaacaaaagcttaggcttaagatgtggattcaataatgttatcttgacacaattattcctttatggagattgtatactaaaactattccacaatgaggggttctacataataaaagaggtagagggatttattatgtctctaattttaaatataacagaagaagatcaattcagaaaacggttttataatagtatgctcaacaacatcacagatgccgccaacaaagctcaaaaaaatctgctatcaagagtatgtcatacattattagataagacaatatcagataatataataaatggcagatggataattctattgagtaagttcctaaaattaattaagcttgcaggtgacaataacctcaacaatctgagtgaattatattttttgttcagaatatttggacacccaatggtagatgaaagacaagccatggatgctgttaaagttaattgcaacgagaccaaattttatttgttaagtagtttgagtatgttaagaggagcttttatatatagaattataaaagggtttgtaaataattacaacagatggcctactttaagaaatgccattgtcttacccttaagatggttaacttactataaactaaacacttatccttccttgttggaacttacagaaagagatttgattgttctatcaggactacgtttctatcgagagtttcggttgcctaaaaaagtggatcttgaaatgatcataaatgataaggctatatcacctcctaaaaatttaatatggactagtttccctagaaattatatgccgtcacacatacaaaattatatagaacatgaaaaattaaaattctctgatagtgataaatcaagaagagtattagagtattatttaagagataacaaattcaatgaatgtgatttacacaactgtgtagttaatcaaagttatcttaacaacccgaatcatgtggtatcattgacaggcaaagaaagagaactcagtgtaggtagaatgtttgcaatgcaaccaggaatgttcagacaagttcaaatattagcagagaaaatgatagcagaaaacatattacaatttttccctgaaagtcttacaagatatggtgatctagaactacagaaaatattagaattgaaagcaggaataagtaacaaatcaaatcgttacaatgataattacaacaattacattagtaagtgctctatcatcacagatctcagcaaattcaatcaagcatttcgatatgaaacatcatgtatttgtagtgatgtactggatgaactgcatggtgtacaatctctattttcctggttacatttaactattcctcatgtcacaataatatgcacatataggcatgcacccccctatataaaggatcatattgtagatcttaacaatgtagatgagcaaagtggactatatagatatcatatgggtggtatcgaagggtggtgtcaaaaactatggaccatagaagctatatcactattagatctaatatctctcaaagggaaattctcaattactgctttaattaatggtgacaatcaatcaatagatataagtaaaccagtcagactcatggaaggtcaaactcatgctcaagcagattatttgctagcattaaatagtctcaaattactgtataaagagtatgcaggaataggccacaaattaaaaggaactgagacttatatatcgagagatatgcaatttatgagtaaaacgatccaacataacggtgtatattacccagctagtataaagaaagtcctaagagtgggaccgtggataaacactatacttgatgacttcaaagtgagtctagaatctataggtagtttgacacaagaattagaatatagaggtgaaagtctattatgcagtttaatatttagaaatgtatggttatataatcaaattgcattacaacttaaaaatcatgcattatgtaacaacaaattatatttggatatattaaaagttctaaaacacttaaaaaccttttttaatcttgataacattgatacagcattaacattgtatatgaatttgcccatgttatttggtggtggtgatcccaacttgttatatcgaagtttctatagaagaactcctgatttcctcacagaggctatagttcactctgtgttcatacttagttattatacaaaccatgatttaaaagataaacttcaagatctgtcagatgatagattgaataagttcttaacatgcataatcacgtttgataaaaaccccaatgctgaattcgttacattgatgagagatcctcaagctttaggatctgagaggcaagctaaaattactagcgaaatcaatagactggcagttaccgaggttttgagcacagctccaaacaaaatattttccaaaagtgcacaacactataccactacagagatagatcttaatgatattatgcaaaatatagaacctacatatcctcacgggctaagagttgtttatgagagtttacccttttataaagcagagaaaatagtaaatcttatatccggtacaaaatctataactaacatactggaaaagacttctgccatagacttaacagatattgatagagccactgagatgatgaggaaaaacataactttgcttataaggatattaccattagattgtaacagagataaaagagaaatattgagtatggaaaacctaagtattactgaattaagcaaatacgttagagaaagatcttggtctttatccaatatagttggtgttacatcacccagtatcatgtatacaatggacataaaatatacaacaagcactatagctagtggcataatcatagagaaatataatgtcaacagtttaacacgtggtgagagaggacccactaaaccatgggttggttcatctacacaagagaaaaagacaatgccagtttataatagacaagttttaaccaaaaaacagagagatcaaatagatctattagcaaaattggattgggtgtatgcatctatagataacaaggatgaatttatggaggaacttagcataggaactcttgggttaacatatgagaaggccaaaaaattattcccacaatatttgagtgttaactatttgcatcgtcttacagtcagtagtagaccatgtgaattccctgcatctataccagcttatagaactacaaattatcactttgatactagccctattaatcgcatattaacagaaaagtatggtgatgaagatattgatatagtattccaaaactgtataagctttggccttagcttaatgtctgtagtagaacaatttactaatgtatgtcctaacagaattattctcatacccaagcttaatgagatacatttgatgaaacctcccatattcacaggcgatgttgatattcacaagttaaaacaagtgatacaaaaacaacatatgtttttaccagacaaaataagtttgactcaatatgtggaattattcttaagtaataaaacactcaaatctggatctaatgttaattctaatttaatattggcgcataagatatctgactattttcataatacttacattttgagtactaatttagctggacattggattcttattatacaacttatgaaagattctaagggtatttttgaaaaagattggggagagggatatataactgatcatatgttcattaatttgaaagttttcttcaatgcttataagacatatctcttgtgttttcataaaggttacggcagagcaaagctggagtgtgatatgaatacttcagatctcctatgtgtattggaattaatagacagtagttattggaagtctatgtctaaggtgtttttagaacaaaaagttatcaaatacattcttagccaggatgcaagtttacatagagtaaaaggatgtcatagcttcaaactatggtttcttaaacgtcttaatgtagcagaattcacagtttgcccttgggttgttaacatagattatcatccaacacatatgaaagcaatattaacttatattgatcttgttagaatgggattgataaatatagatagaatatacattaaaaataaacacaagttcaatgatgagttttatacttctaatctgttttacattaattataacttctcagataatactcatctattaactaaacatataaggattgctaattccgaattagaaagtaattacaacaaattatatcatcctacaccagaaaccctagaaaatatactaaccaatccggttaaaagtaatgagaaaaagacactgagtgactattgtataggtaaaaatgttgactcaataatgttaccatcgttatctaataagaagcttattaaatcgtctacaatgattagaaccaattacagcagacaagatttgtataatttatttcctacggttgtgattgataaaattatagatcattcaggtaatacagccaaatctaaccaactttacactactacttctcatcaaatatccttagtgcacaatagcacatcactttattgcatgcttccttggcatcatattaatagattcaattttgtatttagttctacaggttgtaaaattagtatagagtatattttaaaagatcttaaaattaaggatcctaattgtatagcattcataggtgaaggagcagggaatttattattgcgtacagtagtggaacttcatcctgatataagatatatttacagaagtctgaaagattgcaatgatcatagtttaccaattgagtttttaaggctgtacaatggacatatcaacattgattatggtgaaaatttgaccattcctgctacagatgcaaccaacaacattcattggtcttatttacatataaagtttgctgaacctatcagtctttttgtctgtgatgctgaattgcctgtaacagtcaactggagtaagattataatagagtggagcaagcatgtaagaaaatgcaagtactgttcttcagttaataaatgtacattgatagtaaaatatcatgctcaagatgatatcgatttcaaattagacaacataactatattaaaaacttatgtatgcttaggtagtaagttaaagggatctgaagtttacttagtccttacaataggtcctgcaaatgtgttcccagtatttaatgtagtacaaaatgctaaattgatactatcaagaactaaaaatttcatcatgcctaaaaaagctgataaagagtctattgatgcaaatattaagagtttgataccctttctttgttaccctataacaaaaaaaggaattaatactgcattgtctaaattaaagagtgttgttagtggagatatactatcatattctatagctggacgtaatgaagttttcagcaataaacttataaatcataagcatatgaacatcttaaagtggttcaatcatgttttaaatttcagatcaacagaattaaactataatcatttatatatggtagaatctacttatcctcatctaagtgaattgttaaacagcttgacaaccaatgaacttaaaaaactgattaaaatcacaggtagtttgttatacaacttttataatgaataatgagcaaaaatcttataacaaaaatagctacacactaacattgtattcaattatagttattgaaaattaataattatataatttttaataacttctagtgaactaatcctaaaattatcattttgatctaggaagaataagtttaaatccaaatctaattggtttatatgtatattaactaaattacgagatattagtttttgacactttttttctcgtggccggcatggtcccagcctcctcgctggcgccggctgggcaacatgcttcggcatggcgaatgggactagcataaccccttggggcctctaaacgggtcttgaggggttttttg

SEQ ID NO: 28 - DNA, 1638 bp, synthetic construct
  misc_feature 1..1638: note = cDNA encoding a soluble pre F trimer
  source 1..1638: mol_type = other DNA
atggagttgccaatcctcaaaacaaatgctattaccacaatccttgctgcagtcacactctgtttcgcttccagtcaaaacatcactgaagaattttatcaatcaacatgcagtgcagtcagcaaaggctatcttagtgctctaagaactggttggtatactagtgttataactatagaattaagtaatatcaaggaaaataagtgtaatggtacagacgctaaggtaaaattaataaaacaagaattagataaatataaaaatgctgtaacagaattgcagttgctcatgcaaagcacaccagcagccaacaatcgagccagaagagaactaccaagatttatgaattatacactcaacaataccaaaaacaccaatgtaacattaagtaagaaaaggaaaagaagatttcttggatttttgttaggtgttggatctgcaatcgccagtggcattgccgtatccaaggtcctgcacctagaaggggaagtgaacaaaatcaaaagtgctctactatccacaaacaaggctgtagtcagcttatctaatggagtcagtgtcttaaccagcaaggtgttagacctcaaaaactatatagataaacagttgttacctattgttaacaagcaaagctgcagcatatcaaacattgaaactgtgatagagttccaacaaaagaacaacagactactagagattaccagagaatttagtgttaatgcaggtgtaactactcctgtaagcacttatatgttaactaatagtgagttattatcattaatcaatgatatgcctataacaaatgatcagaaaaagttaatgtccagcaatgttcaaatagttagacagcaaagttactctatcatgtcaataataaaagaggaagtcttggcatatgtagtacaattaccactatatggtgtaatagatactccttgttggaaactacacacatcccctttatgtacaaccaacacaaaggaaggatccaacatctgcttaacaagaaccgacagaggatggtactgtgacaatgcaggatcagtatcctttttcccacaagctgaaacatgtaaagttcaatcgaatcgggtgttttgtgacacaatgaacagtttaacattaccaagtgaggtaaatctctgcaacattgacatattcaaccccaaatatgattgcaaaattatgacttcaaaaacagatgtaagcagctccgttatcacatctctaggagccattgtgtcatgctatggcaaaaccaaatgtacagcatccaataaaaatcgtgggatcataaagacattctctaacgggtgtgattatgtatcaaataagggggtggatactgtgtctgtaggtaatacattatattatgtaaataagcaagaaggcaaaagtctctatgtaaaaggtgaaccaataataaatttctatgatccattagtgttcccctctctcctgtgggatgcatcaatatctcaagtcaatgagaaaattaatcagagtctagcatttatccgtaaatcagatgaattattaggctctggcggaagcggatacatccctgaggcaccaagggacggacaggcctacgtgcgcaaggatggcgagtgggtgctgctgtccacctttctgtga

SEQ ID NO: 29 - protein, 545 aa, synthetic construct
  REGION 1..545: note = soluble pre F trimer
MELPILKTNAITTILAAVTLCFASSQNITEEFYQSTCSAVSKGYLSALRTGWYTSVITIELSNIKENKCNGTDAKVKLIKQELDKYKNAVTELQLLMQSTPAANNRARRELPRFMNYTLNNTKNTNVTLSKKRKRRFLGFLLGVGSAIASGIAVSKVLHLEGEVNKIKSALLSTNKAVVSLSNGVSVLTSKVLDLKNYIDKQLLPIVNKQSCSISNIETVIEFQQKNNRLLEITREFSVNAGVTTPVSTYMLTNSELLSLINDMPITNDQKKLMSSNVQIVRQQSYSIMSIIKEEVLAYVVQLPLYGVIDTPCWKLHTSPLCTTNTKEGSNICLTRTDRGWYCDNAGSVSFFPQAETCKVQSNRVFCDTMNSLTLPSEVNLCNIDIFNPKYDCKIMTSKTDVSSSVITSLGAIVSCYGKTKCTASNKNRGIIKTFSNGCDYVSNKGVDTVSVGNTLYYVNKQEGKSLYVKGEPIINFYDPLVFPSLLWDASISQVNEKINQSLAFIRKSDELLGSGGSGYIPEAPRDGQAYVRKDGEWVLLSTFL

SEQ ID NO: 30 - DNA, 1656 bp, synthetic construct
  misc_feature 1..1656: note = cDNA encoding a preFsc
  source 1..1656: mol_type = other DNA
atggagttgccaatcctcaaaacaaatgctattaccacaatccttgctgcagtcacactctgtttcgcttccagtcaaaacatcactgaagaattttatcaatcaacatgcagtgcagtcagcaaaggctatcttagtgctctaagaactggttggtatactagtgttataactatagaattaagtaatatcaaggaaaataagtgtaatggtacagacgctaaggtaaaattaataaaacaagaattagataaatataaaaatgctgtaacagaattgcagttgctcatgcaaagcacaccagcagccaacaatggagccagaggctctggcggaagcggacttggatttttgttaggtgttggatctgcaatcgccagtggcattgccgtatccaaggtcctgcacctagaaggggaagtgaacaaaatcaaaagtgctctactatccacaaacaaggctgtagtcagcttatctaatggagtcagtgtcttaaccagcaaggtgttagacctcaaaaactatatagataaacagttgttacctattgttaacaagcaaagctgcagcatatcaaacattgaaactgtgatagagttccaacaaaagaacaacagactactagagattaccagagaatttagtgttaatgcaggtgtaactactcctgtaagcacttatatgttaactaatagtgagttattatcattaatcaatgatatgcctataacaaatgatcagaaaaagttaatgtccagcaatgttcaaatagttagacagcaaagttactctatcatgtcaataataaaagaggaagtcttggcatatgtagtacaattaccactatatggtgtaatagatactccttgttggaaactacacacatcccctttatgtacaaccaacacaaaggaaggatccaacatctgcttaacaagaaccgacagaggatggtactgtgacaatgcaggatcagtatcctttttcccacaagctgaaacatgtaaagttcaatcgaatcgggtgttttgtgacacaatgaacagtttaacattaccaagtgaggtaaatctctgcaacattgacatattcaaccccaaatatgattgcaaaattatgacttcaaaaacagatgtaagcagctccgttatcacatctctaggagccattgtgtcatgctatggcaaaaccaaatgtacagcatccaataaaaatcgtgggatcataaagacattctctaacgggtgtgattatgtatcaaataagggggtggatactgtgtctgtaggtaatacattatattatgtaaataagcaagaaggcaaaagtctctatgtaaaaggtgaaccaataataaatttctatgatccattagtgttcccctctgatgaatttgatgcatcaatatctcaagtcaatgagaaaattaatcagagtctagcatttatccgtaaatcagatgaattattacataatgtaaatgctggtaaatccaccacaaatatcatgataactaccataattatagtaattatagtaatattgttagcattaattgcagttggactgcttctatactgcaaggccagaagcacaccagtcacattaagtaaggatcaactgagtggtataaataatattgcatttagtaactga

SEQ ID NO: 31 - protein, 551 aa, synthetic construct
  REGION 1..551: note = preFsc
MELPILKTNAITTILAAVTLCFASSQNITEEFYQSTCSAVSKGYLSALRTGWYTSVITIELSNIKENKCNGTDAKVKLIKQELDKYKNAVTELQLLMQSTPAANNGARGSGGSGLGFLLGVGSAIASGIAVSKVLHLEGEVNKIKSALLSTNKAVVSLSNGVSVLTSKVLDLKNYIDKQLLPIVNKQSCSISNIETVIEFQQKNNRLLEITREFSVNAGVTTPVSTYMLTNSELLSLINDMPITNDQKKLMSSNVQIVRQQSYSIMSIIKEEVLAYVVQLPLYGVIDTPCWKLHTSPLCTTNTKEGSNICLTRTDRGWYCDNAGSVSFFPQAETCKVQSNRVFCDTMNSLTLPSEVNLCNIDIFNPKYDCKIMTSKTDVSSSVITSLGAIVSCYGKTKCTASNKNRGIIKTFSNGCDYVSNKGVDTVSVGNTLYYVNKQEGKSLYVKGEPIINFYDPLVFPSDEFDASISQVNEKINQSLAFIRKSDELLHNVNAGKSTTNIMITTIIIVIIVILLALIAVGLLLYCKARSTPVTLSKDQLSGINNIAFSN

SEQ ID NO: 32 - DNA, 420 bp, synthetic construct
  misc_feature 1..420: note = deoptimized NS1
  source 1..420: mol_type = other DNA
atgggttcgaattcgctatcgatgataaaagtacgtctacaaaatctatttgataatgatgaagtagcgctactaaaaataacgtgttatacggataaactaatacaactaacgaatgcgctagcgaaagcggtaatacatacgataaaactaaatggtatagtatttgtacatgtaataacgtcgtcggatatatgtccgaataataatatagtagtaaaatcgaattttacgacgatgccggtactacaaaatggtggttatatatgggaaatgatggaactaacgcattgttcgcaaccgaatggtctaatagatgataattgtgaaataaaattttcgaaaaaactatcggattcgacgatgacgaattatatgaatcaactatcggaactactaggttttgatctaaatccgtaa

SEQ ID NO: 33 - DNA, 375 bp, synthetic construct
  misc_feature 1..375: note = deoptimized NS2
  source 1..375: mol_type = other DNA
atggatacgacgcataatgatacgacgccgcaacgtctaatgataacggatatgcgtccgctatcgctagaaacgataataacgtcgctaacgcgagatataataacgcataaatttatatatctaataaatcatgaatgtatagtacgtaaactagatgaacgtcaagcgacgtttacgtttctagtaaattatgaaatgaaactactacataaagtaggttcgacgaaatataaaaaatatacggaatataatacgaaatatggtacgtttccgatgccgatatttataaatcatgatggttttctagaatgtataggtataaaaccgacgaaacatacgccgataatatataaatatgatctaaatccgtga

SEQ ID NO: 34 - DNA, 1176 bp, respiratory syncytial virus
  source 1..1176: mol_type = genomic DNA
atggctcttagcaaagtcaagttgaatgatacactcaacaaagatcaacttctatcatccagcaaatataccatccaacggagcacaggagacagcattgacactcctaattatgatgtgcagaaacacattaataagttatgtggcatgttattaatcacagaagatgctaatcataaattcactgggttaataggtatgttatatgctatgtctagattaggaagagaagacaccataaaaatactcaaagatgcgggatatcatgttaaggcaaatggagtggatgtaacaacacatcgtcaagacattaatgggaaagaaatgaaatttgaagtgttaacattagcaagcttaacaactgaaattcaaatcaacattgagatagaatctagaaaatcctacaaaaaaatgctaaaagaaatgggagaggtggctccagaatacaggcatgactctcctgattgtgggatgataatattatgtatagcggcattagtaataaccaaattagcagcaggagatagatcaggtcttacagctgtgattaggagagctaataatgtcctaaaaaatgaaatgaaacgttataaaggtttattacccaaggatatagccaacagcttctatgaagtgtttgaaaaatatcctcactttatagatgtttttgttcattttggtatagcacaatcttctaccagaggtggcagtagagttgaagggatttttgcaggattgtttatgaatgcctatggtgcagggcaagtgatgttacggtggggggtcttagcaaaatcagttaaaaacattatgttaggacacgctagtgtacaagcagaaatggaacaagttgtggaggtgtatgagtatgctcagaaattgggtggagaagcaggattctaccatatattgaacaacccaaaagcatcactattatctttgactcaatttcctcacttctctagtgtagtattgggcaatgctgctggcctaggcataatgggagaatacagaggtacaccaaggaatcaagatttatatgatgctgcaaaagcatatgctgaacaactcaaagaaaatggtgtgattaactacagtgtattagatttgacagcagaagaactagaggctatcaaacatcagcttaatccaaaagataatgatgtagagctttga

SEQ ID NO: 35 - DNA, 726 bp, respiratory syncytial virus
  source 1..726: mol_type = genomic DNA
atggaaaagtttgctcctgaattccatggagaagatgcaaacaacagagccaccaaattcctagaatcaataaagggcaaattcacatcacccaaagatcccaagaaaaaagatagtatcatatctgtcaactcaatagatatagaagtaaccaaagaaagccctataacatcaaattcaaccattataaacccaataaatgagacagatgatactgtagggaacaagcccaattatcaaagaaagcctctagtaagtttcaaagaagaccctacgccaagtgataatcctttttcaaaactatacaaagaaaccatagaaacatttgataacaatgaagaagaatctagctattcatatgaagaaataaatgatcagacaaacgataatataacagcaagattagataggattgatgagaaattaagtgaaatactaggaatgcttcacacattagtagtagcgagtgcaggacccacatctgctcgggatggtataagagatgccatggttggtttaagagaagaaatgatagaaaaaatcagaactgaagcattaatgaccaatgacagactagaagctatggcaagactcaggaatgaagaaagtgaaaagatggcaaaagacacatcagatgaagtgtctctcaatccaacatcagagaaactgaacaacctgttggaagggaatgatagtgacaatgatctatcacttgaagatttctga

SEQ ID NO: 36 - DNA, 585 bp, respiratory syncytial virus
  source 1..585: mol_type = genomic DNA
atgtcacgaaggaatccttgcaaattcgaaattcgaggtcattgcttgaatggtaaaaggtgtcattttagtcataattattttgaatggccaccccatgcactgcttgtaagacaaaactttatgttaaacagaatacttaagtctatggataaaagcatagatactttgtcagaaataagtggagctgcagagttggacagaacagaagagtatgccctcggtgtagttggagtgctagagagttatataggatcaataaataatataactaaacaatcagcatgtgttgccatgagcaaactccttactgaactcaacagcgatgacatcaaaaaactaagggacaatgaagagccaaactcacccaaagtaagagtgtacaatactgtcatatcatatattgaaagcaacaggaagaacaataaacaaactatccatctgttaaaaagattgccagcagacgtattgaagaaaaccatcaaaaacacattggatatccacaagagcataaccatcaataacccaaaagaatcaactgttagtgatacgaacgaccatgccaaaaataatgatactacctga

SEQ ID NO: 37 - DNA, 6498 bp, respiratory syncytial virus
  source 1..6498: mol_type = genomic DNA
atggatcccattattagtggaaattctgctaatgtttatctaactgatagttatttaaaaggtgttatttctttctcagaatgtaacgctttaggaagttacatattcaatggtccttatctcaaaaatgattataccaacttaattagtagacaaaatccattaatagaacacataaatctaaagaaactaaatataacacagtccttaatatctaagtatcataaaggtgaaataaaaatagaagaacctacttactttcagtcattacttatgacatacaagagtatgacctcttcagaacagactactactactaatttacttaaaaagataataagaagagctatagaaatcagtgatgtcaaagtctatgctatattgaataaactggggctcaaagaaaaagacaagattaaatccaataatggacaagatgaagacaactcagtcattactaccataatcaaagatgatatacttttagctgtcaaggataatcaatctcatcttaaagcagacaaaaatcaatccacaaaacaaaaagatacaatcaaaacaacacttttgaagaaattaatgtgttcgatgcaacatcctccatcatggttaatacattggtttaatttatacacaaaattaaacagcatattaacacaatatcgatctagtgaggtaaaaaaccatggttttatattgatagataatcatactcttagtggattccaatttattttgaatcaatatggttgtatagtttatcataaggaactcaaaagaattactgtgacaacttataatcaattcttgacatggaaagatattagccttagtagattaaatgtttgtttgattacatggattagtaactgtttgaacacattaaacaaaagcttaggcttaagatgtggattcaataatgttatcttgacacaattattcctttatggagattgtatactaaaactattccacaatgaggggttctacataataaaagaggtagagggatttattatgtctctaattttaaatataacagaagaagatcaattcagaaaacggttttataatagtatgctcaacaacatcacagatgccgccaacaaagctcaaaaaaatctgctatcaagagtatgtcatacattattagataagacaatatcagataatataataaatggcagatggataattctattgagtaagttcctaaaattaattaagcttgcaggtgacaataacctcaacaatctgagtgaattatattttttgttcagaatatttggacacccaatggtagatgaaagacaagccatggatgctgttaaagttaattgcaacgagaccaaattttatttgttaagtagtttgagtatgttaagaggagcttttatatatagaattataaaagggtttgtaaataattacaacagatggcctactttaagaaatgccattgtcttacccttaagatggttaacttactataaactaaacacttatccttccttgttggaacttacagaaagagatttgattgttctatcaggactacgtttctatcgagagtttcggttgcctaaaaaagtggatcttgaaatgatcataaatgataaggctatatcacctcctaaaaatttaatatggactagtttccctagaaattatatgccgtcacacatacaaaattatatagaacatgaaaaattaaaattctctgatagtgataaatcaagaagagtattagagtattatttaagagataacaaattcaatgaatgtgatttacacaactgtgtagttaatcaaagttatcttaacaacccgaatcatgtggtatcattgacaggcaaagaaagagaactcagtgtaggtagaatgtttgcaatgcaaccaggaatgttcagacaagttcaaatattagcagagaaaatgatagcagaaaacatattacaatttttccctgaaagtcttacaagatatggtgatctagaactacagaaaatattagaattgaaagcaggaataagtaacaaatcaaatcgttacaatgataattacaacaattacattagtaagtgctctatcatcacagatctcagcaaattcaatcaagcatttcgatatgaaacatcatgtatttgtagtgatgtactggatgaactgcatggtgtacaatctctattttcctggttacatttaactattcctcatgtcacaataatatgcacatataggcatgcacccccctatataaaggatcatattgtagatcttaacaatgtagatgagcaaagtggactatatagatatcatatgggtggtatcgaagggtggtgtcaaaaactatggaccatagaagctatatcactattagatctaatatctctcaaagggaaattctcaattactgctttaattaatggtgacaatcaatcaatagatataagtaaaccagtcagactcatggaaggtcaaactcatgctcaagcagattatttgctagcattaaatagtctcaaattactgtataaagagtatgcaggaataggccacaaattaaaaggaactgagacttatatatcgagagatatgcaatttatgagtaaaacgatccaacataacggtgtatattacccagctagtataaagaaagtcctaagagtgggaccgtggataaacactatacttgatgacttcaaagtgagtctagaatctataggtagtttgacacaagaattagaatatagaggtgaaagtctattatgcagtttaatatttagaaatgtatggttatataatcaaattgcattacaacttaaaaatcatgcattatgtaacaacaaattatatttggatatattaaaagttctaaaacacttaaaaaccttttttaatcttgataacattgatacagcattaacattgtatatgaatttgcccatgttatttggtggtggtgatcccaacttgttatatcgaagtttctatagaagaactcctgatttcctcacagaggctatagttcactctgtgttcatacttagttattatacaaaccatgatttaaaagataaacttcaagatctgtcagatgatagattgaataagttcttaacatgcataatcacgtttgataaaaaccccaatgctgaattcgttacattgatgagagatcctcaagctttaggatctgagaggcaagctaaaattactagcgaaatcaatagactggcagttaccgaggttttgagcacagctccaaacaaaatattttccaaaagtgcacaacactataccactacagagatagatcttaatgatattatgcaaaatatagaacctacatatcctcacgggctaagagttgtttatgagagtttacccttttataaagcagagaaaatagtaaatcttatatccggtacaaaatctataactaacatactggaaaagacttctgccatagacttaacagatattgatagagccactgagatgatgaggaaaaacataactttgcttataaggatattaccattagattgtaacagagataaaagagaaatattgagtatggaaaacctaagtattactgaattaagcaaatacgttagagaaagatcttggtctttatccaatatagttggtgttacatcacccagtatcatgtatacaatggacataaaatatacaacaagcactatagctagtggcataatcatagagaaatataatgtcaacagtttaacacgtggtgagagaggacccactaaaccatgggttggttcatctacacaagagaaaaagacaatgccagtttataatagacaagttttaaccaaaaaacagagagatcaaatagatctattagcaaaattggattgggtgtatgcatctatagataacaaggatgaatttatggaggaacttagcataggaactcttgggttaacatatgagaaggccaaaaaattattcccacaatatttgagtgttaactatttgcatcgtcttacagtcagtagtagaccatgtgaattccctgcatctataccagcttatagaactacaaattatcactttgatactagccctattaatcgcatattaacagaaaagtatggtgatgaagatattgatatagtattccaaaactgtataagctttggccttagcttaatgtctgtagtagaacaatttactaatgtatgtcctaacagaattattctcatacccaagcttaatgagatacatttgatgaaacctcccatattcacaggcgatgttgatattcacaagttaaaacaagtgatacaaaaacaacatatgtttttaccagacaaaataagtttgactcaatatgtggaattattcttaagtaataaaacactcaaatctggatctaatgttaattctaatttaatattggcgcataagatatctgactattttcataatacttacattttgagtactaatttagctggacattggattcttattatacaacttatgaaagattctaagggtatttttgaaaaagattggggagagggatatataactgatcatatgttcattaatttgaaagttttcttcaatgcttataagacatatctcttgtgttttcataaaggttacggcagagcaaagctggagtgtgatatgaatacttcagatctcctatgtgtattggaattaatagacagtagttattggaagtctatgtctaaggtgtttttagaacaaaaagttatcaaatacattcttagccaggatgcaagtttacatagagtaaaaggatgtcatagcttcaaactatggtttcttaaacgtcttaatgtagcagaattcacagtttgcccttgggttgttaacatagattatcatccaacacatatgaaagcaatattaacttatattgatcttgttagaatgggattgataaatatagatagaatatacattaaaaataaacacaagttcaatgatgagttttatacttctaatctgttttacattaattataacttctcagataatactcatctattaactaaacatataaggattgctaattccgaattagaaagtaattacaacaaattatatcatcctacaccagaaaccctagaaaatatactaaccaatccggttaaaagtaatgagaaaaagacactgagtgactattgtataggtaaaaatgttgactcaataatgttaccatcgttatctaataagaagcttattaaatcgtctacaatgattagaaccaattacagcagacaagatttgtataatttatttcctacggttgtgattgataaaattatagatcattcaggtaatacagccaaatctaaccaactttacactactacttctcatcaaatatccttagtgcacaatagcacatcactttattgcatgcttccttggcatcatattaatagattcaattttgtatttagttctacaggttgtaaaattagtatagagtatattttaaaagatcttaaaattaaggatcctaattgtatagcattcataggtgaaggagcagggaatttattattgcgtacagtagtggaacttcatcctgatataagatatatttacagaagtctgaaagattgcaatgatcatagtttaccaattgagtttttaaggctgtacaatggacatatcaacattgattatggtgaaaatttgaccattcctgctacagatgcaaccaacaacattcattggtcttatttacatataaagtttgctgaacctatcagtctttttgtctgtgatgctgaattgcctgtaacagtcaactggagtaagattataatagagtggagcaagcatgtaagaaaatgcaagtactgttcttcagttaataaatgtacattgatagtaaaatatcatgctcaagatgatatcgatttcaaattagacaacataactatattaaaaacttatgtatgcttaggtagtaagttaaagggatctgaagtttacttagtccttacaataggtcctgcaaatgtgttcccagtatttaatgtagtacaaaatgctaaattgatactatcaagaactaaaaatttcatcatgcctaaaaaagctgataaagagtctattgatgcaaatattaagagtttgataccctttctttgttaccctataacaaaaaaaggaattaatactgcattgtctaaattaaagagtgttgttagtggagatatactatcatattctatagctggacgtaatgaagttttcagcaataaacttataaatcataagcatatgaacatcttaaagtggttcaatcatgttttaaatttcagatcaacagaattaaactataatcatttatatatggtagaatctacttatcctcatctaagtgaattgttaaacagcttgacaaccaatgaacttaaaaaactgattaaaatcacaggtagtttgttatacaacttttataatgaataa

SEQ ID NO: 38 - DNA, 19 bp, unidentified
  source 1..19: mol_type = other DNA; note = T7 promoter
taatacgactcactatagg

SEQ ID NO: 39 - DNA, 49 bp, unidentified
  source 1..49: mol_type = other DNA; note = hammerhead ribozyme
ttttttcgcgtctgatgaggccgttaggccgaaactcctctccggagtc

SEQ ID NO: 40 - DNA, 68 bp, hepatitis delta virus
  source 1..68: mol_type = genomic DNA; note = hepatitis delta virus ribozyme
ggccggcatggtcccagcctcctcgctggcgccggctgggcaacatgcttcggcatggcgaatgggac

SEQ ID NO: 41 - DNA, 47 bp, unidentified
  source 1..47: mol_type = other DNA; note = T7 terminator
tagcataaccccttggggcctctaaacgggtcttgaggggttttttg

SEQ ID NO: 42 - DNA, 21 bp, synthetic construct
  source 1..21: mol_type = other DNA; note = 3' leader
acgcgaaaaaatgcgtacaac

SEQ ID NO: 43 - DNA, 23 bp, synthetic construct
  source 1..23: mol_type = other DNA; note = 5' trailer
gtttttgacactttttttctcgt

SEQ ID NO: 44 - protein, 20 aa, Vesicular Stomatitis Virus
  source 1..20: note = cytoplasmic tail region of Vesicular Stomatitis Virus G protein
LKHTKKRQIYTDIEMNRLGK

SEQ ID NO: 45 - protein, 23 aa, respiratory syncytial virus
  source 1..23: note = cytoplasmic tail region of human respiratory syncytial virus strain RSVA/TH_10654
ARSTPVTLSKDQLSGINNIAFSN

SEQ ID NO: 46 - DNA, 51 bp, respiratory syncytial virus
  source 1..51: mol_type = genomic DNA; note = the inter-gene between the G protein gene and the F protein gene
gtattgttgcaaaaagccatgaccaaatcaaacagaatcaaaatcaactct

SEQ ID NO: 47 - DNA, 43 bp, respiratory syncytial virus
  source 1..43: mol_type = genomic DNA; note = the inter-gene between SH gene and G gene
agtcataacaatgaactaggatattaagaccaaaaacaacgct

SEQ ID NO: 48 - protein, 29 aa, respiratory syncytial virus
  source 1..29: note = 29 amino acids corresponding to R109 to F137 containing two furin cleavage sites and a p27 region
RELPRFMNYTLNNTKNTNVTLSKKRKRRF

SEQ ID NO: 49 - protein, 6 aa, synthetic construct
GSGGSG

SEQ ID NO: 50 - DNA, 12 bp, respiratory syncytial virus
  source 1..12: mol_type = genomic DNA; note = furin cleavage site II
cgagccagaaga

SEQ ID NO: 51 - DNA, 12 bp, synthetic construct
  source 1..12: mol_type = other DNA
cgaccctccaag

SEQ ID NO: 52 - DNA, 12 bp, respiratory syncytial virus
  source 1..12: mol_type = genomic DNA; note = furin cleavage site I
aggaaaagaaga

SEQ ID NO: 53 - DNA, 12 bp, synthetic construct
  source 1..12: mol_type = other DNA
aggaaaagaaag

SEQ ID NO: 54 - protein, 5 aa, synthetic construct
GSGGS

SEQ ID NO: 55 - protein, 4 aa, respiratory syncytial virus
  source 1..4: note = furin cleavage site II
RARR

SEQ ID NO: 56 - protein, 4 aa, synthetic construct
RPSK

SEQ ID NO: 57 - protein, 4 aa, respiratory syncytial virus
  source 1..4: note = furin cleavage site I
RKRR

SEQ ID NO: 58 - protein, 4 aa, synthetic construct
RKRK